European Patent Application EP 4 306 637 A1, published January 17, 2024. Title: BACTERIOPHAGE(S) TARGETING CAPSULAR DEFICIENT KLEBSIELLA PNEUMONIAE (KP), COMPOSITIONS COMPRISING IT(THEM) AND USE(S) THEREOF. Applicant: INSTITUT PASTEUR. Application EP, filed July 13, 2022. The sequence listing filed with the application follows.

SEQUENCE LISTING (14 sequences)

SEQ ID NO: 1 - protein, 1277 aa, unidentified
MADLEKIQFLRSTVAGKTPTTSQLADGELAINMADYAIYTKNGSSIVQLAGKGIPETNTKKLTVDGPSALNDTVTVAEGKTITFTNENLSGEITRHIVGKCASNDGWYIGSGGTSNNGILEIGTIDDGTETIQFVQRGAGNVEARKLVLLDSSGNTTLPGDLRLSTNKTVKINNGSSLVLEMGVGANDAYIKNLRGSGVLQLTNDGNLTFRNSQVYYATDGRGPGKDGTLLTNVENARQLEQDNFPVTTGNESRWIKVALLKDPGSGQSRLQLMVTNGGNYGSTCSSIDFIDCSARSIPSTLTSSNIRSYLQIRRIGDPGIDNTNQMRYSLVRTSEGLELWFTQRAFIGGVKVALLSIAGGAVTEYYLPTGYTTSATAPEGLVESVAIRIYDEINKPNLDNGTDGILSIAKGGTGASTASAARTNLGLGTAATRDVGEGAGNVLENGAYGLGGNGGKSINDIISNADMLTRLKSYGGTFWRGVTKSGVSVQNGLYSHGSGIFMNAGDTMSAINIDYASAKVRVYAANNAALAAGDVKYNELYGTANKPSKADVGLGNLTNDTQVKKAGDTMTGDLTVPNLHASGTGTASVYVNAGTGNAHVWFRTDSNERGVIWATPNTADLGQINIRARTTGGTSAGDFSFRSDGRLDVPVAVKIGGAAMLTKDGNITSGSMFGGNLNNYLTSIKNDIVAGDNKQVSKTGDTMTGNLTINANLKVENPNGTMVDLGSENSDKYSRLTLARKVGSGATVAMLKVTPEGHVQFGYQDAVATPAPSKYILVKSSGLEVEGDLVFNQTYSGAEDAVDITDKTVDLNSLVIKKSGLGTRQLYKCMSSGGGNNISNKPTYDGNFVLEVLSLRKVSETDWTCKQTFTTKNGDVEGTYVRYCQNGTWSAWKEVVAGVQPINLGGTGATSVAAARNNLGVGEGQSVKFGGLVVDGNINVASGNFVIAGQAPTDNSHLTNKKYVDDRVASAISNAGDTYLPLAGGTVTGRLTITGDQLKTTSLWVTGDAAVNGVLTVDGRARFNQEFSVSTSVNVQNNGNSHVFFRKADGTEKGLLWVDDPGNVSIRAGGGSGPVWNFWNSGSCQFPGAISNFNGVNSTTNYPGGGIGAYLNTAGLTSRFSNGAYVSLYFQEYVGNYHQAILNVNGYGQDNSFYFRAGGDFICTRNGSFDNVEIRSDRRAKSDIKVIENALEKVEKLTGNTYELHNTSGGTTRSAGLIAQEVQEILPEAVTQDNEEDGGMLRLNYNSVIALLVESVKELSAEVKNLKAEIEELKSK

SEQ ID NO: 2 - protein, 1267 aa, unidentified
MADLEKIQFLRSTVAGKTPTTSQLADGELAINMADYAIYTKNGSSIVQLAGKGIPETNTKKLTVDGPSALNDTVTVAEGKTITFTNENLSGEITRHIVGKCASNDGWYIGSGGTSNNGILEIGTIDDGTETIQFVQRGAGNVEARKLVLLDGSGNTTLPGELRLTTNKTVKINNGSTLVLEMGVGSNDAYIKNQRGVGVLQLTNDSNLTFRNSQVYYAMSGRGPGKDGTLLTNVENARQLEQDNFPVTTGNETRWIKVALLKDPGSGTSRLQLMVTNGGNYGNTHSSIDFIDCSARSIPATLTSANISSYLQIRRIGDPGIDNTNQMRYSLVRTSEGLELWFAQRAFIGGVKVALLSIAGGTVTEYYLPTGYTISATAPEGLVESVAIRIYDEMNKPNLDNGTDGILSIAKGGTGASTADAARTNLGLGTAATRDVGTGSGQVMLVGAYGLGGKGTSYTVANSRDYLKQLRADGSQFMRNTLGTEINYGMGASFYSSVSDVHAVISVDWATGRVKVGATNDANLNSDTGKISSQELYGTAFKPTPDDVGAVARAGDTMTGNLTIKANLKVENPNGTMVDLGSENSDKYSRLTLARKVGSGATVAMLKVTPEGHVQFGYQDAVATPAPSKYILVKSSGLEVEGDLVFNQTYRGTEEAVDITDKTVDLNGLVIKGTDPGTRQMYKCFSYGGGSNISNKPTSDGNFVLEVLSLRKISDTDWTCKQTFTTKGNVEGTYVRYCQNGTWSAWKEVVAGVQPINLGGTGATSVDAARNNFTIGKTQSVEFGSLILNGVGDNDATLDFKGGARIRGGQRTGEGAMILSAAAGAVGKYIAFRPFGDSSVTEIRVKANESSEPLLEWSYGPGIRSNSSGAFVIYAKTGQALHLRPNGDNSNQATVIDQNGKMTVGGEFEAQNSKITGNLNVSEDNRMIVLGRNTDIGLVKKSNMPGKMAISKSNSFTVMVSTNTNNQINPADTFNDIFKVDADGNQTVYGNAQVNRQLTVSSSATVAGVINANGGIIVPTTKYVQIADAPTQNNQATNKKYVDDKVASAISNAGDTYLPLTGGTVTGRLIITGDQLKTTSLWATGDAAVNGALTVDGNVVSNYGIGSFVGAVDVKAPAADNGTTHLWFRHSNGGERGVIYMPRDNNTMMGLRAGGSEWQLHGSAGQMVGPGARWRIHPDGNIQGDVYGGYITNYINDRFNQCAQWVRTGAQQDFGPIGRPAPGKTVPAGWVLVGLNGNSNEANQNMQLIGGRLQVWKPGVQWVDSAT

SEQ ID NO: 3 - protein, 222 aa, unidentified
  source 1..222: note = corresponds to translation of nucleic acid sequence between positions 165829 and 166497 of SEQ ID NO: 11
MADLKAGSTVGGLPIWHSGTFPLVPVGNTLTYRGYKVYTENDKPQASNNDFVSKASGGQYLGVVAFKQGLQINATFTGGSDQNGLYSGDGDGATLSKANIDLVSWYGIGIRSSSGTNGRVLVINARNGDLNTQGNITVEKQISITTANPTDASHATRKSYVDGQINNVTTNANSRVLRAGDTMTGLLTAPQFASTGAASRPEHVPRLDQVITKGTIIDFGSY

SEQ ID NO: 4 - protein, 222 aa, unidentified
  source 1..222: note = corresponds to translation of nucleic acid sequence between positions 168589 and 169257of SEQ ID NO: 12
MADLKAGSTVGGLPIWHSGTFPLVPVGNTLTYRGYKVYTENDKPQASNNDFVSKASGGQYLGVVAFKQGLQINATFTGGSDQNGLYSGDGDGATLSKANIDLVSWYGIGIRSSFGTNGRVLVINARNGDLNTQGNITVEKQISITTANPTDASHATRKSYVDGQINNVTTNANSRVLRAGDTMTGLLTAPQFASTGAASRPEHVPRLDQVITKGTIIDFGSY

SEQ ID NO: 5 - protein, 374 aa, unidentified
  source 1..374: note = corresponds to translation of nucleic acid sequence between positions 164655..165779 of SEQ ID NO: 11
MSNLMAGFGPDFVETQILSETNSVTYRITAKATHPNSVPNQYEFTLNQKAVGTPPSVGINVWRINNAVVDPIKTFTLSNDNSATANKAFVEYMDAQTSGLYLIMTNGEYKTSQIVDDWFAKKRSVMWQGADFAQRFPNSAYVALYGASKSRILIESFYANDGVLKEDSRASIDLVYDNVGDVGRTGVPFRSVEDTEEYNSTNGSEYKVYPVANPVISKLADYGMAPGLAMMIAGDFYASKALLDAGSTTRVTVRWFTGTAQTSSSVIEVPANKPDEWLRFEQFYTIPSGCDGFNVAVSRYPKPATDSLSAIRNFVMVQVSAAEADQNFAAQFGVNGIRMNNMIDGGTPYIFELPNTKVYPGGDYSASEFREVDA

SEQ ID NO: 6 - protein, 374 aa, unidentified
  source 1..374: note = corresponds to translation of nucleic acid sequence between positions 167415..168539 of SEQ ID NO: 12
MSNLMAGFGPDFVETQILSETNSVTYRITAKATHPNAVPNQYEFTLNQKAVGTPPSVGINVWRINNAVVDPIKTFTLSNDNSATANKAFVEYMDAQPSGLYLIMTNGEYKTSQIVDDWFAKNRSVMWQGADFAQRFPNSAYVALYGASKSRILIESFYANDGILKEDSRASIDLVYDNVGDVGRTGVPFRSVEDTEEYNSTNGSEYKVYPVANPVISKLADYGMAPGLAMMITGDFYASKALLDAGSTTRVTVRWFTGTAQTSSSVIEVPANKPDEWLRFEQFYTIPSGCDGFNVAVSRYPKPATDSLSAIRNFVMVQVSAAEADQNFAAQFGVNGIRMNNMIDGGTPYIFELPNTKVYPGGDYTASEFREVDA

SEQ ID NO: 7 - protein, 1257 aa, unidentified
  source 1..1257: note = corresponds to translation of nucleic acid sequence between positions 160882..164655 of SEQ ID NO: 11
MVAKSFRARSGLDAAGEKVINVGKADRNTLSDGVNVDFFNEFNGIQQYDPTRGYSQDMAIIYARRIWYAKQNIASPAGAFDESKWIATRNDPKWVYSNVTTPDGSIIESGSYIMADGRFTELLYLLPDNPTEGDVITFKDCGGLVGVNSILVKSNTRQIRLRTVQSAQYRLTHPYMIATFIYNGNVWRVAETLDNRDSEIVNATGTGSFQLQSGMTVFRNSATGKITLQLPKYANDGDVITTYDADKMNSINVAVLQIYPGSGHTISDGAITGVTSVTSQKSGFGMFIFDAQNSQWKVYDADNRVRLRRIYSDLNTVPNDYVFVTANPSGTIPNVTVTLPTDVADGDRVYVSLYMMGKNQNCTIKVKDGTTDKIRTNKNMMQFPQRKDYPPDDWFSVTSLAFNAASDYLPYIEFSYMKATKEWVVANYRPIVERVDATNRSRTGVIALAAQAEVNKNLEDNPNDETAITPMTLANKTATETRRGIARLATTAEVNKLSTDTYLDDVIVTPKKLNERTATETRRGLAEIATQAETNGSTDDITIVTPKKLHNRIASPTLTGILALVATGGAPNTNTDRAQAGTGVYDHSDYQKAVTPKTLREYKATQLQSGAVWLASETEVINGTVASANIPTVVTPEMLHKKTSTDGRIGLIEIATQAETNAGTDYTRAVTPKTLNDRAATETLTGIIAIATTAEVSAGTVTDKAIVPSKLKGYLDDTSHITVATADGLTQSGTIWTTVNIGIQSATETQRGTLRVATQSETNAGTLDTVFVTPKKLHAKKATESAEGIIQVATAAETTAGTVANKAVSPKNLKNTIQVDTSWQATDLVRGTVKLSKGLGTWSGNDVAGSTLPDDGYAAVGVAVSPYELNLTLKHYLPIGAKAVDADKLDNLDSSQFIRRDVDQTVNGALTLTRTTTVQANIDSSADATFRVMNVNGDLNVGDGSSMGKLRLNGGSSNDWSIQASSASGRIAMISTGNTGTVHLSVYNDTRGVVANVKFQAPEIQAISKVTLGNDTVITAAGSVLSMGTNNKTTKILTSDAGNIVAEESANSYKVFTEKNAQTLLNPTYVRKAGDTMSGRLTVNNSSIIIAGQAAWSTLDAVTEASRGNWTAEITASAQYNLLPGYAVPVLEPDPINPEIMIVTRYTYVKAPGTLTQFGNGTAFTYQIWAPRPTSGTGVDALAQSFWIRQMNPITGKFDGWGRMYTSNNPPTAGEIGATSAVGTTVKNMTVTDWIKVGNVKIYPDPVTQTVKFEWVA

SEQ ID NO: 8 - protein, 1257 aa, unidentified
  source 1..1257: note = corresponds to translation of nucleic acid sequence between positions 163642..167415 of SEQ ID NO: 12
MVAKSFRARSGLDAAGEKVINVGKADRNTLSDGVNVDFFNEFNGIQQYDPTRGYSQDMAIIYARRIWYAKQNIASPAGAFDESKWIATRNDPKWVYSNVTTPDGSIIESGSYIMADGRFTELLYLLPDNPTEGDVITFKDCGGLVGVNSILVKSNTRQIRLRTVQSAQYRLTHPYMIATFIYNGNVWRVAETLDNRDSEIVNATGTGSFQLQSGMTVFRNSATGKITLQLPKYANDGDVITTYDADKMNSINVAVLQIYPGSGHTISDGAITGVTSVTSQKSGFGMFIFDAQNSQWKVYDADNRVRLRRIYSDLNTVPNDYVFVTANPSGTIPNVTVTLPTDVADGDRVYVSLYMMGKNQNCTIKVKDGTTDKIRTNKNMMQFPQRKDYPPDDWFSVTSLAFNAASDYLPYIEFSYMKATKEWVVANYRPIVERVDATNRSRTGVIALAAQAEVNKNLEDNPNDETAITPMTLANKTATETRRGIARLATTAEVNKLSTDTYLDDVIVTPKKLNERTATETRRGLAEIATQAETNGSTDDITIVTPKKLHNRIASPTLTGILALVATGGAPNTNTDRSQAGTGVYDHSDYQKAVTPKTLREYKATQLQSGVVWLASETEVINGTVASSNVPTVVTPEMLHKKTSTDGRIGLIEIATQTETNAGTDYTRAVTPKTLNDRAATETLTGIIAIATTAEVSAGTVTNKAIVPSKLKGYLDDTSHITVATADGLTQSGTIWTTVNIGIQSATETQRGTLRVATQSETNAGTLDTVFVTPKKLHAKKATESAEGIIQVATAAETTAGTVANKAVSPKNLKNTIQVDTSWQATDLVRGTVKLSKGLGTWSGNDVAGSTLPDDGYAAVGVAVSPYELNLTLKHYLPIGAKAVDADKLDNLDSSQFIRRDIDQTVNGALTLTKETTVQANINSTADASFRVMNVSGDLNVGDGSSMGKLRLNGGSSNDWSIQASSSSGRIAMISTGNTGTVHLSVYNDTRGVVANVKFQAPEIQAIGKVTLGNDTVITAAGSVLSMGTNNKTTKILTSDAGNILAEESGNSYKVFTEKNAQTLLNPTYVRKAGDTMSGRLTVSNSSIIIAGQAAWSTLDAVTEASRGNWTAEITASAQYNLLPGYAVPVLEPDPINPEIMIVTRYTYVKAPGTLTQFGNGTAFTYQIWAPRPTSGTGVNALAQSFWIRQMNPITGKFDGWGRMYTSNNPPTAGEIGATSAVGTTVKNMTVTDWIKVGNVKIYPDPVTQTVKFEWVA

SEQ ID NO: 9 - protein, 179 aa, unidentified
  source 1..179: note = corresponds to translation of nucleic acid sequence between positions 170379 and 170918 of SEQ ID NO: 11
MAVTGPWVGSSAKAETGESWMAQAGAKLRLGTPFWMSNMIGRSVFNFSLTVQYRNWNNIYYRGSWQVGGWNWSPKPTTQNTVQGNFEGKEVTLFVSVSGQGGVNYWNGDPQGTTLGIRNGDAINLRVMMSDGTTFDFTPGKMDGDVRNYQIASNDEANKLKNWFSDRTDQYWQGLITRR

SEQ ID NO: 10 - protein, 133 aa, unidentified
  source 1..133: note = corresponds to translation of nucleic acid sequence between positions 173111 and 173512 of SEQ ID NO: 12
MIVKQMKGIKWHHNFEGGAYYRDCNDKCWYSFRNSLDKNSHIIIVDAKTNKIINYYNGEDPTMIGLFADKEMILDVYQLDDFPVDSWDEFSKRKFEFIDGKTIMTKDVEVEKERTKEDILADLIKLQKELESM

SEQ ID NO: 11 - DNA, 175100 bp, unidentified
  source 1..175100: mol_type = genomic DNA
ttagtaatggctaaaaccatatgtaacatcaatcatgactttataacggcatacacgcatttttgcgttattgtaatccactgggatcgctaccacgtcagcaggatccacctttacctgaatgactctaccaacaccgcccccgtagtgtggaaggtatgatttagccgcaacgtgtaggccagtagaacaggtgcgcgttttatcttcgtctaccatgtttcgaggcatggagacagtcacaccaggactattatcaaatttgccagtagcgagatctttatagttatcgcgcacacgtttccaggcaaggaaacaaccatcatcggtcagttcaatgtcattatgtacaaggaacccataaagctggtatacagcatcgcgtgaagggtttcgcatcaaccgttcaaagaagttcaccagatgttcatacggacgatcgttatacatttcgcgaatgattcgttgagtgatatcagaatcaaacactacatctttatatagaagctgatgaccaatgattttaatgttgcctttgctataggttcggatcgcttcttgagtatccaaacaagttacagcacctttgacatcaccagctttcagcatttcatgcgctttcttaaagttcggatgtgtttcacccgccatgaaaacgcgcccttcgtatacaaccgtaatgaacgattcagatccgatcatacgcggtacagtgtctgatactttaggcttttgttttacatcccttttcttagggaattccgctaacttgcggttgataacgcgcccaatggttcgggcgcttacgttgaactgttgggccagtgctgttttacttgcccccgtcaaccatccattatagatagctttctgttgtacttcgtcgagaattttgaccattatttccaccgtattaatttcttaaactcactgagattcttttcgttgttgtaaatcggacgaattgaataagaatcgctatgttcaacaagtgaagccagtaacgggtttagtgatttaaagatttcccatgcctgatcaacacgttttttcatattgctgcgtttaacgcgcattgatgctacagattcacgcagaatcggacaacgcgccctggaaagatttttaccatctttctcatacccttccagacacactatacgttcgagggtatcaacaatcttatacagtttttcattatatcggtttttcacaatccgatcaagcgatacaccgaaacggctatgcaatgcgtctgtttctgttgagtgatccttcccaatccatccaggcaagcaattatctttcaatgccttttcagatttaacatactgcttgcacagcatatcatcaaagcataccagatttgaatccgggatccacttccataggctgttacgtatagcaaacacaacagggatcccagtatggcgcatgatacgcgataaagtagattctttcattgctgaatccatagacaacctggaattttcaccatctaagcggctatattcatcaataccatacaaccgaacacctggggctttatccagtgataaaaactctgattttgtcataaacagagaagtttttgccagattgccgttactatccaactcataacgatatacggtcggggtttttgggcgcggttctgaatttttcggtgcatatagcgcttttgatttttcgcgatctgcatcatagatctctttttcttttgtcatttcactggtacggagatacacaatttccgattcatcaaaatgacctttccgaacgatatcattaacaatctcacgctttgaatcactatcgtaatatgcaacaaagctaacacggcttaggttatgcattttcgcatacccgacgatatacggtttaaccgtgttggtatccacttttaacagaatgagtttcttctgtttccacggataataaatgcgtgtgatgtcctggcgtttggttgtttctggcttatacttgctccagcggcctccgctacccgttacctgataccatgcatctttaccgtcgtattcgttcgcccaatacccagcaacataatcatcattatatttgttgggtttgactagttcgctatggatccagccaatagaatcaccgttgatgcgaaaattagcatctttaccaacaaagttttgtaccattgaaggcagagaatggaaccacgtcagtttatcacgaacggtttgtaacttatcgaattctgatttaactcgattgaaatatacccggctgatttgtttcagacgttctttaacaatccctactgtcattttatccatactcaactcttcgcgagaaggcatgaaatcaagttcgccgatcgggaagtcaataatatacgtatactggctttctgtatagcaatagaacatcgaggtatcatacaaatctttatccagaggataaatgatgttacccatgcgagcatatacaccgctagtgtatgctgatttatgacggatcaccccgctatcgttggttgcttctttcggctgatagttgattttgagaatagaagcaccaacaaagttaggacgaatatcagtaaatgattcgtatacccttgctgcttcgttttcccattctttgatatcttcaactttaaccggaacagtgatagtaaccccgttaggttcatcactttcaatctcatacagaggatcgcagaacggttccccatcatccatatagattgtgtaaccgcatttgataccgtcttttacagattcaactgtgaacgcatcggcatagcaaagcggagatttgcaacccagacccatagaaccgatcaggtcgtttgaatcatttttagttgattcgaagtaaacggtaaacgcatcactaacgaaatcaggagacataccgatcccgtagtcacgaataacaaaacgaggatcaacagcagttggcaactggacatcaaacgggttctgatttcccgcttctttgtgtccatcgatcgcattacaagacagttcgcgaatgattgcgcggatcttgtatttgtatactgtcgaagaaaggatcttatacgctttcttgtttgcgcgtagagatagtttgtttcgtcccttgctggtatctgtaccaactcggtagattgtttgcggtgtatcttcgcgtaatttcattgtttatttctcacttaacattaaaaataacttggtcacaagagtacttcgttggctttttgttcaggccatattctactacttcgcaatatgtgtcaaggaattttactaatttttcttcctcgacctgctgtttcttcatatcaagtataccccacacgatagccccgataatgatagaaaagaacgcacaaaatccgaatatggtcagatattttcccaacttaggcgcattacaacgtgtcataccttacccctctttgcgaatgtatgcaagttcttcatgggttactggacggatatacagacggccttttgtatatgccttgcgcccactgatccaaatgtttttcatatccttaacaccgttcatcacatcgttgtaaaacttcttatcagctttagcctgatagacttcacggccttgataatctttcatgaacaaacagtaaaggatctcattcttatcaaccagattagcatcctttgtagttgttttactcggtgaaggtttagcacccaggcgcaaggccatagcttgccacactttaccatgttcataacctcgcccgacaagagcatgagcgatttcgtgtaaaagagtgtctaaaatatcctcgtagatatcttccgcaacatgacgaccagatagttcgatcagttttttggcataactgcaacggcccagagtttttgtaatgcgtccattgatccggaatgtccaaccattactgatcaaaccgtgtttttccatcatggtacgcgcccagtgggttacttccattgcactacgagttttcaacattttagaatctcctttgcttggtacaaaaccaatatagcaaaaagccccctgcattgcaagaggctttgtaattatttcaatttcttagaaagttcttttaaatcattgagatactcaattttaggggttgtttcttcccagtatttcaactgtttacgcaattcttcggcttcgtcttccagctttttgctttcgtccgtggttagatggtagatgttcatagccactaacatttcggcatgattctcgcaacctatccacgtagacacgaatttaaccgcttcgctgcgactaaggccacgcagagaatcaggagattctaccatttgagcaataaacgcaacctttgccagtgctttatctaacgcttccttagtttcctggatacgcttattgatacgctgttgatatacattcatacgaatatcaacgaaatcctttagaagcgtttcagggcgttcatatgagtatagtttgccctcaaagataacgttaatgtttgggtttgaattttcaatcaacccgaaatctttcaggatcttttcgcgggttaacccattggcatactctcgcttgagcgttacttcataacgaaaatcttctttcgatagatccttgtagctaacgataacgcctttttcttccagcttgtcaaggattgcaatgtatttcacacggtcatacttcactgggatctcggtgatcaccaatttggttttaccttgcaattcatacgtgccgtaaattgtcccgtctgtgatttcacctttaaagtaagggtatttcagttccagtgtgaaatctttatcattcagatatgcaatgcacccgttaacaacagatttaggatcatgaggcggaatgtttgttgcatatgcttttgcaatcccgctaaacccgttaaccagtaccatcgggatgatcgggagatagtacgctggcggtacatgttccggatcttcatgaactggcgttaaatcaccatccatataaattgctttgaatattggcgatagtttgcacttgatgtaacgaggtgcgccaggtttcttaaccaaacgggaaccaaagaacccatcacggtcgaataacggaatgttattgcaccagtgcgccgccataagggataacgcttcttctacagaggtttccccgtggtgatacccatacatagcaacaccgccagcgatagaagctactttctgaaatcccgttccgccctgcatcgcagagtgaataaagaaacggtgaacgggtttaaacccgtctaccaggtgcgggatcgcacgtgaataaatcgtgtaaagggcaaacgttagcccttccacctgtacaacatctttaatacttctttccattagtcaaccttagaaaatttgtgttttccattaacccaatctttacgcggatcagattcgtcgccgaagcatagttctaacacttctttgtattcgtcgtcaagtacgatgacatcatacttcaactgatcacccagaacacgatcgtaatcttctttgcgtaaagaacccagccccttgatatatcgtacatcttttgctttatcgcggaacggtgcaaactcatcaagagaatagaaccatttttcctcgcgcccaactttagcgataacgatcggggttcgaatatatcggatccgtttctcagtgaacaaagaaggccaacggctaaagaatgcaagcaacagggttaagatatcaccgccgtcaacgtcagcatcgaccatgatgccgatattatcataagtcattccggaagtatcaccaggatgaatattgaggatagccattagctcaaacagttctttgtttttgataatgtctgtaaaactcataccccatgtattcagaggcttaccacgtagcgggaaagcgccttgtgtttcttcattacggcattcgatgaactgtccaacagcggaatcaccttctgtcagaaacaatgttgtttctaccccaggggtatcaataccggaagccggaacgtgtttagcaatctttgcctttttcgctttctttttcgctttggtgatcgcggcggcttctgctgcttgtttacgaatcaatgcggattcaatgatcggagtaatgatttctggagtatccataatcatttttgcgatctttttgtagttcaaattcgcatgattgttaaactcacctgctgtatttgctaatcgctcttttgtttggctatcgaatgcaggtgcattaaagttatgcaggaataccacaagagttaagcattcttttacacgtgctttcgggatctcgatactatgctttttcttgatcatcggttcaagttcagaatagataccatcaatcatacactcaacatgaacaccgccgtttttcgtatccagaccgttaacaaaggatttctgtttaaacccgtcctcagtgctcgccagaatgaagctgaggcgattatttgtctggacaatggttttatccccatacatggaagcgtacagcgggaagcgattagagagcgtttcgccgttatatgtgaatttcacggacgggaaagcaacggcaagggccattaagcgatccttaatcacttctttggtttcttcatcgataccagttacaccaaacatagagaagtctggagtaaacttaacagtagtaccctgttctttactggggctggttcggtaatcgatgttctgtgcgccgtccgtacagttaatggttactttgcgtttcccgtttgcagtctcgccaataaaaatcgagctataacagtttgtcaggaaagaaccaacaccattcatacccatcgttacgcggtttttatcatcgaagttagaacccgattttgccatagtccatgccgcaactggtttaggaactattttcccatctggggtttttacatcatcctggggaataccgcgcccgttatcagagattttaaccagattatgatcaatggttacatcaatcttattagcatgtttgaattcagttcggatcgcttcatcaatcgagttatcaaggatttcgttgatgattttaaccaacccttccacgtactcaaccttgcgatattggcccattatgaaacgttcatgcgcttctttgttaaccgatccgacgtacatatttggacgcaaccgaatatgatcgcgatcgctcatacaaaatgattcgtcaacctttgcgccttttttggctggttgtggtttctgttctggttcatcatctgccagaagaaaatctaaactcatattcacctctttgtttaatcactgacattatatagggttctatgaaaaagaaaacccctttcggggtttacttgttataagggaaaccatcacgaaccatttgaggtttatcaaccgttcgttttgcttcgcctccgcaatcgcaatctttcggtgcatcacgggtagcaatgcttgccatttttggaaattctttattacacttggtgcatttataggtataggtaggcattaataaatctcttttaaacttaacatcttaactaaacgggctttgtctatgtcaaaaacacattgacgtgcgcccggatacaacttttcaacttcgtataccatgcagacgaaaccaacattgtgcatgtactcgcgttcatatgcattgaaccaacgagaaaggcgctgtattgactgaaaaccaaagtataacccagccgcttgaaagtctatgttatctttttcaaggttgcgcatcaatcgattatcgtcatccggcgctggatgtcggttatcatccatatcaatatagatatcaggattcatacagaattgatccaaccattcagcagtatccattgacacataacgattgacatatgggccgctttttgtttgccatttttctgtacaatcattccagaaagaacaagaaaattccacacgatatacgaacatgatataatcctcacaagtaaactcaaggtttacaagtacgataccacttatctaatttttctgcaagcatttcgttgataatttttgcaatttcgtaccgtccgtgagtagtacccagttccaggtaaatcacatcaagtgcgcacacaatcgcatcaatactttcttcaacgatattaccgccgcgttgaggctgaatgagacattcgctgatctcgccaacttccgctgataggtgatgaaccacatcactcttcgtgcgtttcttcactttatgagcgatttcaaaaaacttatcaagtacgatcgccgtttcttctcgcgttgcagtattctcggatgtcgtctccgtttgttgaacaacgtattttgtaaaatagttttcaaacacgttgaaagggatcacatgaggaacaccattcaaaaacaccccttctttacaaacataatggatttggcgcggaatagacaacccgccgctgcgttccaaatgtcgtttaacgcttgctacaaaatcgaactctttcccgtatccagccgacatactgtgatacgtgagtaggccaaatgcagaaacatagagatcattttctttatacagattcatttacaatacctttatggtagccaaaaatataacaatcaattgaaggacgttcaccagggaagtgaatgcattgcatgatgcgttcagccattagatcttctcccatgtataccgaagtagtttcttcgttgtaatgggtatcatacgacgttttaagcgtcatgcccggaagccctgcaatgtgcatgaatttagaattggtgcaaggttttcctacttcaccgttaatcatcaacactgcattagttttacgtgcttttctcatttgaatttcaccccgatttgcgatacgttccattcttttacttcatcaacaatatcataatggttgatgtatggtaaagcaatttttaaattactcgcgtcttgaatgttgcgtaagaaacgagtaggagaaagaagacacaaccgctcggatccgttgtttcctttagcggcaaatgatagggtttctcccccgtcaatcttcatatcaacagaaatcgttttgaattctggtgcgtatgacgtgattttgccgttgtctcttggcgtactatagaaacatacactttgtgggacattataacgatctgtttcaatgtacatataatcgccgtcagtcattccccacgcggtataaagggatccggtatagtcaccaaaggaatttttaaaatcttccttcgtggtgtatcccagcgagcgcaattgcataagctggttatgctgttcgattgcgtcggctttttgttgttcctgtacttgcgcatcaatcgtttcttgccaggaattatacgcatagtaacccacaacagcgattacagccataacccctacagctttccagattttagcgtcttcgtttttgttactcatgctatattccttttaagaaaaagggccgaagcccctttgttaacgaagataaaccacataaccgctttggtcaatcgcgcggtctgcgtcattgaagatattgccacgaatgccttttgctggtgctttccagcttgcaggtttcaggatattaccatcattatcgatgaaggcggcaacagaacgctgattgaacatttcgcctgtttctttgttgcgagtatcctgaacaacacgatgatatttgcggcctttctccagaacgaaaacagtttcgaaaggagaatcttggaaacgagcgttacgcgctttgtacattgcttccatgaaaggggctgctttttctgcgaggatttcgaaagtgttcatggtatatctcctaaagtgtgtttcatttcgatgtaagtactatatcaaagatggttattctatgcaaggctttttttcgttatccatcaaatattttaagtgttcttttaatgcagggagttcgttcaaatggcgttgcttaactttctcgtactctttgcgttcccagttttcaagattgcttgccaacgcttcatcacaataagcgatcccgcgttctgcatcctgaactttctgtttccattgtgcaactgcttgttgataaagagaaccgttaaccatcataataatttcctcccttgtttcgatggggtaactataccaaagctaccccagaatgttttaacaaaaagtgctattagtaggtatccagtttatacattttgcaccagttcatgaattcttcgaaagtctgagtattaacacgtttttccttcttcactttcttagtgattacaggacggttagtaaaacgtttttgcattttcacagtgattgctactttatcgcccaggtcttctaccttttcaaccagcgcccactgagaaccaatttcagcaccgaaagttaaaccaacaatctcacctgctttaacgtgtgctgcatattttactttaaccattttcgtattcctttctctgtttcgtttcgatgaatacaagataccaaaaagcctcccgcaatgcaagaggctttttaacaaaaagtgctattttatttctttgagcaatttacggatcccgccgccctgtgtcttatcaaagattttctttgcatcaataacagaagtgattatgtggtagttgttcccttttccgtcaaactcaaactcgaccttgtagtcactacgaaatttcacaaaaacaaattcacctgcaaagtgcttacggaactgtttttcgttaatgtccaaccattcctgtgtatcatctaactgatacatgcgacaaaacaggatcgaacccattacagcaatcacgacaaggatagctaacgcgaattctgacatcatttacccctgtttactgattgacggtgcaatgatttaggcacaaccggatttcggtatggtttgactttatggatcgtgggttcttccccaaccaaattaggaaattggttgttccattccatcgaaaatggatagggtgatgactttaactcttcgatcatacagtttactaaacggtcgccgattacacccaaagccgccccaataatcgctatacgcataaatcaccccttaattgtgtcaagtacagtaaaccagtcatgaagccatatcgttgttcttacagcgatatacgttaacaaactaatcaatgataccgctccgcaaatagccagcgtaatcaacagccggatttcaaatttagtaaaattcatatcaatctcctttctgagaacccaatataacaaaagccctcaaccgaagtcaagggctttgttttaaatttttaccagttttggcaatcgaagaactataccaggatggatcagacgtgcatccggaatagaatcacggttgattttagcgatatcaggccaaagttcaccaacaccatacagtttctttgctatagaatataggctatcacctggttgcacgacatagcgatcagattcaatcttaaccagatcctggttaatgatatcatcaaaggcttttgctttcgcttcgttaatcgtgttcccgtagtaatggcgatccataatagttaatgtgatcatcgtttctttcctatgctgttttcgtctgtctcttctaaggatggaggttcttccagccccagagcataacgtttagcatagattagcatcaatgcatctttagcgcaatcatgaatcgaatcatgctgaatgaatccatctaacatgcctttacgaagtggacacgtggtcactccgcgagttagtaaacggttttcaatagctgtacgcacatcacggctattccagaacacggtcggcatatcttcaaacgtgtcaagtttccctgtcatagttcgtacaacatcggttagcatagaacggtcgaattcagggccgcgagtataatcgtatgactgccaacgactcacaccgtcagccgctaaatcagcaaagaattgtcgatgaccttcgtacaaatccatgtcaatatcggaagggaacaaaaccctttgtgcttctttagattgttgtttccaccattcgatcgttttttcatctttgattcgttctggttgtttccggatgtcaaatttgtactttcttcctttagcaatcagttcctggaaggtaggcggatcataaggatcatcaacaaacggaacatagctaagttcagctagttttccttttggaaacgggccaatactttcataatcaaatacaaaatctacgggtaaatgactcattcgcgaccccgcttatacgattccatgaaataggccaatgatagcgcgacttccggagtaacatcaacggatttgatcatgtctggagttactgccatcatcccgaactgacgaagcccacaacgagcaatcgatttttccagtcggatcatgttttctacagcctctgcaaaattgtccagatgttcccaatcgtggtaatcttccattgtagaacgatcacttttcaaaatcagatcggcaacggattcagcataaaggcgcggaaggtgaatattcatttaaaacccctcaagcatgtttttgttttcacgaatgttacgacccattttcaaagtatcaatgatcactgcatactcttcaaaagtgaattcgatatcttgtgaaatgtttccccacgtgtaggtcggcccgttaggacagtataacccaacttctttgtttgcgttgacaatgcagcgcaattttgcaaacaacaaattgatatcgatagaattgaacccttcgagataatcaagcccctctctaccaatacggtcaacttctcgcaaaatcttttctacatctttgactttaacaataattttcataataacctcaaagggccgaagcccttagacataatcaacagtgaatcgtgcgcgggtagttcctacataaagcaactgcttacacaattcataatcggcgtatgcgtatgcatcgcgcgtatacatgtatgaatgatcatacgtgcttccctgacctttgtgatacgtacaaaccggaagcgccttaaccgtctggaacttgtttttgatttgccagaacgaataccagggggctttgtatccggtttcctgtttcatctttttatactgaaacgcgacgtagttcaaataatcgcctaaacgttcctgcataaccggatccgcgataacctgaatatccgctttcgtatcctcgaacatcgattctgttttcatcaagaaataatcgatttgtaccggatcgcatcggtcagctttgatagtatcagaacgcggtatgatttcaaggattttaatttgctcgttgttgttatagataacttcaacaaacgaaaccccattcacacggccttctgtcactaacggttcttgcatcacaaccacttcaccaacaatgaacggctgatcagttttgtacaagtgtttacggatcactgcgtttaacttgtctacgtttgcgttagtgtaagcaaacatacggttattgttcaggtcatccggagtcttaacacggctaaaataacgtctcaggaagtcaccagcgttttcgtgcttcattacccctagttcaccattcatgaggggcattaacggcttaccgtcgcgtatagcgcgtgatacctggatgattgggtttccttctgcctgacgcataatcttatccatgcgaatgacatcaaaaatttcctcatcaaagaacggtgaaagctcggtgatcccttcggtattaaccggacggatctgatccttatcacctaatcccaggatcaccgcacaactcggaatagtacgcttgatgatccggaatagttctttgtcaaccatcgagacttcttcaacaacaaacacacgacattcagacagatcagcggcttttttgcctttttgctgttcaaatactcgtaactcttcgttggttacggggctgattttcagtgctgagtgaatggtcgttgcatccatacccaccgcctcagagagaacgtttttagcctggtgcgtcggtgctgtcaaccagatcccactaatacccagttttttcaatgtttcaaacacaaattttaccagagtagttttaccaacacccggcccacctgtgatagtagtatggattttgtttctgatatttttaatcactcgatcatgtgcatttttctggtcttcgctcagatcgtcaaaagttaattcgctcatactttaatcaataccccttgaatacttgcgtgttcaataaaccaacgcatatctttctttttcttttcggttacggtttcaacttcttcctttcgaaagaatcggctaagaccactttgtttaactggattcatcttatcatgatattctttgataatcgaatttttatactcgttagcatcgtccggagatagaaacaacaaaggtgttaactctccttccttaatgaagggaattttaaacccgtctttatccttactaacgacgatataatattttgtaatcattctcgcccctcataacaaacgtagaatattccaacaaaccaaaacactgatagtataatcagtaaaagttttctttcaacgccatttacgtgaaacacacaccaaccgaaaagatatgtgatcatcgcgcaaacaccataagaaagaaccccaacagctactagcgcgatgatcggatccattagtagttgttagcccaacggcggaggttttcggcttgtttcagtgcatacagtttgtagatggtttccgcatccatacccagcgccaggaatttgcacataaagaaatgccattgatcgataagttcaaacagaacttctaaacgatcctcttcactcagatccgcaaatttagtattgcgcaattcctggtgatttgctttccacggtttccaaacaccggatgcaggtttaacaccgcgagacattccacccagagcggtatacaattcgcgggtttcgtcggcgatcgcgtcgtcttgcagtttcagccaatcaaggatttctccgcaagtttccagattatccggacgcggaacccaatgcagggtatcagacaggctttgttgcgcatggttttgtaaatccagcatggattgtaaaggatcgccattacgggccagaaccttttgatattcggaatctacaaattccagatcttccgggttaaccaggtgcgcacatgaattaaatacaggagttttatcagtagtcatatcaatctcattttttcggtgatttgtcccacgacttaaatcgaagttttgccgtgagtccggaaacagtattatctttcaaatactgcataatttcaagtttagttgcgccgtccgtttttatcatttcgttgatatctttggaaggccacgggcatttatcccacattacaaccttttctccagcctcaatcaatttaaagaggcggtgagtagtatccggatgacgtgcttcattgtcaagaacccagacacgcatatttttatacggaacctcagaaagtgcaagctgtccaccagtgatagcgccagcattatcaacaaacaggctatctaatggcccctcaagaagataaaccgtttttagcggatctatcgtatcctgtccgtaaatcttggttgattcttcacaggctttgattgtgatatatttcgactttgccccgtcgcgtaaagcacggccctggaaagattcaattttccctttcttatcgaagatagggatcactaatctcggttctggttttgcgatcggataggtatccggattcaccgtattaaccagttgttgccattcgcgagtaaaccacaaccgatcccacttgtcacgggggatacaacgattctgcacatattttatgatcggatgttcatccggcaaggtatctaacctttcgcagaattgaagagtaggaataaatttcttctcttccttcggttgttctgtatgcgttggctttaacgaattgcgatccttaaacgattccatgagataatcacggtaatcgtctggataatattctttcaggaatacgctaaacggtacaccataaccacagttaaaacaaccacaattcatatgatcaccctttttagaagggtagatccaaaatcgttttttgtacttgtctttcattgagtcgccgcaaataggacaacgcgcattgatgcttaatgcccccgatttacgaacgatttcgctttgaggcagtgatcccatgattcgggttgcaaattctatatcaagatacatttcttacctcagttgactatctttagatcctcgtcgattataccccgcgctgatcatttcgtcatgttctttttggcattcaatacaataacggcaacccttcacgatagccctacgtttttcgggtatcggatccccacaatcaaaacaatgcgttaatgattctccgtttctgatttgagaacgtgcaaaatctatcgcattgtctattgttgcctgaatggtatcttgaacaccgtcagcagggccaaatccaaccgccattgtaaatcctcctaatcaaatgatttcaatatcatagactaagaggatttttctgtcaagaacttacttgcttttctgttccgtcaagcattaacttccaaccacgaaatgcctgtttaaacgaataatttattgcaatatcaattttatcagaaccttttcgacgattctgataaacggtcgcgttgtcactcatatacatgatacaaattggaaaccatgtataatcgttagcagtagcccagatagtgatattcagcggaggaattatcatttctttttccttttccctgcacgggtaacgcctaatactttcggcccgatgttggttactgctccagtagtcacaccagaagcaatcttttctgtatcgccgccagaatcacccgcgaccatatcctctaacatgcgccccttatcataatattctttgaggcgtggaacgttcaacatgatttcttcatgctcttgttctgtcagattgtagcgattgcgtagggtatcatatgaacttgttaagttcataaacccagtcatatacggaacagaattcattctacgcttgatatggcgtactgaacgatgaaaaggagaatacgcttctaactcttcttttgttttggggttacgaattacttcgccttgaccatcaaggatccccagtttataagcagtccattcagtccagggctttttgagtagccggatcatccggacgctatatgttaaatccatatttttaactaattgatcactcatgattattactctattgtgaaagtgaataaatcagatttggtttcaggttcaaactccatacaaacaacctcgcatagtggtttaacccctttccaatcctccaggtaatacccagtatctataccgcatccaggattcataacgaggccagtttcatcaagaaactttttgcatttacttgatgtggtgctgtcatcttgtcggaaacagtgtgttttcgaataccggaaatttgcagacatttgagggattatgaaagttccctgacgcgcgatctgtgatgcacgttcgattactttatactcaaattccgcccctgtatacttacccttaaaatcagatgttttgattttaccaaaaggcggattactgatcgccatatcaaacacctgattaaattcagttgttaaggcgtctccatgcacccaggaggcttctggtacgatacgcttacctaactcatagtatgtgtgatttaactcaacacagacgatttcacgcggcgtattgtacatcatgtaatgaaccatagcgaaagataacccaccgataccagcacacaggtcaataacacttccacctgtgcaagcatcgattgtgaaatcgcgagcaagtccaataggggtaaagaacgcccctaattcagaattgtttgtaaacgcgccttcatgaaagttttcaataatgaacaacttctcttcgtaagttagcgctttgtcagagtgaaccagatccattatctgattgtgtttcttggtttctgctttcgttaactttgccattttcccagctatacaataatgttgattcgttagggtagaattcccatccgtctacatatccggtttcccaatcagtagtttgttcaaaaccacagatccattcatatacaccaggaggcatttcgacggaatcaggaagcccgatatcttccgcgctgcgtccacattcaaagaatgcatcatgaatgaatggtcgagataataccgtaacataaccttcatcgtcaacagctacgatccagcgggaactatgaggactatcgaacttcggttcttcttcgtctgcgtcagcttttatttcagccttacaaaaatctaaattcatcatttcaaaccctctttaacaccctctttcatagctttccaggtagaacctgcttcaccattcagggcggcaaatacaaataataagatagcaaggacaagattcacgccagcaatcaccatgattttgctatacacgaaaatgtaaggcattgccaccacccaccaactaaaagaattaccagttacgatgttgagtgctgcaagtaagaaagtgataacgaatgcgattttcataatgtcctcctttgttatgattaaggtatcatcttttttgaaagaatgcaatacctatagatacaaaaaagccccgaaaggggcttaattttttatgcgttattgatgagataccgaagaacgtttttcgcttgttcctcattacaaccaactttgaaaccaggttcgatagggaggaagttccagaggaaatcaacacttccttcaacgtcatctttgcctttttccagcatcgctaacagcaaacctttgtttttgatgctgtttacgattgcgtcaaaataaccatcgctgaaatcaacattcgggttcagcatttcgttgtaagggttgttgaatacgttcattttgaatctcctttgtttaactcagtatcttgtctacgtgagttatattaccacaatggagattcaggtcaatacctttttacgattttttgaaaagtttttcgtatttggcttttacccagcgatacatatcttcggccttgtcactggcaagcagtgagaacagcagatagatcgcagcacccaccaacacaacgcctactacaatgtagacgggtaagagaactgggaagagaacccagaaccatgacatttgcgagaagccaaacactttagcggctgcaaaaatcagagttagtccagtcagcagtttgatagccggaataggaatagttatagtcttagtcatttcattaccttacattctttatggggctattcgccccagtcaattaaaattgaatgtcagattttgcaatctgtgccattttatcacgtcgggtagattcagcctgtttaatcatcgggccttgtgtctgttctactgttttaggcatagtgttgccgtggtagtcagatttaaacccgtattcactgttgtcagtatccatccagcgctgattacccttgcgaacttccaacttgaacttgttgaaagtgttcttatcaccataacgggatttgatttgcttgaacagttgcataccctgatcagctaactcttccgtctcgattacagctaacataaaatcagccgtagcaggtaaaccagcggattccgcaacatcacccatactcacatccgaactatcccatgcagaacgcccaacctgtgcgcctgtccacattacggtattagtttcaacagcaagaccgcgtagttcttcggcaattgctttaaccagaatataggtattttcagcacctttaacgcgggttgaagtacagatccccaggtaatcgacaatgatcacatccggcacaaactgtttcttcaatttaagctctttcacaagcgctctaaagtggtttgcacccgcaccagatgtagggtactgcttgaccaccaaacgcccaaccttacccgctttaaggcgctccattttgttcttatagtctgcgtatgtaatgttcccttcgtcgatgtcatccatagtcacatcaagaaggttagcatcgatacgcttagagcaaacatgctctgccatttccatagaaatgtaaagaacgtttttaccctgttgcagataatcagccgcaagagaacataagcccagtgatttaccaacgttaacaccagccatgatgatattcagtgtaccacgttccgcgccgcctttggtgattgcgttcaggatcgggataccaaacggaattttcatcgccttcgattggtaaagcatccaccgtttttcataatcttcgaaatagtcatgacctactgaactatcgaatgaaattgctaatgcttcctccatgatttcagggatagccccaacaccaggaagtttcttgttctgttctgccagtggtttttctgcgttagcctggatctcgattgcgcgagaaagagcacgatacattgctttgtctttgcaatatgtttccgtttccttcattagccaatctaaatcttctggcgcatttttcagcgactgaatcgcctttttcgtgtcttcgtagactacatcacttagatttcgtttgtcaagcgcaacctctaaagcagtttttgacggaataccgttgaattcctgtacatgtttatcaatgaggtcaaacaaaacttgtgcattgccttcgaaatattcctttttcagatgaggccatgcttggacaaaatacgtcccgttataaatcaggttagaaaatattgtatcaacgatcattgtattgccttataccaggttgctgaacatcatgaaaaagttgtaaaccttttgtttgaatacatcccataatgtcagcttaggctttgggacaactgaacccttttcaagctctttaatctgtgcataaattgcatcatgcaccagcgggatcaacgcttctttgtcttcgtctggggtactgaattctactttcagaccatgatcccaaaacaccttatgaatataaaccagatgcgcaacacctttttcatcgttaatcagaagttcctgaataacatctttcatcgcttcatcaatataattctttgctttgctctcgatatccatacattgcctcggttatggggccgaagccccatagtttttataaaatttcgttgtcttcttcgatatcatcaaatgattctgggatatcgtcatcatccagatcaggatctgggatgctatcagtgctgtataaatcttccagcgcggaaccatcactgatttcacgatcagggatcttatacttttcttcgatagctttcaagaatggttgatgagtaaacagaggacgccagaattcaacgctatttgtttctgactcacgccatttcttttcttcaacttcgagttcgccagtctcggtattcaggaaagcacggttgcgccagcctttggttacggtctgtacaaagttcatttccattgccagatccagaaggccagaatacatactaataccgccttcataggtaacatgcagcgggaattttgatttctctttcacgaatcgagatttttcgatgttcatgatgaaatcataacccactacctcagtaccttctttcacctgttgtttacccaggatgatcgcagtatcagcggaatacattaaaccagtaccaccggaaataactttcttgctgtacatttcttgtgtgtcataggtatgacagatacaaaccatcgggatatccaggtcagccaaataaggcgtaaccatacggaacataccttttaatgcttttgctcgcgtcatatcctgtttatcgttatcagacagcgcgtcagcaagttcttttttacttgccgtgttgcctactgagtcaacgaatacaatcactttatcaccgcgttcaagcgcgttaagctggcttacaacgtcattacgcaactgctcgaccgtcgtgatacgagtatacacaacacgatccggatcaacacccattgatttcagataggatttagtaacacctttttctgaatcgtagaacaggcacacagcatcttcatacgttttgagataagccgctacagtcagcaaacctaagttggatttgaagtgtttggacgggccagcgaaaagggtaagaccagaagttaggccaccgttaaacgcaccggacaacgccagattcagaatcggcacacgggttcgcgtgatggtaatattgttgaatacgtcgctttcagaaagtacagatgcagtttggctattcgagtttttgatcagtttttttagtagtgctttgtttgacatttaatttttccgatttattcattctcattctatatatctcactagttaatgaaaggggccgaagcccctagagtttaccagtcaccgaacagatcgtttaaactggcacgtttttcataatcaattttacatacttctgtgatgttagtcaatggactaataacatgtttttcaaacatacccggataatctacccatgccagaatatcactttcgatctctgctggtagtctatttccagattgccacgcgatgcaatcagcttgccacgggtttttatcccttaatggtagaaccattaccttttcaccttccatgattggcgtaacaccatcaatatcagcagtgaaacggttaaagaacagcacccctttaatatggtttggtgttccttttattggatatccagccccatcacgatatttcgaaatgttgttggcagatgatacaccagcaatttccctgtagtcaagttccttatattcttcttcgaactttttataatgttcgtgtaaagataattcaccttcttgcaggatacggcggatcgcttctttcaggaatactttcacagaggtcggagtactcgaacgctgtgtttccatacccatgattttcaatttcggtttttcatagcgagttccttcggagtcccacacgttagccgcatatcgttttttagcagtccagaaacttcccaacccttcggaacccaacggaggcccagaaatgatttcacgatccataaacatcaggtgttccacgttgttcatgtattcgcaaagttcacgataccctttatcgatcattggttccattctttctttagcaaagcgatccaggaagtcaacccaatggttattatccttaaatttagcctcaccaccaacttttgcaatcacgttatccatacaaacataaatggagtcagtatcacagtatcgaacatatgcatgatccgtagtaccgcacaggtcgttaagatattcgtttaccttacgttcaatccactggatagccaactgcccgaacatggtgatcgcgctggcgtttcgtagatcgaagtatcggaagtgttcgttacccaacgcaccataaagggagttgatagaaatcttacggttaagctgtgctgtgttcgcttgtgcgatcttcttctcacatacgcgcttaactgctttaagcatttgttttgtaagagttttcagaactgctttcgattcatcactgaaatctgtatagaaatcaaagtcaggatcaatcatttggttatgcgcgtctgttaagtgttcgagttcgtgcttgatgagttcaagatttcgctcacccgccatcattcgttttttccacatcttacgctgatcaaatactttcttgatctctactgggatcacgcctttgatatcacggcggaacatccacccgttaggagaacagctaaattcatcgctagggcgcggcgcggtcttattaatatactcttcaagagcacgtaccgcaaaacttcccataatcgtttcagggctgatattcacctgtcggatgatggaagggtacaggcttgttaagtcaaacgataccatgtatttgtaaggcccaggaacgggatccttcacaaatgccccagggtaaggggttttagtatggcgtctgttttccggaataacaaccttatcttcacgcagagagttataaatgatcgcgtcccacgttttcagcggagacataaccccagggaagttaatttttgcatagtacgctacagacagaaccagttcaataaagtttcgtttaccgtcgatatcaagtacacggataacgtcaacaatgttgtacgtgatgtacagttggtgatcgcgctggcgtagttcagacagagaaccttcatactcaactttatttttaccagtttcgtattccgcgatcgcgtccaggcggtaagatggttgcggggtaaagctgaatttcttatacagcgccataccatccatttgagcaacgccgaaaatatcatatcctaattgttcgttgccgtaagcgtcagtagtggttctggcggttactttaccaaacgggctaaaatgccttaccacgttttgaccgaaaatgttcaggtatcgcgtgatgatatatgcaatatcgaatttgtcagagttccatccggttacaataacaggggttcgctctttccaatctttgatatacgcagacaataacgacttctcggtctggaaagaccgataaacaattttgtttaaatcttcttcgctaatatcttttcggtcaacgtttgccgcgcaccattcagcaaggccaccctcaaccagatcgtatacatagaatttatcttcgatgctatcgtaatgggtaatcgcatcgattggatattttgcttcacgtggatccggaaattctggggcggtcacctcgatatcgatagaagcaatgcgaatgtgttcgcggttgtactcaatttcactctggtacatgtcagaaatgtaagccagtcggtaatcatccatacctagagcttccatcccaacatcacgcatacgttgcatccagtttttagcttctttgatgctgtcaaactgttttttgaggcaaggcttgccgtaaatgtctttgtatggggtttctacgccattcatagcgtgttgatacattacgggcgcatatttcgtcttacgtacctgttcggtgccgttagagtcaacgaagcgctcgtaaatggtatctcccatttgttcaactgataggtaaaattcattcattggatcttgtcttctccattaatataatgttccattgtaacaccacctacagcaaattcaagtttactcgatgttctaaaaccaacaacccttctgctaacaagtcacggatctttctcagttgaacaagctggcgttcaagtttaaacccgtcgaataacatgctaaaaatactggaattgatactatgatattttgcttctgcaatgccctggttaaccatcatgatagctttgttaaccagtattttcctttccgttactgtatgttcatccagttgacaggttgcaagggaaaccaaatcatcataagcacgttggtcaataacgttatccatacgggccgcgaaaatcttattcatgtaagtgcggatcattgcgcgtcctccattcttttcataaagacttcttttgcttgttggatcaagcccagagattttttaatacgctcatagaaatgagtggtttcaacttgattgcataacaatgtgtactctgaaatgttacgatcgtaaaatccaggaaagtagtgttgtgcatagctgtaagtgcgggtatctgacagattgcaagttaacgataacaagatgtcatcttttacaatcgggatgatcaaagtttcgttggatttgattgaatccatgatttcgttaatagtcataatatatccctctcaatggtgtacaccaaatataacaaagcccttgcacgaatgcaagggctttttgattagtgaccgatccggtacttgtacttgaggatccaatctgctttttgcgagtgagtcagtacgcggaagttgttttcttctgcaaacttcaacccagtggttacgatcttaaccatgccccactcttcgagaagtcgcgcaatgttgttccggcgtagttcgtcttcttccgtcatatcgacttgacgaccatcaagtttcaacagttctttaaaatgcacgataaaatacttaccttgctttttcagaatgtggcacgattgccagagcattttctttttgttgttcgcaataccaatacgggttagcgtttcacggatctttaaaaaagaatcgtcgctgattagttgaatttctaacatacatcaccattgtttaatcaatttttccaatttcttttgttcagctttgtttttcacaatacccaacaaagacagagcgacctttgcgtgttttcttttccaatcctcgaacattccgaggtctttaagttcctgcaaatattccatcgctgtacgtgtatttacactgtatttttcgcgaaggatttcgataataattttctcttcaaaatcttccgatagtttagcccatgcaccgaagcgtttagccttcctaacagagttgagataatagttatagtgcatttggtcagagatactaccgcctaccagattcatcacatacgcgttgtatatcgtgtctatgtgctggctcattgcgttgtctacaaagtacttatcatacacttcatcgataaccaacggcgttttgccgttgttgatttcgtctatgatgttaaacaaggtgttttctttatccttgccgtactctttgaccagttcttcaaccttatcccaatctttagaaagccaagcggattcatgcggggataactcttcttcatccagaaattccgccaggctcatgattacgcctcccagaccatagaaagcatcaggttcatcaacagatattgcagatgaatttctttattcatcgccagcccgtattgcgcgttgttttcgcctacaatctggatcagtgcgattttagaatcctgattcacgataggataaatcgtatcagtcaattttccgataaaggtatcgtattctgacgcatatttaataacctcagagcgcaaccctttatagttcttttctttcaacagggtaatgatatgagacacatcagaaccaacgatctcatttaggatccccgcatcaatttcaccacgtttcgagtagaacccgatcgctttgataatagaacgcgcatccggataatgctctttaacaaacgctgcaatgactttaggatcatacttgatattctcgatttcaaggataccgaaacaacgcttgattaactgtttcatcagttcgatacgttcagcatcagacggaacaccgaatttaacaggaggacaacgagaaagcagagcactatgcacaccgttaatgttgttcgccgttacaataacagaaacgtttttactgtatgcttcgataaagctacgcaagtgtttctgtgcttccgccataccagaacgatcgaattcatcaatgatgataatctttccgcctggtttctgcgtcattgatgaagcaaaacgatccagttcattacgaatgaagtttacaccacagttcgaaccgttgacaaagaacacctcagcatcaacctcacgggccaacacaagcgcgagggtcgttttaccagtgccaggggaatcagatacaagggtcatgttctcaacacgcccagatttgattatgccccgcatagcggctttgtcaccagaaggtaaaatacactcttcaatcgttgttgggcgatagcgctgatcccatgcaaattcatcaggagatcgagatattttaccgtatttggtttcgatgatttcaatattttcactaagttccataatataccttcaaaataaatggtgtaaaagaaaggggccgtagccccttaaaactatcttacttgaatgtgctacttgcttcaagtactacgacgtaagcaacgccgttatcagaagagaatttcgcggcccctttggaggaaatctctactttgtaatcgctgttgatgaactgcatgttatcaatcttcatatcaaaattgaaaacattgtcgccttcatactcaccgacttcaacagagaaagttgattgactttctttgcttttcgcggtgatgaccagtttaccatcaatcggttcaacggacaggtcggtcagtttcatcatgcgagacgctttgatcagtttttcgaaatcgttagccgtaatctggaaaatcagatctgctactggcatcaccaaacgttttttcggtttcgggatcgtggttgcgtctgctgaacgttcgatgatcttcatcttgtcaccgcgaatcacgatttcaccagtggaaatatcgtgagtgatttccgcgtcagtgccgacgatgttcagcatgttcaggaatgagttgagatcgtagataccaacatcgtcatcaatcacatcagcaatttcagcttctgcgtatacaacgctgttgattgatttcgtcatgatgaatgaacctttggtcagcatgatcgaagagttgatttgagaaaagtttttcaggatatcaatagtttgtttagagaatttcatattcagcctttagttttcaataagtgttacttaataagtgattttacaacggtttccgctgctgtgtcaagcatatcagccatttctttaacggttgtacgcttcggatcttcgcggcgttcgctggtaagtttacgatgttccgcaaccactttttcatcaatgtcacgataatgtttaaaacgttcctcttgaggcatagctttaaacagttcttttgtttcgtccgagagtttagcaacccaggatttacggacgcggttcatgtagtcaacaaaaacattactttcattcatatatttcttctctaacttagaattctttgagtgggggccgaagcccccgcttgtattacatgtctaacagtttatccaggtcatcatcaccggagctatcagaatcatccagatcgaacggtacgccgtcatcttcacctaccggaaccgatgcaacaccaccagatgatttcacatcagatgtctgattgtcaaacttagccatttcgttatcgaagttgctcagttcgctatcaaggtcagcggaagcgctggaaccagcagaaccgatcgaactacccataactttattgaagcgagtagtcaggtcagccagcggtttgaattcgctttcggcagtgatcgggcggagatcgctcataccttcgaaaattgctttctgaacttcttcatcgtcgatgtttttgatcttagccggaacaccaaacgagctatcgtcatagttaggccaatcaccaacttttttcgctttcagggtgaagttagcaccatcaaacggacaggttacagcaatacccggttcatcaagttctggattaccgttaattgcggcggtgatcttgtccatgattttcttaccgaagcggtatttgaacaccttaccttcgttttctggagcgcctgggtctttaacgatcaggacgttagcccagaaactttgtttacgaccgatctggctcagtagcttatcttctggcccgtttttgttggctttagccttctcatacagatcgttttcggaaatgtacttacatgcaggacagccgtcataatcgccgtgggtagaggaacagttctcaatgtaccactggttgtttttcttgaaagagtggctcacgatacggacgaacgccagttcatcatcggaacgtgctgggaggaatcgaataacggcggaaccgtttttctgtgcgtccagggtcagtttccattctttctcatctttctggaagccggaaccacctttcagatttgctacctgtgcctggagtttagcgggatcttgacgtttaaaaatgctgctcatattctgttttctcgtttagtttagtttgattaacgtttgtttcattaagtttcgatattttatgatatctttttcagtaaggtcaaatatttttctgtatgcctttaacttaatgctaaagtcagaccaaataatatcatcagctacttgatcgtgtttatttatgatacctaaaaatgagtcaaaaatcaaaaacgattcgtaagatatcacatttgacaggacaagtttgcttatgtaggacgttgatgatttttcgctgtacttgaacaccagagacacggggatctctttcattttggcgaattcgtacacgtttttaacgtcatccacaaacacgttatctagtctttgtaactttcctatgtactgcctgtaaaagacaatactatcttcatcaacatcgcctacccagaaatccggattggctacgaagttggagaggaatataaaatagatttctttgaatgtaaagcgttgagctaattttacaaagaaatatctatcctttcgcttgttaaaggcgttttcactaactttgatctgccagttgtattgaaggacatcaaaacgcccctggaaatgagttttcatcgccagatataacttgtatacagacaaaggcacaagccgtgaattcgcctcgctatcagcaaacggagctttgaatctcacatgaagccgtccagagtggttgatgaactatgttcaagcgcaaccgatgggcgaagcatgtttcctttgatcgcttcgtcgctaatcttatcaaggatcgcgcgaggaaccgttttattcagcatcgcataatcaatagaattttcatccatccattgtagcgttgcttccatgtaggttgccccctcagaggcaaccagattttcgatatacaaaccgacttcggtcttatttccgatcatgctttacgccttatcgatcatatcatacagttcgatcagttcgttgttttcttcttcgaaagcggtacgggcctgttcgtgatacagtttgaacagtttcccgaaggtttttccatcgataccgaaatcagtttttgctttggatttgatatccttgaacgtaccgttgaagatctcaacttgagttttcacgttggatgcttctttgatcagttcttttacctgttttgctacatcagggtttgtttgtaaaaattctacactcattttgttacctcaaaaatcactcagtttttcgaacatacgggaaagtttgttatccatgaagtaacgttccattttggctttacttccggattttggagtattatacgcttcaataatcgaattttcaatatcttttggtataaattcgaaatcgcgtagttcctcattttctttgtaacgtgcggcccattcaggggtcatcaatgttgtcggatcgtctgcctccagccatgcctctaactcagaggattttaccgctggggcgcgttcaccttcaaccttcgtcacaatataatcatttctaattttaatgcaagcgatactatcttttttatcgcctttgatatttttgtatcgcagatcgttacgtggcgaaccgtacttaggcgttacccattttttctggggaggcgaccattgacgaacaccgttatatttctgtagttgtgtaaagtcgctatcagcagaaaccactaatactcgtctaccttcaccaacagcttttttcgtaacaacagcaattatatcatcagcttccgcgaattcaacctttaatccgagataaggcatattctgacggatttcttcgaacacagggttcaggaagttgttcagacgatcccaatcccattctgattcttcgtgttcgatctgacgacgttttttgtagtaccaggctttttgcctacgccagtaatttctgtcatcgaaggcaatcacgatttctggatactcacctttaaattttacaacgttaaaccgtaaagtgtcaagcaccagatgacgaatcatttcgatcgtgatggatgcttgttcctttggtttgaagttgttcatcagtgtagcgatggaaatgttagagatatcgatgatcatagtatcatcgggttccccttcatcttgcatcagcttgttcaagttaaacatgcttgcaaaactgctcatacatacctcaatttttcaaagaacggggttattgtagtaacttacgaaatgaagtcaatacaaaagaccataaaaattttgatcaataatacttgatctgatcaaatttatgatctataatttattaattaataattattttactacaatgatcattgtaggtcaagtactaaaatcaataaattttatataatttagatctgatctatagatcattagatctactttaaccttaaataatatagaatgaaatttgattttgtctacagttattatataatattcttaacttcaaagaggaaatatgaatactatgactaaagaaacaaccaatatctacgcagacaatgaaaaattataccctatcctctgtgcatggaaaaagcaaatcgccgaaacaggtgatcgcaaaatgcctaatgagttgggggctgctattatggatattgcaaacgggctatcacgtcgttacaacttcaaccgttattccgaagattggaaaatggatatgatcgatgacggaatttccgctgcaatctcaggactgcataacttcgatgaaactcgttataccaacgtttacggttacattaacaaagcatgttggcaagcattcgtaacacgtattctgtacgagaaaaaagagaacgcgaagaaatataaattcttccttgagcacgtttacgactgcgaagattcggatatggttagtattgcagacgaaggtttcattcaagatctacatgacaaactatctcagtacgaggcttccgccaccaaaaccaaagacaaggaagcggaagtattcccaacattggaagattttctatgaaagcaataattgacttaaacaaaatattaactgatatcgattacgaaattgacttgctaccctacttcgtaaaattggagttgcaaaacgtgggaatcccggttatcatcgatccaactgacgtaagaaaccccgatttcgaagtagaagaaggggttttgtcttatatgataaacgccgaaactatgatcatggagatcacttatgattgatgaagagaaagaagtactaaccagtgtggaagaagtggatccggaagaggaaattcgacaaaagatccaggcacgtgtagaagccgacgcattgaagcgagcacaaaaattcattaagaagaaccggactgagatcaaacgcctccgtagacacgcagaggaagccctattcaggggtaataaagttcagtatgtgtatgcggttaagaaacttcgtgatatgctcaaacagccgtatacagaggatttcattgatacgatgtggaacacttcactagcatcaattcgaaatatcgtagcttcacaacagaagcaataacaaacaagtagccccgaaaggggctatgagggtcttatgagaaagtacttaatgatcggggatactcacgctggcttgcgtcaggacaacccctggaatgaagaaaacctatacaatgtattcgtacaaatcgtagaacactgcaaagcaaacggcattaccgaggctttccatgctggtgatttctttgatgtgcgcaaggccaccacacaaaccacgatgaaattcattcgtgaacgtattgtgccactactggaagaagccggattacatatctatgttctggttgggaaccacgattgccagtttaaagacaagatccgccctaactcaccgcgagagattcttgatcagtatgattgcttcacggttgttgatgaaccgatgacagtaaatcttgatacttctccgctgcaatcaatcgatttgatcccgtggatttgtcaagaaaacacacaacagatttttgatttcatcaaaaagtcaaaatctcaatactgcttaggacactttgaactgtccggatactatttctataagaacagtaaagcggatcatgggcttgaacctgatttcttaaagaaatatgatatcgtgtattcaggccactatcatcacgctaacgaaggcgctaacgttttctatatcggtacacctcttaccatgagtgcgaacgatgaggacgaaaccaggggcttctatgagctatcttatggcgacggtaaacgtgaattaactttcattgctaacccagtatgccaccatcgccggatcacctatccggatcaaaaagatgttgatgttgcagattacaaaaattgctctgttcgcttgattgtgcgcgaagttgataacgatttgcctaagtttcaaacaaaactggaagaaacagtttatgagttgaacattgtcgatcgcgtgatcactgattcagaagtcgatactgattttgaaatcaaaagtgtatctggattgattagtgagtacatcaacaacatgcagatcactccagaagaaaagaccgaagtatctgcaataatgagtgcattgtatgcagaggttacgagcaatggaaatagttgattacgttaatattttaaacgaagaagggcgatataaagccctttataaaatgtttggatttgatgtgattgttgcagtacagcaggattcctataatgagtatgtgtcattggggttcactctgattaaagacaactatcacgaaacaaaggtttggacatttactgtcctgaatagcatggatgaagattccgtgatatactgctttgatagcacgattacaaacatgattagtgatatatcccaaaggataattgatgaaactcaaatttaaaacattgacttatcaaaatatcttgtcggttggtaacgtaccgatcgtcattgattttgattcagcaaagaaaaccctcattacgggtaaaaacggcggtggtaaatccaccatgatcgaagcgcttacatatgctctctttggtaagtcatttcgcgatctgaaagtcggacaactggtgaacagtatcaacaagaaaaaatgtctggttgaactgttgatcgaatacggtaatgatgaatataaaatcatccgtggacaaaagccgaaagtatttgagatctggaagaatggcgaaaaactgccggaagattcagccgctggtgattatcagtcacagcttgaatcaatgttgaatattaacctggtgggctttaaacaggttatcgttctgggtactgctggttatgtacctttcatggaactgaaaacaccagatcgccgtaaactggttgaagatttgttgtctttgtctatcatcagtgaaatggacaaactgaacaaatcatacatccgtggtgttaaccgtgaactggatacgctttcaatgcagattggacacgtacaacagcagatcgcaacacatcaaaagttcattgacgaacaacgggcaaaagcaaatcagaatacggcgcgttaccaggatatctacgattcccacgtagaaacagcaaaacagattaaagcgcaattagttgaacttcaaacccagatcgcagaatgtgtgatcaatggtgaagaccaaacagcaaatattcaaaaactgcgtgatggttatacgcggctctcaatgaacgtagaacagttgcaacgtcttgaggtgatgtatcgcaagggtggcgaatgtccggcctgtaaacagccaattagccccactcctgaacgcatggaagagattgccgagaatattaaaaacggtactcagaaacttacgctgattaagaacaaacaagatcagctacagaaaatcatggatgatttactaacacaacaacgtacactaaatgggctgaaatccaaatacgaatcactacgcggtacacttcaaaatgaagttgcagcggctaaacgtgttcgggctgtcatggataaagcacaggaagacgtggtgatcgacgaatccccagttgaaaaactccgtgaagatgaaaaggaacttgattccaaacgttctggatttgtcaaggaaaaatatttcagaggtattgttacggatctgctgaaagattccggcgttaaagcgagcatcgttaaacgttatattccttacttcaataaacagattgcgtactatctggatctgttgggtgctgattatcagttcactctggatgacgaatttaacgaatcgattaaatcgctgggtcgtaatgattttagttacgcatcgttcagtcaaggcgaaagagcacgtattaaccttgctttgcttatgacgtggcgcgatgtaaccagtaaaatttctggtgttgatttatctcttttgatattagatgaaatttttgatggggccattgaccgtgaaggtggatttgctgtgaaaaaattacttgatgatattgaaggtaacgttattgttatcagtcatcaagaactggatccgcaagatttcaacaggcatattactatggctaaagttggtagatttactaaatgtacgattataaacaatgattactaaaaaatgggacgacgaatttcaagccgagattcgtcgtcggttttaccatgtaggcggggttttgtatcataaaacagagagtagaccaacggtgtctgttcctgctggctactattttaaacccggtgatgtggtaaaattcaacaaaacgagaaaaaagaatccgtacttacagatttgtatgaggtatgaagggaaatctaactatctgtacgtgcatagagttgtctggtttttagaatacgggtatcaagttgatcttattgaccatattgatatgaatccattcaataatgatccttctaacctacgagaagccacgactcaacaaaatcactacaataaaaaaggaaaatctaacacatcctcaatatataaaggtgtatcatgggataaaccaacttgtaaatggaaagttggtatacaatacaataggaaaaagatccatttaggatattttgacgatgaaatagaagctgcaaaggcatatgatgctaaagctatagaaatcagcggaaaatacgcgaggttgaacttttcatgaatatgttagaaaaatcctttgaattagaaaccgctctggaaatagatcggttttatctccacaacaattttcttgaagaaaaacatatagttactatgaaagatgttgaggaagcattcaaagataaccctatagagttgacgcgaatcaagaacaacaaaagttctgtttggttcctcgaaaaaatctattgaccgaaatccataaatacagtaaagtagcccatgtaacgaaacgtgggctttgtttttatttgaggaacaataaatgatcactgaatccaaaatgacttatcaggaagcactgaaagttttgggcgcaactggtagcgaaaccagcgccgaaatgtccagactcttcaaacgcgcatccttacgcaatcaccccgatcgtggtggtagcaatgaattaatgcagaaaattaaccaggcttacgacgtagttacaaaaactgggcctagtggcgcacgttctgagactgctggtgatgttcgcgcacgttatgcacgtcaaaagaaagaatgggaagaaaaagttgatgcttactttgtagtggcgaaaaactatttcagcaccaaatttaacgcacaggaatttgcggaatacttcaccaaatacactggattgcctaccactttcaaacaggaagtaacaaaaggtagtcacggtgtttatgcttcgttccgtttcacttctggtgatgcttactttgatttcggtttcaactgcacccctccgaatggacaagggttagccgctccggattcatctgcactgggtaacgtttctgttagtacctttgtactggttggaactaaaaaacataaaatggcaagccgtgattatcaatggggcaaaaacccagataagatcactccggaaagcctgttcccgtctaaaaaactggaaagcattttcagccctgtacagaaaaatatcaaatacaaacgtgctgattaccttgcatcattccgtaagctgttaggcgctgacattagcggaaacgatatctttgttgaagttggtacactgaaagttcgtttctatcgtcatgtaatgatgcgtaaaggtgcgtatgtgtttagcgcggtgtatgatcctgctgtatctaagtatcgtccggctgcacaacttcgcggaactatgttagaagacgaggacggcgcttgcctggatatgatcgttgatacgttcaaagagttgcagaaactgaaaccgagtgttcaaggcgttgtgaacgcgatcgataagatgaacgcagagtttgcagcgggacatcgttcagcatcttttgttaaacgtgtagctgctcaggaagccgcgccgaagccagaagagaagccaaaacgcactgttaatcgtatcggtaaagaggaatacttcgcagcactaaaagatattggtgctcgtgtaatgcctaccagcggttatgttgaatttgataacggcgctggtgttactatcaacttcaagcgtattgttgtaaaccgtaaagcatactactcattcagtagctttgatttcatgtactctggtcagaaacacattgagtggttgaaaggaatcgatatcgcagaagataccaaaggcgcaagcattagcctactcactgatactctgaaatctttacgtgggatctctgactggaacactgttaagagcgctttagatcaaatgaattctaacttcaaggcgggtaaattctccgcacctcatgtgaagaaggaagcagagcaaaaagcaccgaaacagaaagacgaaatcggcgcacagcctaccaaaccacaggcggctaagaaagatacaccggaagtggaaaaatcacaggctgttcatgcagcacgtgagaaagcgaatatgaacaacactattcgtaaaatgatgactatgttagtcaaagcacagcgcaaagacactccggaagatatcaagaaggaagttgatgcagcaattcaattgtggcgcttgacttactaatcaaatgaactataatgggaactgttaacgcagttccctttttatttgaggaaaatattatgagttgtccaacatggttacgtttggaaaatctgaaagaaggtacacaaaaacggatttatattaatcttggttgggttcctcctaccgattttcaaatggctgagattttaatcaatgctgttaaagaagtaagcgacacttacgaatgggaaaggctctattttcccttgattggtttgtatatgacgcgaaataaatttgaagaaatgaaacttgctgttattcgcgctacgattattaattcccaacaaagatttactttgaaaaatgcatggagttctgaatgattattcaagtatctgtacagggtgacactctgactgtcacacaatccatcaataccgctcttgctgtatgtcgtgaccatatctcacaaaatcctccagtgactgagatcctggaaattgatgtttgggatcagattgggatgatcgacgcatcatatggatttaccccgcgagatgaagaactatctcgtatcgaatcatggctgaatgaacaggaaacggaatgaaactccctaagaacacaacactactaacccgcgaaaaacttcactctgttgattggtgtcctctggatatcatgatttttgatattgaatctcgcgtgatcaatgcaaaatatcaggggtgtagtattttctctgttgaattcgagaagattcgcgggtatgatgagaagtacaaagaaaaactgaaagttatgattgaagcattgggctatattgtaactgttgaagacaacaaaatgtggatcgcaatatgagcatagtaaaagcggtgtttgcgctggggcatgatatctaccacgatgatttcgcttttggatatcagcaaggcttgccgtggggccactgtaaagaagatttacagaacttcaaagaagaaaccgccgatagcgttctgattatgggtgcaaatacgtttacctctcttccgggtaaactacttggtagaattcattgcgttctgtctggttccggtagttttttgaaaaccaaaaaaggcgaggttgctgattacgtgatccacggtggcgggttgtctgctgctattggtacaatgcaagcaacacacccagataaaaatgtgtgtgtcattggtggtaaggggttgcttttagattcaatcaataataaaatggttgatgaagtagttttgacacacatttacggacatgatgtatataatgcccccgcatttaaacgcgatgtttcgtttactgcttctgaattgggtgatgcattgttaaaatatgaattttctgatttcgaaactcagtacatcaaagaacatgaacgcattgaaaaaatcatagtcgatcgatataaaaaggtataaaatgaaacagtatctggatattattaaacttgtacttgataacggtgttgaatcaaccgatcgcactggtgtaggtactattcgtattttcggcgcacaagcccgatgggatctaaacagaggtttccccgcaactacctgtaaaaaactattcttcaaaccgtgcaagcatgaattgcaatggttcctgtccggttcaaccaacgttgaagaacttcgccggatgacctggggtgaaaatagcgataagcgcacaatctgggatgataactatgaaaaacaagctattgatttaggatatgattctggttatctggggccaatctacggtcatcaatggcgttcgtttggttctctttatggggatgatgatagttattatggcggtagtggtgttgaccagatagcaaaagtcattgaacaactgaaatcaaccccagacgatcgtgggatcatcgtttcggcatggaaccccgttgatcttgatgatatggcattgcgtccgtgtcactgtttctttcagttcgttgtaatcaacggtaaactgtctctacagtggtatcagcgttcagttgatgtcttcttagggttgccgttcaatatcgcctcctatgctctcctgacgcatattatcgctgatatttgcgggtacgaagtgggcgatctggtttggactggtggtgatgtccatatctataaaaatgcggttgaacaggcaaaagaacttttacagcctaaccgttcaccaatgccattaccgattctaaaaatgccgaaggtaaatagcttacttgatttagatcaagaattctttgactcgataaccttagaagggtatcataatcacggctctctaaaagctgaaatggcagtatgaaaaatggggcttcggcccctttcttaacaaggtaagagaatgaatgacattaaagtagtagtaaaatcctctggtgtacgccagccgtttgacaaagaaaaaatatacaaagtgctcaagtgggcctgtgatggtcataatatcgatgttcgtgcattccttgaaaatgtattagaactgatccgcgatggtatgactaccaaacaaattcaacgtatcgctatcaagtatgcagcagatcatatttctgttaaagaaccggattggcaatacgtagcatcgaatcttgaaatgtttgcattgcgtaaagacgtttacggtcagttcgatcctatcccgttctacgatcacatcgttaaaatggttgaagcggggaaatacgataaagagatcctggaaaaatacagcaagcaagatattcaagttttcgaacgtgcaattgatcatgataaggattttgaattttcgtatgctggttcccaacagttaatcgggaaatatctggttcaggatcgcgatactggcgaaatctttgaaacccctcagtatgcgtttatgcttattgcgatgtgtctgcatcaggaagaaactgggttagcacaggttacgcatatcgttgatttttataacgcaatttccgatcgcaaactgtctctaccgactccaattatggcgggtgtacgtactcctacgcgccagttctccagttgtgtagtaattgaatcgggtgattctcttggttctcttaacgctgtaacctctgcgatcgtgaagtatatttcacaacgtgctggtattggggttaacgcgggacatattcgcgcaatgggttctaaaatccgtggtggtgaagctgttcatactggtgtgattcctttctggaaacatattcaaaccgctgttaaatcctgttcacagggtggcgttcgtggtggtgctgcaacactgtattatcctttctggcatctggaagttgaaaaccttctggtgttgaagaacaacaaaggcgtagaagaaaaccgcgttcgtcatcttgattatggtgtacagcttaaccaattgatgtataaacgcttaatgaatcgtgattacattacgctgtttagtccggatgttgctaacgatcgtctgtatgatctgttctatgaagctgatcagactgcatttgaagaactgtatgaaagcctggaaaaagatccaactgttcgtaagaaacgcatcaaagcggttgacctgttccaacttttagcacaggaacgcgcacagacaggacgcaaatacattttcaacactcatcacgtcaaccaacagggtagttttacggttcctgtccgtatgtctaacctgtgttgtgagattgcgatcccaacgtcgccgctggatgacgatgataaaatggctggtgaaatcggattgtgtacgctaatggctatcgttctggataacgctgatatcagcgaattcccgaaactcatgcgtattgcagtacgtgcgcttgataacctgttggattaccagaactaccctgtaaaagccgctctgaaagctaaacagcgccgttctctgggtgttggtatcaccaactatgcatcatggttagcgagcaactattgcgactactcagaagcgtatacagacaaagttcatgagctaatggaagcgtttcagtttaaccttctcgttgcttctatggaactggcgaaagaacgtggtgcatgtggattgtacaacgataccaaatacgctcgcgggttactgcctatcgattggtattgcaaaaccgttgatgaactggtagcacctgtttataattgcgattgggaatggttacgtagccagattaagaaatacggcttgcgcaactctactctttctgctttaatgccttgtgaaagtagttcacaggttagtaactctaccaacgggatcgaacctccgcgcggtttagtgagtatcaaatcttcgaaagaaggacactataaccaggttgtgccgaaccagaataaccagattgatttctatgatctgctctgggatatggctaaacgcggtaacaaagggtatctgtctcatgtagcagttatgcagaagtttgtcgaccagtctatttctgcaaacaccaattatgacccggcaaactatgaagacgggaaagttaaaacagaagacatcattgatgatctgctgtatgctaactactacggtgttaaaactctgtactatcataatacgcgtgatggtgctggtgatgaagatgaagccgccgacgattgcgcgggttgtaagatttgattaatgccccttcgggggctttttaaaggtaaagacatgttaacagtaatgaatacaaacccagatcataaccacttagaacaacctatgttttttggtgaagatactggtgttgcacgttatgaatcgcagaaacacaaagttttcgaaagcctgacgcaaaaacagctttctttcttctggcgtccggaagaagtcgatctgtctactgaccgtatgcagtatgcaaaacttcctgaacatgaaaaaatcattttcgattctaacctacagtatcaaaccctgttagataccattcagggacgtgggcctaacctcgcatttttgccaattgcatccgatgtgagcatggaaacctggatcgaaacgtgggcgtttagtgaaaccatccacagccgtagttacacgcatattcaacgtaacttgcacattgatccttctgtacagttcgaccaaatccttcgcaatgaagcgattatgaaacgttctgcatcaatgacacggtattatgatactctgattgatgaatgtcataagctgaaaaccatcatgatgctacaggaacaggttagcggctataaaccaaatgatccggctgtcgtgtattataacgagcaatacactaaacaggccactaagtgcaaagaagctctgtacctgtgtatgcacgctgtgaacgctctggaagcgatccgtttctatgtgtcgtttagtttcacctttaactttgctgaacaaggcaagatggaaggcaacgcgaaaattatgcgcctgattgcgcgtgatgaagcattgcatcagaaaggtactcagagtaaaatccgtttgtggcaaatgggtaaagatgatccagaaatggttgaaatctcccgtaggctgaaaaaagaagcaacggctatcttcctggaagtatatgaacaggaaaaagaatgggctgaacatttattctctgttggtgatgtagaaggtgtatcgctgaaaagcactatcgcttatattgaacaccttacagatcagcgtatgcgagcggtagggcttgattcgccattcaccccgatccctaacccgtatccgtggatgaataaatggctcaaaagtgataacgtacaggttgccccgcaagaggttgaagtaagttcttacctcgtcggaaacttgaatactgaaatcagtgatgaagcgtatgcaaaatgggccagcaaatacgcgtgattgtcgggtagtaaacaagtacaaaactgattgggatgtcgatattcaaagaggtacgaagttcggaaacccttatcacacaggaaccaggggagaaaacattttagcgtttatcccctggttccagaatcaggttcgtactggggcgatcacgattgaagaattgaaagaacttgatggaaagaggcttggttgtacctgtgcgcctcttccctgtcacggtgattacatcgcgcatgtggttaatgttttgtgtggtaagaaaagatcacttgactttttggatatataatgtatgaaatctgaattcaacttaacccttgataaatgtggtcgcatcgatcgaagttttgttaagtgtggtgaacttaggcattgtgtttattttattgcaattaacgatgaaatagtatatgttggtaagtgtagggatatgtggaagcgtttagacacatatcgcaatgcaaagtattggagagaagccaaccccagcaacatcttaaaaacgtgtcgattggaaatggctatcaaaaaacgaaaaactgtgaaacttatcgtgactactcacgatgaaaatacatatcatgattatgaaatcaacatgatacgaaaatacaaccctgaatggaataaacagcactatgacaaaggcacaaactaaaattatcaataccctttacaaacaactcatgcagttgtgtggtgaatccgaaacatttttcttcgttgatcaagtaaccgtgatgggtacacctgttcgaatctttaactatcgcatggcctcatatacagactggctaaagcctggtgctctggaatgtcgcggtatcatgtttgaaatggatggagatacccccgtatcaatcatcagccgccctatggagaagttttttaactatgccgaggtaaaggcatgggaagcgcttaacgagtctcctattgaattaggcgaagttttagacgtgatgattaaagaagatggttccttgatctcaactttccttgacggtggatttctggcggtcaagtctaaaggttcggttaaatcagaacaagctatggatgcgcacagcgtgttaatggcaaatcgtgaattactgacccgcttaactgagatcgctaaagaaaactatacggtgaacatggaatacgtttccccgaaaaaccgtattgtcgttggttatgattctcctgatctgcgtatcctgaacgttcgtcacaacatcacgggtgaatacatcccttatgatgaactctttgctgacgcgctgttacgtgcgtatctggttaagcgtgagaatatcgaagtactggatctggatgcattcgcaaaagaagcatatcagaatgaaggattcgaaggctatgttgttctgacaacgaaagggtttgtaaaaatcaaaacaaactggtatgtcaacctgcatcgcacaaaagatagcatcaccaacaataaggatcttttcctaaatattgttgagaatacggtcgatgacctgaaacagctattcagttcggatctggtctctctgaaaaagattgacgatttcgaaaaacttttccttgatagtctcaatcgtttgagtgcaaaagcattcaaagctattgaagataataaagggaaatcgcgtaaagattttgctatcagtctaagcgcggatttgtcaaacgacggtcggatcatcttcgggcctcttatgaagtacttcgaagaaaccgatccacaaaaactggtcgatcgcatcattgaaatgatggttaaaaattacgatcagttcattcctgaacaatataaatgaggttcataatgcctaagatatcatcttgggtatggcctgtaatcgtggggctatctttgatagcccttttttacattgcagtcgataccaaaattgaaaatgcatcattacgcaaggatataaaatctttgcaagacgatgtgaagaaagtaaaagagacaaatacaagcaatactgtgatctatgtcgaacaaaaaggtaaggatcagcagttggtcaaggatgccggacgtaaagatctgctgtttaaaaaaccaggactgatcgaaatcaagatcaacaaatccttcgaagagtatatggcggaatacgacaaatgaaaattgcaacgttagcccttgttctgggcgttctgttggtcgggtgtgctgagaagcccccagaaaagattttgcctacgctccccgctaaggtgaatccggtgaatgtgaaatggaaagtggttgcagaagtccgagagattgacggtaaaaaataccttgtaatgccctatgacggaaatccttatgttgcattatcatatccagattcattgatttttcgtagctggatgaacgacgttaaaagacaaaaggatcagaccgataatgttctgtgtactttgggataccctgagaaatgcaaatcaaaataaccaaaacattttttcgtgacataacagaaggaaaagtttatactgcgaaaaaggataaagaaggtctatggatagaaaacgattggaatcgtgatatatggctcaatctgacgaatgagtataacaaagaactaattgaatatgagatagtgaaatgaatctgtttatgactattggcgttccgggtagtggaaaaactacctgggcgcatgagaaagcccgtgaattgggtaatactgttacgatctctcgcgatgatctgcgtagctctttgtataatgcgggtaaaggtgctggcggatacaaatacaccaaagcgaaagaagacatgattgcagaaatgcaggatcacgttgttatctccactctgaaagatggtaaaaacgtgatcatacacaacacacatctgaaagaaagtgataaaaatcactggcgtgaaattgcgttggaacacaaagctgattttcatattgaatattttgatgtgtctattgttgaactgcttcgccgtaaccacaaacgcggtcgtgatgcattacccgtttcgcgtctttgggaaatgtttaaccagtatcgtaagatccgtgggttcgtaccagcaatggaaattgttaatccccacaatcagaagtgtgtgatctttgatgtcgatggtactctaaccaaagtgggacaacgtagcccgtatgactttaccaaagtgatcaatgatccgccaaatatcccgatccagcaactgtttcacctgtacaaaaatgcagggtataagtgtgttgttgtgtctgggcgtgaaggtaatccgcaatgcgcacatgatacatgggttagcctgttgagttatggcgttgaaccggatgaaatttttatgcgtcaagaaggtgataccaggacagattttgaagtaaaagaagaaattttgtttgacaagattttagataagtattatcctgttattgcagtggacgatagagacactccggtcggaatgtggcgagcaaacgggattccgtgcttacaagtcgattatggtgatttctgattgacatataatgtgggtatgttaaagtacccacacaaaagaggattatattatgaacgttattcgtgaagataaacacatcatggttgaacttggcgatcgcattcgcgtagaaaatctgggcgattttaaccaaaaagttcgtttgttgtgccaaaaaattgctaacaaaattcaggaacagggtaaagctccgggcgggtttgaagttagcgccactccggtttctcagtactcctatattgtgtatattcatgacgtggatactaacagcacccaatctttcgggctggtgttaaatcctattactggctacgttacatgggcggctgtattatgaacgtaaaaattattgatagagcggtaattacggacgaatctgtatacccggatcctcgttattatggcggtgttttcggatacatcaaaggaactgatattgatgtagtaacaagtccgattgcagaatatgatatcaacaaaaatcagacagaagttcgcgttactacaatcaacggttcagaatatatcgttgaagcgactcctgattttatcaaacagctactaaaggtgatgaaagatgcttgatcatcctggctctatgagtatggtgctcctggaagcattaaaagcatatgatatcccttgtcatttcggtgaagtaactgttaatactatcattgacgaaatcgacaacccaaatactttcattgcttgtcttgttcgaaaatttacaagttgttttcgaccgagtccagaaaaagtagtaatcagttctgtttctgctcatcatcgagtgttagatgatggaaagattcaactttactggaaagttctttatcacgtggtgtatcatgaagattgatgatattatgtttatgcttagagcaataagcgcttctaagttctctcaatgtgtctctgttaatgtcggtgctgcattgagaaatggtaacgggcgtgtgtttgtaggcgcaaataatacggttgatcctagtcatcgttgtacagatcagtgcaatcacttattagatgataacgggaaactgagtgaagaaaagcgccctgaacattcacaatggtcagatcgcaacgaagtacacgcagaaatgcgcgttattatgctggcggcgtctcatgaacaaatcaaagacgcaactttgtatacaactcattccccttgctcacaatgtgcgaaaaatatcgaattttgtgttgcaacaggtatgattaagcgtgtagtatatctacataaatacgatcgtggtggcatcgagtggatatggcgtctacagcaatacggtgccgaagtagtacaacttgaccccgaagaaatgaataaacatttccggatcaaataacaaatgagtaaatgtatgtctgaactgagtgtaaaagcatcctttgaatatgttttgattgaaaccaacgctaaagcggctggaactgaaattgtatcaccttctggtattgtgactggtgttcgtcaacacggcgaggaaccgatctacggcacagtgttatcatgtgggccggatgtaccggaagaatataaaaccctgcttatgggtaagcgcgtaccgcttcctcatgcacaaatggcaaacgtgccggatcctgaactgattgcaggaaaggcaacaaaagaagaagctcgcaagtatccggttaaatatgtaaccgcacactataaagcgattcaagcaatttacgaataagagatccaacatggctaaacaaattcaagcaatcatcgccgataccgtcgcaaaatctaaaaaacttttcgacaaaggcgacatcctcgaagcaccgacccgcatcgatgtaatgacttcaatgatcattgatgctcaccagggaaaactaaattcccgtgcttcggaagtaatggaatacatcgtacagttcgaggatgtatgcaaatacgccaaagctgttgatccggctgttcgcgaaatctaccgcaaacagttctaaaaatatcggccccttagctcaataggtagagctaatcactcataatggttaggttcccggttcaagtcacgggaggggccaccaaacaaggcaaggcacttagagaagcgggaggaacagaatctgattctgttggttgtaggtgcaaatcctacccttgccaccaaattagggtgcgtagcgcaatgccgttaaatggttcggaatatgcaacctttctcacggagaaggctctgttggtatccggtaataggttccccggaatgcggggtgaagtaaagaaactcccagcccactaattttaatgaggtttatatgaaatttcgtgaaactgtgaaataccataacgcggtcgaatatacacagatttttgttgatatgtctcccgcaaaattcaaagaacgttatggcatgacatttaatgaatggaaagatggattgcccgatggggactaccgaaaaaacttcaaattcaatgaatgttatgtggatgatgatccttacgatctggatatttttggtaaaacaacgcctctcattgagaattcgccagaacagctttacgaatcttgtattgactctgcatacgaaatttaaagagataacatgaaaaatttacaaaaactgtttgaaatgtctccggcaattagaaaaatcatcggagaaaatagcaatccaacgaatcgcaataaaaaattgatggaactttttgcaaaagagttcgatgattttgattctgaacttcataaagcgcttgaggcatattctaaacaagggttctttgcatcgccgcaagtaaatagcaagaaagagtatagcgaacgattctttgattgggagattgtcaatctcgttcgtagaacaaatatatctcctagcaatcaccaattgatttctcttgatacttcggtattctttatccagtatcttatcagcggtggtttcaaaaatcctgaaatttcgtttacaaatgaagcggttagcagtgaatttgatgaatcatttgtatacatcaacacaaacaaataatcaaatggctatcttcggatagccttatttttggggtgtctatgcgctttttaaagtatgcaagttggatcgtactcgtccctcttgacattattactggagtattagcaattctgtttgccccgtttgttgtaccgttctacaacgagaaaacagggcatcttcctaaaggcttccggtggatggaaaccttcgataatcctattgatggtgatggtggacatatccgccgttgggcgtctatacgctatcatctgggggattttggggtatacatgcagcgtgttggctggttgtggagaaacaaggcttataacttcgcatatcacgttttaggacgtgaagcgacaagcaaattcaactggaaaggcaacccaaaaacagaaggtgggccgaaccctgtaaatcatgggtatctgctcatgtggaacgaatcagcatggggtttgtacgtttacaaaccgtggctacggatccacaaagtgcaattctgtttgcgcgtttatgctggatggaaactgaaacaagaagttagcgacccagttaacctggatcgtgcaatgctggcgtttcatttcaacccgttcaggtattatgtaatcaagtaaaggtaatacaatgaaagcatttcaaattttagaaggtttgcatactggtacgatctacctggaagaaggtaacaacgttcggatcgtagtatcaaaaacattaactatggattctgtgatcggtaaagctcgcgttactccgtttgcaaagcgagagattgagatcgaatatcagccaactgttaaggtggaaggtggacaacatttaaacgtaaacgtgttgcgccgtgaaactctcctggatgcggttgaacatcctgaaaaatacccacagttaacgatccgtgtttctggttatgcagtgcgttttaactcactgacccctgaacagcaacgcgacgttatcgcccgaacctttacagagagtctataatggcaattgctgatatcaagggttataaaccccatactgataaaaaagtagaaaccgtaaatcgtatcaaagatgctgaaaatgcattaggtgcaatcctggaagatatcgaacagcgactatcaaattcagatattgattcgctgatagaggaagaattagatgaggtgcttgaacgtatccatcaaatccaactggctaaagaccgactgaaagaagcctctatgtgggcgtgtcgtgcggtgtttcagcctgacgaaaaatattaaaaatcaagccgttgccgaaaggtagcggcttttttcgtttttggtgtaaaaagttgttgactcctttctcacattcccttatagttaatcccgtagacaagaaaacacttttatgaggatgacattatgaaacgctcttacaacatgaatgaactggttttcttcaaaactcgtcgtgaagcacgtgcttacgttctggtggctggtaaaaatacttctgctgctatcgatatgggtactgataaagctgttggtgctcgttgggccgctgttatcgttatcgctgctccggttactccggttaaaactctggtacttggtgcgcgtcacgccgaaactcttaacaccgctgcaagcggtaggggccacgaagttaaagtgttcaagaagcgttcttatctttcatgtgcaaggggttaactatggcacgattcatatataaagtggaatacgaaaatactgagttatctgatacctttttgaagatgattcgtgatcacgggcaacgtctggaaagagtaacgattgatactgcttttgattgtcctgttgggttggttctaacattatcttgcagccccgcaaaagaatcagcccgtgtcgaaatgttacataaactaaatgcattttatgaaggtggtagtgtatggcgagtattgtaaaatttttcaccgactcagtgaaagaaattaaaagcgctctggaacaatggaacactcgttgtgacgtatccattaaatcagagtacgaaacaacttatgatcgttatgatccggcccgtggtttgcacaataacccccatgaggtggaagtgtgaaatactacggattcaaaacgagtcattttggtaaagcgtatcgtacagaaaacatcgatcgcaaacgtccttactatgattctttagtacgcgcgggacgcaaacgcgctcgccaggaagggaagaaagaaggtgaagatcgtggataattggaaaacgtggatatcaattattgttggtgttatcatcggtcgcggtttgtatgatttaatcttttcggcgggggttcattatggacattggttcgggtagccaatacccatcatgcgcgttgagcaacttcgcccctcatccattcacgtttgacggggtagaatgtgcatcaatggagggctttttgcaaagcctgaaatttagcaacccagatatgcaagcccatgtatgtactctggtaggtaaggctgcaaagttcaaaggcaaaaagaaaaaatggtggactaaccagaccctatactggaaaggtatccctattcatcgttcctctgaggcgtatcaaatcctgattgaaaacgcatataatgcgttattccttaatgaagggtttcgccgtgcgctggcagcaaccggaaaaagtaccttgacacattcaatgggaaagaataaaataaacgaaactgtacttactgaaagagagtttgtacgcaacttaacccgattgagagatctgttatgagtgaaaaagaaagagtagaatgcgtgtttctgttcaaaggcgcgattaatccattagcgttactgtatgcgcaacatgcattacgttcaacgttgattcagagtgttatctataaagcaggtgtgtattatgttaccatcggcgcaaataacatggttgttattgaatcctacgttaaggaatgtgcatcaaacggcgttgtctttgataaagtcgattttgatgctggggtagatgctgtttatatgtataagggttgatatgagttacgtagtttattttgattgttcggatctcgatccgttcgtgctgcaacaggcaaagaaatatcatcaagatgtcgttggtattggtgtaacaaatgatgatatgctgtgcatcgaatttgaatattatcggacatttgagcgtgattatttcctgggtgaattgaatgcattcaaaagtacccttttctttgatcgttatgaggttatatcttgaaacctgttattcttaccgatattgacgggatcgccgtaaaatggcagtcggggttgccgttctttttgtctaagcacaacatgcctactgatattgcattagaaatggttacagatgaaaaatttcgtgatatgaccgaaatcttcggatgtgatcagcagttggctaaaatccttatggaagaatacaataacagttctttcattcgttatctgaatgcgtatgatgatgcattgattgtgatcaaccgtctgaaaacgcagtatgatttcgttgccgttaccgctctgggaacaacaccaacagcaagccttaaccgaattgctaacctgaatactctttttccttctgcgtttaaagaggtgatggtcgtgggccacggtgaaacaaaaactcatcgttacctggaagcaaaagcaaagtatggtaatcgtctggtttgctttgtcgatgatctcgcgataaacttaaacgaatgtcataacgtcattagccagttgccgttattccatatgttacgtggtgaacgtgaagaaacaaatgcacctcatcagttagtaaaatcgtggtttgaaattgaagagaaattaaatgatcttgtcaatccttaatgaacttgcttccactctgaaaactaaagagaaagaagcaattttaaaacgtaatgcagataatgaattgttgaaagaagttttccgcattacgtatacaaaacagattatgttttatgtgcgtcaattccctctggtagaagagaaaccaggcacaacaccgctttccgatgcaatcaaagcattactggaagatttagcaagccggaaatatacaggcaatgcagctcgtgatcgtttactggatattgtatcatcagtgaacattaacgatcgtgaagtgctacgccgtatcattaaccgcgatctggaatgtggtgctggcacaaccttaccaaacagggtatggaagaaactcattcctgaacagcctcaatgcctcgctacgccgtttagtgaaaaggctttacgtcgcatcattttccctgcttactcgcagcttaaagccgatggtgcgcgttgcatggctgatttgttggaagcattaaaccgtaaggtatcgagggctggtaacgagtacgaagggttaactcagcttgatatcgatctgaaaaagattcgcgattatctgggatatgatgtagttctggatggagaattgatttatgttccttccggaaccgtaccaacattacctgaacctgaaacagacatgcctttttctttatctgctttcatggacgatgatgataacgacattgcgttatttgcggaagaagttcgcaaagtatcgaccccagaagaagaacaggccgaagcaaaacgcgaagaagggaacgggatcgtaaacaaatctctgaaagggacgatcaccgaagaagaacagcgaaacattgtttatgttgtttgggatattattccatatgaggtgtattacggcgaagctgaaagtgttcagacttatgatgagcggtttagcctgttgcgtgatatcctcttggatctttctctgccttctgttcgtttgattcagtctaagctggttaataacattgcagaagcgaagcaggactataacaattaccgtaatgacggtaaagaaggttctattctcaaaaacagaaacttcaaatggaaagattcgcgagtagccgatcaggttaagctgaaaaacaaaaccccgattgaactacggatcattgatatctacgcgcacactaaagaagaccataaggtcggcgggtttgtggtggaagatttatccggaatggctcgaacgaataccggatctgggttaactgataccgattatcgttacgatgatgatggtattacccgtgtatacattccattagatgaacgtggtgaactggatcgcgaatacatcatggcgcataaagatgaatacattggggccattgtagaaatggaagttgacggcctccagaagtcgaaaacgcgtaagaaaggggaaccggaatacagtttcttccttcctattatcaagaagataagacgcgataagaccgaacccgacgatattcatgttgtctttgcagatctattttaataaaaagcccttgactccggtcgggggctttgttatattgcatatcgaaacgtaaatcactgagagaatatattatgactagtagttatcagaaacacaaaacccttatggcaaacctgtccggtaaacatatcgacgaagtaaaatctctgctgacagtaaccgaaggttcccgcttcgaaaccaatcacattatcaaaccttctgtgaagaaagtactgaaagtgatttaccgacatccggtgtatcagtgcgttcatatcatgaacagcaacgcatttattttcgtatataacgaatccgatgataagtgtgttggtattttccgaaaacctaactttgaatgcatgagcgaagcggctgttgcaaccccgatcgttgaagaatatccggattatgttcaacgcaacatgcgttatgtgcaatcccgacttgattatgcatacgatttcaattctgacgcggtagaagcgctggcggatatcctttgcaaaaaccagaaagatcgtcaaatgacaaaatatctgactgatccaacaccgccaacaattcgaatttctgttgaagttccgtttgaaaatcatttcatggcagttgaagcgcttgctaaacttggtttagaagtgaaaacagaagccgtttaatagcactttttgttaaagaagcctcttgcaatgcagggggcttttttgtatattgcacacatcgaaacgaaacagacaaaaggaacatcccatgcaaatcactaaagaactcgaaggcaaagtaatcgttctggtaaatgaagaccgtttggcacaactgggtaacggtggtgaaaaactgccagcggacgcactcgaaagcctttctaaaatgcgcgtgatgcgcgttactgacggttgggttacttgtctgcctctgaacgacgaagacaaagccgtatacgatgcacaagcggattcatgggatatcgaagtacctctggtaaacatcgaagttgaagagtgctacgaaatcgaaaaataatgcttgtgttctgggtaatgtaatggtacattacctacatcgaaacgaaaggagaaacatcatgaaagttatgcacactgcaaatcaacttcaaaacggcaactacgctatccacgatgctatcggtgcgctggttggggtttatcttcatggtatcaaactccttgaagtaagtgggaataccttttatggtgttgaaaacatcgaagcagcgatggaaattatcggtgacctgaaatgagtaagaaactcgaaatattcgaaactatcagcgaagacccgaatcttcgctggtgctgtgcgaaaactgggtttgatgctgcatggggtgatactccagaacaggcgcgtaaaaactgggaacaccaacaattgttttttgcctgtcgggttcctaccaattatgaggggagtcaattgttagcatgaaaaataaagaatatgacccaatagaagttaaagagcggttatcggtagcaagaagattccttgaatctatcgaccctgataaacttggaaaatgccctgatacgatttgccttaattgtgggcgttctgttcttgttggtaagtgttgcgataatccaaatatagttgtgatggaaaaggaacaagtatcccccgaaacatgggatcagatccaggaaatcattaaaaaccctccagcgccaactaagaaattacgtgaattgatgacaaggaaaatgaaatatgagcaaatttaaattgagtgcaaccgttcgccttattcgttggaatggtgaagagatccgttatgatgaccctgaattcgcccatgaaattctttcgcatcgtttgggattgaaaaacgcgtcattggttcaaactgttaaaacatcagcagagccggaaatttggcgttgtgttattctggatctcgataacaacattgattatgatgatcctaagaactatccgcttctggaagcacaagttgagaatgctccagaagacagacagtgttttttggttgagttgccacgcgaacattacgaaaacatcataaaggcccgtaaaaaggtcaataacaatgttttcgatctccacctcggattgtttgaggattaagtactgctagttgtgttcgtagtagcggcgctggtaggttcccccacctgtatacattcaagtgtttgcaggtggaaatcttttgatacgtctcgaacacattcaacgatcagatattttcctgcatactcttccccaaatacctcaatgattgcccctaccttaacatctaaacgaccctgctttatatcgaatcggatccggcgttcatagctggataacaattgcattttagacgcctggaaaggtttaccttctgaatctgggttctgaaagttggtatcatagattgcattacggtttgtgaagatccatgtattctctgtgtctgtatcagccagtatatcaccgtacatctttttatcagtcaatgacagactaaagaaactggcgtctttaaacagcgttgtgttatccttatgggtaatgtactgggcttctgtgaatatgacagtatcgccaacaaacacgttatcaacgttaaatttgtatgctgggatcggtgtctgggccagaatgtcagttgaacttttaaggaaaataccggaaccatcttcccacagataacagaaatcagaagaaactacactttgcccgttgtccctgatataatcgaatatatcctgatatgtaccatttagacatccaggagggatacgtatgttaccgccgtcaacttcgggggtaagtagtttcattttgctatacagtgccgtcatacactctgtaatcgtctgtacggcgttgttactaaatgaacgggcaaacttacgtctgaacgttttatgcagcggagagaggttcatacgcagcacagagcggtttttatcgtcagtatctacgttagagtaaagcaatccgtaataatgttgttcctgtgtaccgttatactggaaagatacctgtatgatcggctggataagttgctgatagattaactgtgcgtcgtatatctgcatcagcgtttccgatgagccgttaatcatcgtcttttcactaaacgagacaagagcgggtagcaattcagtatatgcgttatcaatgtatttttcgtatgatgtatataatttaatcgatgtgactcgattgacgattttttcagccataaaaatccctcctaatatatcctatttactaaatagtaaataatgacccaggttcaatttgaggcaataatgaaaaataaaactcttgataaatttatgactacacggcttgaaatcaagaagactaacgttaaaaccgttcatcttccggatggaacagccattgagatccctaagatgtcgtatcgtcattttgtaaagattaagactctgaaagatgacccagttgcgatcatgcgattcatcattgatgacatcaaaccgcgtgaactaacagcagcggaaattgaatttgtgttgatccatatgtatgcacacaataacgctgattatgccaatacgcttaaagaaattgggctaaatcttgatgacctcaaaatctccgaaccttgctatgattttacgtttgacaatgtgcggttagtctttgacaaacccagcctgttaaatgctcaccttccgttcctcatcaaagaggcatatgttgacggtaagccagtagaattaactgaggataaacgagacgaattaattaattgcctgtaccgattcgaatatgatcaggtatcgcgtggtgtcctccaggaagtatacattattcatgaggggaaaaccatcaaagggcttaacatcattggtgaatgataatggctaactcttatttcaacgaagaacaaaagaaaaagtttctgaacagaaacaacaacaaacaaccagcggtcaccaaagtaacagcctcccttgatgctgaaagcgcccgtgacctaaaggaaatcaacgataacacccttgaaagtgcaatcaatactcttgatatcaaagaagggttgaaatcgttcgaagaaaaattccgtgacaaattcgcggggttcaaagaacaatacgaagaggataaaaaggaatcattagccgaacaactacctgatttcgtcggcccgatccgtcctatatccttaaccgatgataactcaaaaactgttgacaatacagtaaacgttaaccaaaatggtcagtttggtaagctggaagaaaacaccgaatctatttttcatgctattaacaaacttgttgatttatatgaaaatactgataagcataagccgcttcctgaaccagtggaagaacccgatccgtatgtagacactaagaaaaaacgcatcaatgatgatgatgacaaaagaagcaaaactctggatcgtattgctaaaagtctggtttctattaaaggctttacatcgcagatccttagccgtttcattggttactctctggaagcaatggcaaagtttgctaaatggacgctccttattggttcgttaatctttacattcgatgtgttgcgcgtcacaatacgcaaatggttcgaagatatcctgaaagaaggggaatcctcaaaaaaactatttggtacatatctgggtaacgtaaaggctatcgtaacaaagatcgaagaaggtttgaacaacttcaatatgaacaacttaggcgaatcacttcgtgacttgttcgttgagcctatgaagttattgggacaaactgtacaaacggcaatcactgagggtatcggtcgtcttattcaatcattgggtgaatcaactggtatagacagcattaccaatgccggacgcggaatgcagatcaccgctttacgtgataaacagaaatttggtcttgaattgactaaagaagatattcttatgatcaagaaacaggaactagaagaccaaaaagcggcattagaaaaagaagataaagctattgcagcacgccatgcattaacaataactccttctcaaattcctaatggttctatctataaagttgctcctactgattatcaagaaagaaatcagaaaaccgtagatgctgataaagaacggcttgataatatgaagaaagcaacggaagaaatgcagaaacaatacgatttagctaaaagcagcgaagaggaagcacaaaaattagccgatgaggaaaacaaacgcaaccgcgcacgtatagaagaagcaaaaaggttagaacaagcgaggaaggaaggaaaacagccgccagaaggtgaagagaaaaagggtgatgatctgttgggtaaagcaaccaactatgctaactctgaaaatctggatgcagccgatatcaaatacattaacgatgaactgttggatcagcttgaaaaacgtcgtaatgaaggtaatctggacgatgtacagaaggatagaatctctgaccttatcgagcaattgcaaaacaagattgcagcccgtacagaatccagcaccccgatcgacgcacagccaccgttagcagcaaataaaccggatgctgataaagcaagcaacattcaggttaacaacaaaactgttaacaacaacgtaactcattcagtacaacgcacagagcataaaccgctcgtagcgctggcataaggaacatataatgaagttttctattattgatgacagtataaacactctcaaaaatattaaaaatcgcggtatcccctctgggggtgccgcaatcacagaatcagtattaaagcaaactatcgttaccgccgaatttccggcccaacgtgcagcaggtatcgataacgcttataatgcttcgagtctgtataataacggccttctgttcactgcatatgattttaatggtgttggtagtaaagacaactatcgttcattacgtcaggcagcacagaacccaaaacaaatactatcatctgcgacgggtaatgttaagtacaaacaagtgttgaatagttctattggtactatggaacctgtttgccagatcctgctaccgcgaagcctgaacgataacgaagtaaacagccaccgctatcaagatgcaaacgatagtttcttaaccaaagggttgagccgtgttgtttcaaacatggtatggggcgctgtagaatccatttcaggcggtattatggcagaccgaagagaagcccttgatgttggtactaaagccgctttccagggttctgacaagcgaacaaagatgtattacaatacattcgtgatcgaaagccgtaatgatttgctggaactgattaaaatctactatctgtttactgttctgggatatggtacaacttctggcggtactgctaaagaggttgctgcattggttaaacagtattacggtgttctaggtgctaaaaccgcgaacgcaattagcccttccagtaacccagtaacagcgtcagattttgataatagtctgggtaatgatgtggttgatttcatttcgaacgtagaggttattaaatcgcctcctgtctggtttattcgtgatttccagtctggggattccttgcgtttacctcattcaacctttgggccagcgggtattaccagtgttcgctttggtcgttctattgataatattgtaaatacattaagagaatcaccaaataccccgatctcacttgaggtcgaaattcaatttatggaactgatcgatatgcgtcaggattctatttttgatacaaattactaaggagatatgatgttttacaacgtagatgaatttttatcaggtatggctaatcgcgattttcagcgtagcaacctgtttagcgttgtatttgcaaccagccctgcatcacgtatccttgacaacacgatcggtagtattcgagatactttgattgatggatctattagttctatcaacgcaaacaacccgaacgaattcattaatgctatcactggcggtgtgagtaaattgtttagttacaccgtcgataaggcgattatgtcgctgaacaaaacaggatttagcaaaatcatcggggcaattagcccccgtttgattacttccctgtttggtgatagtatgtatggacaactgctatctgaattccgtgatgaaatgatgtataatatgggtttaagcattatgggagttaacctccctggtaaatccattggatacgaatacgtttataatggtggcgtacctcaaatcagattcactcgccctgagaatggggaattgtcattgacgttccgcaccgattcagaagcccgtaacctgaaaatctttaacgaatggatttccgctattcgcgatgatgtaacaggacaatacgccttcattgatgaagtgacaagtactattcaggttaacttacacgatcgtgatggttcaccgcatacaacatacgtatttcagaagtgcttgcccgtcaaaatcagtaacagtgaattgagctatgagaacaacaacgaaatctggacatttactgttgattttgcctataaaacatcatgggttgttgaggctgataaagaaggctgggaagggttcaaacaatccgtagaggaaggtttagccattgcagcacgtaccgcaattacaggacaataaaggggctacggccccttttgaggatcttatgtttgatattattcgagtaacattaccatcagggatcaaacgattccctatgtttacagttaaagaccagtttaaattaatgctgacccgtattgatatggaaggtcggccccttaaagagcaacaggaaatactggatgaagtgctggatctgctttatcctgggtattccaaaacagaacaggaatacattttcagccgggtgtattgtggttcgttcggtaaaaacgttatcaaggttgtgataggcggtaaaggcgggggccactccgaagccttcatggtgattaatgatattcaactagaaaatgaatacaagctgaatgatgaaatcacattagggtttaacttcccccgtacacgcaatacaagcgaagagttgtttcttgaatgtatcagttatgtaatatacaacgaacagcgctatgaatggacatcactaaccgaagaaacgaaagagaatattcttgatatcgtcgaacttgatgatgtcgaaaaaatagttactatgctaacgaaatcggttgatgtgtctatgcgcggtaaatcatttagtggtatgttaaccctgttcaagatattgtttagtcgcggggatctggatgaatttgtgaagaccaactatctgctaaataaaaacggcctgaacctggaacctatcatgaatagtagcccgatggaaaggcaaatttatactgcattgcttgcagaagacttgaaaaaacaaggtgctgttaaatgagaaagcatgaatataaacacgttgagaaatataatgttgattatcgtcctctgacacatacagagtttacccccgacgcagattttatcaaaggggatgtttacctgtatcaaagagaatatcttttcattctggcacttctggaaagtaaaaatattgatacccgtcaactgttcatcaactgtgaagaatgtcaggaaagaatagaattccagcttaaacgcaatcaaatcatggttgaagatttcgacgataagctatacggcaatgacggaatcgcgctatctgttcaccctcgtaagactggtgatgaagagatccccgatcttatcgattacgtaatgatagacggcgaacagatcatgtggagtgattgtagcgacaaagataaagaaatggtgttggatgcaatcgactatgcaacctataaatcgatttctaccgccctggataagccagcagtggtcgcaaacattccggtaaggtgttcgtgtggacatagccatatcgtctctctgagaggcttacagcaatttttaaaggtggtctaaatgggtgtaaatctgaggttgctatatagcgatatagaacctaacatgcaacgagattggaataatgacgtagcggcttcaaaaggggccgcagcagtaagaaatagtttgattggtatcgtaaccacgatcaagggtacacgtccatttgatagtaactttggttgtgctattagtgatatgctgtttgagaacatgaaccctctgacagcggaatcaattagaacttctatcgtatctgcgatccggacatatgagcctagagtatataatctttctgttgaagttattccacagtatgatgataactcagtaacagtaaccatctattacagcatcattgatgacccggatgacgtagagcaaatcaaactacagctttccgcatcataacaaaaagccccttcctttcggttggggctttctcttagaattcaatgaatcccattagtgtttgatatcgcaattcaaacggggagatataactttgcatctggttttgatcggatacgatgtaataatacacctcatcattatcatcatatagcgcttctttgatgatgcaataacgatcggtttccacgttcacataaagagtatccatgtactttgtaactttggaaccctgtgaactgatttcacgaatagcgttatctatgaaaagcgacaatgcttgcatgaagttatcaaactcaccatattcacagcccataatagaaattgcagtgtattggtgccagcctttgattgtgtctccacggcggatccatccaatttgtctacccccgatagatacacaccacactttaccaacgggactatagaacctcacaacttcttttaataacagggacatgatcccacattttgtataaggattcatttcaacctcatttcatatcaagtagccaggaagggctagtttcaagcgaaatcgcagtatattcgtattttacagtataacctttgaaaccgaaaggaatgactgcattttcattgagatattttactttatgctttgcttcttcttcattcagagcagcacagactgttgtttgttcaacgttaccagcaggagaagtaaatttttcaatgatgatatatacgcagttcatcctattgtcctctttccattttttcaagtttcatcgtatccacttgcagttgaagtttaagaatacaacctttcgatatgttatacaagtagtcactaacgatttttgactttacctgatcgtaatcagaagataacgtaatccaatcatacatcgtttggtatgatggaagatacgtacattgttcttcttttgataacgctttaaatgattggtaatcggttggaggttccgaagcaattgcggttgtggtcataagactaagtgcaagtagtagatatttcataatgtattcctcattgttttcgatagaaccaatatagcaaaaagccccgaccgaagtcaagggctttttcatcaatgcaagaaagatttcacgtactgttcgatcttttcacgacatgtatcaactgaggtgctttccgcaattacggcatgacataacgcctcgcctccgacccagaaactcatcatgtactgaatatcacgaccttccatttctttttgatgcgctttgattcgatcgaaagcgttttcgattgtttcagtagcagtaagcatttcggattccccgtcaacctccgccagttccccatcgatcatttcgctttcgacttcttcccagtatactatcgttatcatgcattaccccagtggttaaccgtcgtaatccccgccacaattcacatcgccttcaatgaacagttcgcggttatcacgtaataaattatactttctttcgagttcaggcccgaacgcgtcggcgtcttcataccagctataattgtatcttccgcattcatcatcatattctggttcatctccgcgttcattgaagtgaacaattttgatatcgtccatccccagttctttcaacttatcccagatatacgaaatctcaacgctatgggaaccgaacgcttccagtgagatcgtaccgttgctatcgacttgaggaataccccacttcgaacgagtatcatcggtgatcatatctattaatgactcaatattattctcaccgtagatatcagcaacttccttttctttaccagggcgaacaagaccgatcccgataataaagctactgcttgagctattgctcacaaacccagaacggatcttcatcgcatcaccatattaccaatcatgaatagagggattaacgcgaatatgataccccatagaatgaccttatcttcacgacggtcacacccatgatagataacacctccagcgaaaatcaatacaacaactgaaacgaacgcgaataaagaaatcatttgcgggtatccattctcatagaaacttctttcaggatcttattcagatcgtgaagcgcatcttttacgtcaccttcgttataggtaagcatatcctggtacagccctttcaaacaacgattgataacatatgctttttcagaaggtaacattgttccagaacgattataatctctgaaaatgtccatcatcgtgccgttgttgccaggtaatgacgggttgaagttaaccataccagacatcaaactatcaacatacacaacggttgtgttatcagaacgatacgcgccaccaactttaaaccagttgctgaacacatacggagattcccgcacttcgctcaaatcggttccgatttcatcgatgtttacacgaatgttgttaaaatacaccgattcatcaatagaaccaggacgccataagatagcaccgttgttatttttgaatccgactacatcaacttgccagccgttatctgttaaccggacatcatcaacgacgatgaaatcaggtagctgtgaatgaaagccgatgttttcaggacgggaattacgaaacccatcacgattggagaaataaaggatgtcaccttgattcagtttgcatatattcataagatttttaaagtccaattcaagtaattccacaagtcacctcaaagccccctttcgggggcgagatctcattagagtttaacttctttttcttccagaacgattgtgcaatcaaatttcacatctttccagaattccgctgcaacgatatctgttgcggtaacgcttacgctggtttcttcaaaatccagatccgcaaaccatgcgtgtccgacgacaataccgtacattacacgactcaggcgattattaagggcgcgaacctctttaatagtttcctttgtctgcttatcaagatactcgatcaggtcattcttgtcaagcgcttcgatctctttagatacagtatcataagcccacagaatgatcaggtcgccattgttgagtttcttcttaccttcggcgcgttttgcaacggtagcagcaacagccggaagtgatgaaacgcctttgattttcacgttcagttctttcgacatgtaaacatcagtcgattctgtgcgctcaaccttcggagaaaagccgtaatcacggatcccttgctcagacaaccattcaccagccgcctcaccaaagcgctgtttaagcccttctgcgttgcgtaaaccaatcgcgttatcacggaagaacttcattaccttctgacggcctttcaggatttccagacggacgttatcagcaacaaattccttaccagaaataccgcgagtcatcgaacggttaaccagaggcagagaggtaaagtcaaccagtacagacatacggtcttcaccaattttagccagcggtttgatagtcagaccagaagcacgtaagtttttcagagtcgggatatcggtttccagcggaagtaccttaacgttaacgataccatctttaacaatggtaaagttacgcacttgtttggtttctactttttccggcaatccaaactctttttgtttgctttccggaatggttacgtaaccttgtagatccgtattgatagaaatgttcggacgggaactgttacccaccaggtgtttcactgcaactttcgttgtggtttgggtaaattccggtttccatacttcatgcgctaccagttgcgccgccagtgctttacgttcttccggagtagaagcgtttgcaatctgttctgacagtttatccagtgtatcatcatctttctggacagtctgacggcctgtacgattgtacgcccagtgttcagaagacaggtcgatcactgtgtcggtttctgccagcagttcgagagcatcaaccagagtaaacgcgttttcatcaggaaccatgttgtaatcaacaccatccatcagacgtttagccggatcaacaaccgcttcggagatcatatctttagcgttggaataatcctgtttggtaaagcagttatcgtatgctttaatcagacgcacatcacccagctttttcagaactttccatgccagatctggattcatggtatgaagcgcatgatacagaaccacatacagaacctgttcaccttctgctgttgccggatcgaagccgtcaacgtcattgatcgcgttttcacccagcgcccaaatgttcttgatatgttccggaaccagaacaacaccatttgcagcattcaggacatacacacggccttcatccaagtagatcgcatgggttgcatcgccaactttgacttcaacacgtgcggaggtttgcgcggtaatgatttcatcaaatgcaggtacatacgcatcaaacccttcaacgaatttgtgtaatgcgttggttgcttccgccattttttccagcagaggacggtttacataataaccatattccaggaaagcaatgttgttaaacgtcaacggcagagtagaacacgctttcaggatgtcatcagtacgccagcagttatcataaccatcagtcaggaagatcagactgttcagattgccattatccgcttgcagatcggtagcgacttcaaccgccagttgcagaggttcaacgaagccagtacatccggtcggacgcagataacgatcgatagcatcattgattttgctcaggtcggatacagagctaaccttttcgcccacgaatacagaaccgaactgaccacggctggagaaatacagaatagatacggtatcatcctgcttaaccagcgttgccaggttgtttttcaggtgctgacgaatgcgagggagttcgttatacatcgatccggatacgtcacaaacaaaaacgtggttagtcggggttggtttggctacggcgtttttgaattcaatgttagtgatcataattttctcatttataggtaaattttattaaaatttcgtttacttttttgctaatagtatctaatgcatcatcgcatccaaacttactactcaacaatgaaacaaaatcatccatcgttgttgtttgagactcgccaacgtcaaaagacagagcgtaggcaacaggatttttaatccttacgatttgaatagtatactcattcagatcgaaccgttcaagatattttcgcaaagaaaataaatcaatcggtactggtagagtttgactaaacgttatttcttcccccagttgataggggggcatttttacacagatttcgtattccatcagtgatgactcttcatagtgtgttccagattacggaaaatttgcccgtgttcaagctgtgattggaattctccgcattcatcagagtaagtaaattcataaatgaatacaccgttctgattgccaaatttagcgttgtactcttcatacaaccacatcttgatcagagcgtctttctcttctgtttccagatcataccagtcacgcccatcataagcaagcgcaatttgaggattagaccgatatcgagtttcggcgctatcttcggtttcccattcataacgcttatcatcataatatgattcaaagccattccccatatgaccgcccaggtcgcggtgtacttgctgtacaacttcttccgctgtcgggcaagtcatccagctataaccacagttaggaacacaatcacccatcatttcgcggagattgttgatatcagtcggatccttcgggaaccggacgatgaaactacttgatgaactattgctcacaaaaccagatcggattttcattataatttctcccaacgttcagcatttttaaccttcatctttcacttccttcatgtttttcataacttcttcaaaagttacagggatctcgttgtactgttgcgattcttcatcccatacatcacgatgcccgaatgttgaactttttgcaatgattttttcattttcccatacatcaatagtaacatgatcaccaagataagggaaattaggaactttgttcagcgcatcaacacagttttgcaatgattcagaaacatgaacaatttcagtgaattcataatcagcactataataagctacgtaaatcatcaccaccccctaacgatgctaatcaacagtaaccccaggatccagaacacagcaaccgcacaaatacgggccattactacatttccgcgactagtccactccgcactaaggaacaagagaacaaacgttaacgcgtataaaaccatttcaataacttcggtaatcatataaacctcacgaaaaagcccctttcggggcttgattaatcaatgtccgaacacaccacgaatagactctgcgaatgcatacagttcagggtttttagctttcactgtttcgatttgctccagaatataatctggtttatatttcgcaccgaaccagcagtaagagaaagaacgatcccacatgaacacgttatagtattcaccgttgcgaacttcaaccatcacataaccaggattagaacccagcggataatctttcagaagattgaatttcgcgccagcaccagtacatccgttaaacaggtcattaaaagtcatggtatgttccttttgtcagtttcgtttcaacaaggacactatactattcttctttagcctgtgcaagcgcttttttgatttgttttgctatggcttcaatcactgggatggaaactgaattcccagcctgtttgtaagcctgtattttgctttcagggatgataaacgaatccggaaatccttgtaacctaaaacattctcgcgggcttaatcttctagggttcttaccttcctgcaataccagacattgaacaccgtcctttccatattgggctgttatcgtcccagtacacacagaatcaactgtaacggcctgatagccaaaccccttaccgtttgccttgtttcgttctttacgctctctaaagcccttccaggcacgatctgatatggtgtattgatcattatccggttcgagaatgtcaccgacccttgttggggtacgtggaggaacaggaaaactaaagaacaccggatcgcgaaagcagacaataaacacgcgctctcttcgttgaggcaatccaaaatcttttgtattcattacctgataatggatatcgtacccttcgtcctgtaacagcctgtagatggttttaaacgtgtttcccttgtcatgtgttaatagctggggaacattctcaaagaacagcacagagggctttttagcccgtataatgcggagtatttcaaagatgatagtaccgcgaggatctaacatgccctgttttaaccctgctttactgaacgcctgacaaggaaaccccgccaacaggatatcgtgatcaggtacgtcgttttcatcaatggcgaatatatcaccctgaatattttcatcaccccagttatcagcatatgtttgttgtgcatgtttatcgatttcagacgttaaaaggcattcgaccccgccgaatgccttatcgaaaccgagcctcacgccaccaacaccagcgcaaaggtcaattattttcatacgtcgaaatcaacctcatcgattttgtatgattcttcgccaatatcagcccatagctgaatattcacactttttgcatcacgataaagagattgaccacaaagcccacctgtataacaagtttctgtaatctcgttaacttccaggcggaggctattgcgcataattttaacaacagccttttccattgccgaatctagggttttagtatcacccaatactacatctttaacgttcaaaataacatcactcattatcgccactccgtttcaattccgtgtttgtatgcgtcaacgcccagaggggtgatcactaaacacatatcagtatttttcgttggtgaactaaacgccatagatgcataacctttttgaatcagggcatcacgccccgatttactgggaacatcgttgaaatctaaatccaacatttttgacgagtatttgtaaagtttacacagaacatcaatttcagcgccggataatttcgggtatgtcatttgtagtacctcacaacatgttcagaatacacacgttcaatgaaatcattccagaaatcgcgatcaacttctttcggataaccagatacagccgccagcttttcaacttcacacatcgttgattctagcgcctcttgtacggttgcgaaaggaacaccgccagctttaaccattttcaaaaatgcgctatccggaagaggatacacaatatcaccttctttgaaaatctggatcaattgcataccaccgcgtaatgcatgagaaagagctttccagtcgatcccgttgttggcttctgcttgccgtgcgcgttccccgtattcatcccagagtttatacacggatttcttcatttccgctacggtgattgtagactggaatttacgccccagaacttcataaaattcctgacaacctgatttcagtgttttgtctgtaacgaatcgacaaaactcgttggtcgggaatcggttagaaacctcaccaactttgatgcgcttgccgtagttagattcatctacgttacccagcaatgatgtgccataccagtaatcaggaatcatctgcaacacatcgacaacttcacgtaatgcagccaggcgagaacctttaacgccatacttcgccgcttgcttacgaacataaccaaacaggccagttagttccgtagtgtagaagcgtgaacggttagcgcggagatattgccagatatcagagttagcgatcagtttgctatcatctgcatgaagcatatcaatcgccacggtgtcaccatcacatgcgaggctgataaacttttgcagactgtaaatctgacggtctacgtcattaacaccgttctttgagtttttatcgccagttgatgtatcaatagacttcttcgcagtacctaacaggatttcgcgaggatgagggagataaatccctttgtagtctttatcgcttgttggtgtttccagtccgtacaggtgagaaccaaatacggtttccataatcattttcatcagaattcaacctttaatgtttttgcgatcccgcgcaattcagcggtagtaatatcagggatgtttgttccgtagctgttcccaaatacttttttaatcttatcacacaaatcgcggcggtacaccatttctttatattcttcttcgctacgatacagttgataacccatccacccctcagcccatccggaattgcgcttgattttaatattagtacaacaatcagacccatcttccggtctgaaagatgcatacaggtactgacgcgcaactttttgtacgtaaagggttttggggttgcgattttgtcgctggtcactacggatcccagcatcatacaacgtatcaccaactttcacatcacttaaatcaatcatttacgtctccagcaattagttttttcacagtaatgaacgggaacaggcacacccaacgtttctttactgcttctgttgtatgttatcacaacgaatcggttttcgccacccctaacacactccagatccaaaatctcgcgggttcccttcgtgttaatgtctgcaacataatattcttcgttgttgacaatcactatatccgacataatcaagcgaggtttcatgcagcgtacacctctgattcatcgatccattccagatcctgattgagtgattcaatcagctttttatcgcgtctggaaataacaacggtagaccctttttctgccttcacgatgatatcaccagaagaggtaatatattcaactacataatcacggcgagggcttccgagtttatcaccaactttaacagcacgtctaaccgattcatgagatttttcggtaaacattaattcatcgcctacatgggtaacaataccatcaacagcagaacgagaattaacataaattttgctaatctccgccatgaaaacactatctctcagatatcgagcagtcactttatctaaacactgagaagatactttatctccgccaggatatactgagataatcattacatgaccctgaacacgggcggttcctactttatgcagaatgtaaaccattgaaccatcagaatctttagatacaaggatcacgctgaaagattctttgtgttgcttctgagtttctccacaggtaaaactcacgtccagaaaatcaccaactttaacagcacggggttttgctacttgttcacgagcactaataacagggatcataatcatttcctcacagtttcaaattcttcatcagatttccagtacacgttaaaattacgacaatcatgatcggatgtcaacgtgtatttttcatttgttttttcgtcagtgataaccatagtttcattctcgatcgagttaacaccgtaaacgaaaacattctcaccacgtttgtttaaaaacgcatcacccttttcaatcaactgccaacaggtaacaggcaaaccacccggactaaccgggcggctaacaagacaatagggatgtttaatcatttaaattcttccattgcataggaagtaagatctttgaaataccttgcggtgttgccttctgggttgtttgtaatctccatcaggataacagcactatcaactcctgctttcttagccatgaatgaaagggcttcggtagcaataatcgttgctttcataacatcagctttagaaacgttgatcgtattcatttttcttccttttcattaatcacttggtatgtgtgtataatacaaaagccctcacgagaacgcaagggctttttattaaatttcgtataaatctggattcacaataaccgcacataaaagatcatctatatgtgcggcttcttgttctaaggtttgcttagatgaatgtgctttcaagcaaccccagtaaaggcgtttactatctggaaatgatcatcgaagaattccccttgtcgttgcacgacctcatgcataggtagccagaacgcgtctgctgcatcatcagcaccgcccatgatacgaggcaatgaaccatcgttattaggttcgagcttgatatactgtgctacagtcggttttgagaagtacaccgaacgtttcggatgatcgaacagcatcgaattacggatagaaccacgaataaccttttctggtactttaattcgtacttcttccagcaattcacggatcgcacaatcaaggaacgtttcgttaccgtttttgtgtccacccggaagcgctaacgcatctttaccaggcgcaaacttacgacggattactaacacgtggttattacatacgaccactgagtcagccgtgcaacagttcagagaatccggatacggatattttttgaacttgtcaatctctctttgccagtgcgcatcttcatgggacaaacgctggaattcttttgtttgtgtccattcatcgataaaggaaaccgtagtgctaggcgcatattttaacaaatcttcgtcccagccttcatggtgttcccagataattttgcgtaaattggtcgaggatagatcctgatctccaaccttcacaggttcaaccgtaatatgattccatccgaatgctttaagccagtaagaatctttgtctttttcgtacccgacgatcgcaattcgatcatttcgagtttcatcgattgccatacgaacacgggatttccatttttcctcgttatagaggtaatccggaatgtacgcgaatttgattctggctgcatctccaacatcaagtttgcagatagaccagcgagtgatcattgcttgacgctgtttagcggtcaatgggtttaatgtgttcggatatgcataagcagaaccgatcagaatgtaaaccgtatcagcaacagcaagggcttcccttaccattttctcatgaccatagtgaaaaggttgaaaacgtccaattactacagctttatcatatttgtgtttcataacgtgctccacgtttaaaggttaatcataaaacagacgcaattatcaacacaccaaacaatccaccaatgaaaccaaagaatagtgaaatgagtatagtcagtacgatctgttttatgttcattatagtattctcgttttagatgtcaagcccccaaagagggggctttaaaacattatttacgagaatcgaaaatcactttacccgcataatccgaacccattacagtttgaggtacgccacctttatagcgggtagagtagttcatctgtacatccagttctttccagcggatcatttccggtgtaatggtgcgttgcagggcggcgttggcttctgcttctttcttcgctgcatacagacgggcatcagcatcacgttcgttagcgattgcagcgttttcacgcgcctggcgatcggcttccgcttgttttactgcttgtaatgaagtctgttctactttttgcagttcagctttagcagcgttaacctgttcttcgcggatcttcgtgttagttacctgttccatgataacttccggcagggtgatatcctgcaagaatacctgtttcacagtgtaaccgtaaggccgtgcataatcttctacttcctgctgaatcgcaatttgcagttggttttggatcttcgcatcaaacaggtcttgcgcttttggtacggatttaccaaattcgcgaacagtggaaagtagtttttcagttacatacttatccagtgcctgatcctgattacccgcgttgatacggttgatcggtgctttgctaccgtcgaattgcagcattacggtcatatccacagtggatttaaatttatcctgggacggaacctgtaatttgtcgaacttcatcgcgatgtctttggtgctgaacgtatcaaacgttgccagcgggtttacaatgtggaaaccaggcagtacgggtttcggtgatactttacccatgaaggtttcagttttaaccgtaccgtcttgcacaatggtatacatgttaggcactaaccacagtgctgcgactacgcccagagcgatcagagaggttttcttcgggttgttcacgatagtgtttaagttcatcataatttccataagttgttgttcaattcgatagttattctatcatcacatttcacgctgtcaaactatttttaagaaagttttgtcagcttgtagattgtttgatagcacaagcccttaatctcgtccaggatgttcttcaaagaactatctactgattcgtagatctcgtttgcttcgttggctattttacggagatacgccaccgtgtcaagcacattttcggtttttagcacaggtttgtatcttcccgtgattcctatgtggatttcggtgaatttatcaaccaaatcctgcatatcttcgtaaaaaccctcatatgctttatgttgtgagtatgaacctgttgcaaaatgtgcgctatgcatataggtaacggacataaggcacatgccaataaaggcatctatcttgcttgagttctcagattctgtaatttgtttaaatgattgcatgatgatccctttatgaacgatggatacttgcaaactcatacgcgaccctaatccctagctttgcgcattcggattcagatcggcattgtttttggcgccattttcgttccatgtagttgtagaatagttcgcttgtatttacgctgggagggatcgttgtgatgtatacttgaagggccgcattgatataatcgtcaaattctttctgaaccggacggtcggcggcgtgtgttgtgggtgtcatcatcaacaatccaaacaacacagccattgatatgcgtttaatgttcataacaattactcttttactcatagacccactataggtctactcctgtatatatttatagcaaaaacgaggccgaagcctcgttataatatttttgttgtaaagtcaatcaagtaatgtcataccaacacaaacttctttcgaaagcgcgtattttgttcacgttttctacgttttcatcccaaccgatcacaccagctttcatacgtttcagttcctgacttaaacgggtacgtacttttgaatcaattttctttactgcaatagaaagcattgcgttcagatcgccatgagctttgttaccgtcgcgacacaaattattatcaaatcgaatgtatgcacatcctgatttgtgtttccagttggttgagtaccaacgtaacccatccggatcaataccatgttgagcataataacgagaatactcttttacttcttcgatcttttcgttagatgaacggtcacgaagaggattgtatttcttacggtaagtgcgactcataatgatctccttttgtttatgcttccactgtatcagggttgttctttagttgcaagtagtgttttcgacaaagtgaaacatatttgtcttctgccccgatctcaatctggtcgccattagcaacaaatttgccattcgcatcaatacgggcaacggtagttgctttctttccacaatgacaaacccctcgcaactccctgatctcatcagccagcgccagcaacatataagaaccttcgaacaagttcaactgaaaatcggttcttagtccataagtcattacgggtatatctaattcgtcaacaacccgacacagatccatgacatttttcctggaaaggaattgcgcttcatccacaaacacgcaagaaaccagattcgggctgtcgctataaaaatgattgttgtgaacatcataatacaagtccatatcaggcgtgatcatggtgcatgttgcttccaacccaatgcgcgaagagatactctgtttaccttctcgcgtatcaattgctggtttgtacatcaggatccgcataccgcgttcctggtagttgtatgcatcagtgagtaaacgagcactcttgccagcattcattgatgcataatgaaaatacaatttagccatttatcctctcaacaaaatctggggtattctggaattttccttccccttcatggtttttgcatgttttgtttgaacagtagatccaccaatcccactcatcataagggggtttggtaatgttcattacgcaaattaaagggaaatgacaatcccgacaacgaactttttctataatgtgtgcgttagccaattgaaaaccatcctttacccatgagtttttcattatgtcgcgcaagatactctttgatttctggcatccggatcgcagtgtcatactcttctttcgtcatggtatgatttgcgcaacccatacacccgcacacctgcgcgttgcaccaacggagtgttccatatgtcgcaatcaccttcattgctttagctttgattttgtcagtcatgattataaccactcatttcgttatcttgtgcttgatgtatatcaagataccacatattgattttacttttcagttcgtccatttccttactcagacaattgtcaacgatacatagaacattaacagtttctttacgctgcataatgttgatgttattcgctttcatcgcttgcgccaatgcattacaggttttaaccagtgcggcgcgttgtcctttgattacggcgatccgtttgttcgctttcttaatctcccgacctgctttgataggatccatcatgattaattcgccttacgaggatcgaaatgaacgacaatgatcgggtaatcaccagtcacctcattaataatgcgcttaatgagttcccagtcgcccccagcgaggccagcaccgattaaaggtgtgatgataggctttccagtcttaacggcgtcagcaagccctacagcctgtttaaaagcattgccgattgcgtcataatcgacacgcggcccaggtgtccagaaatcatattgagtatatgcattgaaaacaatgttgcctttttcgccaatgtaaacagaacaagttccgagcttatcacgggaaccttttaacgtgttggcatcaacttgaaatgcaccaggaatacgatcgcggatctcgcgagcaataccagcacccatattgcaataacagttgcatccgtggatcaaatggccttcaccgttcagatacatgttgacagcattacctttcacttctttaatgatcatttttatttttccgatatagtagggccacaacaaggcccatcaaaatcacaaggatccacaatacagtgaattgaacccctacgctcattttctcgctttccgttcacggcggcgatcttcttgatgacacatatataaaacaccaccaaaaattataaaaccgataacaacgcctataaagtatccagcactaaacatagtcatcatccccgcaatagtaacaaggcccagtgctctcatgcttaccagcattgtacgccaagaacaccacaaccgccgccataataataaaaatccagatagccattagtaaagtcctatgccagcattgaattcgtcaaccaaataagtacggaacttttcgcaccgttccttatttgacgcttgtttgcatagattcatcattggttcagactgcaaaaactctttttgtttcagcaacttgccgcgtttatacaggtgagcattttcctctccccacatataagcaacatctaactgttctgcgataacttgcttacatactgcgacatctttgatatcacgattgttgcataactcatccaggcgagcatcacccgcgtgagcaaatccagcaaccagagttaaaagcagtgctaactttttcatgatgattccttattcatcctcttcgataggggtataataatgcgcattgcagatatacgcaagaacttttttcagagacatatccgagaatgtcggatcctgatttcgtctcatcccactaccagtttcaacagcccaacgtttgttagctggattgtatgtcagccagtaacaatcccattcagacagagtatgttcgaacagatcgaaacgcttacgcccatttgcttgcggcctgacaaaaggttcaaccatttctaaagcggttaaaactcgattaaggtttgaaccgtcttcatccatcgcgatccgcaaacagtattggttaatgtccggatccataccatcgatacccagaccgatagattcgaaaaattttgttgccgcgtgataagacacactggaagaacgatattccaacatcacggggatcttttccccgtccttgacgttgttaatgatatcctgatcgatgagttcaatcaggtctcttttctccttgatcaaggtagaaatttcttcttgcagcggggctatctgtgcatgaagttctttgatccgttgatcaatcacggtcacttcgaacgctaagtttctcattgtacccattccccgtttttatcaatgtacatgatccaatcagcaaccgcccaatgggaagtattgcctttcggagtagctacgatgtaggaaccagctttaaacagtacgcgtttagtttcgttcaggatcaggtcgctcataatgtattcctcatttaaccaaagtgaatcgtgattcataagcatcgttcgggcgctcatacacagtatccgaacttgtaatgacagtgtacacggtttctttcacaagatccatgattttctgtgattctccccagacattgatactaaaataaatcccatttttaggaataggattgtattccatatcataatacatatccatgagttcacaaatgaacaggcggcgctgttcgttatcatatgtgaaataaatgttaaaacaatcgagagatttactcaaagtaatctctttgataacgatgttgtcttgtttgctaaaatgatcgcggattgcttgcacacaacgcaacaggttagggtaatcatatttttgtgaaacaatgacttgatgtgaaacgctcataatgtattcctctcaattagatgcactcataataaaaaagcccccgaccgaagtcaagggctttttgtcaaatgatttgtttttcttctaacagcttcgcggttgtattaaccatacgagcataatcacgggcttctttctttgtatacttgaaaccagcgttatagctcgcaagcgcctttttcaagtcgcctttgtggtaatcaagccagtactccagttcatagatcgcatacttcgatccaccttgaagagtttcgagctttttgattactacgcgtttaggatatgacttatccattcgtgcgctggcgctccttgcggtaacttgccagcatccataagcgtgatggccttttttacctttaccgacattctcacatgcgcgagactcgatccagacaatagccgctaaatgatagcctaaacgtttagccttatctttttctacaggttttgcagtcttcaaatcatagttgtgtccaactcgataagcatactccaaaacctctttctgcttcggtgtgatattatccaaatccttgatgtaggatggagaatttttgtttgccggaggcttcacagtagccttttgtaaaggcaattgatgagtaggcaaatccgcaatgaaatcccctagcggatccgtcgcagcgttgccagaaaaagagcacaagaaaatgctggcagcaataataattttcttcattttaatacctatgttgcaaaaagagtggcaataatacaccccactttatatttatgcaactattttagatagttttcgcgtcacgtagtttatcgttgataaactcagcaatgttataatttgaaatagcctcgttaggatcgtatagtgcaatgatttcatctaacgataccataacggcatgtttaaagtagacgctccagctagtagtaaggatctcacttttgtcaaatccacaatcagggctgaacaatgcgcggtatttgtacccactgtatttcgtcagacgatttgtgctgtgcgcatcactggtgatcagaaaagtcccctggtgagtttccacgacgaaaaagtatccgaggcgttctttgttgtccagcatcttttcaaacttgcgatcggtttcttcgcgaacaatacgagaagtcagcatttccaacactttatcgtattcgggccaatcattctcgatcacgatcgcatcaaatggtttcttaccattgatcccgcgcccgatttcgattttcgtgcaaatttcgttgaacgttttcaaatcttctggcgtcagttctttaagatcgctcaattttgctacataataacgtttttctagtttcatttatggaaacctcaattcaaaaataatttcacagagttaccacatttgggacatgtgataaattttttcacgacataatcagcagcagagaaaaatccattgtaaatcgattctctcttttgctgtatatcagatagttcatattctaacccacttttacagcaactgcaaacagtaatcagttttgggctatggataacagtaatcatatacacctcacaaaaagggggctttcgcccccatcattagaaattgtcttcgacaaacgccgcgagacgggaacgatacactgtatcaagaatgatatggcttgagtgttcgtattctttcagcttttcaacagcccatacaaacccgttgttaacggcagtgtttcgagggttgtcgatctgcttaatgttcccgcatagtatcagaagtgtgttctctccgcaacgagaaatgatagatttaatttcgtggttgctaaggttttgacattcatcaacaattagcacagaacctttgcccggatccggatgaccgatactgcgaccacggaaataatacaggctagggaattgcaccacccctttttcaatcaaaccttcaatgtatttttcagattccggattatccttaaacagaatgttcaggctagtaatacaaggttcgatagaaggccggagtttttcgcccaatgtaccaggaaggaagccaatttcacttgataacgggctatctgacttcacatacatcaagttagcgtaatgtccactattaaccaggtgcatagcaccggaaacagcaagcattgttttaccagaaccagcgccgcccataatggtagcaacatcgatttcattgctcataatggattcgacaaaagccgcttgcagagaatcacggggctggatagctttcatgagtttgcgtttcatagcctgttcgtgcttaacaggtaagacattcaagcaaatctcatcagcagtcaccacacgcccgactaactcaccatttgaggtaatgtactggttaggataaaaatcttcgtcaggaagcgaactgtaagtgatttgggctacattatccgtatatcccaacacttccacggtatcccagaaatcagggatctctacgtaaccggaatacaatacatcgctatcttttaacgtatcgtcgccagtatactgttctaccttacacccacgggacattgcgatcagcaacatcataatatcgcgagtaactaaggttgcatcctgttgcatacaagtttcaatgattctttcgtcttgcttgtcaagagcaaacgttttgtttccgacataatcaaccactttaagggtgatagtgtcagacagtgctgggtttgtcaggtttaaaggaatacctgatttcgtaatcgcatcatatgactgaccgaaaataacttttgacagaagccggatcgccaatcgtgcttcgtgcgctgttcgttctttcgttttcaggtgatctaattcacccatagtagcagaggtaataatgatttctgtaccaggttgagtgaatgaatagattgaataggggttactaatcaaaacattggtgtctaatacgtattttgacatacattaaccttatgtggtttcgttaaaaaatgcaccgaaaacctcttttgctttccggttataaacggattttgcttcttctggagtgttatagtaccccaaaaattttctttttccatctatgtttatctgcgctttgtacttcccattggctttatgataagaaacacctttcaaccctgtactactgtttgagttacatttctttttcatcgcattttgctggttcgtcgctttctgtaaatttcttgctgtatctccattctcaacaccatatacatgatctacgataggaggaagataaccattctcaacgtaaaacactattcggtgtcgcaaatacatagaacctttaaaatgaatttgggaatactcgtttttgcttccggcttcacttccaggagacatagggccgcgctgaactttccaatacactttacctgtagatgtatcaacatctacaaaattcagaagagattcgatcccttgaatctcttcatgtatggttcttgatgaatagccatgacttttcattacatacccagcgaaattacgtgaatatatgctaatgggtgtctcttttgtacacaatgcatgattgtattatatacaatgtccatgcgttcattgtgtgtgagatcacactcatcaaaaataaggtttattgcctggtgctctattcgacgtccacggaaatgattaagaattgcccctttactggtcaatacatcacatccggtagcaccatttagctgtttggcgtcttgtgctgcatttaacgtatgcgctacgtaaatgttaagggaactatgggaacgtttcataaaatcaaacgcgcctttagtcttttgcgtttctctgcccagatccaacctggtttcaaataccataaaatcgttagggccgtaattatgcgttggttcttccaactctcgcataagatgcatcttacgacattcttcaattgtctttacataaaattcactattcatgttttacctttaaggggccaaagcccctttgttacgctaattccacatgcggggcatcaatgaattttgtttcgatcggaaggttcggatcatttttccagttgataccaaaacgcagtttaacacccagttcatcacctgcttgtttaacagcattcaggacaggcaaccacactttagggtttgtttgccagccttgaggcaatacgctaggatacagatccaccgcatcacccgtgatgtgttttgagttcattgtttgagatacacccttacggacgttctcgcgctgttgttcaacagtacgcagaccttcacgtacaccaaaatcaacaggagacagttgcagagcacgttctacgactttcaccagttcaggcttaacgcctttcaggttgttcaggcttttctgactaaatttaaacatacatacctctttatgaaaataccctatgggctacacagggtatttatggtttaagaggcgcaacgttttacatgtaactccaaattgcatcttcctcgcgatcgcgtttccagcgaatcgtcatttcaacactttcctgtttgtcatcaagaggaagtttatcattattgatttgttcaacatatgcttgcgcatctgcttcgctacggaacaacgcatggaaattataatggttgcgccccactacatttcgatccatcaatgaaaaatgactatggttttcccagtcattgtaaatggtaatgccgttaacaaacagcccgattccacgatggttgtacgggaacccagtgacgatatgtttacgacccatttctgctttaacaccagtgatgctaaacacttcatacagaatagcaccaggtttaatgtctttcagttgagcacgtttttcaaaagcattcataatatacacctcataattagttttcatatacagattaccatagtcaggttatctgtcaacagggattatcgttttttgatggaaaagttaactggaacaggcgatcttgtaatgcttcgatccgttcatacgcttgtttcaggatcgtcttatcttctgggttcgttgtctcgatgcagatcagttcgtctgagtcgatagcgatcacatcatccatcagtgaagcgaatatgttcacgtcaggatgtgtcaattcctttatctccgcttccattccgtcatgctgggataacagttcgatgatatcgcgctgtaaatctccctggtacgggaatccggtttgaagatggttaataattctttctgctttggtcatatttcacctacaaaaaaagcccctttcggggctgggattaaatgtctttgcactggcaaacaccgtatttggtgaaaggcttgtcaccgctcaggtaagaccagaaatcgcaagcctgttcagcggtttcgaagattgcagcatcatagaagccgtgttcttcgttaccatctttattgaggaacacaggaagccagctttgcggtttgaagcagtcagtaacaactacccaaccttctttcgctttcattgcttctttgttcgcttcaaccatttccagcatttcgttcagtaagttcattttaatccccttgtttatctgtttcgttgtctacgagagagatattatcacaacggggattagtgtcaacagttattcgaaacgaattgtgctatttttgaaaaacattccagaacacacagcaccagcgatcggtttaccgtttacacccgtagccgtaaatccggttgcgtatgtgtctttttcggaacatgagaaccagctatagccagtgaattcaatgttctcatacccttgcgcttccaggatacgttgcgcttctcgttcatcggtacaactcgattgcaggaatacacagacgacgaccaacaggatacatccaattacttttaacatgttacactctttttaagttagttttgcttgctttgacccagctaacgccaggatatgcgtcaacattaccaaggcacacagttgtgtgactgaaagtgttaggcaaatcgattttatgatctggactgatacccaaatcatgtacgcttacgtcagttgcatacagataaccaccggacatatacaaagaattaatagatccaaaagcatcgttaggccatttgaaacggtatttttctccccacaattcgacttcatacacatcgtattcatcgaacagaggatcgttacccttcgttgcattatacaaagcactgcgccattcatacagttttgcttcaatgtcgctaacgttgatctcttcaccagcgcttaaattatcaagcactttctcaagggtgcggattgctccgcttaactcacggtcaagattcattctataccttcctcttttaacacttcccagatcagcttatccatgtgcatgagattccacataacggaatcatgagaacccagagatcgagagtagatcactccccatgaacgatacgccttttggaattctgctgcattggttgcatcatacggcatatcatcaccagaagcaatcaacagtttaagaatcattaaactgttcagcaattttgcactgggatcttgtgcctgtattttcgaacagtaattttcaatgattgcttttacctttggttcggtaatacgagctttttcgcaacgttctctgtacacgtacatcagttcatcgattatttcttgcatataacgcctcccgttctactgctgataacccgcgaatgtagttctgtgattctctatgcgcatctgctacagcgcgtcctgctcgttccgacgccagtatataagtaacaacttcattacgaatgtgccataggtaatccatcattacaagatcttcttctgtatgaaaacctttaatgtcacactcgcagcaaatagcgtctctttccgatagtgccagttgcgcggattgcgcgttgattggcatcatactgtacttgtcgatcaaactatccaacgttcgcggtttcacaataccaactgttacaggaacaggacgaagagtaggtttatccgaataaatcatagtattcctcttcatcaagtctagatgtcagtttagcgataaagtcgaaaatgtgttgtgaaccatcttcaacataatgacggtatgcaagcaaagttgatacgtgacacatatcgaccgattcaactttgatgcttgatgcgatcattgtatcatcatttccatatccgtcaatatcacggagtaccatttcttcagtcgggaaacgctgaaggagtgacgcttcccgatccgataccagagcaactaagcgattatgtcgcgtgttgtacgataatattttcatttcaattccaccgcgtaaacatcaggttcaggggctttgtgtacgcgcatatctttaccgcataccgcataagccggacagttacgacaaccgttatgatccttattaccgatcagttcattacggaactgtttggttttcggatgttcccagatatccttaatgaaatcgttcgcttccaggacattcaaaccttcttcccaaccaccttcaacccagcgttcggtaaacgaacaagggaagaactcgcctttctcgttaatgtacgagctaaacatagttgcttcgcaatcttcggcatattgcttgtactgttcgaagtttgggtgtccttccatcgcttcaacaaaagcaggggctgaacagctatcgaaaccaaatcctacaccagaatcgaggcaatattcaacaagttttttatattgttcgcgggtaactgtgtcccagttcttgcctcgtcccttttgtttcagacccaggaatacgatcgcgttaacttgtttcaagcgcggatcattctttacagcatcaaccacgttaaacgcgtcatcataggttttagagctaaccatgaaatgaaggttgatttgctgttgtccggcttctgcaagattagccactgaattaaacgctacatcgaatccagcatgtttgtatactgataccgcaacagccccagcaacagccgctaaacgtgctgcaacgtcttttgatacatcagcaatagtaaggttaggtacaatgcctttagaacgcgcataggccatcatatcaaacatatcagggtttgtttgtccctgtgcatcagcaccgagggcgcattgtgttaaccagggcattttatcaatgatagatttgaatgtatcaagatccatattgaagccgttagggttattagacttgtagcagaaaccgcaaagtttaccagcagggccattgcatttagttgtgatctcgatatcgagaatttctgggaatggggcataggtaggatcagtttcaaacgatgttccccagcgagcaaactcaccagttttaacgttgaaattgtagttataccacttagagcgagcgtaacggatatcaccatcttgatagatgaacagggtaggagctttcagaacagtttgtgcgttattcataatataattctcaaaatctaacatgggattggaagacagcgcgagcgagactttcattatcaaacggtattgattggtgctgccctttgctatcgatgttaacgcgccaaaattcactagaacaattttcagtggagtagttcaacagcgttaccgttttattattttccaaaaatacgcgtttgtcaatctctgttttgattacgtgttccatcattttacccaccgttgtttgcgttcgtcagccagttcttttttgtacaccttgatgtattcaccgttcaaggcacggagatttgaaaatacacgattgaaaagatttttcttttctttgtatgccggagacatacggatcgattcaatagtcatacccatttcatttttaggatacgctcttaactctgcaccgatctcatcaatccatttttggtaaagatcgcgcttttctttgtactgttcaaaagtcaacatataatttcctcacatttcgttgggttcaatataaccctataaagaaccaaacgcaagagttatttgtacttcataaagaatttaactgcttcttccggtgtcatatcgtcagagaacaacccgaagaaagtacgatgatgatctttgtacgaaatgttaagtgggttcaataaacatctaacctcttcaacccattgatagtattttttgctgaacggttgatctctcattcttcatccccttgcgcgtagtattcacacactgcatcttctggggtgcaaccgtccgagtaaagagcatacatcagatcttcgtcataatcagaagaacccagcatatgttgaacagagcgtttccatttgttgtaatctttttcgccctgggtttcgctgttttctgatttaagcatttcgtacatgttcataggaatctcccgtagtcggttgcagcatcttccggatccgcatcaagttcgtacagttcgcgagctagtgcgctgggtttaatatcgcgccctaagtgggcgctaacattacgtagccatttcatatagggttcgaatttgttcattttatacgtaccgcgttaaaagcctggttccggagatcatacgctttttcaagctgttcagtagtgaacagaggactatcagtgttagtggtgaaactgcaaatggttttgttgtcggcgttgacttcttcgacaacgatttcataaccccagatcccgctatactcacatttcacgttccggtacttgatgtaaaccgcagcaacatcttcttttttgtagttccggcttttgtagatgatttccatgatttcctccttcgtttcgatgtgtgtacaataacagatcagggttatcgagttttagcaatttgtgctaattatgccattttcttagcgattttccaggaggctttgaacgccggaacgtcttcaatatcaatccagaaaccagatccgaaaccatcactatagcaagggcaaccgtcgcagtagttttcccaggtcatcacttcaccaccaacagaagcaccagtttccatagcacgtaatgcatcttcaactttttccagtttttcggcgttgtcgtcgtaaatgacaaagtaccatttaccgttgtattcgttacccagtttgattgattcgcgaacaagtttcatgataatttccttttgtctgtttcgtttctatgtgtgtaatataacaaaacccctcaccataggcaaggggttttgcaaaaaattatcgtttgatttgggtattatctataaccctttgaatttccgaacgcatcgtagaatactgacacaattcggtaagcgcccgatccaggtgcatcatagcataagaaaactcttttccgcatttgtcacatcgagcgtataaatgtaaatggatgcgcccgatcccatctacctgactatatttctggaatatgtaaggatctgcacctcgatagccagttgcttgatgcttacactctcgtttgaaccatgacattaataatatccttgtacgttgaagcgatcacataacaattttcttgtttggttagtatcgctttggatagaatgcaacatagcgctgatcatgtttaggttattttgcatcatttccgcgctcatgagaacttccatacgcgcacgtaagcgtttattttcttcttccaactcaaccatacggtcatatgctttgatgcgctctaagggcatatcaggacgctctttgagtacgcgagcacgttcaacctcacaagcatgatttgctttccagtggttcgattccgcttcaaatttattaaggcggcggatctcttcaaccagctttttgatcatgtgtggatccatcatgtcgatgaatttcatcaagcaattggattttgtttggttgtcagcaacagaccaagacgaattatacgtaaccgtaaacgtgcggcccatttcatcaacaaccccgatcttgttatcatcggtgattgtagccgcccatttctccctcatggctgtacaggttccgctggcgacactatgcaacttgtttaatgttgcgtcatcaaacacaatttcatcactcatgtatgcctcacatagatttcaaaatacgcagaagtgcgttagtaaagatatcaggaacacaaccaccaaacaacttatgattcatcagcgctaatttcatgctgtgattttcagtatatcgcccgttatggatcccccaggcaacgacattaccaggttcatgaataactaagttagtgagagtaacggtcatgcgctctttatcattgatagagaatgaatagcgataaccggatccgatgtcgccgtaaaggttaaggtctttcaatttcccttgctcatgcaagcgtttcatatgaactgcacatgcatgattaatagtcatttcgtcatccctagcccagtcatcaataccagaggtataacgaatattgaagtagttagtcagttcatttgatacgctcattagaaacctcacttttataaaattctttaccagacccattacagctactgcatttgggggaacggttgttatcataccgccccgaaccgttacatgcaacacatttccttaatttccagccatacacgaacctcatgtaataatcggttcgtgcggccttgcgttcatggaaattcatgctttgtaaacctgaaccaaccacatttcgatgttaggcgcgtaagtaacgtttaccttatgcatagtgcggtatttgtaagcggctttgtacgcatcgagttcagtcggaacacagaaagaaaaaccgttatcatagcgttctgcgttagaaacttcacaaccaactacagcggcaatgtttttattcatgttcatgatgttttcctttctctgtttcgtttcgatgtgtgtaatataacaaagcccctgcacgaatgcaagggctttttgattattttggtaatttttcgatggttgctttcaactcattgattttattaaagagttcatcgctatatttcatcaactcactacggcgtttttcggcccacttgatcaggaattcatgagaatctacaccatacgtgtaaccttctgcactcagttgaatacgagcacgggaaccataatcaacagaactttgttcaatgagaaacttaaccgcatcaagcagggctaaatcttcatgacttaccatgattccttctgcctttggaagatccacaacttcatcctgaatgagttcacgacgggttgtttcttccagtgtttcatgattctggatcatcgtttcgaccggatcctttaccacggctggtttgttttcacctacttcttccaaaaacatcaacatccatccaggaattttagtccggaaagaactttgtacttcactggtgcatgaatttcccagaatgtggatcgcgttaccatgcatatcaactttattgatatagataacgttctgctgttcctgtcggttgctaccataagaaaggaagcggcgtaacgatgtgttatgaccatacttccctaaatcgatttcagccaggcaatcaatgatcccacggttagaaaccttgtaacgcttaccctgtttgaaaaataacgattcttccaggtgagtaggggtaaactcttcataaagaacatagaattctttaggaattttgcgctgaaccaggctcagtttacaattattagaaggaacaataacagcgtgaatgtttccttctgcgtcacacatagcttgcattacttgcggatagtaaagatggtctttcttgcaagtatagctatggatacgactctgccgttttttgaagtaccatttaccagtttcaaaaggcgctgttgtaaaattcattttgcattctcatacatagttaaaattgcttgcatatgttccggtgattgtggaacccctgcaaagttcactttcaaaaagaaattcaaccgatcttttatgttgcactcatcgagtccaagcgctggtaatgaaatgttttcaaaagcacgttgttcatgtctttccatttcaccccaaaacaaacgggaaccgttaggcatcggtattccaatttcattgttccagaatttcatgatagttgtcaagcgttgttttccgtcgatgacttctacccatcgagattcgttgaattcactatcaaccgcgatcgcgatgataccgcaaggaaacccagtaatcaaagtcttcatgaaagcatcttgctctttctgcttccacacgtagggccgctgataggacggattcagatccagatcgttgttcttgaaccagtgaatgtaactaccaaccatgatcgcatgatcgcgactttggaaagtttttaactcacgaatacggtttcttacaatttcgtctgtcattataaaatcaccatccagtatataatcgtaatcataaccgctacagtgaaacacattgcagcgtacacccgcgcattatgaacctgtgttttcaattctgcgatctcttgatccttttcgctttcaaactcttcgcgagtaccataatacccaggatcgttagcagttgccaatctaaccgcatctttttcaaccagcgttgcataaccgctttttatttgtgtcgccccgtaccatccaccccgatcgttgttaatgatcagatgatcgcctttttcgttatgctttgattcaccaacgacaataacccgcttaccattcataatatgatcctcaaaggggccgaagcccctattttgcgttcttccgtagataatctaacagatttccgctttgatgtaaatccaaaactttagaaaacttctctgcgtttctttcgtttgtgagttcgtcgaaatgccatacaccatcatcagctattaacgcgccaggtgatgaacctgtttctacatcacgggaaagcgcaagccccagagggtgtaagatttcgcggttaatgcgccaaacaaggcccatttcagatagagtattaaaatcgacgtatttcatattatgcctttggtttcacaccgtaggccaacataccaaaacgatgatcattatctgcatctttaaacagaacttcgttaccatcaatgcagatgacctttgcttccggatcgatgtatggaagcaaccacaaagggatcaggcgtaggccgctatgttcatcccagcgactgaaattgagttcttccagttcatcaagggaaagctcattaggatcgatataacggaaccatttggtatttttgaggcggtcggggaagtttacaatttcttcatagccgaattcagcactccatgaagagtaaatagtgacttcggatgctttggttaaaacagcatcgcgaattgatttgcagatatcgattaaagtcagttgattttccatgatatatttctcatcttgctaaaattttaggcagtagttgccccatcgttttacgtgcatgtgacggaatctgtgagatcgggacatatttaaaatcatccatttcacgtatagtccgtccgttcttaacgaaagttgatgcacaatagcattcttccgctactgggtaatcttgccctacatagaggaataaagcaaggttttttgttttcgtgtaatcgagaacacccaggctaaccaattcctccgcgaacacttcaaatcctgtttcttcgaagcattcgcggatcgccgcgtcaatatgagtttcgcccttttcaacatgccccttcggaatatcccaatggggcgtttcagtggcatggcccatcaacacggcaccatctttaacaaagataatacccgctgatagttccatttattcacccgcaaaagcgttatcaaatgcttcaagtgcgttgttagcgcgagcactggcttttgtcacaccagcctggagattttcaaagaaggtatgtttccacacttcgcggcgactggattcatgttccagactgtttttgtgatcaccgcgaatctgttcttccatgtcataacggtacagatcgagttctgcgtttaatttctgctctaatgcctgtgcaaatacatgttcaatattcattttgtatagcctatttcagatttaaggttttcgagggtggagtgataaacaacattcccttcgtgtcgagtataccatacttttccgttctggttacactcattcattacattttcatctaaaccagggatcggcttcatgctgggagaaaacgtgatagacatcatttgttctgcactatcagcaaacccacaagggaaaacagatccagttggtttatcaagatacatcaactctactttagccatagatttcttcgaaatcctcacaatcaggcaaatacgtttcacagaaggtgcaaagcgtaaagaatgcaggttgacgaataccaggattatccggtagatacatccagaaggtgttagcaaacacgatgaatgttttcaggttttcggtggtaatttcgctaacaccatcatacccggattgattgatcgcgcgttgcagtggcacctcgtactgttcgcaatagtcggcataatgatcgcttgttacaaggccattagccattttaatcaaatcgacgattttcatgattttacatattccactttaacaggttttgcaacaaatttatctttggtgcgcccatgaccattacacaggtcacattctttgttgaaatctttcatatcttcgacccatccagaatctggcaacccagacggatatgcgttataacgaatggtttcataaccttttccgttgcatttcgggcaaacatgaggacgttcttttttagcagactctgccagttcgcgaagggtggtagaactaccataagcccgacacatgttttcaaagtcttttaaagtcattctataaacatcaatgacgttatattttttaccggatggtttagccataatatatttctcacttaaagaattttttgatgaaagagatagcaaggccgataccaaagaaaattaagtaaccttttccgtcaccgtgcgccaaaacatagagtgagctgccgtatgcgatgagttctgcgatgttcattaagtttctcatgatatcctcctttttctatattaagtatcttaccataatataaaccaaagtcaacaacaaagttttatcaacccacttatcaccagtcattagtaatcccctacaggttgagacgccgcaacactcaggatcttgaaagtgcaattgttccactcacaatacgtttttgcacagtgaacagttcctttcataacaaacccgtttgagaaaattaaccagtaaagtttcatgatagcctcctttgtttcgacaaggccaatataacaaagcccctgcacgaatgcaagggcttttttcagtttttcaacatccaaagttgcggaggacaatctttagaagcgattagacgatccaggcgggacataacccgacgataaccgtcgtattcaaaattaatttttggtggaacgtagtttacctggattgtttttctgttagctaaagaaacatactcagggatcactgttcgcaaccgtatagcgatgactggcttctcttcgccttcgttaaagaatatttgaacagttataggacaagcaaagattttaccatttacccgacgataaacaataacttcctgtgtcccttctgttttggccttcacagcgtaggttagaacataacacgaataatgatttgctagactcatcatgatatcgcgataagtttcaatatcttttttaatcgatactgaacggtctttaaagcgatctgaaatgtggtcagcagtagccgctaccttgattgtataccagtcacctaacgcgctagtaaacgcctcgctaacttcttttcgtacactgttaacaagatacattaaacgtgttctgttcatataatcctcactgatttttgaagtattcgatctgacgcaaacgcttttcagcggcggctttcgaatcgtattcaccaagttcttttgtgcgatcgtgattcaaaacaacccacttatcgccacgctgttcaatgtgttctgtaatatcttttaacgacttatccagatccagtgattcagcctcttcacagataatagtcaaatccacgggcagtgtcaacaaccttttcactccgctgatatcatcaagcatcgaatcgtatgcaagggttacgtgcggcttgtaatccggataatcgtatgttgcgccagcatcaatagaatctttgaaacggctatgcaggtattcagattccaggatccctacaatagtgctaccgtattttgtgtcccacttttcaacatcaaccagtttagcaggttctgtgatgtcctgttgcgggaacaaatcaaccgttttccggctgtatacgatcgttgtatgcatcttttcggctgaaacagcattctttgtgatacctaatgtcttttgaacatttttcaaagcctcacatgaagcctgatcgaatttagcacacatgtagataccaggatctacaacaggttttgtgatttcaagaaatgatttcataaaacaccccaataaaaaaggggccgaagcccctttgtaataaatttgtttttacgcttcttcgccaaaggcggcttcatcttccgcgactttttcgacttcaacggaagggatcagagcggataccgcgccaattaccgcttctggggttactggctggcttgcgtcaatacccagtaccgaacacaggtcggacagaagttgacgatgaacagagagttcactttctttttgcgcgataacttcgttcagatcgaatgcgcggcctttcagtaccagtacttcattttgcagtttttgaatatcagacattttattacccattgttaaaatttaaaagtatcgagcactttgctctttagttgtttcaaagtaccttcgttagtgatgatactatctcccggttgaggtgtcaaacctttttccgtggaatgttcatcaacaattccggtatcctttacaataaacacaaacttagcacccaagcgtttcaggtatttatattcgtgttcttgacgacagtcagtgaccagaagatggttgtattcgtcaccagtatatttattgacgaatctttccaacgtgtaacgaacccaaaccgtgttatcatacttgcatacgatatcagttccaaacacttgcatcaagcgtctgatactccagggagtatcgttactcataatcagattatcaatatcatcaggactataaacaatattgtatccacgttctttgaggatttcaagcccgattttgaaaatatttagaacatcttcattagacatcacaagaggtttctctcgatcgcctttgtaaaaaatagcatccggatcagaatattgtccttcaatcatattgcgaatgtatggtttatcgtaaccatatcgctgcattgctattcttagcgttcttttgataccaaatgccagtgcttcacactgaacatcattgtacgcctcttgaataaatttagcaaccgtatctttaccagttcgcttttttccactaatcacataaatcattagctcattctcttttgagaagtgactacttttccgtcaatttcaacttccatatgaaggaagccaaaagttgccatacacgtaaccgcttcatcactatcgttagtataacccaattcaacctcacccaagtttgttgggaaggcaccataaaatctaaatgtggcgatcgttttcatctgggagttatccaggatatgcacagcgaatgattgcttaggatcatcccacgcaacagagttaaactcattgtaatcgtttgtgctcaacatccatatgtaaatcccaagatacgatctcatttcctcatcgactacaaagcggatcatcaaaggatcaaactcaaaagccgaaccaggtactttacctcgaaccatcatatttgcaggaatatcaactgctgggaggttcattgatggtagtgtaaccccttgaacttgtaaagtcaaacctttcatgtaactgttatcaggaatatcaacccgaaagtttgtaggtgagatttggtttaaaatcatttctgtagacataggatctcctttcctctatttagcggggaacgggatcaaagcggcctgacggggtaatataaaaatttgaagaaaatgcttgaccttttaaaatctttgatctataataattattaattaaaattttatcaaaaagatctaacaagatcaagtaaaatttaataaataatttatcaaaaatttttagatctgatcttgaattaataaattttgtgatctataatatattaatattttattttatcataaatttttatgaagatcaatacttagatctaataaattttatgctttttctgaaaacttttcctttaccccgtcactaaatactggtactatgttcccatattggaaatcaggaaaaacaaaatgactcatttgaaaaaattcaaagaatttctgaccgaaggtaaacccctcgctcgtaccgtagtacgtggtcaacgcgctaaaacttccgataaacattcaatcggttttcttcacttcaaacatggttctgacttcgaagttttagcaccggattctcacgatctggcatacttcggtaaaaacattgtacgtttgaaaggtatgactactggtaaagttcaagcggcttatgtcgattgggctaaaggtactgtttctttctacagtggcaatccggatgatgatctggatttcgacaaaccagaaaaattcaaagctgctactctgtatgaagaggcggaagaaaatctggatctgtataaccagttagcagaagatttcgaaatcgagatccctatgaatgaagctctggtgaaaggtaaagtttacaaactcccaagcaacgatatgcgtcttctgtacactgggcgttctaaaactaaagcaagcggtgaatatgcagtgtttaccgtagtcgatgcttccggcaaacctcgcctggtatctggtaaaaaattcacccaggaatataaaggcgatatggtttctaaactagttctggctgaatccgaagatctgaatgaagcggctaaaggcattcgcgaaaaagttattgctgtgatggtgaaacgcgggtttaacgaaaaagatgcagaaaagatggttgacaaaaacctgaaagatgctatgaaagttagacctggtgcgacccctggcaaacttgcagaaatagttagcatcctgtaaaaataaagccccttcctttcggttggggctttttgattagtatttgctccagacttttttcgcgccgtaaggtttccctttggacataaattgctgagtcggtagccaaacagctttcgcccaatctttaggggcaatctctgctaatggtgatttgaggtgtgatggtagatatgctttgatcatttctgttgcgcctcgcatacctttcacgttaccccagttaattttaagcacggtcttgttagagaggcgtttggtggatccgtacccacgcttcaataactcttctaaaaactcctgtcgtgctctgggtggcgcatagtgcaagttcaaaccatagaacactaagttacccgctttcgatcttccggatcctaagaaaatgatcagtggaaatctatcccaatacggcagggtgtctttatattttgcatcatatgcaaacgtgtacaggcgacccgttgctggttttgccacacggtgtgttttgatactggttttgatgaaattaccaaaccattctgttgaatctttctgtcgctttgccgccgatacaccaacagtgatctttttcagactattacggaaatcgttgatgatctcgatcccgtgttttttacggtagtcattacgttttttacgggcttctgtctctgcggaacgtcgttcaatctcatcatcaatctgttttttgtaacgatgcattgactttgtgaacgttgcgtagtttaatccctcagaatcggcaaaacgtttagcagaaacacctttcgtttttgccttgcggaatttgatccccagttcaacccaatcactcaatttgcgtttgggtggtgcttttggtttatcctcttccgcgatgatctcaaactcaaaaataaaactcatgtttccctccagggattactgacctcgccacccaaaaacttttttgagtgattcttctgttacgattttgaactgccagcctttttgacggcatagctcatttgcggctttccacttatcaatattaactgtataggtgtaaagagcatcaataaatttctttttattgtgtacgttgttgtttactggcttcggtgggggcatggtttctttaaggggtttaacctcccaaagatatgtagtaccattttccatttccacatagaaatccatgtaatagcgtcttctcttaccgtctgcattgcagaaatacgggatcactatacattcagaattccaacgttttacgtgtgggtttttatccagccacttcataacgtagcgctcccacgatgacctatacgtaatctttcgcggatcgcctttatacttctgtatgttttcgggtacaaacgaccctttatacgtctgtcttccagccattgcgtaaatcctaaatagaataatataacgtttagataggggaacttatcgtgctattttcatacttcccgcctgttgattacaaaggcacccagacaactgatattttccgagactatcgattttattttaatcgtgtgattggaaaatataaaacccgtagttaccagataacaggcacactacgacctgaacaacttgcagaatcattatatggaaaccagcaatactactggatcctgttgatgcttaactctgtttatgaccctttctatggttggatctccgatcaggaagccgcgtatcagtgcgctatacagcgttattctgaggttggcggtgaacaggttctgtatcatgtagatgaaaacaacaacaagtattataaccttgtcgaagaccccaataaccctggtcattggtatgacaaaggtgacaaaccaatgctgtatttacagtatcaaggtgtattagctcctgtagatatttatgaagatgcagtgttgcaaaatgaagcaaaacgaacaataaaaatcattagtccgtctgacatccaggcgtttctgaatgattttattaaagaaatggaaaaggctaactcatgaaattaggcggaaatttacactcccctttctttgatggggtggttgaaaacgttgatgatccgcgcgggttgggccgtgttcaagtccgtgtatttggacaacacccagcccaaaaacaaaaatccgatgcaatcggtgttcctgttgaagatttaccctggatgatgcctattcaggatattagaagcgctgcgatctctggtgtgggcttctctccaactggtatcactcgcggatcctttgttgttggttattggcgtgacaaatggcaccaagatggtatgataatcggtactgtcgctggtgaatatgtcgaacaaccagacacacagaaaggtttttgcgatcctatgggtgaataccctcgctatgttggtaacgatgttaactcccttgcattaggtggtttgaaaggcaaaggatcatcaagtgtcatcattcgtgattcaaacacaagcatagcagtaaacccagacgatcgcccactggatgagataccagaagataaccgccctgatacgggtggatttacgatcgaaaagatgctcaagcaggatgaggggatccgcacacgatggtatacagacagtgaaggatatccgacaatcgggatcgggcatttgcttatccgcgaaaagactcgcgacactgcaaaaattaacgctgcgatcagtaaagcggtaggtcgagaagtaacaaacggaacaatcacggcagaagaggtatcaaccttatttgctcaagatttagccaaagtaagatctgatattcagagaaccgctaacgtccgtgaagtgtatgtgaacctaaaccgtcctcgtcaaatggcgatcgaaaacatgtcgtttcaaatgggtgtcggtggtgttgctaaattcaccaataccctgaaagcgatgaaaaatcaagattggcaagcggcttataatggtcttcgaaattcactgtgggctagtcaaactccaggccgttcttctcgcgtgtctaaaatcgtcctcacgggcaaccttgaatcatatggggtgcaagtaccagatccggaagggcgctctctgagtgctgcttacgctgcgtataacggtgctacattgtcggctactagtccggaagatccgtttactcctggtgatacccgtgtgatgtttgaagaaccagcatcatcttataatgcggaatatccgtataacatggtgtttgaatcgagatccggacacattcaggaattcgatgataccccaggatacgaacgatataaccgtgttcacccagcagggagttacgaagaaattcgcccggatggaacccgcgttgttaaaatcgtaggggatgattatcagatcgtgatgcagggccggaaactcaacgttaaaggcaacttacaggtagttattgaaggcgatgcattcatttacaacatgggtaacgttcaacaaacggttgatggtaacgtaactgaatttgttcgtggaaacgttcaacaaacggttgaaggtgagtacgttggcctgattaaaggcaatgctgaactaactgtaaacaaagatgcaacagttaacgttgatcagaatcttaccgcaaatgtgaaacagaatgcaaccgtggctgtaacagaagacgcaacggtcactgcaaaaaatgcgaaaattgagattgaagaaacgatggatatcggtgctaaagatatcaatatcaaagcaacgaataacacgtttattgattctggcgcattaacaaaaatcactggcggcacagtacaggtaggctaacatgattatggattatgaatcaataattgatggaattatgcaaaattatcagcatccttgtgatgctgagatccccgctggctattatcggcgggttatctggcaagggcatacagaaaattatccggctgttggggttgagtgggataccgagataatcaaaatcggtactcatctttatactcaagaaccattcggacatagaagcacggatctacctgttgtcaattcaccaggaacagatccaaataccggacaaccaacagggatccttgttccaaagattggctattatttcaacactcaagcagaaattgatgcttacattacatctattggtgcaactaaaatcaatggtggtaatgattggtatggcgcggatctgtcaaaatcaaacctatacaaaaaccctggcgaactggctatgtataaggtcgaaaacagtggtgggtatctttccggaacaaaccctgtatgtgatgctcgcatacgtcagacgtataatcaggacactggcgcattcaccaatattgattattattggaatggtaatcgtatagcctatatgaagcatgatgaaacaggggcgcaccaatgcaaatatacgggtatgcaggttaacaccaacgcagatacaagcattcctcctgttcctcctgcaatgccttccacttatggggcattaccgagtgaattaagccgtgctgatatttcgtgcattccggcaactgttggtttcgcatatacaaatatcagtgatgctatgttacaggcatggaacgaaacccgtaatacgttcaagctacagtttaacatgttaacgggtgctgtacagaatggattcgggatcgcgacaatgtttgatggtttatccgtatcgatggaagaagtaatggcgggggcgatcgcattgtcacagcaagcatggcaaactgctatgaaagttttcagacaagtgattagcgctgcatttaacattatcggtggtgcatggggattgattaatcagttcttgcctcaagtaaccatcttaggtgttgcgatcaacatttacgatctggtgtttggtgataattctgttcagactttgaaagatgcgtttaatgcaatcatcaaatccggacaacaaacatatgaaaccgtcataaacgcaatatacggggccataggaagcgcatacaattactctgtggaatatgtcaaagctggcgctcgcgaccttgtggatgcttgtagcgcgttatttgattggtgtttaacgatgttccaaaacggttgcgttgcattaatcgacttatacggtcggatcatgcaaacatgggctatccctccggaagtcccaaacccgttatggtctgcggtgctggctatccgtaacatcatgatgcaaatcaaaccacttgatataattctgggcggtaacttccctggattcactgcaatggatttgtatcaacaagcacaggaaaaagtcaaggcttttgttgatgagtcatacgaacagatccgagggctttatgaacaggggcaggaactttacaaaacgttaaaaagtcagattttcgaacgtgatgcaattcagagaaaattcaaccagtacttaaactggatgtggggcgctgtaacagacgaagcaacagcggcttatcaatctgcattggatgctgcaaacgctgctgtagctgcaacacaggccgcgtatgacgctatacaggaacagattggatctctacaagacgcaatgaaagatacatacagcatggcgatggaagaattaaagaaattgcctttgatgagtacaataaacgagtttttaggcttctgtggtgtcgcatttgacgatcttctcaagtcatatgaaaatgcgattactggtgctcagtctctgtacaaaaatttcattgatagttcgcgctcgtttaaagatcactgcaaagtaatctataaccaaatttgtacgttggcgttgagtaaagtcacacaatatgtgaataaattgctgtctctcataggattagcaatcaacttcggttcgattagtgtatgtgttccagtactgaaatactaaatagtcgaatgatcaagaggaatttataataatggctactgctaagactaagactgtcaaaaaacagattaaccaaatccccgatatctttatcgggggtactttcgaagaaattaaaacagatctgattgattggctgggtggacaagaagagtttaaggattacgatttttccggctcgcgaatgaacgtactgatcgaccttctgtcgtatgctactctttatattcagcagatgggtaacacagctctatttgaatcgtttattcgcacggctgcattgcgtagttctgttgtacagtctgctcaagaactgggatatatgccagattcgcgcacggctgcaagtacagcagttatgattacggctgctaacccactgaccccaacatcgatccgtatcccgcgcggtacaaaattcatcggtactgtaaagaatacagacagttattcttttgttgtatcagatgacgttgttatcgttcgtgatagtaataacaactatacatcaatgctgaacctggtgcaaggccgtttagttcgtactgaactaatttatgacggttcgagtatcctgatccgagatccaaacattgaccgtagtcaggtacgtttaactgtaaacggcgcacaatgggacgactggacaaacgaaagcattgtaaacgcaacaggcgcaagcacgatttactacatgcgtgaaactgttgatggacataccgaagtttatttcggtgaaggtgaagcaagtcaacaagtggcgggtggcgcactaaccgccgaatatatcgggggcttgaaacctgctaatggttcgactatcgttattgaatatctgtcaaccgatggggaagcggctaacggtgcaaaagattttatctatgtcgatacattaaccaatattagcatcacggcgattaaagagaacccaaccaacacccctgattatgtcggtgctgatggtggtggtgacccggaagatatcgagcgtattcgagaactagcccctgttatgcgtgaaacacaacgccgttgtgtaactgcatcggattatgaatccttcctgtctcacaggtttggatctatcatccaggcggtacagtgctttactgataacgaaaaacctggttatgctttcatttctgttaaaccaaagtcaggtttacgcctaacatcggtacagaaagaagatatgcaaacgtatctttcgaaatataacctcgcgacgatcaccccgtcgattatggatcctaactatctgtatattgtgcaatctgtaaaagtaacgtatgatatcagtaagttgacggaatcagaggaatggttacgcggtcaggttatttcgtcgatcgactcttactatactgacaacgttgaaattttcaacaaatcgttcagtgtatctaagatgttgacttatgtcgatcagtctgatacttctattatcggttcggaagcagatattaaattgctccgtgaaattgacaactattacagtgctcctatgtctgggatccatttcttgaaccaggtggaatcgaaatcaatcatttccagtacgttcaagttcaccaacgaagaagacgaaagttatgttgttcgttatgcttctacggaaatggatcaggatggtaacgcaaaaattgtaataggcccgttcaaggatggggatatttcgatcgctgcttatacaggtgatgactttgaaaaattaacagatgcaggaacccgtaataaatattacgaagtcggatcggtgtctcattataccgatttcattagctttgatctgggtgttctgaacgtatccgccgatagtttcagtgctgcttatatcgagctaaccgcaaagcctctcgaagaaaccatttttactcgcgatggatcgttgatcgtgtttgaaaatgacctgcgtcctcaatacaccacattgactatgaatcctatcagtcaataatcgttaacccctgtcttcggataggggtttttctttttataaatacgtgatatacataaccgcaaatttggagaaatataatgattaaagcgccttcgattacgagtttgcgcgttgataagctggctgctaacttcgtttaccttaaatgggatgatgttggcatggatttctattatgtggttgaatttgcccgtagccgtgatatggacggaactattattccagacgaagagttaatctggacgcagttgggttatagctacgaaaacgaatggtttagcgatcaggttgccccaaatacacgttataaattccgtattcaaacaactcatgaagggtttgacccttctgattgggtgatcagcgatgaattatggacgtttgatgagaacgcctacgcatatacaaccatgcgtgaattcacccctgctgattcgtttatcaatgaaaaattcgcaaaaaacaatcgtgattacgtcgattttaacgatgatgttattatggcttctctgatggttgaggattttgtatactctcccctgtattctgatgtaagccagatcagcgataagatcctgaaacaagaaagctaccatgaaattcaagatcacatcgaacacgtttgtaatgatatagatcgcacgttcctggtatactcaaacggattgctttacctgtttgaacgttttcagaatatggctaaagtgtcaaatgacaaaggccaaacgtggtattactacaaagcattaaacgatcgtgtaggcaatccggtttcccgtaccgtttcttatcagagcactaacactacgtatgtgttaggatacgatcgcatattttacgggcgcacgtcaacagatattcgttggtcttctgatgaagttcgtttttcttctgatgatgtaacgtttgcgaagctggggaaccagtcagggttagattttgatcttctgatgaagttcgtttttcttctgatgatgtaacgtttgcgaagctggggaaccagtcagggttagattttgatgttgattcatacaacacatatgcgcgtctaccgggaggagtgtcgaagtatgccgaagctatagcttgttctaatgaatggctctacgtggctgctaagaacgttatgcgccgtattgcgttacgtaacacaccaattgatactgatcctggttcgccgacctttggtgaacgtatttttgatgaagtttcatataccatcgtaccaggaaatgataaaattgttgttaaaaaaatggacgtgctgaatgaccgtctatacgttctggtaactggtgaagttaaaacggcgatgatggatccgactgtcaaggctaacgtgatcccatcaaacgatgctggcgtttatctgtgggatgagaatgcaaagacgtttacccgtgtttatggtaaaaccgaagatgaacgtttttatatcactcatgaatataccaatatgtcaaccaatggcgatgaagtttacatttctgttggtaactacaaatatccaggcactttgccagatccagatctggttgaaaagtatccggaagatgtgcattcagcggtgaaatacgatcttgttactggttatactgcgagcatttcgattaactttgctacagttcgtgcaaatcagaacgatcctacagtatggaactttgggccgcaagagtactacaatgaagcaaactttagctggcatttccgcgataaggttagcacatggatcaccaatgataaccgtcctctggtggtttatccggaaaccctgtatactctggttactgatagcgcgtctcctgcgtcaacgattcgtgtaaaccatgaagtttgggacaaaggaacagttactatctacttgaataatatcaagtttactggttttacgaagtacacaaacggtgttctgttgtatcgctcaggtggtaggataattggattctatgaactgtcataccgcgcaagggatgaactcactattttctggaaacccgataacactttaatggtggcaagtctggttaatcaggaacgtgaaaacccatatacgccggatattgaacctggattaatcgaccctgatctgagtcacatgatcactcgttttgctccgcaaagctatctggacaaccaacagttcgaaaaatttggtgaatactatctgcaatacatttcgttgggaagcaacagttactataacaaattgctgaacctcatccggaacaagtatccgagagagaaaaacaacgttgaatatttgtggtctgaaattaaccgccgtaacatttacctggataaaaccaaacgtgaggcagtggttagatttttcgaatcacgtgcaagtgatttctattcaacaaaagggatcgaagcaagttatacgttcctgtttaaattgctgtataacgaagatgtttccgttgagatcgaaagctccaacagtctcgaatatgatattttggttagttcaacaaatatcagtcaggatatcgtaggccggacgatctatacaccaactggacgcgctaacgttacgtacatcgaacgtgaatatgaaaatggtcaattgcgttggtcaatgactctgcataatgctcaaggtaactttatcgaagggcaggttgtcaagtcagaaaaaaccaatttcaccggaatggtaattcgtggtgttcgcggtaaacaaatggctaacaactcgatcgactatatcaaccgtggacgatcttactatgtgatgaaaattcgttcaaatctaccgacttcccgttataaggatgacgtattgaggtttgttcatccggtaggatttggctttatgggtatcacgatgttaacagtattcatcaactctggtttgtcaatgactcataacgagacaatcattgatattctgagaaactaccgtttcgatagtggttatcctaagttctggcctgatcgcattgcgagtatggacggtaacggaaaccaacaattcgacctggttactggtgaacctctgtacaccgtacacccgcgagcgggggaaccttttgatgtacctccggaatatgacattgaagaaaaaccgcttaacggtgttcttccttctgcgcgacggttcgatcaaagtccgttgttcgattgctcaggcgttaaatattcacagttccgtaatttggtggataaacgactgaaagatgatgcaggaaacccacgtgatccaaatcctccatcacagattaaggtaggaaattaaatggcacaacaaaacttgtatcggtcggtaattactgcaaaattccgaaccgaaaacttgatgaacttcaaagatatgatcggcgatgccgccgatctaaacacgatttacatgtctattggacgaactgaatcgtggtcggataacgaatccgaccctaacttcgcccctccatatccaaatgatagcaccgatggtgttagtgatatgtggacgcatatgatcggggctactaaagttcctggtgatatgatagatgcaattttaccacgtaaagactggggtgatactcgttatccaaacccgaaaatcttttactttaacgatattgttgttgtaaacaccgcaccttataaccgtactgatccgggtaaaggttggatggtttatcgtgtggttgatgttcctgatatcggttcttgctccatttcgagcattaccggaaaacttgaatgtatcaggatcggcggtatctggagtccgtctcatgaatctagtgaacctccacgcggagaagctaacgggatcgacatgggagacggttataaatgggaatacctctacacaatcccgccagatgtcgtgatcaaccgctgtacaaatgaacatatcgtagttcctttccctggcgaactggaagaggatccggtacgttggggttatgataacgtgattcaatggtatccaggacaatacgatctagtgtatcggttgaaggtgaattcaatgcgttttcgtgcatacatggattctcttttcttcccgcaatctacgcttcctggtaacaaagggttccgtcagataagtattattgtaaacccgttgattaaaaaggcaagcccgaccgagcctgaaaagaaagcaactggtgattactataatgctaacgcgcttgaacctgattccggacgtatgatttacatggaaaacagacaacctattattcgctcccttgatcagactgaggaagtgagtattgtattcgaattctaaggaaaaacaatggcttaccaaacagcaaaaaaactaattgatgtcggtgaaatcggcaacccatcaacaggcgacccgctttatgatggtggtgttaaactgaacgaaatgatcaccaacgtttataatgcgtttggtgatgtgcgtatgctgtctgcaaacgaaggtgtcggtaacatggtgatccatgctaccggatactatcagaaactaccacgcacttactattcaagcacaccgatcgaactgggttccctgcatgacatagatacttcaacaggttcgattaccgttgttcttccttctggtaaggttggcgaaggttgctacttcataaatagtacgggtagtgtctctgttgatcgtcctatcgcgtttcgtcctcaagttggggatactatcgcgggggttgcagaccagttgtatatcacgtcaccttacacctttgtaaaaatctggtgtaccaaaaaagaaggtgcggtaacaaaatgggattattctgtagaatctatgttcggttctaaaacgatgcctgttgacactacggcgcttgtactgaaagcaaacccgactgctattcctatgtttggatatagcgaatttagcggggctaaggtgcttgtatacgcagaaaacttagctggtacagttaccaaaatggcagaagttttaatgaccgtggatcgtgtacacaaaacgatttattcaacggaatacgctattttgaaaaacagtgaagatgaaatgtttacattaaactttactgtcggtgctggtgatgtcgtatacgctaacgtgcaagcgatcaaagaagatcgaattaaattcacgattaaagcaatagatacgattaaatcagggatcgcgtcatgaaacaagaaattttaataggtcagattgtagacgatggtacaggcgattacctgcgtcgaggtggtcaaaagactaacaacaactttacagaattgtataacatgctgggggatggtgagatcccccatccagcaggtgcctggaaaacttttgcgggtacgacgctatcaccaaaatttggtgaatcatgggcgttgaataccagtgcaaacaaaatcaccgtaaacctcccgaaaggcggcgtaggcgattataacaaggttattcgtctgcgtgatgtgtggtcgcgttgggctaccaacaacgttagactgatccccgcaactggtgatactatcaaaggttccccaactcctaaagatctgtttaaagattttatggatgtggaattggtgtattgttctccgggccgttgggaatacgtcgaaaacaaacagattgacaaaatcacaacttcggatctggcaacagtagcaaaagaaacgtatattgctactcagggacaaactgacttccctaacgtattcggtgttggtaatgaatacaacctgcaatcgttcgaagtttactatcgcggtaacttgctgttcatcgatgagaaagacggattcaatgctgataactcagactatgggtcgattggctctgctcctggtgaactggttgcacttgatggtaattcagtacgtcttaaaaacccgtgtaacgctggtgacacgcttcaatttgttacctatctagatgggttagcaacatggcgttcgagctatgaagcgtatgtgatgcgcatgtatcagactggcgatacttctctggaaaccgttcctggtgaacagtgggtaggtgatctggcaaccaaaaaagagtttacacctgctgaatttggtgttaaccctcgcgtgttgattaaccctaactcgtttgaactgcttctcaacggtaaacaactggttaaaggcggtgacgctgactatccggcgttttcctgtgaaggtgcggaaggtgttgatgaaagtacgtgtgttggtaactctggtgtatgggttccgtcaggacaggattatagtttaatattcactgattctgtagtgacttcaatcaagtttgcccaggaactggaatccggcgacgttgtaacgatccgttggtttaacaatgatattggtactctgatggattgggaaggaactggcggtattaaagaaaaagctgataaggtttatctcaataacgaagaagaagttatattgacgaaccgtatcgaatataccgattataataacccttctcagaaaacaatgcgtaatacaggggaaacctatcaggggcgtattctggatattcaggctatgtttgatattatccacccgatcggaaccatctatgaaaacgcacacaacccggcaaaccctgctgattatatgggatttggtggttggaaacgttacgcagaaggttatttcctggctggctggacatcaaatgcaacggatcctgatttcgcattaaacaataatgatttagatagtggtggtcaaccgagtcatacggcaggtggtactggtggcgatcgtggtacagaaatcaaaatcatcaacgttcctgaacttgtatcaaaagataaagttcttattgctgatgaaaatggtgctgtgatcattggtggttgtcagttagatcctgatgcttctggccctggatacactaaataccgtgaggatacattgaaagtgaatcatggtaacacattacctgataaaatcaaaactattccaccgtatatgactgcacatcgctggataagggttgcataatggcttacaaaaatatttcaaaaacaagggagggcgctcgcgtcctctctaaagaagcagattacttacagtatgatacttatggtaagttgcctctgatcggcggtaaacgttcgatcggcgaaccaaacattgaccaaacaaaacgcggtgttctgtatggaaacgtacaatccgcaattgatgacctgtatacgcttatcgagcaaatcccgattaacggcgttgttaccatgactgaggatgcccctccaatcgctgtacagcaggttgagagcgtttcttttgatggtattgtacagaacatcgattcagaccaagaacaggctgtagttcacgtgtacggctttcctttcatctttgataatgggactaacgccgcaactgtttgtgaaacggcatacaacaaatttactgaatttgttgcagcggaaaaatatttcgcagaagttaaccgtaaaggtgttgatggtacgatcctagaatgtcgatttattgatagtgtttcgcacccggcaacaaatatctccgaaaacggtattcgtcaaatcggaaccatcgacgtagccgcaaaaagtggctatggttcatgggttaagttgggttctggtttcttacctaatgttactccgcaagtaaccgtgtattacttcaaacgaattgcataaggataacacatgagtaacaatacaatcaaccacgtaagtgataaatccatttacgtgacatttgacccaacaggtactgattggcctgataccataaccaacgtacaagatgcgttggaaaaaataggtagttgggcgcgtactgatactgggcttcctatcgcaacaacttctgttcgtggtattgctcagatcgcaaccgaagctgatattgacgctggcacggataacactaagattgttactccgaaactgttagcataccgtatgcagaaccctaaagcatcgcaaaccgtatggggttatacgaagtattcgactgatgcggaatctacaaccgtaactaacgatgcatcgtctattactccgcgatctctgaactatgtgttcaataaccgtaaaggtacagaatcggtttggggttcttctaaaattgccaccactgcacaggcggttgctggtacagataacactgtaactatgactccgcttaaagtcaagcaagcgatcgcgtccctggttccggttcagtcaagcgcgaccgaaagctcgcaaggtttggtacaactggcaacagttgcacaggttcaggctggtacgatccgtgaagggtatgcaatttcaccttatacgtttattcgtttaactgcaactgaaagcaacctgggcgttattcgtatcgcatcacaggcagaagcaaacgcgggtactgatgacaccaaagcgattactgcgaaaaaattaatcaatacccgtgcaactggatctcagttcggtgttgtcaaattagcaacaactgttggttatgtggcaaacactgcactttcttcaaacgctgctgtattacctagtgatcgaaatgcggtaattaacggttctctttatgagaatagcgcaatatataacaacaaatatcagacgtggacagatcttgattggcatttcccagtaggtgctattgtcatgactggttttcagactgaccacggtagtttgtatatttgtgatggtcgctcactgaataaaaataactatccgttactttttgagcgtataggttatacatttggtggtggcggtgattggtttaaccttccagattgtcgaggcgttgcagtacgtggtcatgaccgtgggcgtggactaaaccctaatcgtgggtatggtacatatgaaggagatatgttgggctggcatgaacacccattacagcttatctaccagaacggcggtaatattcctaaatggcaagcagtttacgaactgaaaagcgccgaaaagaatgaccaaagcgctcgcgtatttgatgcttctataactaaagccactggtgtgggtggggaagaaacccgcatgaaaaacatcgcattaaactacgtaattcgtactcaatagaggttattaaatgatcatcgacaaattaaacccgttgccgaagatcccgtttgttgatggcgtcccagatgacgccacgactcaaacgaagattatttggatcaaaaacggtgaaactctggacggttcgccagataaagtgtcaaacactggtagtcttaaccgaactggtgtaaacatccagcagaacgcggttcagttagaacaaaataccatcacccataatgataaaatcaacgaagtaatcgatcaggttaacttgattactgaaaacattgatgctattggtgatgagagcgtaatcaaaaaagttaaccagttggatcaggatgttcgggcattaactttatctaacacccaaacacagaacaaggtagcacagttaaccctttctgtaaatgctcaaaacgatgaaattggtgaatacgatccagaaaaagatcctaaacaccgcacaattcgtaatgatatcatttacatcaagaaagaagttggttcatatcctggatttaacgttgatggtgatgttgacccctcttctactggtactggccttaaataccgcgtactgagtaaccaacgtgctatttctatgcaggaaacccgtataaccaagctggaagatgattgggcgctttccgaagtaggacaactgacagaagaggtaaaagaacttcgtgctgaaatgggtgattctggtcttgccacaacccgttcaatctatgcgcgaattaagatccttgaggatggttctgttgtaatgcaaaatgaacttgatgcgattaatagttatataggtcgcacgtcaggttcaaccagttccattaacgatcgtgtgaacagtctggaaaactccgttagttctctggttacacaaatcaatgatccggtaactggtatcactgcacaaattgcaaccattaacggtcaaatcggtacggcttctgctcagggtagtatccgttatgatattgcggaaactaaacgcagattgatggatatggaaatgattctgggtgaatccggcgatgatggattgcagggacaagttgcgatcttaactggtgacgttggtgaagattcagatcctaccagtatcaaaggccgtttgagtgttgttgagggtgaattgcgcaccaacactagcgcactctgggaactgcaaggcattgtaggtaactcttctagtggcctcgttgcaactagccagcagattaacaaagaaatctatggtgatggtgttagttccgatcctgttactcgcgctggtttgaaaaagacaacccgcaacctgttcactcaggtaggcgataacgcagaaggtaacgaaactggcatttatgcactgattgccgaccttaataaacgtgttgaggatttagaagcgttgaacattgcacaggcacttgcagatcgcgtaactatcgaagatctgaatgctaaactggctctgtacatcaaagaagctgacgcagatctccgttatgagagcaaaaacccgcctctgttattcggtactaacctaactggtgatactgaatacactactggcgatccattgtctctaagcgtaactatgaatggtggtgtttctccgctgtcttaccagtggacgaaaaacggtgtaaacgttggcacaaactccaacacatttaccatcgattcgctacagccttctgattccggaacttacaaagtaacggtaactgatgcaagccataaagtcattgtttctgatgaactggcgatcactgtcgcttaacgattaacaaggggcttcggccccttttgaggatctttatgattacgaacaacccagcacaattaaaagatgaaattctgcgccgtttaggtgctccgatcgtcaaaatcgaagtgacaacagatcaggtttatgactgcattcaacgagcattagacctatatgcagaatatcattacaatggatctaacaaagggtatatcattcttaccctggggccggataacccgaaaaatattttcgatctgagtaaagaacacattttcgcaattactaaagtgttgcgtactaacatgggttcccttgtatcgatggatggtactgcggtttatccgtggtttactgatttcctgatgggccttactggtggttctctgggcggtggtggttgtgcatcacgtacctacggaatgaacgcatatggcgcggatatgggctattttacccagatgatgagctatcagcggtcaatgcaagatctcctgtctccgcttccggattactggtataacgacgacacaggacagtttgcagtatacggaaccgttaaagatggtgatattgttgttatcgaagcaatgatcagatcctttgttgatgtacccagtatggtcggtaacgtctctggatacgctacagcgggttctgatggcgaagataagccaactatagcagatatatacaataacccctacaaagctgtctcaggcggtgtgaaggctggtcaaggtacaagcgttcagggttcatcctctgcgtataacaaccgttgggtgaaagattacgcaactgctcttgttaaagaggtaaacggtcaggtgctggctaagtttcagggtatgcaattacctggtggtgttgctccggatggaacccgactgattcaggaagctatgcaagaaaaagaaaacctccgtcaagaacttctgttactgtctgatgcacttccagtgttgatgatgtaaggaggaaaaatgcattatagattgtatcttgttgtttttgaaacttctactggattaaaaatttatggggggaagcggcattccccttatgacaatccacataatgacccatatacaggatcagggacatatataaaaagagctattaaaaagtatagccattcttgtattaaatgcattcgatggtctaaagaatttcccaacagagaattactagcagaagcagaagaattattagttgatgagataatggattattattccagttgtgttaatctagtacggggaggaaaaggcggagtttctttttatgatccatcaaaaaacccaaatataggttcaaaacgaagtaaagaatctagagataaaatgtctatgattgccaaaaatagaaaatatagcgaaattggccttaaaaatagacaagaagccacccgtataatgacaagaaatagaaaacaccatgatgtttctggtgataaaaatcccgctgcaagaaaagttatcgttgatggcgttgaatacccaacattgaaagaatgcggagaccactacggcataacaaaaaattctgtatttcacagaataaactctaagaaatgggagggatggaactatgcgtgattgggatgaaaacttatttgcacaactggaatctggggaaggtgtagacaataacctaaaaacagaagttactaataagtatgttaactggtacaagtataaccctactcaacagttgcatgattcactaacagccgaagcaattcaaatgaaatctccggatatgtattacgtccgtcgagaatttgttaatattgataaaattttgggtgaagaccgtgaatcgaagtttacaaaatcgtggaaaattgcagcatacatcgattcgtatgcaaactacgaaggacagagagacttttacagcaaattcggtatgatgtcaaacgatgaaatgacacttgtgatcaatcctcgtttatttgcacatcaaactgatggcgggatccctgttctgggagatttgatttatttccctatggataacagtctgtttgaaattacatggattgagtttgacccgttcttccagttcggcgatcgtcctcaacgtaaaatcaacctcgttaaatttatctatactggtgaagaattggatcctaaactgcaacgaaatgaagggattaacctttctcccgatgccgatctggatctcgaacctattcgaaatcttgatgggttggcggataccaatattgaacaatacgaagaagatcaagcctttgaagatgaaggtgatgaattcattgaatcgtttgatgttgttaacgggcgcggatcaccgttcgcacagttcccataaatataaccaggggaaaccctatacatgtagggtataggagaaatcttatacccgctttaacccatacaggaaaaagaaaatgtttggctactggtataatagttcgctgcgaaattatattgtcttgatgggttgtcttttcaatcacgtgcaagttaaacgcgttcgcggcgaacaagaaaaatttatcaaggttccgattacctacgcatcaaaagaaaaattcctggcatccatgaacaagctgaactatgcatacagtcaggaaaatgttgctaaaacggaaacaattttaccacgtatgaatctatccctcgttgatttgcagtataacgcaattcgtaaaactgggatcgcggtaaaccaaaaaatgacgcagttacgcgcacctggaaaaacagtaacgcagtttaaccctgctccgtatcgtctcatgttcgaactgggagtgtatacccgttacgaagatgatgtgtttcagatcatagaacagatactgccatacttccagccgcatttcaactgtcgtattacagaattacataaaaacgacattaaaatagaccgagatattaaaatatctctgcaatctgtttcccctgataccacgtttgaaggtgatacaacgacacggcgacacattgaatggtctttaatgtttgaattacagggctacctgtatccgcctgttaacgagattaaaggcgagatcagaacagtatacacggatttcttttccaatatgaacccgttggacaaagacaattttgaatccgttgatgctcaggtggatccggttgatatgcctatacaggattacacgggagaagaatacgttcaaacgtatgctaatgatatcccaattcctagcggtgatcaacctcctaaaccgaggggccaataatggaagaatttagcgtaaaacaactacttgatcttgaaaatctccctggtgctgaaactggggaagaaatggttgtatatgaaaaactcgaactcgttgatgtcgagtcacacccagcagatcgaaaacctgatttagaggaagactatgcacttgcgcgtaaaaccgcgcattacatgaatcagatgatcatggatatggcacaaattgccttgcataacgctaaaaactctgaatctccgagacacgttgaagtttttacaaccctgatgaatcagttaaacaattctaaccagggattgatgaaaattcataaagaaatgcgagaaattaccgaagaaacaacaaaaccaggatctgaaaaaggtaatggcggcggtaatgaaatgaacatagagaatgcaactgtatttgttggttcccctacggaattaatgcagaaatatggtagtgcatacgaaccaaaagaaggcttcattaatggtgaagcggtagaggtaaaccctgatggaaatggaaccgacgatcgatccgagtaaggaatcagatcacccaatcggattaatacatcccgattatctgaaaaagaaaattgatgaatttgggatggagtggacgcaaagcgaacatgataaaaaatggtatccgacaaagtttagcgattacctaaaaattaacggtatccataaagttgatattcaagcaaaagacagttcaaactttgcgacgtataaaaacaaaggaaacaagaaaactcgatataacggaaacccaaacctgaaacgcgcgtacatccaaacgaaatggacgcaacagatgttgatggagtgggttaaatgtcgtgatgatattgtttattttgctgaaacatattgcgcgatcacccacattgactatggtacaattaaggttcagttgcgtgactatcagcgcgaaatgctgatcgaaatgcataaaaaccgtatggttgcctgtaacctgtctcgccagttgggtaaaacaaccgttgttgctatcttccttgcacactttgtgtgtttcaacgaggataaatatgttggcgttttggctcataaagcctctatgtctgcggaagttctggatcgtacaaaacaggcgattgaacttctccccgatttcttgcaacctggtatcgttgaatggaacaaaggttctattgaacttgataacaaatgtaaaattggtgcgtttgcatcttctcccgatgcggtgcgtggtaactccttcgcaatgatctacattgacgaatgtgcgtttattccaaactttattgatgcgtggttagcgattcagccagtaatttcttctggtcgtaaatcgaaaatccttatcacaacgacacctaacgggcttaaccacttctatgatatctggaacgctgctatagaaggaaaatccggcttcgtaccatacacggcgatctggacatcggttaaagagcgtttgtatacagacggtgatgatggcgtatttgatgacggctattcatggtcttcgaagatgatcgccagttcaagtaaagaagcatttttacaggaacattgtgctgaattcatgggaaccaacggaaccctgatcgctggctggaaattgtcaaaactctcatgggttgatactgatgaaacggaaactaatttttatcagtataaagctcctgtagagggacataaatatattgcggtactcgacccagccgaagggcgcggtcaggactatcacgcgatgcatattatagatattacatctatgccgtttgaacaggttgctgtatatcattcaaacaaaacatcgcaccttattttgcctgatgtcctgttacgttatcttatgatgtacaacgaagcatgggtttatatcgagctaaatagcacaggccactcagtggctaaatctttgttttctgagttggattacgataacgttatttgtgatagctataatgatttggggatgaaacaaagtaaacgatcgaaagcgattggatgctcaaccctaaaagacttgatagagaaagataaactcatcataaataacaaaaagacaatacttgaatttcgtactttctcagaaaaaggtgtttcgtgggctgcggaagaaggtttccatgacgatctcgttatggcgctggtttgctttgcatggctaacaacacaaatgaaattcgcagaattttgcgagaaagacgatttgcggttggcaaatgaggtattcgcacgtgagcgcgaactgctttatgaagatatgttatgtcctgttatcgtaacgagtggcgacgaaacaatatctgtcggccaacacggtatttcgtttatataaatttagaggaaacttaataatggctttaatctctccaggcattgaaactaaagaaacatcggtacaatctaccgttgttcgaaattcaactggtcgtgctgctattgttggtaaattttcatgggggccagcttaccagatccgtcagatttctaacgaagtcgaactggtaaactattttggctccccagacaatgacaccgctgattatttcatgaacgctgtaaactttttacagttcggtcaggatctgcgtgttgttcgtgtcgtcgataaagaagccgcaaaaaacgcaaccgcgatctataatcagatcaaaaccacgatcaccgctgctggttctaactatgcagtagacgatcagatcaaagttaaacacaataacgttgttattgaagaagatggtgttgttaccagcgttgatgatcagggtaaagtcctgtctgtgttcattccgagcactaagatcatcgcacacgctaaacaggttggtgtatatccggatctgtctagtggctggactacagaaatcgtttccagttcttctggtgtttctgctacgattacaatcgacggcgtagaagttgatccgggtattactctgctcaacctggacaccgcaaaagaaactattcaggcaactgctttccaggaactttgcaccaaatacaagctaccgtctgttattgcaatttatcctggcgaaatgggtagcaccgtaacggttgaaattctgtctaaagctgtatacgattcttcggctgtcattaagtcttatccttctggtaagtctggtaaaaacagcggtcgcagttcgatgaactttggccctcagaatgataaccaatacgcgtttatcgttcgccgtggtggtattatccaagaaacgtttatcgtgtcaaccgctaaaggtgataaagatatctacggttcaacgatctacatggatgatttctttgcaaacggtggttctcagtatctgtatggtacgtccctaaactggcctgtcggattctccggcgttctggaactgggcggcggtacttctgcaaactccactgtaggcgctgatgaactcatggctggttgggatatgttcgcagatcgtgaatctctgcatgttcctctgctgattgctggtgcttgtgctggcgaaactgccgaaatttcgtctactgtacagaaacacgctgtgtctatcggtgaaacccgttcagattgcgttgtattcgtttctccgccgcgttctgctctggttaatatcccactggctcaggccgttgataacctcgtagaatggcgtacaggctacaaaatcggtaatactaccccagttgataacaacatgaacgtaagttcaagttatgcgttcatcgacggtaactataagttccagtatgataaatacaacgatgttaaccgttggatcccgctcgcgggtgatatggctggcctctgtgtttataccgatcaggtatcgcaaccgtggatgtctccggctggctacaaccgtggtcaactgcgtaactgcatcaaactggctatcgaaccgactaacgcgcatcgcgattctatgtaccaggtacagattaacgcggttactggtttctctggtggtgctggatacattctgtacggtgataaaaccgcaacgactgttccaagcccgtttgaccgtatcaacgttcgtcgcttgttcaacatgatcaagaaagacattggcgataacgcaaaatataaactgtttgagaataacgatgatttcactcgttcttccttccgtatggatgcaggacagtatatgtctaacgttcgcgctctgggcggtgtatacgattaccgtgtggtttgtgacactacgaacaacacgccggatgttattgatcgcaatgagtttattgcatcaatctacgtcaaaccagcacgttctatcaactacatcacactgaacttcgtagcaacctcaactggtgcggatttcgatgagttgattggttcaacgtcagtataacatgtaaggggctgaaaagcccctataaatacacatagaggttagaaaatgcttactgatattgtacgcgcctttgaatccggtgatttcgcacgtccgaacctgttcgaagtagagatcccgtacctgggcaaaaactttaaattaaaatgtaaagccgctactatgccagcgtctaccgttgaaaaagttccggtaggttacatgaaccgcaaaattaacgttgctggtgaccgtacctatgatgactggacaatcacggtatataacgacgatgcacacacaacccgtgatgcaatcgtagcatggtcaaacatgctgcatggtatgggtgaagacattacaggggatatccctgcaaactacaaaaaaaccgctacggttaaacagaaaaaccgtaacgacgaagtaaccgccgaacataccatttatggcctgttcccgaccaacgttggtgaggttactttagactgggatagcaacaacgaagtgagcacttttgagtgtactttcgcgctagactggtgggtttaaacgctataaatacaggggtagcaataccccttatcattatttttcggagttgtaaatgaacttttttggattagacaatgtgttagggtttttcaaaaatttcgccaaacaggatgaaatggaatttgaagcccaattaaaagatgatacaggttcgattgcgcctccgaaaaataacgatggggcgcacgaaatcgaaacggacttatcaaaccagcgttattcttctgtgttccaacagttctattccggacaggatccgcgaattcagaacaaaacacagctaataaatacataccgtggtatcatgacatatccggaagtggaaaacgctgtttctgaaatcattaacgaagcgattgttaatgaacaaggaaaagatattgttacgatggatcttactaaaacgaattttagtaaaaatatccaagataagatcatggaagaactcgataccgtaatgaatattcacgatttcgataaccgaggatctcgtttattccgtgattggtatgttgattcgcgtatctatttccataaaatcatgcacaaaaatgaagctgacggcatcaaagaattgcgccagttagatccccgttgcatggaactgatccgagaatcggttacagaaaccctacccggtggggttaaaattttccgtggctatcgtgaatacttcgtatacaccgcaccgaaaaacggttatagctacaacggacagatttatagtcacaatgacaaggtaaaaattcctcgctctgcgattgtttacgctcatagcggccttgaagattgcgacaacaacattataggctacctgcaccgcgcggtcaagccagctaaccagttgcgtttgctggaagatgctatggtgatttaccgcattacccgtgcgcctgaacgtcgtgtgttctatatcgacgtaggtcagatgggtggccctaaagctacacagtacgtaaataacattgcacagggcttaaaaaaccgtgttgtatatgacgcgagcactggtaaagttaagaatcagcaaaataacctgtcaatgacagaggactattggctgatgcgtcgtgatggtaaagcagttaccgaagtttcaacgcttcccggtggcactgccttctctgatatcgacgatgttaaatggtttaaccgtaagctgtacgaagcattgcgtattccgttaagccgtatgcctcgcgatgatggcggtatccagttgggtaacgatggcggtattacccgcgacgaattgaactttagcaaatttattcgcgaattgcaaattcaattcaaccctgttcttgcggatccgttaaaaactaacttgatcgcgaagaaaatcattacagaagatgaatgggatgaaaacgtaagtaagattgcttttgtatatcagcaagattcttactattccgaaatcaaagatattgagattttggaacgccgtttaaacctgatgggccaacttgaaggggtggtcggcaaatatatctcccataaatacgtaatgaaagaagttctccggatgtctgatgaggaaattcaaagcgaagccaaacagatagaagaagaatcaaaagaagaacgttttaaaaatccagaagcggaagaggaaaacttttgatgaaagaatttatcgaagcaatcaaaagcggtaatctggtggaagctaaaaaaactttttactccatcatggaagaccgcacagaagcgcttcgtcacgaattacgcgttgaacttgccgaagctgtacgcatcgaaggcgaagaagacaaagaaaaagacgacgaaggcgctgataaagatgacgaaaagggcgataaaaagccagccgaggatgataaatccgataaagatgatgagtgaggtgtgtaaatgcaacttgacatcgaaatcaccgccgaagatctccaggaacatttagacgaagcgaaagcccgtgtagatattctgggtatcgatgaaggcacggttaaaatcatcgaaaatttggcggtcaccgaaccaaatttagcccttgctatgatggcggttgttgaaggtttaacacttgatgaggtaattgtcaagcatgttgattcccgtggcaacgtagaacgcctcaaagacaggaaaacccgtgagcgtaatgcgtatcagactaccggattaactaaatcccaacgtcgccagatcgcgcgtcgtgctctcaaaacaaaacgtgctaacccgtcaattgctactcgcgcacaacgtaagcgcaagaaagcattgcgtaaacgtgctgcactggggctataaatatgaatgaatcccaaatcaacgaaaacggcgatatgcttttaatcgaagaatggggtttaccttgcggtgacgtttcagaatctattttagaatctgttggggaatcaaaagacggtaaattgcggatcgaaggtattttccttcaagccgaaaaggttaaccgtaaccgtcgtttgtatcctaaaaacgtacttgaagaagcagttaacgattatattataactcaagttaacacccgtcaagcattaggtgaaatgaatcaccctccgcgcccgaatgtggatccgcgaaatgcttgcatcctgattgaaaaattgtggtggaagggtaacgatgtttggggccgcgctgttgttgttgaaggcgacggtggtgatggtgacaaactggcggcgttgattcgtgctggttgggttcctggtgtttcttcccgtggattaggtaagctctccgattccggcaaaggctacggcgttgtacaaaagggctttaaattagctgtaggcgttgatgtcgtctgggggccaagcgcacctgatgcatatgttaagcctatagtggaaaatcagcaaagcaaaccgcttgttgagaataatagtgctgatgacgcttttctggcattgtccgagcgtttgaaaggtctataaatacattaaacaaaacaacaggaaaatcaaaaatgcttaaagaacaactgctggcggaagcccagaacctggatactccggtcgagttagacagcattttcgaatcagttgaactttctgatgacgtgaaagcgacattcaccactgtattcgaacaagctgtaaaagctggcgctgcaaaactcgctgaatcccacattacccagatcgcggaacgttccgacgaactggtcgaagctcaggtaactgaacgtgccgctgaaatcgaaactaagctgtacgaagatgctgataaatattttgcgcacatttccgaagaatggctgaaagaaaacaaagaagccgtttcccgtgacatcaaagccgacctgtttgaatccctgatcatgggcctcaaagaagttctggttgaacataacgttgtcattccggaagaacaggttgatgtagtcgccgaactggaagacgaactgactgagaatcagcaggaagttaaaaccctgtttgaagcgaatcaggaactgaccaaagaaatttcagaaatgaaacgcaatgcagtagtttcagagaaaactaaaggtttgaccgaatctcaggtcgaaaaagtagaatctctgattgaagggctggaatattccgcaaccttcgaaaataaactcagcgcaattgttgaaatggtagcaaccaaagctgaaaaacccgttgacgagtctgtaaatactcctcaaacgaaagatgactttgttccggtagttgaaagtgttccggcagagaaatccaagatcaataaatatgtacaagcggcaaaagccctttcttaatttcaaaaggtaagaaacaatgtctaagaaaaacgaattgatggaaaaatggaacgatcttctggagtctcaggaaggcttaccggatatcgctaccaaatccaaaaaacaactgattgctgccattatggaagcacaggaaaaagacgcagaagttgatccggtttaccgcgacgagaaaatcgttgaatccttcggtggtttcctggcggaagctgaaattgctggtgaccacggttacgacgcaaccaaaatcgcttctggtaactcaagcggtgctatcaccaacatcggccctgctgtaatcggtatggttcgccgtgcgattcctaacctgattgcgttcgatatctgcggtgttcagcctatgactggccctactggtcaggtgttcgctctccgcgcagtgtacggtaaagatccgctggcttccggtgctaaagaagcattccatccgatgttctccccggatagcatgtactccggtcagggcgcggatccgagcaacggctttaccaaactgacttctgctcaggctattgctgacggcgctattgtgttccacgatttcgttgaaactggtcgtgtattcctccagaacgtttctggcgctccggttactgtaactggttctaccgacgatgctctggatgctgctgttatcgccgaacaggaaaaaggtactctggctgaaatttcttacggtatggctaccagtgtagcagaactgcaagaacagttcaacggttctactggcaacccgtggaacgaaatgggcttccgtatcgataagcaggttatcgaagcacgtagccgccaactgaaagcacagtactctgtagaactggctcaggatctccgcgctgttcacggtatggacgctgacgccgaactgtctgctattctggcaaccgaaatcatgctggaaatcaaccgcgaaatcgttgacatgatcaactataccgcacaggttggtaaaactggtttcactcagaccgttggctctaaagctggtgcgtttgacttccaggatccgattgatgttcgtggcgctcgttgggctggtgaaagctacaaagctctgctgattcagatcgacaaagaagcaaacgaaatcgcacgtcaaactggtcgtggtgctggtaacttcatcatcgcttcccgtaacgtggtttccgctctggctcgtatcgatagcggtatcactccggcaggtcaaggtctccagaagactctgaacgttgacaccactaaagcagtattcgctggtgttctgggtggcgtgtataaagtatacatcgaccagtatgcacgtggtgattacttcaccgtgggttacaaaggcgataacgaaatggatgctggtatctactacgctccgtatgttgcgctgaccccgctgcgtggttctgatccgaagaacttccagccagtaatgggcttcaaaactcgttacggtgtaggtatcaacccgtttgcgaactctcgctctcaggctccgtccgaccgtatcacttctggtatgattaccaaagaaatgttcggtaaaaacgcatacttccgcaaggtttatgtgaaagggctgtaatagccaacttttccaagagggaaccgcaaggttcccttttttattacataaataaagaaaagtttgtcaataacgcaggaacataaaatgagtgaaaaattttacacaattaacaagctggtgcgtcagtcacagctaccgcctggcctgtctaaaaaggttcttgatgaggcaaccggaacagaaacaattaacgtagctaatacccgtccagatctggtatctcttacccgtgcggtaaacaacctgatctacggtgaacttgtagcgattcaggaaactaatttgcctaccgcaaccctgtttggtgtgcgttatcgtaaccctaaaggcgatatgacgttttccagcgctgctacctattccggtaagtatgcaagccgtgataacattccagttggtgcggttggtactgcctataccaaaggccaagtttttaaacatccgacaagcgatgtcgtatacgaagcaactgatagcgtaactctcgcaggtgctgatattgatgaagcaattatggtcgcagtattcagcaataaattacgcctggcaagcgaagccgcgccaacaagtcagtatgaaaccagcgaagatattagcacaacttctttcgaaatggatcgttggaatatcaacgttcgttcccgtaaattcaaaactgaaatgaccgtggaacttatgcaggatctggaagcaaaccaattcaacgcagaaaatgtgattgaagatgttctgggtactgttgccagcgaagaagtaaacaaagatatcattcagactctgatcaacgtatcacatcgttacaacgttgatggtgtggtaacaaatggcattttcgatgctacaaccgcatacactgcaaaggatgctccggctttaggtcgtttcctgtatcaattagtgtgtgaaatggggcaggaaatgaatagaacgacttcatttgaagctacctatgtcctggcctcttctcgcgttgtaggcgttctggctgcgtctggttggatgcatgaaactgatgaaacccacccgttagcaacaggccgacttaaaaacggttattatgtctatactgacaccaatacaccgtttgattacctgctgactggttgcaagtacgatctgggtgaaatggatcatgttggctctctgttctatacgccatacacagaagctgatcaggcaggttcgatcaagatttctgttgatcctcaatccttacagcctaaagttgctattctgatgcgctacggtttatcggttaacccgtataccactgctgctaatgaaagacttgtgaaaggtgatgactgggtaaacctctcaggcaaatctaaaatgagtcagattgttggtatcaaacttcctaaactgggttgatagtataacccaacggggataatattcaataggtggagtagggaaacttactccatcttttaataattattataattaatattaaattagatcttgaatttataaatgatttatgataaaatttattaattataattataatagatcaaataatttttgaaatcaagtaaaaataaatttgattttataaattagatcatgtataattattcttttaatatattatattagatcaaataaaatttgactacaaattaatatagtatattatagatcaactgggtaaattggtgagtatgttatgagtttgaaattagaagatctgcaaaatgaacttgagaaggatatgctgatagatcccctcaagttgcaatcagaatcagcggatatcccgaagatttgggctaaatggcttcgataccattcaaacgctaagaaaaaattgatccaacttcatgcgaaaaaagaagctgatgtgaaggatcgtatgttgtactacaccggaagacatgacaaagaaatgtgcgaagtggtgtatactgggactactgaaatcaaaatcgcgatcgctggggatccgaagattgtagaaaccaacaagctgatccagtattatgacatggtggtagatttcaccagcaaagcactggatatcgtcaaaaacaaaggatactctatcaaaaacatgttagagatccgtaaattagaaagtggtgcataatgtctactgaaaatgaaaaatgcgtagtgtgcaagtgtccggttccttctactggttttgtgactgaatccgggcgcgtgtgtagtactatctgtgctgactacatcgcagaaaaaacaaaaaacggcgagatcaacgaatctgatgatctgaatgaagttcaaatgttgctgtaggtacaatatgaaaaattattcgaacattgattttaatgaagttaatcgtcttcttgatttgatggaaggttgctataatgaaatcaaggcaatccgcaaatcatgggaaatcgggtatggagaaggctaacatgaaagaaattgatttgggtatttttgatgaacgtccagatcttttagaatctgacgaacatcctgatttttaataatcataaatagtattgtagtagggcaagggcatgtttatcgatggatgcatttccataatcgaataaaccttatggcctatatagaatgcaatatatatccgtgattgagatttatctcaacctggaacctttaagctaacagtgtgcaacggcacggactactataactttagtacccgaaaggggcttgataaaagaatgctggatgataggcgtactcttttgcgccgtccgatggagtttaccttcggcggggtgattgataacataccttcgatcaagggcatgagtaaaaaaagccagaatagtacctcactggctataatcaaatgtacgtgttgggctgattgcgtcccaaaattaaaaagccccttcctttcggttggggctttttttagaacttttcttcttctccgctttcgagttcggcctttaattcttcggctcgacctttcagcgcatcgcgcatagaaatatcgtctgacggcgcaacatcaacttcttttacacgatttttgtaatatttttcaagctctttaaggccgtccatagtacggcaagaggcgaccttgctcatgaaatcatcaatagccgcctcataaagtcgaaaatcgttgaaactcttcattttgacctctaaatttcgatttgtttgatcacgtagtcaaacttttcttcattgtaaatgcgtactcgttcgattgcgtgtttcataccatagtttttgtatgaatatttatttttagcatttttggactttgccagcgttgctaagttatcaaccaaatcccaaacagtagcaagagatttagaatcatgtttacgcagtacgcgcccaattgactgtttgactataacagcagatttgcaaggatgtccgaagatgatgtgatgcaggttcttgacagaaatacctgtactcagtacaccaatagaaccgattacgatcagccccttcgttgattccgcgatccgtttcatttcgtttcgctcatcaatccccgtttccccagaaatgtatacaacgttgtcatatacctttttgagttgctcatacagccatttaccatgtttgatctgattgaacatcacaaacacgttttcatctttttcccttgccagtttcaacgccagcttacagatccatgcgttacgcctggtatgcgatgttatatacttgatttcgctttggtaatcggcccccttcattttcttaatctcatcctctttgtatctcatgaagatggtattaattcgaaggttggtaacttgaccttcctgcatcaaccgatttgtatcaactggcttgaagatttgaccaaaagcgccaatgtattgcatcatgtttgctttgccttctttcagagaaccagaaaggccaaacttgaaaatacactgatccattgtgttgatgatcttctgtatgctttgtcctgttgatttgtggcattcatccaccatcaaacacatgaactgctgaaaccactcaggaggcattttaacagccgattgccacgtagacacgtagatcaatgcattactgtttttagcagttcctgaccgtattccaagcattgcctcgcgaggtaaaaggcgatagttgacaatatcaccgatcatctgatcaacaagggcggttgttgggacaatgattagtactttgcctgtgtaattttccagacaccaacgagatatcaacccctggataagagatttacccgctgacgttgggaggttaagcacagcacggcggtttttaatcgcatggaacaccgattgtttttgataccaatacggatcaatctgcttgtttccgtcgtatactgggtgttcttctaaccacttgtcaaaatctggctgggtaatttcttctgtttcgtggatcttaggatccatccagatagaatacccgcgagactccgcgaattttgttacaagataggctaaaccgtagggcagtttcccgttatagtccatcaagtatatgtagccgttccatccaccatatttgtattttgcctggtactgataacctggcggctggaagctgaaatagtcgcgcaattcatagactatgttagcctctgcctgaatctgcacatgactagtgttaaggaatttgacttcgatatccactatgtgtatcctatatacggtttatatgaatatttataggctaaataatgataaacattggagaactacaatgagtattgattacgaaaaggttgaaggtttcaaagccttagaacaaaaagaagccaaattacagcttgctacctacgcgcaagaaacgtttgatgtcaaactgaaccgtcagaagtcattcgaaaatatgcttgctgatctggaagctgccgtaccggaagaaaaaccggaactgttgatcgactcccctgatccggaaattgttacatacgaaggtgaaccatctgttcctgatattgctccggaaattgaaattgttcccgacgctctacaagctcctataagcgattctgagacggtttctgatgaactggcatggatggaagggtttaccccgtctatcatcatgatgggccgctctgtttcgaatactggcttttatacgtgtccgtattggatctatgattggatgaaacaaaatccggattggtacaagcatcctgatggttgccctcattattcagcgcgtcaaaccctcaagtcgctggcatggtacatgcaccgtgatgggatggttactgtacgcgaaaccagaaatagccagttcgacacgttcaaaaaataattttaaaaagtagttgaccttaccctgctgttcgagtatatttgtattcgaaggcgggggaatggctctcgcagtgaagaaggaaatacaaaatgaacatgatgaaaaatgcttactacccagttctgtttgtttggactaatggtgaagttaagaaaatcgtcaattctaaagctccttattacactgtaggtgaagcacttcgccacgctgcggaagcaaattatcctgttcatgctgaacctggttatgctcgttggaacggttctaaatgggttgctgatacctgggacaactacgaagaagaaagaatggagtgtgatcctgattacatatctcgtcaaatggaagctcatatgattgcagatcgtagactggataatgaagctcgcggattctattgattaacaaggggctacggccccttttcttttaggtgaaatatgaacttaaatcacgaatgtttaaaagatttgagcgatggtaacgagattggtaacgttatttttcttgatatcgatggcgttctaaataatatgcggtgcatgaaatttggtgaacatatggacatcgaatgcgcacgacacttacgccggatagtgaatcacgctaattgtgatatcgtcatttcctctacgtggagaatcggcaacagtacccataatctacgtgaaatattttatccgtggggattgtatcggatcattggtaaaacttgcactaacttccctcatagtactggaatgcgtggtgatgaaatcaaggcatggatcgatactttcggatgtaaaaactatctcattcttgatgatgataccgatatgctttcttcacaaaaagaacattttattaaaactgatgggtttgttgggttgaccgaagaacaatccacttatgcgatccgtaacattttcggggttactactccgttttgtcctgaatgcaatgggtatggacgtgttaacggctacgacaaatgcggaacgtgtaacggtaaaatactccggctataaataccaataaacataagaggttaaatttatggcaattccttctgtaacaattagcgccaacaaaaacgaacttttgattggcgaaactttgaccttagaggttgaaactactgaactagatctgggtgatgtgtttctggcctatcgttggcaaaaagacggtgtagatattccaggcgcaaccgccgatacttacacaactacggttgacggtacaactgctggcgattataccctgatcttaaaacacggtgctgatgaagaatcagcaacagaaaccacgtctgatacaatcaccgtgaccacttattctgatgatcttgtttctaaatggacggttcacccgattccgtggcgtgataccagctttaccccgatcggttattgggtacttgatgaaattctgtatcaaaaagcacagggtaaagattggaaaactgattatgctgattacaagtatagtgaggaagtacaaacgatcctgaaagcgttcatggaaaacggtgaatgtgagatccaggattcacgaaacggctatattcataaaatgagtgaaatctaagaggctttaaatggcaactgaaaaatggactacggttcatcctattccgtggagaaataccagttttacatatcttccatactggctatacgatattatcgttgatgcttttgagaaaggcgacgactggcgcgattatgcggaagaaaaatataaattagagtttgatactctgaaagaggcgtttgaagattatggtgatattcatgtaatcgaatctcgtaatggtaaactggttagtctgttgtcattgactcctgctcctgaaccagatcctgaccaataaaataaggcaaacaatgaatacacttctttttgatttcgacgacactttagcagaattttctcagactttttatgataagttcggtgtacgtccggaaggaacgccaaaagaacgatatgacgaaatggcggcttctttggtgcgtactgatttttataaaaaccttccccgtattcaggctgggattgacctccttcaatggagtttccaacgccgaatcggtgatcctgctactttgctgcttcgcgcggaagcggtcagccctctttgggttatgaaagaaaaactgaactatacagataagatttgcgctgaactggggatccctcgtctcgattttagtcgcattgactatccggaacagttcgcagaacatgcctatcgtggtgttctgatttcccgcaaccagaaacatcttgaaatctggaacaattctcatctagctaataaagttcctggtattttccttgcggaaaccctggaagaaaatattcagctagtcacggaagcgcttgcaaaggctaatcaataacaaaaaagggaaccgcaatggttccctttcttttacaatctttttaattcatcaagcgctgttttcttatcaccaacaaagaggattgctttacctcctgcttttctgaaaggcaacaccgcttttgcccgatcgtcaaacagaattcctttaccagcgaatgctgctttttcatggctacttttaacgtagtggaattctggaacgtaacccaatactttttgcaatgctttacgtttttgttcggcaacaccgtcagaattgaatttaccaacactggttagtattgctacatcaccaagtgttcttaaatgatggaataattcaaatccttctttgattggttccagattttcgtagaaatcagttttggcaatttttgctttgcactttttcaactcatcttctgtcatcatagagggttcgccatacattggcacaaatgaaccttcccagtcgaacaatacaccatccatatcaaagaaaaacttattcatatcaattcctcagtttgtgtatgcatactataatgtttaatcattaatgtcaaccccaagtgtcagttttcggtgcgtatgctgcaactttagccacaatttccttatccagttcagctacagatttctgaggcttaccacgggctttaactttgatgtagtttgacttaacaacaaacatccctttgttacttgatttcttgatctcgctatcaacaccaactttgttaaagctgatccaaatgtcgccgtccatatactgtttaagagaatcacccatgttcaggatcttcgccatagtaagggccgcgccttcgtgggtatccatgagaatttctttaggaactacacgatcgcgtttctggttctgctgcatagcaatatgcacatcgttcataacccatacgatatgtacgttttcttttttgtatcccagcgtttcgacatcacgcgcgatgcttgccagcttgctcatgccttttaacgttacgtcaaagatgaggttaggtttacgatcttctggtgctgccataataccggaataaacacggttttggtttttgttggaaatgttgaaaacgtcggcgatcacatgatggagggtagatacgttttctgggtttttgaggttcattgttttgacatcatgacccgtttgtttcttgatctctgctgcgagtttatcgctacccattacaagttttttcagggcgtcaacgtccagggtaataccttcgatgcctagcagtttttccagtgtgaaccctttacctgaaccagcaccgccagcaagaataacaacctgaccgaacttaggataagcacggcctccgaaggtgatcagcgcttcggttaaggtgctttctgtgaattgtttaaatgacttcatgtaaaattctccagtttattttctattatttattgacatgctttctgacagtggtgtatggttagggtgttcgacggataggccggaagaactttaaaccataaggtatatgatatgaaaatcaatttacatcgcttcattgtagaattttcccgcaaccgtgacatggactcttacaactattactcccgtgagattgaagatctttttgcggctcacgttggattccttcgccaccatacccctaaaatgcgtcctgaccacgatccgatatatagccctattacatggcaagcccctatcgatggttacgttgaagggatccggatcatgacgtttaacgcgatgtatggaaacgcgttgatccatatcgcacgtgagaaaagggccgaattccctaacggatggcgtattgatgaagtgattcaaaaccttatgcagttacgacgtgaatacaaagcgggtatgtgtctgcgtaatgaacagtatcagatgtataaaacgtatgcatatatctctaagcacctaattaactccatgttttacatcgttggtaatcatggttccgctatagatatcggttcttatgaaatcgtggcttatgctcgcgaacaaggaaaggccgctgcactgaaaatcattgaatctggtgctatcattcttaaccatcgcattgatactattgcttactatggtgatcaggttgaggttgaaggcgtacaccatgaacgattcaacaaagccgtatttactaaaaatggttatgcgtatggtaatgacattataacttctgcggttcctttcgttcgtctaactgttgaaggatttggagaaaggttgccttataaaccgtcagaagctcaaatgtgtgcggctgctgaaagaatagccagaaagcggaaaatgtataccgatgaatacctggcgtatgtcaacaaaacaaaagaagatgtagatcgagaaatttcttgcatggatttatccatttgatataatgtaagcatctttttaagggaggatacatgaaaacgatacattgcagaaatgaaaacgttgtttattatcacggttcgtgtactgctgctggtattgaaagcatgttattgcctccctgtgattctgatactctgtctgaaaaaggcagaaagaaaaatttagaccgtgttttctttaccgctgatatcgggttagctcgtatatatgctggaagggccgcacgttctataggtggggatcctgttctgtacagggttgtgtgtccggttgatgttgtatgcatgaacgaagacaaaggcgcgagcgtttaccatgcagcatgggcgttttgtgaggaattatgaatgataaagtgttggcgtatctcgttttcttgttgggatatcgcttagaagtgatgggcgcgtattcatcaatgtatggtgatttaacggctatctggatggttgggttaggggttgcttttacattcctttcctttgcaattgttaatgaatcggaagaggatattgtatgaaactatatcatgtgatctactctggtgttttaggcattgacaaacaaatgttagttgatgtaatgtgtaaaaaactcgatgaacgaattggaacccgatacaaaaatcatgtatcggaaagtattttcatcaacgttgaccatccaaatgacatggaagaaatggtcaatactcttgatgatcagcagatcccgtttgttgacaatttcaacatgagcgctggagtgtatacggtagtaacttttgttctaaaaaatgttgacagccgaaacgatagcgtgttgaatgtagttgcaaaaatcgattctaccaaaggaaaataatatgaaaattgtacaccgtagcatttccgaactgtctcaagccgaaaaagtgcaaatccatttcaaattcaatgatttgcgtaaaggttatgccgaaattgcccgtgaacatgggttagataacggcgatatttaccaggtagtacaggaaattgaacgtatccgcgcgttccgttctgcaaatctacctgttaaaaatgcaatgcgccgcgaagcgatcgaaatccatcgtaagcgtgtgtacaatttagaacgtgctaaacgtccgatgaagaaagaaaagaaacctcgcccgtttaaacgcgaacatcttaacacctctatggcgctggcgtttcaagatgcggggattatctgatgcgtaaatctgcgatggatcgttgggctagtattgctacttcaaacgtaaaaccaaatcaagccgctcctgatgtagaagcggttcgtaaagcaaaagaacctgagattgtggcccttagccccgaactcattgagcatcgccgccgtgcgtctgctattgaactggatctgcgtattgcgcgttcatacaatctcaagcatgaacacgccgcaaagaacaaccattcttttgaccttactctggaagattggaaagtattgatgacaactgaacgttgtcagtattcaggcaagatgtttagcaataaacccggtagcccgtatgcccgtacaatggaacgtattaatccacgtctgggatatacacaagaaaatacaatagcggttatcaatgctgctaatgctgaaaaatcaaatctagatgcattcgttaagggtgatgtcattctggatgaagtaaaagtgaagttgctgcgtaaagcactttatcaagtcgaaaaacgtgtgaaaatgaaaggttaaattatgtttaagaaatattcttctcttactaaccattatgaaggtaagttcatcaatggtgtaattatgaacgggcttactggcggtgtgtgggttgcacgtgaaaagatccacggtgctaactttagctttatcaccgatgacggtattaccgttacccccgcaaagcgtactgatgttgttaagccagccgaagatttttatggctgttcagcagtagttgcaaagtattccccagggatccgtaagatgtgggaaaccctcaaaaagaccggaacttatgatgatttggttattcaagtctacggcgaatttgcggggcgcggtgtacagaaagatgttgattacggcgaaaaagatttctacgtattcgatatccgtgtaaatggcgaattccttcctgataacctgtgctcgctgatctctcgatctcatggcctgaaaatggccccgctgttgggatatggtacttttgaagagatcaaagaactgccgatcacgtttgaatctgttgtgaataaagcaaatagcggcattggtagcgataatacagtatatggtgaattcgtatatcctatcatggaagttgaagagggcaacattgcagaaggttttgtaatgaaacctgtttcacctgcttttatgccaaacggtgaacgcgttgcaatcaaatgcaaaacaaccaaattcactgagaagaaagcgaagaaagcaacccgctttaatgctccggtttcactgtcagaaaaagacaaaaaccaactcgatgagtttgtttgttaccttacagagaaccgtgtgaaaaacgttctttcgaaactggatctggcttcgatcactgctaaagatttcggtcgcattatgggcttaactgttcaggatgctatcgaagaaatcagccgtaatcacgggcctttcctcgaacagttcgaagacccagcaatggctaaaaagctgtttgtaaccgaagcccaaaacatgattcgccctgtatggggcaaaatcctgaaccatgaattttaatcagattctggttgatgcaaaagcggctaccctgatcggtagccgtaaacctcctgaacgtatcgcaaacattgctgttaaaatcggacgtgctttgaacgaacgcgggatcagggcttattctggcggcgctcctggtatggatagtcactttctgtttgactatagtccggataacagatgtataatccttcctgagaacgggtttaacggccttttctcaaacggaaaggatatcatcgactttcgagatttaaacacacagaaagccgctgacgaagccagaaaggtagcaggtaacttcgatacacagaatgaatacgttcaaagaaggtatgcgcgaaacacgattcaagttcttcgtgaaaatcttgacaatccaactgattttgttttattttgggcggaagaacgtgaaggatgtgttaaaggtggaaccgcgattgctgtaagattggctaggttgtacagggttccatgtttcaatctcttcaaagaaagtgtattgaacgatgtgtgtgatacgttagggatcaatatcaaacccccaacgttggattttttatggtaattgaacatgcgcccttacttcgtgaaacatacgaaagatgggctgttaataacgcaataggtgaaaatatgattcatgtacgtagtatcggtactgacggcgaaactccggtagaaggccgatcccccactctcgcagaacgagcaagagaaattatcaacgatcagaatactaagatgatcgaacatgcgcgggatacaatcacaaaaggtgttctgaaacacgcgacaaaacaaaaccttatctatgatatgaagcacgatatcggctcttgtctgggtattgaatgtactcgctatgcattccaacgagtttctgaatggttggaagaagaagggctaaaattcgatacagaagaaaaacgcaacgccgctaagatcacaaattctctggctagtaagtacaatcaaacgtatcgaaaccatgaagaacgtgaagtgttttctgaaaggaaaatagatcgccgtgtaagtgaattcactttttacattagttggtaaaaaggtgttgacgggggttggttatagtagtattctaactcccgtagacaagacactaactcagaaggataaacatcatggaaatcgtaatgaaagcaacttatgctggatactgcctggaagcaaaaggtgttgctaacaacggcaaaggcttacgggccaatgttgaagcaatgctggatgaattacatgcaatgtacgaatacgacaacgtagcgggtagcgttcttatccaggcgttggaagttgatggtgttgattgtgctggttggtgggatgcttacattgactacaacgataaccgggtttacctgttgagcaacaaagattatttctaaggaaccactatgagcgatgaagctgaggctttagaagattgggctgattttgatgacgaagaagacggtgaatatttctgcgttaatcgtggtgcttataaagaccgtttagaactccgtaaacttttatcgggttcctctcaaatatcaggatccaaacgaaaaagtagtaaacaaaaagttcagtatagtgatggttctgtacgtgatgaaactgttgttgctgaattccgtggtcgggttatcacaaaagaaagacaaattgatgtaaagaacttgtatgaagtggctaaggctgctaaaataggttctgtgattgtttgccctgtgtgcaaagaaaaacacacaaagacaacgtatcacaaagttttctgttcgaatggcagaaaaaccagtaaggattgtaagtctaaatatcacaatacaatccatcccgaacgactggatcgggtattttaaaataaacctaaaacgtggagtacgtttatgaacaacaaaactttcgaagaactgaacagcatcatcacttccgtagattcctataaggtttctcactggtcgcaatatccaactggctccgaagaggcgctgttttatattgaatctcgtggtggtaaatttgatcaagtagttacggctggctgtaaccgccttgcgcaaatcctatcacgtccggtgactatggaaaacgtggattttgctaatcggttgtacaaaatgcactttgggcgcgaaatcttcaactacaaaggttggaaagaaattgcagaactgggttacatccctcttgaattcagagcgattccggaaggaaccccagtagcggttaaaaatccggttgcaactttccatgctgggaaaaatgcgctgtggttagcaggacacgtagaaaccctggcgatcaggggagtatggttcccttcaaccgtagcaactctatcccgtgaatgtaaaaaagtgttgaagaaatatctcaagaaaacctccgatctcgaaggtgaagcatttgatatggtgttacgtacccgtttgcatgacttcggcgcacgtggaacctcttctgctgaatccgctggtattggtggcctcgcgcacctgtataacttcctcggtactgataccgtagaagcgctgattatggctatctctctgtttgaagattgtcagaaagcgtttgatgatggtgaaatggcggctggtatttcaattcctgctcgcgaacattccactaccgtttcttacggcaaagaaaacgaagaccttgcgtacaaaaacagtattgagatcttcggtgaagggatgtatgcatgtgtgtatgattcctgggattttaaagcggcggttcgccgtatcgcagaatataaagattcgattctttctaagggcggtactctggtagttcgtccggattctggtgatatggtagacaatatcatgtacgctcttgaagaactgggccgtatctttggctatacagtgaactcaaaagggtataaagtactacacccagcagtaaggatcattcaaggcgatgaaattcatggccctgaaacaatcaatcgggtgttgaactggatggagtctaaccgttgggcgtctgaaaacatcgcgtttggtatgggcggcggattgcttcaagaagttacccgcgacactcaaaaatatgcgatgaaaatgtgcgcaatcaaaattaacggtgtgtggactggtgtgtataaatgtccaaaaggcgctgaatggaaaaagagtaaaaaagggttgttgatgactatcactgatggtgttaactttaaaaccattgatactctggaacagaaagtgccggaaggctggaaagatgctatgatcacatactatgtcaacggaaagattacttcccgtgacactttagaggaaattaggaaccgtgccgggatttagtatccgcaaaaacaacaaaggaaccgtgattttctatgacaacattccccttgtagctcgcaaggggctttttgctaaaatcgctgggtattcctttaaactggaagaagtcaacgacgaaacactaaaagagatcgtaagaattgccttacaattaagaggtaagaaagacgaacagaaagctattgacatgatcaataaattgggtgaaactcaatgctttatagtgaatcgtggttacaagtacgataccattgcaaaatttgaaaaagggctttgtgaattatgagttattatggtgtgatcccatacacaggaaacaagcaatcgctattacctgaactattcaagctgttccccgaaagaagttcatacatgcgtttcattgattgtttttgcggtggccttagtgtgtcgctaaacgtccctaaacccgttctaagcaacgattatgataagacgctgattgatatgtatgagcgtcttaaaacgcttcctgacctgtctccggtgcgagaattgattgcatcgaaggggctggggaaagacaagaaagaagagtatctgaaattccgtgatgaatacaaccagaacaaagatcctttatggctctatgtcctgatcctgcattcattcagcaacgttaaccggacaaacgacaaaggcgattttaacgctgctgtaggaaaacgaaccctcaactttatgacagaaaaacgtttcgaacatttcaaaaagaatgtgacaggaattgaatttcgttctggttcatactctgatattgaaatcaacgataacgattttgtttattgcgatcctccgtatctgatcactgatgcggtgtataacaaattctggaacgcagatcacgaacgcgagttatatgctttccttgactccctgcatgagcggggtatcaagtttggtttatcaaacgtgacacatcatgcaggaaagcaaaatgatatcctgatcgagtggatgcaaaaatataatgtgcataacctcgataaaaagtatctgttaggccagcatactgattcttacgaacaaaataaaacgcaagaagtctacgtgtgtaactaccagaaacgcgacgtaaatacataccctgaaacactggatgacttaatgtaaggtaacatatgtttaagatttttggttatatcccttctgtttataattgcgctccatgcctgaattctaaacgtctcctggacgcaaaacgaaaagaatatgagtttgtttctgtagccgatgaaaaagacgcagacggcaaaccgatcctgaatgaaacggtcatttctgaactcgaaagcctgttaggtactcgtagactgaccatgccccaaattttccacgatggtaagcacatcggcggctttgaccaactgcgtgagtacgttcgcacgttgggataaatattaacacctttatttgattggtgttattatgctcactaaacgtattactaagaaagattatccatccattaaacaagctctttttgaacagcaaaacggcttgtgcgcgttatgtggtcgccctttagagggtgaccttgaaaaacatcaccttgaccatgatcatgctctatctggctctaatgccggacgtgtgcgcggcctcctatgtaacctatgcaacggtacagaaggtattgtaaagcacaaatttaatcgttctggtctggtttcccgtgatgttgattatatcgaatggctagaaagcctggtagcatacctcaaacgcgactattcacaaaaccgtatgcacgacaaatttatacccgataaggttaaatggtttacacgccttactaaatcggatatgatagccgaaatgatttctatgggttttgagtacgccgacaaagacgaacgcaaagccttaaccgcaaaatatagaaagcaattaatgaaggcaacgaaatgaaatatctaaacgctcgattatcaacgcaacagaagaaaaagctgatgatgttgatatcctccactgacaaaaagatcatatctctacatgattggatgcttggaaggggtgactctgatttgtgttatgtcaaaccgaaagaccgaacgatgtttgatgatcgcggtcgcacattgactaatttttctcctatcaccgttattgatatgtgggaactccttgagattgtaggacgggatatacctgttgacggggttgaactgatcaaatatcttaacgagattggacacaatttagatattatccataaggcaacgaaatgaaagtagaaaaacgcgacggtaaaaacgtcgatttcgataaagaaaaaattcgcaacgctgtgtataaagctggcgggactatgacggatgctgatgccgcaatcatgctggttcagtacaatcagatccgcgatggtagcgcaatgaagatcgcccgtatccaggaactcgttgaagaatccctgatgaaaacgaacccagcggtcgcccgtgcatacatcgaatatcgccacgatcgcgatattgcccgtgaacagaaaagtaagctgttcaaagatatctccggtatggtgaatctgtccaacaaagagatcaccaacgagaacgcgaacaaagacgcaagggtattcccgacacagcgcgatttgctggcgggtattgtggcgaagcatttcgcccgtaatcatatccttccgaaacacatcgtagaagcgcatgattccggtgacatccattatcacgatctggattacagcccgttcaccccttacactaactgctgtctggttgacctgaaaggtatgcttgagaatggtttcaaaatgggtaacgcggatatcgaaccgcctaaatcgatcggtgttgctaccgctctcatggcgcagatcaccgcacagattgcttctcaccagtacggcgggacaacctttgcaaacgtggataaggtgctggctccatacgtggaaatgacgttctttaaacatctgcgcgatgctgaacattatggtatcgaacactataacgattatgtgtatgcaatcgagaagactgaaaaagacgtgtatgacgcgttccagtcctacgaatatgaagtaaacaccctgcatactgccaacggacaaaccccgtttgttaccatcactttcggtactggtacaagcgactacgaacgcatgatccagaaagcaattttgaaaaaccgtattcgcggcctgggtaaagagggtatcactccggtattccctaaactggttatgttcatggaaaaaggaatcaaccttgatccagaggatcagaactatgacatcaaacaacttgccctggaatgtgcttcgaaacgcatgtacccagatatcattagttcagctaacaaccgtgctattactggttctagcgttcctgtatctcctatgggttgtcgcagtttccttagcgtgtggcatgatgataacggtaatgaaattcttgatggacgtaataacctgggcgttgtgacaatcaaccttcctcgtattgcgattgaagccgaagcacaggaagatgaagacgcgcatgatgcattttggcgtatccttgatgaacgtctggaactgtgctttgaagccctgatgactcgtatcgatagcctacgcggtgttaaagccagtgtagccccgatcctttatacagaaggtgcgtttggtgtaaggttgaaacccgatgatgaaattctggaactgttcaaaaatgggcgtagttctatcagtctgggatacatcggattgcatgaaaccctgatgcttttcggatctggacagcacccattcgaccggatcggttctcagaacatgggtagactgatcctggaatatctacgcgctgcgaccgaagcatggaaaaagaaaaccggatttgggtttagtctgtattcaacccctgcggaatctctctgccatcgcttctgtaagctggactttgagaagttcggaagtatcaaggggatcacggataagggctggtatacaaacagtttccatctggacgttgaccgcaaggtaacaccgttcgagaaaatcgactatgaagccgattatcattacattgcaactgctggacatatcagctatgtagaattccctgatatgaaaaacaacctagaagcccttgaaaaagtatgggattatgcaatggataaactggactacttcggaactaaccttccggttgataaatgttttgaatgtggctcggatgatgaatttaagccaacagaagacggttttcattgtacccattgtgggaaccatgatccggaaaaaatgagcgtcacgcgccgtacatgcggctatttgggtgctcctgctgtccgtgggttcaacgaaggtaagaacaaagaaatgatgcatcgcactaagcatcaaaattaatcaaaaagcccttgacttcggttgagggcttttgttatattgggcctatcgaaaaggagacatattatgaaactgactaagaaaatgaccgatgtagtggcatgtgcgtttgcattaggctacaaagttgaaaatcatccaactcgcgttgaagtcatcaaccctatcaagggccgtcctggtttggttctgtgtgaagacggtacagcatatcgtaatgatgtctctttagaactggcaactactatccgcaccgcaaaacaaatgaaagatgttctcattagcggcgcaaaattgagggatttatgatgtattggacaaaagataaatttgtttttcgtgatgatacgtgctttgggactgcataccgaaacttagctattcgtggcggttcgttttcggctaatgatttgtctaaggtagtattccctattaaagttactgagtatgacgtattcggtgttaaaggatttactgattactttggtacaaagtttgaatcagaatcttacatttttactaatagcgatcgtgaattattcaaaaaacacgttgttgttaaagagaaaccgttattaccaaaagaggatgaagcaaaggaaatctatgatctcctgaacatgcttgacaatctcggtacttgtcatctgttcggtaaacgcgcccgtaaagcgaaagatgttctcaacttgttgcgctctcgccggaattacctgatccgggaagctgaacgcaatctgaaaaattcagaaaaacaggctgaaatccataaatccacccttgctaaattaaaggctttgtgatgtttccgttatacgctaaagtgcgtcgaaatgtcggtaattcatatcaggaatggagtgaatggctacgcgaaacgaagtcattctacatttcaaaagccactgatatgaaaggccgtaacattcgctatcgtaaacccagtggtaaacgagtgaatgggatagattacattgttcttgattcgattcgggatgatatacgataatttaactttgaggcaatattatgattttcaacaaaacaaattcacgtaatttgaactatctacgctgtgaactggaagctaacgaaattgaactgtttttctgtggggctacagatccggaacacaaattgcattgggtatccggtgagattgtaagcctaaccgatcagattgtcgaagaggctacccgccgcgatgcaatcgttaaaattggtgctgttgatgtgaactacgaaggacatccttcatttttcattcaatattatccataaaagtattgacctgtatatctgaatgtagtaacatccttcttgtcaactaaggaggatgttatgaaaatcaaaaacactgctactgaaactctttgcaacgaaattgcagaaatgtactggagtaaaggtcacttagaggctatgaaagagtttcaaaagtggtgtgatacccaaaagttagctaaatgggaatacatcgttattgttgaacggatcaaagaactgatcctcgtgaagaaaggtaacatgaaatgattcaactgaaattagacacaaatgcggtgttaagcctgtttccggaaggttcaaccgcccgcgtagacctccaatctgctatcatcaaaaacgtggtgaatagcgtagttggtaagcgtgttagcgaagaaatcaacaaacggatccaggaacagttagctgttctaatgccgaactcatccgaaattacacagatcatcaaatctgaattctcggattacgtcgaaaaacgttatggttattcgaatgttttcgatgtcaactatggcaatgttcgcgaactgtctggtaaaatcaaagaatcggtaaaacagcaatgccaaaccattcttaaagatatcgagaaagaggcgattgctcatgcaacagaaaacattattgcagacgaagccgcgtttatcgctcgcgtctcgaataacctggaagttactgtacgcaaagcagtaatgcaacgggttaacactcagttcccagacattattgacgaagcgatcagagaacgtctgtttggcgaaaaagcatgaattacgaccgcatctataatatggatgtggtcaacggaaaagggatccgtgttgttttgtttgtgactggttgcaatcataaatgcgaaggttgttataacaaatcgacgtggaatccttgcaacggaacaccgtacacggaagagacagaaaaccatctgatttctctgttgagtaatccgcatgttgatggacttacattaactggcggcgatccgctttaccgtgacaactatcctactatcctaaaactgcttgagcgcgtttctaaggaacttccaaagaaaaacgtatggttatggacaggatataccctggaggctttacaggccgacccagaacgttctaagctacttccttacattgatgttctgattgatggtaagtatgaaaaagatttgccaacgaaaaagccgtttcgcggttcagataatcaacgtatgatcgaattcgctaaaaattcgatagaaattaaaaatattgcttgacctaatgtgtaactatggtaatcttaccacatcgtaaatgacgattaactttaattgagagataatatcatgatcctgaatttcaaaacccgtaaagaagcacgtaactattgctggaagtggaacattcccctgaaaaccatccgtaatacagggcgcggttcttgcccgtggacagttcaagcaaatgaactgaaaacgttcgtggttggtaaaacttacaaactggttgaccgtgaagggtttactaccaattcacatggcggatctaacatagcaaacactatccaggcgaagcagatcgaaaaattcctgaataacgaggtaaaaattatctcgaaaacccattcagatactttcaaaattgatcatcctcctgaaatgacttatatctctctgcgttcgtgggaagctcgttatttcgtcgaagttggcgcggctccagctaagaaaaagaaagccaaaccgaaaaaagccaacgttgcggcttcggttgcgcctgttgcaccagcaaccgcagatcttgatcaaatgcttgatggcggttcggcaatgtcggttgaactggatccgactaaatttgttgaaggccgttcgtatgttctggttaaaccgcagcaatttaaaaatcgttgtggcgctaaccctgggatcaaatcatataccgatgaacacagtaatggtatatacaccgtttaccatacgaattcgctcggtcatcatcaattgagcaaaacggtagaaaccattgattccccgaccggaattgttggttactatctgcttgattctgaacgttcgttcttccgtgaactggcaaccggaactgttgatgaacctgttagcgtttccggtaatagcgctatcgctatcaatgtagacgaagcggctaagaaagaagaaatcgcaaaagcaatggtacagcttgaagaagcggttaaagcccatgaggacgcgcttcaaaatctgcgtactgcttccgacctggttcgcaaagctgctcgaaaagtagcagaagtaagcaagtaaattaaactgggtgctccggcaccctttttttatgaggtgacacatggaattattagaaggtaaatcttataccctgaacatcgacgctaaagaatttgcagaaaaaacctggcgaaatgctttagctgaattgatcaaaaacaacggctatattacaatcgatcgtattgcgattggggatactgaggacattgcttatgttctgcaagatgatttcgaatatgagatccctagccatatctggaaatacttcaaaccatatgatttaccggaagaagaaccgaagattgctactaaagaagaaatcgccgcgcctgatttaaatttcgtatcttccgatcctaaaatgtggatgactgtaaaacctgttcaacaagatatcaatgatctgcgatttgattatccttttgtcaagcggatcacttcgatttctgtactatcagcgccgacggattcacaggcacttgaatttgcattacagcatgttttcggtgataataagctgtacgcgattgacaaggaagctgctattgatgaacagaaaaaggaaatcatcaaccttctttctctgcatcaacaacttgaagcggtggaattgattgagcgtatgctttctgatacaaagaaagatatcattagcaaaatcactccggcacgaaggaaagcaattgatgaaaatcgagatttacggtattcccgaatcgcttcataaatgttatggttgtattgaagctcggaaattacttgatgagcatggattagaatacgaattttattctgttctaaagccagcaaataacagtgtggggtttgattacgatagaccccgcattgaagagttagcgaaacgtgttcgtagtcgaagcatggcatttacttaccctcggatctttgtagatggtaattttattggcggttatatgcaattgaaagagtatttgggtgaagcatgaataaagaatacattcgcaaagtagcaaacgctattcacgcaacaacgattgattttctggaagggtttgatcatattatccatcctgaaacgctggatagttgggaagccaaactgtttaaaagtatcaatgaacagtttccggaaaaggttaagcgctggtttatcagacaggaaatcgtagcaacgatccttaatgaacgtggtgttgaggcgttcggtgtaacccctctatataagcgaaaccagattacagacgaaacaatcaagaaatataaaaagatggttcggaagtaataaataatcagttaaatggccttcgggccattttttgtatataaatattggtattgaatacaatataggaaaaaagataatggtagctaaatcattccgcgcacgaagtggccttgatgctgctggtgaaaaagttatcaacgttgggaaggctgatcgtaatacgctgagtgacggcgttaacgttgactttttcaatgaatttaacggaatccagcagtatgacccgacccgtggctattctcaagacatggcgatcatttatgcgcgtcgtatctggtacgcaaaacagaatattgcttcccctgctggggctttcgacgaatccaaatggatcgcaactcgtaatgacccgaaatgggtttatagtaacgtaaccactccagacggtagcattattgaatctggtagttacattatggctgatggacgctttactgaacttctgtacctgctgccggacaacccgacagagggcgacgtaatcacgtttaaagattgcggtggtttagtaggtgtgaacagtatccttgttaagtctaacacccgtcagatccgtttacgtactgtacaatcggcacagtatcgactgacccacccgtacatgatcgcaacgtttatctataacggtaacgtatggcgtgttgctgaaactctggataaccgcgattctgagatcgtgaacgcaaccggaacaggttcattccagttacaatctggtatgacagttttccgtaacagtgctacgggtaaaatcactctccagttgccgaaatatgcaaatgatggtgatgtgatcacaacctatgacgctgataaaatgaactctatcaacgtagccgttttgcagatttatccaggtagtggacacactatttctgacggtgcaattactggtgttacttcggtaactagccagaaatctggctttggtatgttcatctttgatgcacagaatagccaatggaaagtatatgatgctgataatcgtgttcgtctgcgtcgtatctatagtgatttaaacacagttcctaacgattacgtttttgttactgcaaacccttctgggactataccaaacgttacagttacccttccaactgatgttgctgatggtgatcgcgtttacgtatccctttatatgatgggtaaaaaccagaactgtacaatcaaagttaaagatggtacaacggacaagatccgcaccaacaaaaatatgatgcagttcccgcagcgcaaagactatccgcctgatgattggtttagtgtaacttcattagcatttaatgctgctagtgattacctcccgtatatcgagttttcttacatgaaagctacgaaagaatgggttgttgctaattatcgtccgatcgttgaacgtgttgacgcaactaacagatcgcgtactggtgttattgctctggctgcacaggcagaagtaaacaaaaacttggaagacaacccgaacgacgaaactgctattactccaatgacgttagcaaataaaactgctacagaaacccgtcgtggtattgcacggttagcaacaactgctgaggttaacaaactttcaaccgatacctatttggatgatgtgattgttactcctaagaagctgaacgaaagaacagcgactgaaacccgtcgtggattggcagaaatcgcaactcaggcagaaacaaacggaagcaccgatgatattacgattgtaaccccgaaaaagttgcataaccgtattgcatcgccgaccttaactggtatacttgcccttgttgctacaggtggtgctcctaacaccaacacggatcgtgctcaggctggtactggggtttatgatcattcagattatcagaaagcggtaacgcctaaaactcttcgtgagtataaagcgactcagttacaatctggtgctgtatggctggcttctgaaaccgaagttattaatggtactgttgcaagtgcaaacattccgaccgtagttactccggaaatgctgcacaagaaaacctctactgatggtcgtattggtttgatcgagattgcaactcaggcagaaacaaacgctggtactgattacacgcgagcggtaacgcctaaaacgcttaacgatcgtgctgcaacggaaacgctgacaggtatcattgcaattgcaaccactgccgaagtatcagcaggtactgtaacggataaagcgatcgtaccgtctaaactgaaaggttatctggacgatacaagccatattactgttgctactgctgacgggttaactcaatctggaactatttggactacggttaacatcggtattcaatcagcaactgaaacacaacgtggtactttacgcgtcgctacgcagtccgagacgaacgcagggacattagatacagtatttgtcacccctaagaagttacacgctaagaaagcgactgagagcgcagaaggtatcattcaggtggctacggctgctgaaactaccgctggcaccgttgcaaacaaggctgtttctcctaagaacttgaaaaatacaattcaggttgatacttcatggcaagctaccgatctggtacgcggtactgtgaaactgtctaaggggcttggtacttggtctggtaatgatgtggctggttctactcttccggatgatggttatgccgctgtaggtgttgctgtttctccttatgaattgaacctgacgctgaaacattatctgccgatcggggctaaagcggttgatgctgataagctggataacctggattcttcccagttcattcgtcgtgatgttgatcagacggtcaacggggcgttgactctaacgagaacaaccactgtacaggccaacattgattcaagcgctgatgcaacattccgcgtaatgaatgttaatggagatctgaacgttggtgatggttcgtcaatgggtaaacttcgtttgaatggtggttcatctaacgactggtcaattcaagcaagttcagcctctgggcgtattgcaatgatctcaacgggtaacactggcacagttcatctttctgtgtataatgatactcgcggcgttgtagctaacgttaaattccaggctcctgaaattcaggcgattagcaaagtgactctgggtaatgataccgtgatcactgctgctggttctgttctatctatgggtacgaacaacaagacaactaagatcctgacctctgatgctggcaacatcgtagcggaagaatctgcgaactcttataaagtctttactgagaagaacgcgcaaaccttgcttaaccctacgtatgtacgcaaagcaggtgatacgatgtctggacggttgacagtaaacaacagttcaattatcatcgcaggtcaagcggcttggtcaacactggatgcagtaacagaagcatccaggggcaactggacggctgagatcacagcatcggcacaatacaacttgcttcctggttatgcggttccggttcttgaaccagatccgattaatccagaaatcatgattgtgacccgttatacctatgttaaagcaccgggtactttaacgcagtttggtaacggaactgcattcacttatcagatttgggcacctcgtccgacctctggtactggtgttgatgcgctggcgcaatccttctggatccgccaaatgaacccaatcacgggtaaatttgatggttggggccgcatgtatactagcaacaacccgcctactgctggcgagattggtgcaacgtctgctgttggtactacggttaaaaacatgactgttaccgattggatcaaagttggtaatgttaagatttacccagatccggttactcagacagttaaatttgagtgggtggcataatgtcaaacttaatggcggggttcggccccgattttgtagaaacgcaaattctatcggaaacaaacagcgtaacttacagaataaccgcaaaggcaacacatcccaattcggttcctaatcagtatgagtttacactaaatcaaaaggcggtagggacaccgcctagtgttgggatcaacgtatggagaattaacaatgctgtagttgatccaattaaaaccttcacattatcgaatgataattcagcaactgcaaacaaagcgtttgttgaatatatggatgctcaaacttctgggctgtatttgataatgactaacggtgaatacaaaacaagccaaatcgttgatgattggtttgctaaaaaaagatccgttatgtggcaaggcgctgatttcgctcagagattcccaaattctgcatatgttgcattgtatggggcttcaaaatctcgtatactgattgaatcgttttacgcgaacgatggagttttaaaagaagattcacgcgcatcaatcgatcttgtctatgataacgttggtgatgttgggcgaactggtgtacctttccgatctgttgaagatacggaagaatacaattcaaccaatggatctgaatataaagtatatcctgttgcaaacccagtgatctctaaactggctgattatggtatggctcctggattagctatgatgattgctggtgatttttacgccagcaaagcattattggatgctggatcaacaacaagggttactgttcgatggtttacgggtactgctcaaacttcatcatcggtgattgaagttcctgcaaataaacctgatgagtggttacgatttgaacagttctatacgatccctagtggttgtgatggatttaacgttgctgtatctcgttatcctaaacccgctacggatagtttatctgcgatccgtaactttgtgatggttcaggtatctgctgccgaagctgatcaaaactttgctgcacagtttggggttaacggtatcagaatgaacaacatgatcgatggcggaacaccgtatatatttgaattgccgaatactaaggtttatcctggtggcgattattctgcttccgaattccgtgaagttgatgcataaacaaaggctcggatcatcgggccttataaatatgtaaaaaggggttattatggcagatttaaaagctggttctacagtcgggggtttacctatttggcactccggcacatttccgctggttccggttggtaatactctaacctatcgcggatataaggtttatactgaaaacgataaaccgcaagcatcaaataacgacttcgtttctaaagcaagcggtggtcaatatttgggtgtagttgcctttaaacaggggctacaaattaacgctactttcacaggcggaagtgaccagaacggtttatattctggtgatggtgatggcgcgacattatcaaaagccaacattgatcttgtatcatggtatggtattggtattcgttcatcttccggtactaatggtcgcgtattagtcatcaacgctcgaaatggtgatttaaacactcagggtaatattacggttgaaaagcaaatcagtattacaaccgctaaccctactgacgcaagtcatgcaacacgaaaaagttatgttgatggacagataaataatgtcacaacaaatgctaatagcagggtattacgcgctggcgatacaatgacagggctgttaactgccccgcaattcgcgagcacaggcgcggcttcccgtcccgaacacgtaccacggctcgaccaggtaattactaaagggactatcatagattttggatcttattaaggtgaaacatggctgatttagaaaaaattcaattcctacgtagcacagttgcggggaaaacacctactacaagtcagcttgcagatggtgaactggcgatcaacatggctgattatgccatttacacgaaaaatggttcttcgatcgttcagttagcgggtaaaggtatcccagaaacaaataccaaaaaattaacagttgatgggcctagtgctcttaatgataccgttaccgtagcggaaggtaaaactattactttcaccaacgagaatttaagtggtgaaataactcgtcatatcgtcggtaaatgtgccagcaatgatggatggtacatcggttccggtggtacaagcaataacggcattcttgaaatcggtactattgacgatggtactgaaacaatccagtttgtacaacgcggtgctggtaacgtagaagccagaaaattagtcttacttgatagctctggtaatactactcttcctggggatttaagattatccactaataaaaccgttaaaattaacaacggaagctctcttgtccttgaaatgggtgtaggtgctaatgacgcttacattaaaaacttgagaggctctggcgttcttcaattaactaatgacggcaatctgacattcagaaattcccaggtttattatgccacggatggaagaggccctggtaaagatggtactcttctgactaatgtagaaaacgcgcgtcagcttgagcaagataatttccctgtaactacaggcaacgaatctcgttggattaaagttgctctgttaaaagatcccggctcaggtcagagtcgcttgcaactgatggtgactaacggcggtaactatggttctacgtgtagttctatcgactttatcgattgtagtgctcgaagcattccatcgacattaacaagcagtaacatacgttcttatctgcaaattcgtcgaatcggcgatcctggaattgataacactaaccaaatgcgttatagtctggttcgtacctctgagggtttagaactgtggtttactcaacgcgcgtttattggtggtgttaaagttgctctgctgtctatcgctggcggtgctgttactgaatattatctgcctactggttacacaacttctgcaactgctccggaaggtttagttgagagtgtggctattcgtatctatgacgaaattaataaacctaaccttgacaatggtactgatggtattctgtctattgctaaaggtggtacaggcgcaagtacagcctctgctgctcgcacaaacttaggtttgggtacggctgcaacccgcgatgtcggcgaaggtgctggtaatgttttagaaaatggcgcttatggcttaggcggtaatggtggtaaatccatcaacgacattatctctaatgcggatatgttgacccgcttaaaatcatacggcggtactttctggcgtggtgttactaaatctggtgttagcgttcaaaatggtctttatagtcatggctctggtatttttatgaatgctggtgataccatgtcagccattaatatcgactatgctagtgctaaagttcgtgtatacgcggctaacaacgcggctcttgccgcaggagatgtcaaatacaacgaactttacggtacagcaaataaaccgtctaaggccgacgtagggcttggtaatctgacaaacgacactcaggttaaaaaagctggcgacaccatgactggtgatttaactgttcctaatttacatgcttccggtacggggactgcatcggtatatgttaatgccggaaccggaaatgctcatgtatggtttagaacagacagtaatgaacgtggtgtaatttgggcaactccaaatacagcggacttaggacaaattaatattcgcgcaagaaccactggaggcacttctgctggtgattttagcttccgttctgatggccgccttgatgttcctgtagcagttaaaattggtggagcagcaatgctaaccaaagacgggaatattacctctggttcgatgtttggtggtaaccttaacaactatttgacttctattaaaaacgatatcgttgctggtgataataagcaagtaagcaagactggtgataccatgaccggtaacttgactattaacgctaacttaaaagtcgaaaaccctaatggaacgatggttgatttaggttcagagaactctgataagtatagcagattaacccttgctcgtaaagttggtagcggtgctaccgtagcaatgcttaaagttactcctgaaggacacgtgcaatttggctatcaagatgcagttgctactccagctcctagtaaatatattctagttaaatctagcggccttgaggtagaaggggacttggtttttaaccagacatatagtggtgctgaagacgcagttgatattactgataagactgttgaccttaacagtttggttattaaaaaatccggtttaggcacccgtcagctgtataaatgcatgtcatctggtggcggaaataacatatctaataaacctacatatgacggcaactttgttcttgaagttctgtctttgcgtaaggtttctgaaactgactggacatgtaagcagacctttactacaaagaacggtgatgttgaaggcacatatgttcgatactgccaaaacggtacatggtctgcatggaaagaggttgttgctggtgttcaaccaattaatttaggtggtactggagcaacttctgtagctgctgctcgtaataacctcggtgttggtgaaggacagagcgttaagttcggcggattagttgttgatggaaacatcaacgttgcttctggtaattttgttattgcaggccaagctcctactgataactcgcatctgaccaacaaaaaatacgttgatgatcgggttgcttctgccattagtaatgcgggtgatacttatcttccattagcaggtggtactgtaactgggcggttaacaattacaggcgatcagttaaaaactacatcactttgggttacgggagacgctgctgttaatggtgttttaactgttgatggaagggctaggtttaatcaagagttcagtgtatcaacctcagttaacgttcagaacaatggcaacagtcatgtgttcttccgtaaagcggatggtacagaaaaaggacttctttgggttgatgaccctggtaacgttagtataagagcaggtggtggttctgggccagtatggaatttctggaacagtggttcttgccaattcccaggtgctattagtaactttaatggtgttaatagtactactaattaccctggcggcggtattggcgcatatttaaatacagcgggcctaacaagtagatttagtaatggtgcttatgtttccttatacttccaagaatatgtaggaaattatcaccaggctattcttaatgttaacggctatgggcaagataacagcttttatttccgggctggtggtgatttcatatgtacccgtaatggttcattcgataacgtcgagattcgttctgaccgtagagccaaatcggatatcaaagttattgaaaatgctttggaaaaagtagaaaaactaaccggtaatacttatgagcttcacaacacatccggtggtactactcgttctgctgggttgattgctcaggaagttcaagaaatcttaccggaagcagttactcaagataatgaagaagatggcggtatgcttcgtctgaattataactcagtaattgcacttctcgttgaatctgttaaagaactttctgccgaagttaaaaatcttaaagcagaaattgaagaacttaaatctaaataatgcatggggcttcggccccatcttttaggagaaataactatggcagtaacagggccgtgggtcggaagttcagcaaaggctgaaactggtgagtcgtggatggctcaagctggagcaaaattaagattaggaacacctttctggatgtctaatatgataggacgaagtgtttttaactttagtttaacagtgcaatatcgtaactggaacaatatttactatagaggttcatggcaagttggtggttggaactggagccctaaaccgacaacccaaaatacagtgcaaggtaacttcgaaggtaaagaggttactttatttgtgtctgtatccggacaaggtggggttaactattggaacggtgaccctcaaggtacaaccttgggaataagaaatggcgacgcaataaatcttcgggtaatgatgtcagatggcactacctttgattttactccaggtaaaatggatggagatgtaagaaactatcaaatagcttcaaatgacgaagctaataagcttaaaaactggtttagtgacagaactgaccaatactggcaaggtcttataactagaagatagcaataaatagctctgtaaggagagcaatatgatgtttatttcagtggaactactatgattgacggttggagaagatatggtgtgaaaatgctggaggtctcaatgggtattttgaggctagaatgaataatcagtttggtgctttattagaatacgtttgatagataaaccaacaaactcacactattaaatagattaaaaggctaccatataggtagcctttttgttgcatcctaaatatacctatagtaaactaagaagagtcttataaaatggctgagagaaatcccgtagataaactagccttatttgatcgggtaatatcgtttgtgatgggtgtgaaaacatggaaacaattgctgataaaaataattctaataatggttatgtttcttatggtagtaacttggtataaatggactgatatattcccgatgataaaaggtgcccttgtagtcgatacaagggctatcgaaattgaaagaacagaaaagtttaatcaatccgcgttggaacagttgagcatagttcatcttacttccaacgcggatttttcggcggtactggcattcagaccaaagaacataaactattttgttgacattgtagaatatcagggaaaattaccatcccagatcgatcctaaaaacctcggcggttatccgatcgataaaacatccgaagaatacacgaatcatataaatggcttgtattattcatccactaaagcaagttcctacctaccgacacgtgattttgtgccagtagcttatacttttagttgcccttatttcaatcttgataactactattctggatcggttttgatggaatggtatgcaaagcggcctgatataccagatatgaagataaacatcatatgtggacaggccgcgcgcattttaggtcgagcgaggtgattaacgtaatgctggtgttaaattgtgtgatcttccaatagcccgtttgattgctttaaagaagttcatcaccgggctatttttctcgtaaatatcccaaactttcaatttgtcccacggatccggaacataatcttcattccttgccgaaacccccaacgtaacccgcctgtatccagcgctgtcgtgataatacacgaagaatggcctacctattggcgcaaccttacaacctctcttagcggctctcatagcctcatcgaacgtcatggattcccccaaaaatttctatgcatgaatggtcgaattccgatagtttcactcaaaatgaatatcggatgatctagctcatcgtggttttcttcgtcaatgacgatatcccaatcagtagccttttgttcttctaccgtggcaatgaatacctggtttacttcacacttgcggtgtgtacgtctgatgattgtatccccttcacgaaacacaatcatatcaggattggtagtacggtacgcggttttacccgcgcacacttcattaagcatatcttcgtatgtcattataaaacctttacacgttgaacgatggtttgtttaacgtctttgtattctccgtgctctttaacggttgctttgaacgtgatttcatcaccttcgtttgcaatgttattaccgaagtaaacaacaacattaccatcaacattaattttggtcatgaatctttctacagaagtgtagtaagaaacttgagtatatcccagtgaaatcactttctcaacggttccggtcatttccagacgttgtttgatttcaccgatgtggttagctttagaaatgcgttcctggcgctcttgttcccactgttcgcggatttcttcgcgtttggcgatataatccttctccagtgcaacacccatgcagtaagcgcacacggcgtcaaatacagggctgtttttgttgtcttctttagactggtcagcccaccaaagaacagtaaacattggcatttctgcaattacttcgcctttacgcttgccaatcggcatgatccctttttccagcagttccagtttttcagtatcgaacactgacagtttaccgcgacgttcgaacagatcgaaatctgcaaagccctggaataccattttgaaagtatcagtttcagttaaacgggctgaaacacggtcgaaatactcacgcgctttcgcttccgctttctccggatcggtagataagttgcagatatagttatcagaagtataaccgccacctctacgctcaacacgcaaggtgtacattgcatttttacgaccagaagaaatgaagtaagtggtagtaactacggttgcgttagtcatggtatttctccttaaagggtatctcgtttcgatatggctaatatagcaaaagcccctgaccgaagtcaagggctttttcatcattcattcgaatctttcattgttttatgaagatgaatatcaaaaattttccagtacgcctttccgcgaggataaatttttgctttgtcaatatcgttgttgcttccccatgtgttgtttgggccacgacatcgattttttatataatctgtatgccagaataagcgctgaaccgatgattccgtacctaatggatcttctttactgaacagaatttgtatactcataagaagaacccagtgcgaacaatcagatcgattttattttctggttcaaacggtgatttgctatcgatgttacactgatagaacataccaacatacttttcaggaatgttggattcacgcgcccatttcaggttatcatcggtattcggccccagcatgaggttaacaacatcaacagcataatcctgttctttggtgttgccggaaccgtttacataatgcccgtgggcggttttgaggatctcaattacttcgctatcgtcagtttcgactttgtaaagcgttgtattttcaggaatttcttcaagaatgatcaaagcggttttcatcacacttacctttgtgtttctgtttacgttttgcttctttaaatgctcgcttgcgatcgcggtgagtagaagcgcggttgaaatcatgtttcgctaccaaattattcatataagccccttaaagaaaaatatttaggggctttcgcccctgtattaatccagcaatttgcggatcttgtctgcgatacgtccggcacgggttgcgctttcggtatgattgctttctttggtagccagttcagccagcttacgctgatgttcttcttctgctgcttggcgatctgctgcaacctgtgcaacctgctcattatcgtgagcaatacgcgcttccagttcagacagggttttgtcgaaagttgctacgatttcatctacagaacgaattttattaaacagtttcataatttatctcaattggttagttttaatcagtatacatcaatacggctggaattcaaaatcataaatgtcattcagtgcgcggttccactcggtgtagttttcaccagcaccataacgcatttgaatagcactttcgaacgttgatccgttgaggttcgggaaaccgaacaggtttttgattttgtcatgtgctacataatacagagaagcactttccagcatcgcaaccatcgcagacggttcgtgttcgcggcgcttgatacgtaacagagtacgactagcaccagttttacggcgttgatttggtgctacgtagaaacggaatactacgcgccctgttttatcatcaactaccaggtaaaacccgttttctttcagatccacgccttcgaatttcttgaaggttccgcgtttcatgtcaccaattttaattgcatatttgtgaatgtcaagtcttgtcagaattcttttcatatttttttagataccagtttgcctaattttgtaatttcgcctgtttttacgttaacaaacaaggcgatgctcagaaatgggatgctaatcactacgctgatcaatgtaaacagaaaacgtatcacaaaaagaacagcacgttcaagatatcgttgcatccacgcgattcctaaacaactataccctactataaaggtggttgcaacataaaatgcaccaaatcctttacgaaatacgtaacctttcccggattctatccggtcgtcggcccacatttcacgggcagttttcagaatagattcaccactagcgcgagtttcgttagccgaaggcatgtttttaaatttcatgatagtctcctatgcgcccagaactctccaggcgcggttgtttag

SEQ ID NO: 12 - DNA, 177152 bp, unidentified
  source 1..177152: mol_type = genomic DNA
ttagtaatggctaaaaccatatgtaacatcaatcatgactttataacggcatacacgcatttttgcgttattgtaatccactgggatcgctaccacgtcagcaggatccacctttacctgaatgactctaccaataccgcccccgtagtgtggaaggtatgatttagccgcaacgtgtaggccagtagaacaggtgcgcgttttatcttcgtctaccatgtttcgaggcatggagacagtcacaccaggactattatcaaatttgccagtagcgagatctttatagttatcgcgtacacgtttccaggcaagaaaacaaccatcatcggtcagttcaatgtcattatgtacaaggaacccgtaaagctggtatacagcatcgcgtgaagggtttcgcatcaaccgttcaaagaagttcaccagatgttcatacggacgatcgttatacatttcgcgaatgattcgttgagtgatatcagaatcaaacactacatctttatatagaagctgatgaccaatgattttaatgttgcctttgctataggttcggatcgcttcttgagtatccaaacaagttacagcacctttgacatcaccagctttcagcatttcatgcgctttcttaaagttcggatgtgtttcacccgccatgaaaacgcgcccttcgtatacaaccgtaatgaacgattcagatccgatcatacgcggtacagtgtctgatactttaggcttttgttttacatcccttttcttagggaattccgctaacttgcggttgataacgcgcccaatggttcgggcgcttacgttgaactgttgggccagtgctgttttacttgcccccgtcaaccatccattatagatagctttctgttgtacttcgtcaagaattttgaccattatttccaccgtattaatttcttaaactcactgagattcttttcgttgttgtaaatcggacgaattgaataagaatcgctatgttcaacaagtgaagccagtaacgggtttagtgatttaaagatttcccatgcctgatcaacacgttttttcatattgctgcgtttaacgcgcattgatgctacagattcacgcagaatcggacaacgcgccctggaaagatttttaccatctttctcatacccttccagacacactataagttcgagggtatcaacaatcttatacagtttttcattatatcggtttttcacaatccgatcaagcgatacaccaaaacggctatgcaatgcgtttgtttctgttgagtgttccttgccaatccatccaggcaagcaattgtctttcaatgccttttcggatttaacatactgcttgcacagcatatcatcaaagcataccagatttgaatctgggatccacttccagaggctgttacggatagcaaacacaacagggatcccagtatggcgcatgatacgcgataaagtagattctttcattgctgaatccatagacaacctggaattttcaccatctaagcggctatattcatcaataccatacaaccgaacacctggggctttatccagtgataaaaactctgattttgtcataaacagagaagtttttgccagattgccgttactatccaactcataacgatatacggtcggggtttttgggcgcggttctgaatttttcggtgcatatagcgcttttgatttttcgcgatctgcatcatagatctctttttcttttgtcatttcactggtacggagatacacaatttccgattcatcaaaatgacctttccgaacgatatcattaacaatctcacgctttgaatcactatcgtaatatgcaacaaagctaacacggcttaggttatgcattttagcatacccaacgatatacggtttaaccgtgttggtatccacttttaacagaatgagtttcttttgtttccacggataataaatgcgtgtgatgtcctggcgcttggttgtttctggcttatacttgctccagcggcctccgctacccgttacctgataccatgcatctttaccgtcgtattcgttcgcccaatacccagcaatataatcatcattatatttgttgggtttgactagttcgctatggatccagccaatagaatcaccgttggtgcgaaaattagcatctttaccaacaaagttttgtaccattgaaggcagagaatggaaccacgtcagtttatcacgaacggtttgtaacttatcgaattctgatttaactcgattgaaatacacccggctgatttgtttcagacgttctttaataatccctactgtcattttatccatactcaactcttcgcgagaaggcatgaaatcaagttcaccgatcgggaagtcaataatatacgtatactggctttctgtatagcaatagaacatcgaggtatcatacaaatctttatccagaggataaatgatgttacccatgcgagcatatacaccgctagtgtatgctgatttatgacggatcaccccgctatcgttggttgcttctttcggctgatagttgattttgagaatagaagcaccaacaaagttaggacgaatatcagtaaatgattcgtatacccttgctgcttcgttttcccattctttgatatcttcaaccttaaccggaacagtgatagtaaccccgttaggttcatcgctttcaatctcatacagaggatcgcagaacggttccccatcatccatatagattgtgtaaccgcatttgataccgtcttttacagattcaactgtgaacgcatcggcatagcaaagcggagatttgcaacccagacccatagaaccgatcaggtcgtttgaatcatttttggttgattcgaagtaaacggtaaacgcatcactaacgaaatcaggagacataccgatcccgtagtcacgaataacaaaacgaggatcaacagcagttggcaactggacatcaaacgggttctgatttcccgcttctttgtgtccatcgatcgcattacaagacagttcgcgaatgattgcgcggatcttgtatttgtatactgtcgaagaaaggatcttatacgctttcttgtttgcgcgtagagatagtttgtttcgtcccttgctggtatctgtaccaactcggtagattgtttgcggtgtatcttcgcgtaatttcattgtttatttctcacttaacattaaaaataacttggtcacaagagtacttcgttggctttttgttcaggccatattctactacttcgcaataagtgtcaaggaattttaccaatttttcttcctcgacctgctgtttcttcatatcaagtataccccacacgatagccccgataatgatagaaaagaacgcacaaaatccgaatatggtcagatattttcccaacttaggcgcattacaacgtgtcataccttacccctctttgcgaatatatgcaagttcttcatgggttactggacggatatacagacggccttttgtgtatgccttgcgcccactgatccaaatgtttttcatatccttaacaccgttcatcacatcgttgtaaaacttcttatcagctttagcctgatagacttcacggccttgataatctttcatgaacaaacagtaaaggatctcattcttatcaaccagattagcatcctttgtagttgttttactcggtgaaggtttagcacccaggcgcaaggccatagcttgccacactttaccatgttcataaccgcgcccgacaagagcatgagcgatttcgtgtaaaagagtgtctaaaatatcctcgtagatatcttccgcaacatgacgaccagatagttcgatcaattttttggtataactgcaacggcccagagtttttgtaatgcgtccattgatccggaatgtccaaccattactgatcaaaccgtgtttttccatcatggtacgcgcccagtgggttacttccattgcactacgagttttcaacattttagaatctcctttgcttggtacaaaaccaatatagcaaaaagccccctgcattgcaagaggctttgttattatttcaacttcttagaaagttcttttaaatcattgagatactcaattttaggggttgtttcttcccagtatttcaactgtttacgcaattcttcggcttcgtcttccagctttttgctttcgtccgtggttagatggtagatgttcatagccactaacatttcggcatgattctcgcaacctatccacgtagacacaaatttaaccgcttcgctgcgactaaggccacgcagagaatcaggagattctaccatttgagcaataaacgcaacctttgccagtgctttatctaacgcttccttagtttcctggatacgcttattgatacgctgttgatatacattcatacgaatatcaacgaaatcctttagaagcgtttcagggcgttcatatgagtataatttaccctcaaagataacgttaatgtttgggtttgagttttcaatcaacccgaaatctttcaggatcttttcgcgggttaacccgttggcatactctcgcttgagcgttacttcataacgaaaatcttctttcgatagatccttgtagctaacgataacgcctttttcttccagcttgtcaaggattgcaatgtatttcacacggtcatatttcactgggatctcggtgatcaccaatttggttttaccttgcaattcatacgtgccgtaaattgtaccgtctgtgatttcacctttaaagtaagggtatttcagatccagtgtgaaatctttatcattcagatatgcaatgcacccgttaacaaccgatttaggatcatgaggcggaatgtttgttgcatatgcttttgcaatcccgctaaacccgttaaccagtaccatcgggatgatcgggagatagtacgctggcggtacatgttccggatcttcatgaactggcgttaaatcaccatccatataaattgctttgaatattggcgatagtttgcacttgatgtaacgaggtgcgccaggtttcttaaccaaacgggaaccaaagaacccatcacggtcgaataacggaatgttattgcaccagtgcgccgccataagggataacgcttcttctacagaggtttccccgtggtgatacccatacatagcaacaccgccagcgatagaagctactttctgaaatcccgttccgccctgcatcgcagagtgaataaagaaacggtgaacgggtttaaacccgtctaccaggtgcgggatcgcacgtgaataaatcgtgtaaagggcaaacgttagcccttccacctgtacaacatctttaatacttctttccattagtcaaccttagaaaatttgtgttttccattaacccaatctttacgcggatcagattcgtcgccgaagcatagttctaacacttctttgtattcgtcgtcaagtacaatgacatcatacttcaactgatcacccagaacacggtcgtaatcttctttgcgtaaagaacccagccccttgatatatcgtacatcttttgctttatcgcggaacggcgcaaactcatcaagagaatagaaccatttttcctcgcgcccaactttagcgataacgatcggggttcgaatatatcggatccgtttctcagtgaacaaagaaggccaacggctaaagaatgcaagcaacagagttaaaatgtcgccgccgtcaacgtcagcatcgaccatgatgccgatattatcataagtcattccggaagtatcaccaggatgaatattgaggatagccattagctcaaacagttctttgtttttgataatgtctgtaaaactcataccccatgtattcagaggcttaccacgtagcgggaaagcgccttgtgtttcttcattacggcattcgatgaactgaccaacagcggaatcaccttctgtcagaaacaatgttgtttctaccccaggggtatcaataccggaagccggaacgtgtttagcaatttttgcctttttcgctttctttttcgctttggtgatcgcggcggcttctgctgcttgtttacgaatcaatgcggattcaatgatcggagtaatgatttctggggtatccataatcatttttgcgatctttttgtagttcaaattcgcatgattgttaaactcacctgctgtatttgctaatcgctcttttgtttggctatcgaatgcaggtgcattaaagttatgcaggaataccacaagagttaagcattcttttacacgtgctttcgggatctcgatactatgctttttcttgatcatcggttcaagttcagaatagataccatcaatcatacactcaacatgaacaccgccgtttttcgtatccagaccgttaacaaaggatttctgtttaaacccgtcctcagtgctcgccagaatgaagctgaggcgattatttgtctggacaatggttttatccccatacatggaagcgtacagcgggaagcgattagagagcgtttcgccgttatatgtgaatttcacagacgggaaagcaacggcaagggccattaagcgatccttaatcacttctttggtttcttcatcgataccagttacaccaaacatagagaagtctggagtaaacttaacagtagtaccctgttctttactggggctggttcggtaatcgatgttctgtgcgccgtccgtacagttaatggttactttgcgtttcccgtttgcagtctcgccaataaaaatcgagctataacagtttgtcaggaaagaaccaacaccattcatacccaacgttacgcggtttttatcatcgaagttagaacccgattttgccatagtccatgccgcaactggtttaggaactattttcccatctggggtttttacatcatcctggggaataccgcgcccgttatcagagattttaaccagattatgatcaatggttacatcaatcttattagcatgtttgaattcagttcggatcgcttcatcaatcgagttatcaaggatttcgttgatgattttaaccaacccttccacgtactcaaccttgcgatattggcccattatgaaacgttcatgcgcttctttgttaaccgatccgacgtacatatttggacgcaaccgaatatgatcgcgatcgctcatacaaaatgattcgtcaacctttgcgccttttttggctggttgtggtttctgttctggttcatcatctgccagaagaaaatctaaactcatattcacctctttgtttaatcactgacattatatagggttctatgaaaaagaaaacccctttcggggtttacttgttataagggaaaccatcacgaaccatttgaggtttatcaaccgttcgttttgcttcgcctccgcaatcacactctttcggttcgtcgcggcttgcgatgcttgccatttttggaaattctttattacacttggtgcatttataggtataggtaggcattaataaatctcttttaaacttaacatcttaactaaacgggctttgtctatgtcaaaaacacattgacgtgcgcccggatacaacttttcaacttcgtataccatgcagacgaaaccaacattgtgcatgtactcgcgttcatatgcattgaaccaacgagaaaggcgctgtattgactgaaaaccaaagtataacccagcctcttgaaagtctatgttatctttttcaaggttgcgcatcaatcgattatcgtcatccggtgctggatgtcggttatcatccatatcaatatagatatcaggattcatacagaattgatccagccattcagcggtatccattgacacataacgattgacatatgggccgctttttgtttgccatttttctgtacaatcattccagaaagaacaagaaaattccacacgatatacgaacatgatataatcctcacaagtaaactcaaggtttacaagtacgataccacttatctaatttttctgcaagcatttcgttgataatttttgcaatttcgtaccgtccgtgagtagtacccagttccaggtaaatcacatcaagtgcgcacacaatcgcatcaatactttcttcaacgatattaccgccgcgttgaggctgaatgagacattcgctgatctcgccaacttccgctgataggtgatgaaccacatcactcttcgtgcgtttcttcactttatgagcgatttcaaaaaacttatcaagtacgatcgccgtttcttctcgcgttgcagtattctcggatgtcgtctccgtttgttgaacaacgtattttgtaaaatagttttcaaacacgttgaaagggatcacatgaggaacaccattcaaaaacaccccttctttacaaacataatggatttggcgcggaatagacaacccgccgctgcgttccaaatgtcgtttaacgcttgctacaaaatcgaactctttcccgtatccagccgacatactgtgatacgtgagtaggccaaatgcagaaacatagagatcattttctttatacagattcatttacaatacctttatggtagccaaaaatataacaatcaattgaaggacgttcaccagggaagtgaatgcattgcatgatgcgttcagccattagatcttctcccatgtataccgaagtagtttcttcgttgtaatgggtatcatacgacgttttaagcgtcatgcccggaagccctgcaatgtgcatgaatttagaattggtgcaaggttttcctacttcaccgttaatcatcaacactgcattagttttacgtgcttttctcatttgaatttcaccccgatttgcgatacgttccattcttttacttcatcaacaatatcataatggttgatgtatggtaaagcaatttttaaattactcgcgtcttgaatgttgcgtaagaaacgagtaggagaaagaagacacaaccgctcggatccgttgtttcctttagcggcaaatgatagggtttctcccccgtcaatcttcatatcaacagaaatcgttttgaattctggtgcatatgacgtgattttgccgttgtctctcggtgtactatagaaacatacactttgtgggacattataacggtctgtttcaatgtacatgtaatcgccgtcagccattccccacgcggtataaagggatccggtatagtcaccaaaggaatttttaaaatcttccttcgtggtatatcccagcgagcgcaattgcataagctggttatgctgttcgattgcgtcggctttttgttgttcctgtacttgcgcatcaatcgtttcttgccaggaattatacgcatagtaacccacaacagcgattacagccataacccctacagctttccagattttagcgtcttcgtttttgttactcatgctatattccttttaagaaaaagggccgaagcccctttgttaacgaagataaaccacataaccgctttggtcaatcgcgcggtctgcgtcattgaagatattaccacgaatgccttttgctggtgctttccagcttgcaggtttcaggatattaccatcattatcgatgaaggcggcaacagaacgctgattgaacatttcaccagtttctttgttgcgagtatcctgaacaacacgatgatatttgcggcctttctccagaaagaaaacagtttcgaaaggagaatcttggaaacgagcgttacgcgctttgtgcattgcttccatgaaaggtgctgctttttctgcgaggatttcgaaagtgttcatggtatatctcctaaagtgtgtttcgtttcgatgtaagtactatatcaaagatggttattctatgcaaggcttttttcgttatccatcaaatattttaagtgttcttttaatgcagggagttcgttcaaatggcgttgcttaactttctcgtactctttgcgttcccagttttcaagattgcttgccaacgcttcatcacaataagcgatcccgcgttctgcatcctgaactttctgtttccattgtgcaactgcttgttgataaagagaaccgttaaccatcataataatttcctcccttgtttcgatggggtaactataccaaagctaccccagaatgttttaacaaaaagtgctattagtaggtatccagtttatacattttgcaccagttcatgaattcttcgaaagtctgagtattaacacgtttttccttcttcactttcttagtgattacaggacggttagtaaaacgtttttgcattttcacagtgattgctactttatcgcccaggtcttcaaccttttcaaccagcgcccactgagaaccaatttcagcgccgaaagtcaaaccaacaatctcacctgctttaacgtgtgctgcatattttactttaaccattttcgtattcctttctctgtttcgtttcgatgaatacaagataccaaaaagcctcccgcattgcaagaggcttctttaacaaaaagtgctattttatttctttgagcaatttacggatcccgccgccctgtgtcttatcaaagattttctttgcatcaataacagaagtgattatgtggtagttgttcccttttccgtcaaactcaaactcgaccttgtagtcactacgaaatttcacaaaaacaaattcacctgcaaagtgcttacgaaactgtttttcgttaatgtccaaccattcctgtgtatcatctaactgatacatgcgacaaaacaggatcgaacccattacagcaatcacgacaaggatagctaacgcgaattctgacatcatttacccctgtttactgattgacggtgcaatgatttaggcacaaccggatttcggtatggtttgactttatggatcgtgggttcttccccaaccaaattaggaaattggttgttccattccatcgaaaatggatagggtgatgactttaactcttcgatcatacagtttactaaacggtcgccgattacacccaaagccgccccaataatcgctatacgcataaatcaccccttaattgtgtcaagtacagtaaaccagtcatgaagccatatcgttgttcttacagcgatatacgttaacaaactaatcaatgataccgctccgcaaatagccaggcgtaatcaacagccggatttcaaatttagtaaaattcatatcaatctcctttctgagaacccaatataacaaaagccctcaaccgaagtcaagggctttgttttaaatttttaccagttttggcaatcgaagaactataccaggatggatcagacgtgcatccggaatagaatcacggttgattttagcgatatcaggccaaagttcaccaacaccatacagtttctttgctatagaatataggctatcacctggttgcacgacatagcgatcagattcaatcttaaccagatcctggttaatgatatcatcaaaggcttttgctttcgcttcgttaatcgtgttcccgtagtaatggcgatccataatagttaatgtgatcatcgtttctttcctatgctgttttcgtctgtctcttctaaggatggaggttcttccagccccagggcataacgtttagcatagattaacatcaatgcatctttagcgcaatcatgaatcgaatcatgctgaatgaatccatctaacatgcctttacgtagtggacacgtggtcactccgcgagtcagtaaacggttttcaatagctgtacgcacatcacggctattccagaacacggtcggcatatcttcaaacgtgtcaagtttccctgtcatagttcgtacaacatcggttagcatagaacggtcgaattcagggccgcgagtataatcgtatgactgccaacgactcacaccgtcagccgctaaatcagcaaagaattgtcgatgaccttcgtacaaatccatgtcaatatcggaagggaacaaaaccctttgtgcttctttagattgttgtttccaccattcgatcgttttttcatctttgattcgttctggttgtttccggatgtcaaatttgtactttcttcctttagcaatcagttcctggaaggtaggcggatcataaggatcatcaacaaacggaacatagctaagttcagctagttttccttttggaaacgggccaatactttcataatcaaatacaaaatctacgggtaaatgactcattcgcgaccccgcttatacgattccatgaaataggccaatgatagcgcgacttccggagtaacatcaacggatttgatcatgtctggagttactgccatcatcccgaactgacgaagcccacaacgagcaatcgatttttccagtcggatcatgttttctacagcctctgcaaaattgtccagatgttcccaatcgtggtaatcttccattgtagaacgatcacttttcaaaatcagatcggcaacggattcagcataaaggcgcggaaggtgaatattcatttaaaacccctcaagcatgtttttgttttcacgaatgttacgacccattttcaaagtatcaatgatcactgcatactcttcaaaagtgaattcgatatcttgtgaaatgtttccccacgtgtaggtcggcccgttaggacagtataacccaacttctttgtttgcgttgacaatgcagcgcaattttgcaaacaacaaattgatatcgatagaattgaacccttcgagataatcaagcccctctctaccaatacggtcaacttctcgcaaaatcttttctacatctttgactttaacaataattttcataataacctcaaagggccgaagcccttagacataatcaacagtgaatcgtgcgcgggtagttcctacataaagcaactgcttacacaattcataatcggcgtatgcgtatgcatcgcgcgtatacatgtatgaatgatcatacgtgcttccctgacctttgtgatacgtacaaaccggaagcgccttaaccgtctggaacttgtttttgatttgccagaacgaataccagggggctttgtatccggtttcctgtttcatctttttatactgaaacgcgacgtagttcaaataatcgcctaaacgttcctgcataaccggatccgcgataacctgaatatccgctttcgtatcctcgaacatcgattctgttttcatcaagaaataatcgatttgtaccggatcgcatcggtcagctttgatagtatcagaacgcgggatgatttcaaggattttaatttgctcgttgttgttatagataacttcaacaaacgaaaccccattcacacggccttctgtcactaacggttcttgcatcacaaccacttcaccaacaatgaacggctgatcagttttgtacaagtgtttgcggatcactgcatttaacttgtctacgtttgcgttagtgtaagcaaacatacggttattgttcaggtcatccggagtcttaacacggctaaaataacgtctcaggaagtcaccagcgttttcgtgcttcattacccctagttcaccattcatgaggggcattaacggcttaccgtcgcgtatagcgcgtgatacctggatgattgggtttccttctgcctgacgcataatcttatccatgcgaatgacatcaaaaatttcctcatcaaagaacggtgaaagctcggtgatcccttcggtattaaccggacggatctgatccttatcacccaatcccaggatcactgcacaactcggaatagtacgcttgattatccggaatagttctttgtcaaccatcgatacttcttcaaccacaaacacacgacattcagacagatcagcggcctttttgcctttttgctgttcaaatactcgtaactcttcgttggttacggggctgattttcagtgctgagtgaatggtcgttgcatccatacctaccgcctcagagagaacgtttttagcctggtgtgtcggcgctgtcaaccagatcccactaatacccagttttttcaatgtttcaaacacaaattttaccagagtagttttaccaacacccggcccacctgtgatagtagtatggattttgtttctgatatttttaatcactcgatcatgtgcgtttttctggtcttcgctcagatcgtcaaaagttaattcgctcatactttaatcaataccccttgaatacttgcgtgttcaataaaccaacgcatatctttctttttcttttcggttacggtttccacttcttcctttcgaaagaatcggctaagaccactttgtttaactggattcatcttatcattatattctttgataatcgaatttttatactcgttagcatcgtccggagatagaaacaacaaaggtgttaactctccttccttaatgaagggaattttaaacccgtctttatccttactaacgacgatataatattttgtaatcattctcgcccctcataacaaacgtagaatattccaacaaaccaaaacactgatagtataatcagtaaaagttttctttcaacgccatttacgtgaaacacacaccaaccgaaaagatatgtgatcatcgcgcaaacaccataagaaagaaccccaacagctactagcatcaaaaagtgccattgatcgatactataaatataataaaggagattatacatgatatcgaccgtaagcacaatagttgttcatgctcattatacaacaactcccgtatttgaaggagatatctacacgttcaaatacacttttcctatcgaacagatagttcaattaatgaaaaatagacatcctatcggatggattaccccagcaacaaaacatctactaaggaacaccatcgatggactaccgtaaaatttacaccaatcttatagaaaaagcaagagatagaacactaaattgttacacagaaaagcatcatatcatcccccgatgtatgggaggttgtgacgatcatgataatttagtagaacttaccgcagaagaacattatgtagcccatcaacttcttgtcaagatgtatccacacaataataagttgatatatgctgctaatatgatgtgcgtcaacgcaacacagagaaataataaagcatatggatggatccgcagaaagtggatatctcagatatcaaaagacagaacagggacaaaggcaacagaagaacaacgcaaaaagatgtcagaatcccataggggagacaaaaactctatgtatgggttacgcggtgataatcatcctgcttatggtcaaaaaccctggagaaatcaaataacaatgaaaggaaagcatgaatggaggtatgctgggattttctatgactggtatattaacgatattaaagctggaatctataaaagacaaggacacaagagaatgctacaagaattgcaaattgcaacaatctcccgtgttcctagaacatcaatcgagttattcaaaaaggggtggaacccttacgaagataccgattgggttgagtgggctaataatcaatagctgttggcccaacgacgaagattttcggcttgtttaagagcgtacatcttataaattgtttctgcatccatacccaatgcaataaacttacatagtacaaagtggaattggtcgatcatttcaaacagaacttctaaacgatcctcttcactcagatccgcaaatttagtattgcgcaattcctggtgatttgctttccacggtttccaaacaccggatgcaggtttaacaccgcgagacattccacccagagcggtatacaattcgcgggtttcgtcggcgatcgcgtcgtcttgcagtttcagccaatcaaggatttctccgcaagtttccagattatccggacgcggaacccaatgcagggtatcagacaggctttgctgtgcatggttttgtaaatccagcatggattgtaaaggatcgccattacgggccagaaccttttgatattcggaatctacaaattccagatcttccgggttaaccaggtgcgcacatgaattaaatacaggagttttatcagtagtcatatcaatctcattttttcggtgatttgtcccacgacttaaatcgaagttttgccgtgagtccagaaacagtattatctttcaaatactgcataatttcaagtttagttgcgccgtccgtttttatcatttcgttgatatctttggaaggccacgggcatttatcccacattacaaccttttctccagcctcaatcaatttaaagaggcggtgagtagtatccggatgacgtgcttcattgtcaagaacccagacacgcatatttttatacggaacctcagaaagtgcaagctgtccaccagtgatagcgccagcattatcaacaaacaggctatctaatggcccctcaagaagataaaccgtttttagcggatctatcgtatcctgtccgtaaatcttggttgattcttcacaggctttgattgtgatatatttcgactttgccccgtcgcgtaaagcacgaccctggaaagattcaattttccctttcttatcgaagatagggatcactaatctcggttctggttttgcgatcggataggtatccggattcaccgtattaaccagttgttgccattcgcgagtaaaccacaaccgatcccacttgtcacgggggatacaacgattctgcacatattttatgatcggatgttcatccggcaaggtatccaacctttcgcagaattgaagagtaggaataaatttcttctcttccttcggttgttctgtatgtgttggctttaacgaattgcgatccttaaacgattccatgagataatcacggtaatcatctggataatattctttcaggaatacgctaaacggtacaccataaccacagttaaaacaaccacaattcatgtgatcgccctttttggaagggtagatccaaaatcgttttttgtacttgtctttcattgagtcgccgcaaataggacaacgcgcattgatgcttaatgcccccgatttacgaacgatttcgctttgaggcagtgatcccatgattcgggttgcaaattctatatcaagatacatttcttacctcagttgactatctttagatcctcgtcgattataccccgcgctgatcatttcgtcatgttctttttggcattcaatacaataacggcaacccttcacgatagccctacgtttttcgggtatcggatccccacaatcaaaacaatgcgttaatgattctccgtttctgatttgagaacgtgcaaaatctatcgcattgtctattgttgcctgaatggtatcttgaacaccgtcagcagggccaaatccaaccgccattgtaaatcctcctaatcaaatgatttcaatatcatagactaagaggatttttctgtcaagaacttacttgcttttctgttccgtcaagcattaacttccaaccacgaaatgcctgtttaaacgaataatttattgcaatatcaattttatcagaaccttttcgacgattctgataaacggtcgcgttgtcactcatatacatgatacaaattggaaaccatgtataatcgttagcagtagcccagatagtgatattcagcggaggaattatcatttctttttccttttccctgcacgggtaacgcctaatactttcggcccgatgttggttactgctccagtagtcacaccagaagcaatcttttctgtatcgccgccagaatcacccgcgaccatatcctctaacatgcgccccttatcataatattctttgaggcgtggaacgttcaacatgatttcttcatgctcttgttccgtcagattgtagcgattgcgtagggtatcatatgaacttgttaagttcataaacccagtcatatacggaacagaattcattctacgcttgatatggcgtactgaacgatgaaaaggagaatacgcttctaactcttcttttgttttggggttacgaattacttcgccttgaccatcaaggatccccagtttgtaagcagtccattcagtccagggctttttgagtagccggatcatccggacgctatatgttaaatccatatttttaactaattgatcactcatgattattactctattgtgaaagtgaataaatcagatttggttttaggttcaaactccatacaaacaacctcgcatagtggtttaacccctttccaatcctccaggtaatacccagtatctataccgcatccaggattcataacaaggccagtttcatcaagaaactttttacatttacttgatgttgtgctgtcatcttgtcggaaacaatgggttttcgaataccggaaatttgcagacatttgagggattatgaaagttccctgacgcgcgatctgtgatgcacgttcgattactttatactcaaattctgcccctgtatacttacccttaaaatcagaggttttgattttaccaaaaggcgggttactgatcgccatatcaaacacctgattaaattcagttgttaaggcgtctccatgcacccaggaggcttctggtacgatacgcttacctaactcatagtatgtgtgatttaactcaacacagacgatttcacgcggtgtattgtacatcatgtaatgaaccatagcgaaagataacccaccgataccagcacacaggtcaataacacttccacctgtgcaagcatcgattgtgaaatcgcgagcaagtccaataggggtaaagaacgcccctaattcagaattgtttgtaaacgcgccttcatgaaagttttcaataatgaacaacttctcttcgtaagttagcgctttgtcagagtgaaccagatccattatctgattgtgtttcttggtttccgctttcgttaactttgccattttcccagctatacaataatgttgattcgttagggtagaattcccatccgtccacatatccggtttcccagtcagtagtttgttcaaaaccacagatccattcatatacaccaggaggcatttcgacagaatcaggaagcccgatatcttccgcgctgcgtccacattcaaagaatgcatcatgaatgaatggtcgagataataccgtaacataaccttcatcgtcaacagctacgatccagcgcgaactgtgaggactatcgaacttcggttcttcttcgtctgcgtcagcttgcatttcggccttacaaaaatctaaatttatcatttcaaaccctctttaacaccctctttcatggctttccaggtagaacctgcttcaccattcagggcggcgaatacaaatagtaagatagcaaggacaagattcacaccagcaatcaccatgattttgctatacacgaaaatgtaaggcattgccaccacccaccaactaaaagaattaccagttacgatgttgagtgctgcaagtaagaaagtgataacgaatgcgattttcataatgtcctcctttgttatgattaaggtatcatcttttttgaaagaatgcaatacctatagatacaaaaaagccccgaaaggggcttaatttttttatgcgttattgatgagataccgaagaacgtttttcgcttgttcctcattacaaccaactttgaaaccaggttcgatagggaggaagttccagaggaaatcaacacttccttcaacgtcatctttgcctttttccagcatcgctaacagcaaacctttgtttttgatgctgtttacgattgcgtcaaaataaccatcgctgaaatcaacattcgggttcagcatttcgttgtaagggttgttgaatacgttcattttgaatctcctttgtttaactcagtatcttgtctacgtgagttatattaccacaatggagattcaggtcaatacctttttacgattttttgaaaagtttttcgtatttggcttttacccagcgatacatatcttcggccttgtcactggcaagcagtgagaacagcagatagatcgcagcacccaccaacacaacgcctactacaatgtagacgggtaagagaactgggaagagaacccagaaccatgacatttgcgagaagccaaacactttagcggctgcaaaaatcagagttagtccagtcagcagtttgatagccggaataggaatcgttatagtcttagtcatttcattaccttacattctttatggggctattcgcccctgtcaattaaaattgaatgtcagattttgcaatctgtgccattttttcacgtcgggtagattcagcctgtttaatcatcgggccttgtgtctgttctactgttttaggcatagtgttgccgtggtagtcagatttaaacccgtattcgctgttgtcggtatccatccagcgctgattaccttttcgaacttccaacttgaacttgttgaaagtgttcttatcgccataacgggatttgatttgcttgaacagttgcataccctgatcagctaactcttccgtctcgattacagctaacataaaatcagccgtagcaggtaaaccagcggattccgcaacatcacccatactcacatccgaactatcccatgcagaacgcccaacctgtgcgcctgtccacattacggtattagtttcaacagcaagaccgcgtagttcttcggcaattgctttaaccagaatataggtattttcagcacctttaacgcgggttgaagtacagatccccaggtaatcgacaatgatcacatccggcacaaactgtttcttcaatttaagctctttcacaagcgctctaaagtggtttgcacccgcacccgatgtagggtactgcttgaccaccaaacgcccaaccttacccgctttaaggcgctccattttgttcttatagtctgcgtatgtaatgttcccttcgtcgatgtcatccatagtcacatcaagaaggttagcatcgatacgcttagagcaaacatgctctgccatttccatagaaatgtaaagaacgtttttaccctgttgcagataatcagccgcaagagaacataagcccagtgatttaccaacgttaacaccagccatgatgatattcagtgtaccacgttccgcgccgcctttggtgattgcgttcaggatcgggataccaaacggaattttcatcgccttcgattggtaaagcatccaccgtttttcataatcttcgaaatagtcatgacctactgaactatcgaatgaaattgctaatgcttcctccatgatttcagggatagccccaacaccaggaagtttcttgttctgttctgccagtggtttttctgcgttagcctggatctcgattgcgcgagaaagagcacgatacattgctttgtctttgcaatatgtttccgtttccttcattagccaatctaaatcttctggcgcatttttcagcgactgaatcgcctttttcgtgtcttcgtagactacatcacttagatttcgtttgtcaagcgcaacctctaaagcagtttttgacggaataccgttgaattcctgtacatgtttatcaatgaggtcaaacaaaacttgtgcattgccttcaaaatattcctttttcagatgaggccatgcttggacaaaatacgtcccgttataaatcaggttagaaaatattgtatcaacgatcattgtattgccttataccaggttgctgaacatcatgaaaaagttgtaaaccttttgtttgaatacatcccataatgtcagcttaggctttgggacaactgaacccttttcaagctctttaatctgtgcataaattgcatcatgcaccagcgggatcaacgcttctttgtcttcgtctggggtactgaattctactttcagaccatgatcccaaaacaccttatgaatataaaccagatgcgcaacacctttttcatcgttaatcagaagttcctgaataacatctttcatcgcttcatcaatataattctttgctttgctctcgatatccatacattgcctcggttatggggccgaagccccatagtttttataaaatttcgttgtcttcttcgatatcatcaaatgattctgggatatcgtcatcatccagatcaggatctgggatgctatcagtgctgtataaatcttccagcgcggaaccatcactgatttcacgatcagggatcttatacttttcttcgatagctttcaagaatggttgatgagtaaacagaggacgccagaattcaacgctatttgtttctgactcacgccatttcttttcttcaacttcgagttcgccagtctcggtattcaggaaagcacggttgcgccagcctttggttacggtctgtacaaagttcatttccattgccagatccagaaggccagaatacatactaataccgccttcataggtaacatgcagcgggaattttgatttctctttcacgaatcgagatttttcgatgttcatgatgaaatcataacccactacctcagtaccttctttcacctgttgtttacccaggatgatcgcagtatcagcggaatacattaaaccagtaccaccggaaataactttcttgctgtacatttcttgtgtgtcataggtatgacagatacaaaccatcgggatatccaggtcagccagataaggcgtaaccatacggaacataccttttaatgcttttgctcgcgtcatatcctgtttatcgttatcagacagcgcgtcagcaagttcttttttacttgccgtgttgcctactgagtcaacgaatacaatcaccttatcaccgcgttcaagcgcgttaagctggcttacaacgtcattacgcaactgctcgaccgtcgtgatacgagtatacacaacacgatccggatcaacacccattgatttcagataggatttagtaacacctttttctgaatcgtagaacaggcacacagcatcttcatacgttttgagataagccgctacagtcagcaaacctaagttggatttgaagtgtttggacgggccagcgaaaagggtaagaccagaagttaggccaccgttaaacgcaccggacaacgccagattcagaatcggcacacgggttcgcgtgatggtaatattgttgaatacgtcgctttcagaaagtacagatgcagtttggctattcgagtttttgatcagtttttttagtagtgctttgtttgacatttaatttttccgatttattcattctcattctatatatctcactagttaatgaaaggggccgaagcccctagagtttaccagtcaccgaacagatcgtttaaactggcacgtttttcataatcaattttacatacttccgtgatattagtcaatggactaataacatgtttttcaaacatacccggataatctacccatgccagaatatcactttcgatctctgacggtagtttatttccggattgccacgcgatgcaatcggcttgccacgggtttttatcccttagtggtagaaccattaccttttcaccttccatgattggcgtaacaccatcaataccagcagtgaaacggttaaagaaaagcacccctttaatatggtttggtgttcccttgattggatagccagccccatcacgatatttcgaaatgttgttggcagatgatacaccagcaatttccctgtagtcaagttccttatattcttcttcgaactttttataatgttcgtgtaaagataattcaccttcttgcaggatacggcggatcgcttctttcaggaatactttcacagaggtcggagtactcgatcgctgtgtttccatacccatgattttcagtttcggtttttcatagcgggttccttcggagtcccacacgttagccgcatatcgttttttagcagtccagaaacttcccaacccttcggaacccaacggaggcccagaaatgatttcacgatccataaacatcaggtgttccacgttgttcatgtattcgcaaagttcacgataccctttatcgatcatcggttccattctttctttagcaaagcgatccaggaagtcaacccaatggttattatccttaaatttagcctcaccaccaacttttgcaatcacgttatccatgcaaacataaatggagtcagtgtcacagtaccgaacatatgcatgatccgtagtaccgcacaggtcgttaaggtattcgtttaccttacgttcaatccactggatagccaactgcccgaacatggtgatcgcgctggcgtttcgcagatcgaagtatcggaaatgttcattacccaacgcaccataaagggagttgatagaaatcttacggttaagctgtgctgtgttcgcttgtgcgatcttcttctcacacacgcgcttaactgctttaagcatttgttttgtaagagttttcagaactgctttcgattcatcactgaaatctgtatagaaatcaaagtcaggatcgatcatttggttatgtgcgtctgttaagtgttcgagttcgtgcttgatgagttcaagatttcgctcacccgccatcattcgttttttccacatcttacgctgatcaaatactttcttgatctctactgggatcacgcctttgatatcacggcggaacatccacccgttaggagaacagctaaattcatcgctagggcgcggcgcggtcttattaatatactcttcaagagcacgtaccgcaaaacttcccataatcgtttcagggcttatattcacctgtcggatgatggaagggtacaggcttgttaagtcaaacgataccatgtatttgtaaggcccaggaactggatccttcacaaatgccccagggtaaggggttttagtatggcgtctgttttccggaataacaaccttatcttcacgcagagagttataaatgatcgcgtcccacgttttcagcggagacataacccctgggaagttaatttttgcatagtacgctacagacagaaccagttcaataaagtttcgtttaccgtcgatatcaagtacgcggataacgtcaacaatgttgtacgtgatgtacagttggtgatcgcgctggcgtagttcagacagggaaccttcatactcaactttatttttaccagtttcgtattccgcgatcgcgtccagacggtaagacggttgcggggtaaagctgaatttcttatacagcgccataccatccatttgagcaacgccgaaaatatcatatcctaattgttcgttgccgtaagcgtcagtagtggttctggcggttactttaccaaatgggctaaaatgccttaccacgttttgaccgaaaatgttcaggtatcgcgtgatgatatatgcaatatcgaatttgtcagagttccatcctgttacaataacaggggttcgctctttccaatctttgatatacgcagacaataacgacttctcggtctggaaagaccgataaacaattttgtttaaatcttcttcgctaatgtctttgcgatcaacgttttccgcgcaccattccgcaaggccaccctcaaccagatcgtatacatagaatttatcttcaatgctatcgtaatgggtaatcgcatcgattggatattttgcttcacgcggatccggaaattctggggcggtcacctcgatatcgatagaagcaatgcgaatgtgttcgcggttgtattcgatttcattccggtacatgtcagaaatgtaagccagtcgataatcgtccatacctagcgcttccatcccaacatcgcgcatacgctgcatccagtttttagcttctttgatgctgtcaaactgttttttgaggcaaggcttgccgtaaatgtctttgtatggggtttctacgccattcatagcgtgttgatacattacgggcgcatatttcgtcttacgtacctgttcggtgccgttagagtcaacgaagcgctcgtaaatggtatctcccatttgttcaactgataggtaaaattcattcattggatcttgtcttctccattaatataatgttccattgtaacaccacctacagcaaattcaagtttactcgatgttctaaaaccaacaacccttctgctaacaagtcacggatctttctcagttgaacaagctggcgttcaagtttaaacccgtcgaataacatgctaaaaatactggaattgatactatgatattttgcttctgcaatgccctgattaaccatcatgatagctttgttaaccagtagtttcctttccgttactgtatgttcatccagttgacaggttgcaagggaaaccagatcatcataagcacgttgatcaataacgttatccatacgggccgcgaaaattttattcatgtaagtgcggatcattgcgcgacctccattcttttcataaagacttcttttgcttgttggatcaagtccagagattttttaatacgctcatagaaatgagtggtttcaacttgattgcataacaatgtgtactctgaaatgttacgatcgtaaaatccaggaaagtagtgttgtgcatagctgtaagtgcgggtatctgacagattgcaagttaacgataacaagatgtcatcttttacaatcgggatgatcaaagtttcgttggatttgattgaatccatgatttcgttaatagtcataatatatccctctcaatggtgtacacccaatataacaaagcccctgcacgaatgcaagggctttttgattagtgaccgatccggtacttgtacttgaggatccaatctgctttttgcgagtgagtcagtacgcggaagttgttttcttctgcaaacttcaacccaggggttacgatcttaaccatgccccactcttcgagaagtcgcgcaatgttgttccggcgtagttcgtcttcttccgtcatatcgacttgacgaccatcgagtttcaacagttctttaaaatgcacgataaaatacttaccttgctttttcagaatgtggcacgattgccagagcattttctttttgttgtttgcaataccaatacgggttagcgtttcacggatctttaaaaaagaatcgtcgctgattagttgaatttctaacatacatcaccattgtttaatcaatttttccaatttcttttgttcagctttgtttttcacaatacccaacaaagacagagcgacctttgcgtgttttcttttccaatcctcgaacattccgaggtctttaagttcctgcaaatattccatcgctgtacgtgtatttacactgtatttttcgcgaaggatttcgataataattttctcttcaaaatcttccgatagtttagcccatgcaccgaagcgtttagccttcctaacagagttgagataatagttatagtgcatttggtcagagatactaccgcctaccagattcatcacatacgcgttgtatatcgtgtctatgtgctggctcattgcgttgtctacaaagtacttatcatacacttcatcgataaccaacggcgttttgccgttgttgatttcgtctatgatgttaaacaaggtgttttctttatccttgccgtactctttgaccagttcttcaaccttatcccaatctttagaaagccaagcggattcatgcggggataactcttcttcatccagaaattccgccaggctcatgattacgcctcccagaccatagaaagcatcaggttcatcaacagatattgcagatgaatttctttattcatcgccagcccgtattgcgcgttgttttcgcctacaatctggatcagtgcgattttcgaatcctgattcacgatagggtaaatcgtatcagtcaattttccgataaaggtatcgtattctgacgcatatttaataacctcagagcgcaaccctttatagttcttttctttcaacagggtaatgatatgagacacatcagaaccaacgatctcatttaggatccccgcatcaatttcaccacgtttcgagtagaacccgatcgctttgataatagaacgcgcatccggataatgctctttaacaaacgctgcaatgactttaggatcatacttgatattctcgatttcaaggataccgaaacaacgcttgattaactgtttcatcagttcgatacgttcagcatcagacggaacaccgaatttaacaggaggacaacgagaaagcagagcactatgcacaccgttaatgttgttcgctgttacaataacagaaacgtttttactgtatgcttcgataaagctacgcaagtgtttctgtgcttccgccataccagaacgatcgaattcatcaatgatgataatctttccgcctggtttctgcgtcattgatgaagcaaaacgatccagttcattacgaatgaagtttacaccacagttcgaaccgttgacaaagaacacctcagcatcaacctcacgggccaacacaagcgcgagggtcgttttaccagtgccaggggaatcagatacaagggtcatgttctcaacacgcccagatttgattatgccccgcatagcggctttgtcaccagaaggtaaaatacactcttcaatcgttgttgggcgatagcgctgatcccatgcaaattcatcaggagatcgggagattttaccgtatttggtttcgatgatttcaatattttcactaagttccataatataccttcaaaataaatggtgtaaaagaaaggggccgtagccccttaaaactatcttacttgaatgtgctacttgcttcaagtacaacgacgtaagcaacgccgttatcagaagagaattttgcagcccctttggaggaaatctctactttgtaatcgctgttgatgaactgcatgttatcaatcttcatatcgaaattgaaaacattgtcgccttcatactcaccgacttcaacggagaaagttgattgactttctttgcttttcgcggtgatgaccagtttaccatcaatcggttcaacggacaggtcggtcagtttcatcatgcgagacgctttgatcagtttttcgaaatcgttagcggtaatctggaaaatcagatctgctactggcatcaccaaacgttttttcggtttcgggattgttgttgcgtctgctgaacgttcgatgatcttcatcttgtcgccgcgaatcacgatttcaccagtggaaatatcatgagtgatttcagcgtcagtgccgacgatgttcagcatgttcaggaatgagttgagatcgtagataccaacatcttcatcaatcacatcagcaatttcagcttctgcgtatacaacgctgttgattgatttcgtcatgatgaatgaacctttggtcagcatgatcgaagagttgatttgagaaaagtttttcaggatatcaatagtttgtttagagaatttcatattcagcctttagttttcaataagtgttacttaataagtgattttacaacggtttccgctgctgtgtcaagcatatcagccatttctttaacggttgtacgcttaggatcttcgcggcgttcgctggtaagtttacgatgttccgcaaccaccttttcatcaatgtcacgatagtgtttaaaacgttcctcttgaggcatagctttaaacagttcttttgtttcgtccgagagtttagcaacccaggatttacggacgcggttcatgtagtcaacaaaaacattactttcattcatatatttcttctctaacttagaattctttgagtgggggccgaagcccccgcttgtattacatgtctaacagtttatccaggtcgtcatcaccggagctatcagaatcatccaggtcgaacggtacgccgtcatcttcgcctaccggaaccgatgcaacaccaccagatgatttcacatcagatgtctgattgtcaaacttagccatttcgctatcgaagttgctcagttcgctatcaaggtcagcggaagcgctggaaccagcagaaccaatcgaactacccataactttattgaagcgagtagtcaggtcagccagcggtttgaattcgctttcggcagtgatcgggcggagatcgctcataccttcgaaaattgctttctgaacttcttcatcgtcgatgtttttgatcttagccggaacaccaaacgagctatcgtcatagttaggccaatcaccaacttttttcgctttcagggtgaagttagcaccatcaaacggacaggttacagcaatacccggttcatcaagttctggattaccgttaattgcggcggtgatcttgtccatgattttcttaccgaagcggtatttgaacaccttaccttcgttttctggagcgcctgggtctttaacgatcaggacgttagcccagaaactttgtttacgaccgatctggctcagtagcttatcttctggcccgtttttgttggctttagccttctcatacagatcgttttcggaaatgtacttacatgcaggacagccgtcataatcgccgtgggtagaggaacagttctcaatgtaccactggttgtttttcttgaaagagtggctcacgatacggacgaacgccagttcatcatcggaacgtgctgggaggaatcgaataacggcggaaccgtttttctgtgcgtccagggtcagtttccattctttctcatctttctggaagccggaaccacctttcagatttgctacctgtgcctggagtttagcgggatcttgacgtttaaaaatgctgctcatattctgttttctcgtttagtttagtttgattaacgtttgtttcattaagtttcgatattttatgatatctttttcagtaaggtcaaatatttttctgtatgcctttaacttaatgctaaagtcagaccaaataatatcatcagctacttgatcgtgtttatttatgatacctaaaaatgagtcaaaaatcaaaaacgattcgtaagatatcacatttgacaggacaagtttgcttatgtaggacgttgatgatttttcgctgtacttgaacaccagagacacggggatctctttcattttggcgaattcgtacacgtttttaacgtcatccacaaacacgttatctagtctttgtaactttcctatgtactgcctgtaaaagacaatactatcttcatcaacatcgcctacccagaaatccggattggctacgaagttggagaggaatataaaatagatttctttgaatgtaaagcgttgagctaattttacaaagaaatatctatcctttcgcttgttaaaggcgttttcactaactttgatctgccagttgtattgaaggacatcaaaacgcccctggaaatgagttttcatcgccagatataacttgtatacagacaaaggcacaagccgtgaattcgcctcgctatcagcaaacggagctttgaatctcacatgaagccgtccagagtggttgatgaactatgttcaagcgcaaccgatgggcgaagcatgtttcctttgatcgcttcgtcgctaatcttatcaaggatcgcgcgaggaaccgttttattcagcatcgcataatcaatagaattttcatccatccattgtagcgttgcttccatgtaggttgccccctcagaggcaaccagattttcgatatacaaaccgacttcggtcttatttccgatcatgctttacgccttatcgatcatatcatacagttcgatcagttcgttgttttcttcttcgaaagcggtacgggcctgttcgtgatacagtttgaacagtttcccgaaggtttttccatcgataccgaaatcagtttttgctttggatttgatatccttgaacgtgccgttgaagatctcaacttgagttttcacgttggatgcttctttgatcagttcttttacctgttttgctacatcagggtttgtttgtaaaaattctacactcattttgttacctcaaaaatcactcagtttttcgaacatacgggaaagtttgttatccatgaagtaacgttccattttggctttacttccggattttggagtattatacgcttcaataatcgaattttcaatatcttttggtataaattcgaaatcgcgtagttcctcattttctttgtaacgtgcggcccattcaggggtcatcaatgttgtcggatcgtctgcctccagccatgcctctaactcagaggattttaccgctggggcgcgttcaccttcaaccttcgtcacaatataatcatttctaattttaatgcaagcgatactatcttttttatcgcctttgatatttttgtatcgcagatcgttacgtggcgaaccgtacttaggcgttacccattttttctggggaggcgaccattgacgaacaccgttatatttctgtagttgtgtaaagtcgctatcagcagaaaccactaatactcgtctaccttcaccaacagcttttttcgtaacaacagcaattatatcatcagcttccgcgaattcaacctttaatccgagataaggcatattctgacggatttcttcgaacacaggattcaggaagttgttcagacgatcccaatcccattctgattcttcgtgttcgatctgacgacgttttttgtagtaccaggctttttgcctacgccagtaatttctgtcatcgaaggcaatcacgatttctggatactcacctttaaattttacaacgttaaaccgtaaagtgtcaagcaccagatgacgaatcatttcgatcgtgatggatgcttgttcctttggtttgaagttgttcatcagtgtagcgatggaaatgttagagatatcgatgatcatagtatcatcgggttccccttcatcttgcatcagcttgttcaagttaaacatgcttgcaaaactgctcatacatacctcaatttttcaaagaacggggttattgtagtaacttacgaaatgaagtcaatacaaaagaccataaaaattttgatcaataatacttgatctgatcaaatttatgatctataatttattaattaataattattttactacaatgatcattgtaggtcaagtactaaaatcaataaattttatataatttagatctgatctatagatcattagatctactttaaccttaaataatatagaatgaaatttgattttgtctacagttattatataatattcttaacttcaaagaggaaatatgaatactatgactaaagaaacaaccaatatctacgcagacaatgaaaaattataccctatcctctgtgcatggaaaaagcaaatcgccgaaacaggtgatcgcaaaatgcctaatgagttaggtgctgctattatggatattgcaaacgggctatcacgtcgttacaacttcaaccgttattccgaagattggaaaatggatatgattgatgacggaatttccgctgcaatctcaggactgcataacttcgatgaaactcgttataccaacgtttacggttacattaacaaagcatgttggcaagcattcgtaacacgtattctgtacgagaaaaaagagaacgcgaagaaatataaattcttccttgagcacgtttacgactgtgaagattcagatatggttagtattgcagacgaaggtttcattcaagatctacatgacaaactatctcagtacgaggcttccgccaccaaaaccaaagacaaggaagcggaagtattcccaacattggaagattttctatgaaagcaataattgacttaaacaaaatattaactgatatcgattacgaaattgacttgctaccctacttcgtaaaattagagttgcaaaacgtgggaatcccggttatcatcgatccaactgacgtaagaaaccccgatttcgaagtagaagaaggggttttgtcttatatgataaacgccgaaactatgatcatggagatcacttatgattgatgaagagaaagaagtactaaccagtgtggaagaagtggatccagaagaggaaattcaacaaaagatccaggaacgtgtagaagccgacgcattgaagcgagcacaaaaattcattaagaagaaccggactgagatcaaacgcctccgtagacacgcagaggaagccctattcaggggtaataaagttcagtatgtgtatgcggttaagaaacttcgtgatatgctcaaacagccgtatacagaggatttcattgatacgatgtggaacacttcactagcatcaattcgaaatatcgtagcttcacaacagaagcaataacaaacaagtagccccgaaaggggctatgagggtcttatgagaaagtacttaatgatcggggatactcacgctggcttgcgtcaggacaacccctggaatgaagaaaacctatacaatgtattcgtacaaatcgtagaacactgcaaagcaaacggcattaccgaggctttccatgctggtgatttctttgatgtgcgcaaggccaccacacaaaccacgatgaaattcattcgtgaacgtattgtgccactactggaagaagccggattacatatctatgttctggttgggaaccacgattgccagtttaaagacaagatccgccctaactcaccgcgagagattcttgatcagtatgattgcttcacggttgttgatgaaccgatgacagtaaatcttgatacttctccgctgcaatcaatcgatttgatcccgtggatttgtcaagaaaacacacaacagatttttgatttcatcaaaaagtcaaaatctcaatactgcttaggacactttgaactgtccggatactatttctataagaacagtaaagcggatcatgggcttgaacctgatttcttaaagaaatatgatatcgtgtattcaggccactatcatcacgctaacgaaggcgctaacgttttctatatcggtacacctcttaccatgagtgcgaacgatgaggacgaaaccaggggcttctatgagctatcttatggcgacggtaaacgtgaattaactttcattgctaacccagtatgccaccatcgccggatcacctatccggatcaaaaagatgttgatgttgcagattacaaaaattgctctgttcgcttgattgtgcgcgaagttgataacgatttgcctaagtttcaaacaaaactggaagaaacagtttatgagttgaacattgtcgatcgcgtgatcactgattcagaagtcgatactgattttgaaatcaaaagtgtatctggattgattagtgagtacatcaacaacatgcagatcactccagaagaaaagaccgaagtatctgcaataatgagtgcattgtatgcagaggttacgagcaatggaaatagttgattacgttaatattttaaacgaagaagggcgatataaagccctttataaaatgtttggatttgatgtgattgttgcagtacagcaggattcctataatgagtatgtgtcattggggttcactctgattaaagacaactatcacgaaacaaaggtttggacatttactgtcctgaatagcatggatgaagattccgtgatatactgctttgatagcacgattacaaacatgattagtgatatatcccaaaggataattgatgaaactcaaatttaaaacattgacttatcaaaatatcttgtcggttggtaacgtaccgatcgtcattgattttgattcagcaaagaaaaccctcattacgggtaaaaacggcggtggtaaatccaccatgatcgaagcgcttacatatgctctctttggtaagtcatttcgcgatctgaaagtcggacaactggtgaacagtatcaacaagaaaaaatgtctggttgaactgttgatcgaatacggtaatgatgaatataaaatcatccgtggacaaaagccgaaagtatttgagatctggaagaatggcgaaaaactgccggaagattcagccgctggtgattatcagtcacagcttgaatcaatgttgaatattaacctggtgggctttaaacaggttatcgttctgggtactgctggttatgtacctttcatggaactgaaaacaccagatcgccgtaaactggttgaagatttgttgtctttgtctatcatcagtgaaatggacaaactgaacaaatcatacatccgtggtgttaaccgtgaactggatacgctttcaatgcagattggacacgtacaacagcagatcgcaacacatcaaaagttcattgacgaacaacgggcaaaagcaaatcagaatacggcgcgttaccaggatatctacgattcccacgtagaaacagcaaaacaaatcaaagcacaattggtcgaactacaaagccagatcgcagaatgtgtgatcaatggcgaagaccaaacagcaaatattcaaaaattgcgtgatggttatacgcggctctcaatgaacgtagaacagttgcaacgtcttgaggtgatgtatcgcaagggtggcgaatgtccggcctgtaaacagccaattagccccactcctgaacgcatggaagaaattgccgagaacattaaaaatggtactcagaaacttacgctgattaagaacaagcaagatcagctacagaaaatcatggatgatttactaacacaacaacgtacactaaatgggctgaaatccaaatacgaatcactacgcggtacacttcaaaatgaagttgcagcggctaaacgtgttcgggctatcatggataaagcacaggaagacgtggtgatcgacgaatccccagttgaaaaactccgtgaagatgaaaaggaacttgattctaaacgttctggatttgtcaaggaaaaatattttagaggtattgttacggatctgctgaaagattccggcgttaaagcgagcatcgttaaacgttatattccttacttcaataaacagattgcgtactatctggatctgttgggtgctgattatcagttcactctggatgacgaatttaacgaatcgattaaatcgctgggtcgtaatgattttagttacgcatcgttcagtcaaggcgaaagagcacgtattaaccttgctttattgttcacctggcgcgatgtaaccagtaaaatttctggtgttgatttatcccttctgatcctggatgaagtgtacgatggtgcaattgatcgtgatggtagttttgctgtaaaagcactattggatgggataaatggtaacgtaattgttatcagtcatcaggatttggatccggaagatttcgaccgacatattgttatgtcaaaagtcggtcgattctctaaaatggaagttaagaagtcttaaacttgcagttatcaaaatgccagcgattcatattgctggcatcaccagatttattgcaatatggacaaatcaactgcttcctttttgctggcgtctttctatttgggttatttctgcaatacggtatatgtgaacgcagataatgtaatgacgattctgttccgcaatatggacaattgccccgttctttaggtacgtttccgttcttatgggaacacgggataccctcgaacttatgtttcaacccttcattacctggtttcagtttgcagttgtcgaagtgccaacgagtcatatttccaattatacctgattttccgcaatgaggacacacaaccctttcttgttgctttttggctttactcattcgctgtctggtttcttcggtgaactctctattcctatgtgcttctgacgcctttttctttaaccattcatagcggcggttagctgttctttcctttgatctattggaaccaactgttaacatatgtgctgcaaaaacaagtttgttgtttcctgggtacatcttgactaataacagatgcgcaatataatgttgacgcgctgtaagattaaccaaattatcatcagaatctgttccacctatgcacttaggtatgatatggtgtgattctgtatatccatcatactgcgtttgtttagcatgttctatgatagagttataaattttgttatagttcataaacatatctcttgtttgatgggccgttagatacccctatttaagaggatgaaattatgttattagaaaaatcttttgaattagaaaccgctctggaaatagagcggttttatctccacaacaattttcttgaagaaaaacatatagttactatgaaagatgttgaggaagcattcaaagataaccctatagagttgacgcgaatcaagaacaacaaaagttctgtttggttcctcgaaaaaatctattgaccgaaatccataaatacagtaaagtagcccatgtaacgaaacgtgggctttgtttttatttgaggaacaataaatgatcactgaatccaaaatgacttatcaggaagcactgaaagttttgggcgcaactggtagcgaaaccagcgctgaaatgtccagactcttcaaacgcgcatccttacgcaatcaccccgaccgtggtggtagcaatgaattaatgcagaaaattaaccaggcttacgacgtagttacaaaaactgggcctagtggcgcacgttctgagactgctggtgatgttcgcgcacgttatgcacgtcaaaagaaagaatgggaagaaaaagttgatgcttactttgtagtggcgaaaaactatttcagcaccaaatttaacgcacaggaatttgcggaatacttcaccaaatacactggattgcctaccactttcaaacaggaagtaacaaaaggtagtcacggtgtttatgcttcgttccgtttcacttctggtgatgcttactttgatttcggtttcaactgcacccctccgaatggacaagggttagccgctccggattcatctgcactgggtaacgtttctgttagtacctttgtactggttggaactaaaaaacataaaatggcaagccgtgattatcaatggggcaaaaacccagataagatcactccggaaagcctgttcccgtctaaaaaactggaaagcattttcagccctgtacagaaaaatatcaaatacaaacgtgctgattaccttgcatcattccgtaagctgttaggcgctgacattagcggaaacgatatctttgttgaagttggtacactgaaagttcgtttctatcgtcatgtaatgatgcgtaaaggtgcgtatgtgtttagcgcggtgtatgatcctgctgtatctaagtatcgtccggctgcacaacttcgcggaactatgttagaagacgaggacggcgcttgcctggatatgatcgttgatacgttcaaagagttgcagaaactgaaaccgagtgttcaaggcgttgtgaacgcgatcgataagatgaacgcagagtttgcagcgggacatcgttcagcatcttttgttaaacgtgtagctgctcaggaagccgcgccgaagccagaagagaagccaaaacgcactgttaatcgtatcggtaaagaggaatacttcgcagcactaaaagatattggtgctcgtgtaatgcctaccagcggttatgttgaatttgataacggcgctggtgttactatcaacttcaagcgtattgttgtaaaccgtaaagcatactactcattcagtagctttgatttcatgtactctggtcagaaacacattgagtggttgaaaggaatcgatatcgcagaagataccaaaggcgcaagcattagcctactcactgatactctgaaatctttacgtgggatctctgactggaacactgttaagagcgctttagatcaaatgaattctaacttcaaggcgggtaaattctccgcacctcatgtgaagaaggaagcagagcaaaaagcaccgaaacagaaagacgaaatcggcgcacagcctaccaaaccacaggcggctaagaaagatacaccggaagtggaaaaatcacaggctgttcatgcagcacgtgagaaagcgaatatgaacaacactattcgtaaaatgatgactatgttagtcaaagcacagcgcaaagacactccggaagatatcaagaaggaagttgatgcagcaattcaattgtggcgcttgacttactaatcaaatgaactataatgggaactgttaacgcagttccctttttatttgaggaaaatattatgagttgtccaacatggttacgtttggaaaatctgaaagaaggtacacaaaaacggatttatattaatcttggttgggttcctcctaccgattttcaaatggctgagattttaatcaatgctgttaaagaagtaagcgacacttacgaatgggaaaggctctattttcccttgattggtttgtatatgacgcgaaataaatttgaagaaatgaaacttgctgttattcgcgctacgattattaattcccaacaaagatttactttgaaaaatgcatggagttctgaatgattattcaagtatctgtacagggtgacactctgactgtcaccgaatccatcaataccgctcttgctgtatgtcgtgaccatatctcacaaaatcctccagtgactgagatcctggaaattgatgtttgggatcagattgggatgatcgacgcatcatatggatttaccccgcgagatgaagaactatctcgtatcgaatcatggctgaatgaacaggaaacggaatgaaactccctaagaacacaacactactaacccgcgaaaaacttcactctgttgattggtgtcctctggatatcatgatttttgatattgaatctcgcgtgatcaatgcaaaatatcaggggtgtagtattttctctgttgaattcgagaagattcgcgggtatgatgagaagtacaaagaaaaactgaaagttatgattgaagcattgggctatattgtaactgttgaagacaacaaaatgtggatcgcaatatgagcatagtaaaagcggtgtttgcgctggggcatgatatctaccacgatgatttcgcttttggatatcagcaaggcttgccgtggggccactgtaaagaagatttacagaacttcaaagaagaaaccgccgatagcgttctgattatgggtgcaaatacgtttacctctcttccgggtaaactacttggtagaattcattgcgttctgtctggttccggtagttttttgaaaaccaaaaaaggcgaggttgctgattacgtgatccacggtggcgggttgtctgctgctattggtacaatgcaagcaacacacccagataaaaatgtgtgtgtcattggtggtaaggggttgcttttagattcaatcaataataaaatggttgatgaagtagttttgacacacatttacggacatgatgtatataatgcccccgcatttaaacgcgatgtttcgtttactgcttctgaattgggtgatgcattgttaaaatatgaattttctgatttcgaaactcagtacatcaaagaacatgaacgcattgaaaaaatcatagtcgatcgatataaaaaggtataaaatgaaacagtatctggatattattaaacttgtacttgataacggtgttgaatcaaccgatcgcactggtgtaggtactattcgtattttcggcgcacaagcccgatgggatctaaacagaggtttccccgcaactacctgtaaaaaactgttcttcaagccgtgcaagcatgaattgcaatggttcctgtccggttcgactaatgtcgaagaacttcgccggatgacctggggtgaaaatagcgataagcgcacgatctgggacgataactatgagaaacaagctattgatttaggctatgaagatggttatctggggccaatctatggtcatcaatggcgttcatttggttctctttatggggatgatgatagttattatggcggtagtggtgttgatcagatcgcaaaagtcattgaacaactgaaatcaaccccagacgatcgcgggatcatcgtttctgcctggaaccctgttgatcttgatgatatggcgttgcgtccgtgtcactgtttcttccagttcgttgtaatcaacggtaaactgtctctacagtggtatcagcgttcagttgatgtcttcttagggttgccgttcaatatcgcctcctatgctctcctgacacatattatcgctgatatttgcgggtacgaagttggcgatctggtttggactggtggtgatgtccatatctataaaaatgcggttgaacaggcaaaagaacttttacagcctaaccgttcaccaatgccattaccgattctaaaaatgccgaaggtaaatagcttacttgatttagatcaagaattctttgactcgataaccttagaagggtatcataatcacggctctctaaaagctgaaatggcagtatgaaaaatggggcttcggcccctttcttaacaaggtaagagaatgaatgacattaaagtagtagtaaaatcctctggtgtacgccagccgtttgacaaagaaaaaatatacaaagtgctcaagtgggcctgtgatggtcataatatcgatgttcgtgcattccttgaaaatgtattagaactgatccgcgatggtatgactaccaaacaaattcaacgtatcgctatcaagtatgcagcagatcatatttctgttaaagaaccggattggcaatacgtagcatcgaatcttgaaatgtttgcattgcgtaaagacgtttacggtcagttcgatcctatcccgttctacgatcacatcgttaaaatggttgaagcggggaaatacgataaagagatcctggaaaaatacagcaagcaagatattcaagttttcgaacgtgcaattgatcatgataaggattttgaattttcgtatgctggttcccaacagttaatcgggaaatatctggttcaggatcgcgatactggcgaaatctttgaaacccctcagtatgcgtttatgcttattgcgatgtgtctgcatcaggaagaaactgggttagcacaggttacgcatatcgttgatttttataacgcaatttccgatcgcaaactgtctctaccgactccaattatggcgggtgtacgtactcctacgcgccagttctccagttgtgtagtaattgaatcgggtgattctcttggttctcttaacgctgtaacctctgcgatcgtgaagtatatttcacaacgtgctggtattggggttaacgcgggacatattcgcgcaatgggttctaaaatccgtggtggtgaagctgttcatactggtgtgattcctttctggaaacatattcaaaccgctgttaaatcctgttcacagggtggcgttcgtggtggtgctgcaacactgtattatcctttctggcatctggaagttgaaaaccttctggtgttgaagaacaacaaaggcgtagaagaaaaccgcgttcgtcatcttgattatggtgtacagcttaaccagttgatgtataaacgcttaatgaatcgtgattacattacgctgtttagtccggatgttgctaacgatcgtctgtatgatctgttctatgaagctgatcagactgcatttgaagaactgtatgaaagcctggaaaaagatccaactgttcgtaagaaacgcatcaaagcggttgacctgttccaacttttagcacaggaacgcgcacagacaggacgcaaatacattttcaacactcatcacgtcaaccaacagggtagttttacggttcctgttcgtatgtctaacctgtgttgtgagattgcgatcccaacgtcgccgctggatgacgatgataaaatggctggtgaaatcggattgtgtacgctaatggctatcgttctggataacgctgatatcagcgaattcccgaaactcacgcgtattgcagtacgtgcgcttgataacctgctggattaccagaactatcctgtaaaagccgctctgaaagctaaacagcgtcgttctctgggtgttggtatcaccaactatgcatcatggttagcaagcaactattgcgactactcagaagcgtataccgacaaagttcatgagttaatggaagcgtttcagtttaaccttctcgttgcttctatggaactggcgaaagaacgtggtgcgtgtggattgtacaacgataccaaatacgctcgcggattactgcctatcgattggtattgcaaaactgttgatgaactggtagcacctgtttataattgcgattgggaatggttacgtagtcagattaagaaatacggcttgcgcaactctactctttctgctttaatgccttgtgaaagtagttcacaggttagtaactctaccaacgggatcgaacctccgcgcggtttagtgagtatcaaatcttcgaaagaaggacactataaccaggttgtgcctaaccagaataaccagattgatttctatgatctgctctgggatatggctaaacgcggtaacaaagggtatctgtctcatgtagcagttatgcagaagtttgtcgatcagtctatttctgcaaacaccaactatgacccggcaaactatgaagacgggaaagttaaaacagaagacatcattgatgatctgctgtatgctaactactacggtgttaaaactctgtactatcataatacgcgtgatggtgctggtgatgaagaagaagccgcagaagattgcgcgggttgtaagatttgattaatgccccttcgggggctttttaaaggtaaagacatgttaacagtaatgaatacaaacccagatcataaccacttagaacaacctatgttttttggtgaagatactggtgttgcacgttatgaatcgcagaaacacaaagttttcgaaagcctgacgcaaaaacagctttctttcttctggcgtccggaagaagtcgatctgtctactgaccgtatgcagtatgcaaaacttcctgaacatgaaaaaatcattttcgattctaacctacagtatcaaaccctgttagatactattcagggacgtgggcctaacctcgcatttttgccaattgcatccgatgtgagcatggaaacctggatcgaaacgtgggcgtttagtgaaaccatccacagccgtagttacacgcatattcaacgtaacttgcacattgatccttctgtacagttcgaccaaatccttcgcaatgaagcgattatgaaacgttccgcatcaatgacacggtattatgatactctgattgatgaatgtcataagctgaaaactatcatgatgctacaggaacaggttagcggctataaaccaaatgatccggctgtcgtgtattataacgagcaatacactaaacaggccactaagtgcaaagaagcactgtacctttgtatgcacgctgtgaacgctctggaagcgatccgtttctatgtgtcgtttagtttcacctttaactttgctgaacaaggcaagatggaaggcaacgcgaaaattatgcgcctgattgcgcgtgatgaagcattgcatcagaaaggtactcagagtaaaatccgtttgtggcaaatgggtaaagatgatccagaaatggttgaaatctcccgtaggctgaaaaaagaagcaacggctatcttcctggaagtatatgaacaggaaaaagaatgggctgaacatttattctctgttggtgatgtagaaggtgtatcgctgaaaagcactatcgcttatattgaacaccttacagatcagcgtatgcgagcggtagggcttgattcgccattcaccccgatccctaacccgtatccgtggatgaataaatggctcaaaagtgataacgtacaggttgccccgcaagaggttgaagtaagttcttacctcgtcggaaacttgaatactgaaatcagtgatgaagcgtatgcaaaatgggccagcaaatacgcgtgattgtcgggtagtaaacaagtacaaaactgattgggatgtcgatattcaaagaggtacgaagttcggcaacccttatcacacaggaaccaggggagaaaacattttagcgtttatcccctggttccagaatcaggttcgtactggggcgatcacgattgaagaattgaaagaacttgatggaaagaggcttggttgtacctgtgcgcctcttccctgtcacggtgattacatcgcgcatgtggttaatgttttgtgtggtaagaaaagatcacttgactttttggatatataatgtatgaaatctgaattcaacttaacccttgataaatgtggtcgcatcgatcgaagttttgttaagtgtggtgaacttaggcattgtgtttattttattgcaattaacgatgaaatagtatatgttggtaagtgtagggatatgtggaagcgtttagacacatatcgcaatgcaaagtattggagagaagccaaccccagtaacatcttaaaaacgtgtcgattggaaatggctatcaaaaaacgaaaaactgtgaaacttatcgtgactactcacgatgaaaatacatatcatgattatgaaatcaacatgatacgaaaatacaaccctgaatggaataaacagcactatgacaaaggcacaaactaaaattatcaataccctttacaaacaactcatgcagttgtgtggtgaatccgaaacatttttcttcgttgatcaagtaaccgtgatgggtacacctgttagaatctttaactatcgcatggcctcatatacagactggctaaagcctggtgctctggaatgtcgcggtatcatgtttgaaatggatggagataccccagtatcaatcatcagccgccctatggagaagttttttaactatgccgaggtaaaggcatgggaagcgcttaacgagtctcctattgaattaggcgaagttttagacgtgatgattaaagaagatggttccttgatctcaactttccttgacggtggatttctggcggtcaagtctaaaggttcggttaaatcagaacaagctatggatgcgcacagcgtgttaatggcaaatcgtgaattgctgacccgcttaactgagatcgctaaagaaaactatacggtgaacatggaatacgtttccccgaaaaaccgtattgtcgttggttatgattctcctgatctgcgtatcctgaacgttcgtcacaacatcacgggtgaatacatcccttatgatgaactctttgctgacgcgctgttacgtgcgtatctggttaagcgtgagaatatcgaagtactggatctggatgcattcgcaaaagaagcatatcagaatgaaggattcgaaggctatgttgttctgacaacgaaagggtttgtaaaaatcaaaacaaactggtatgtcaacctgcatcgcacaaaagatagcatcaccaacaataaggatcttttcctaaatattgttgagaatacggtcgatgacctgaaacagctattcagttcggatctggtctctctgaaaaagattgacgatttcgaaaaacttttccttgatagtctcaatcgtttgagtgcaaaagcattcaaagctattgaagataacaaagggaaatcgcgtaaagattttgctatcagtctaagcgcggatttgtcaaacgacggtcggatcatcttcgggcctcttatgaagtatttcgaagaaaccgatccgcaaaaactggtcgaccgcatcattgaaatgatggttaaaaattacgaccagttcattcctgaacaatataaatgaggttcataatgcctaagatatcatcttgggtatggcctgtaatcgtggggctatctttgatagcccttttttacattgcagtcgataccaaaattgaaaatgcatcattacgcaaggatataaaatctttgcaagacgatgtgaagaaagtaaaagagacaaatacaagcaatactgtgatctatgtcgaacaaaaaggtaaggatcagcagttggtcaaggatgccggacgtaaagatctgctgtttaaaaaaccaggactgatcgaaatcaagatcaacaagtccttcgaagagtatatggcggaatacgacaaatgaaaattgcaacgttagcccttgttctgggcgttctgttggtcgggtgtgctgagaagcccccagaaaagatttttcctacgctccccgctaaggtgaatccggtgaatgtgaaatggaaagtggttgcagaagtccgagagattgacggtaaaaaataccttgtaatgccctatgacggaaatccttatgttgcattatcatatccagattcattgatttttcgtagctggatgaatgacgttaaaagacaaaaggatcaaaccgataatgttctgtgtacgttgggataccctgagaaatgcaaatcaaaataaccaaaacgttttttcgtgacataacagaaggaaaagtttatactgcgaaaaaggataaagaaggtctatggatagaaaacgattggaatcgtgatatatggctcaatctgacgaatgagtataacaaagaactaattgaatatgagatagtgaaatgaatctgtttatgactattggcgttccgggtagtggaaaaactacctgggcgcatgagaaagcccgtgaattgggtaatactgttacgatctctcgcgatgatctgcgtagctctttgtataatgcgggtaaaggtgctggcggatacaaatacaccaaagcgaaagaagacatgattgcagaaatgcaggatcacgttgttatctccactctgaaagatggtaaaaacgtgatcatacacaacacacatctgaaagaaagtgataaaaatcactggcgtgaaattgcgttggaacacaaagctgattttcatattgaatattttgatgtgtctattgttgaactgcttcgccgtaaccacaaacgcggtcgtgatgcattacccgtttctcgtctttgggaaatgtttaaccagtatcgtaagatccgtgggttcgtaccagcaatggaaattgttaatccccacaatcagaagtgtgtgatctttgatgtcgatggtactctaaccaaagtgggacaacgtagcccgtatgactttaccaaagtgatcaatgatccgccaaacatcccgatccagcaactgtttcacctgtacaaaaatgcagggtataaatgtgttgttgtgtctgggcgtgaaggtaatccgcaatgcgcacatgatacatgggttagcctgttgagttatggcgttgaaccggatgaaatttttatgcgtcaagaaggtgataccaggacagattttgaagtaaaagaagaaattttgtttgacaagattttagataagtattatcctgttattgcagtggacgatagagacactccggtcggaatgtggcgagcaaacgggattccgtgcttacaagtcgattatggtgatttctgattgacatataatgtgggtatgttaaagtacccacacaaaagaggattatattatgaacgttattcgtgaagataaacacatcatggttgaacttggcgatcgcattcgcgtagaaaatctgggcgattttaaccaaaaagttcgtttgttgtgccaaaaaattgctaacaaaattcaggaacagggtaaagctccgggcgggtttgaagttagcgccactccggtttctcagtactcctatattgtgtatattcatgacgtggatactaacagcacccaatctttcgggctggtgttaaatcctattactggctacgttacatgggcggctgtattatgaacgtaaaaattattgatagagcggtaattacggacgaatctgtatacccggatcctcgttattatggcggtgttttcggatacatcaaaggaactgatattgatgtagtaacaagtccgattgcagaatatgatatcaacaaaaatcagacagaagttcgcgttactacaatcaacggttcagagtatatcgttgaagcgactcctgattttatcaaacagctactaaaggtgatgaaagatgcttgatcatcctggctctatgagtatggcgctcctggaagcattaaaagcatatgatatcccttgtcatttcggtgaagtaactgttaatactatcattgacgaaatcgacaacccaaatactttcattgcttgtcttgttcgaaaattcacaagttgttttcgaccgagtccagaaaaagtagtaatcagttctgtttctgcacatcatcgagtgttagatgatggaaagattcaagtttactggaaagttctttatcacgtggtgtatcatgaagattgatgatattatgtttatgcttagagcaataagcgcttctaagttctctcaatgtgtctctgttaatgtcggtgctgcattgagaaatggtaacgggcgtgtgtttgtaggcgcaaataatacggttgatcctagtcatcgttgtacagatcagtgcaatcacttattagatgataacgggaaactgagtgaagaaaagcgccctgaacattcacaatggtcagatcgcaacgaagtacacgcagaaatgcgcgttattatgctggcggcgtctcatgaacaaatcaaagacgcaactttgtatacaactcattccccttgctcacaatgtgcgaaaaatatcgaattttgtgttgcaacaggtatgattaagcgtgtagtatatctacataaatacgatcgtggtggcatcgagtggatatggcgtctacagcaatacggtgccgaagtagtacaacttgaccccgaagaaatgaataaacatttccggatcaaataaccaatgagtaaatgtatgtctgaactgagtgtaaaagcatcctttgaatatgttttgattgaaaccaacgctaaagcggctggaactgaaattgtatcaccttctggtattgtgactggtgttcgtcaacacggagaggaaccgatctacggcacagtgttatcatgtgggccggatgtaccggaagaatataaaaccctgcttatgggtaagcgcgtaccgcttcctcatgcacaaatggcaaacgtgccggatcctgaactgattgcaggaaaggcaacaaaagaagaagctcgcaagtatccggttaaatatgtaaccgcacactataaagcgattcaagcaatttacgaataagagatccaacatggctaaacaaattcaagcaatcatcgccgataccgtcgcaaaatccaaaaaacttttcgacaaaggcgacatcctcgaagcaccgacccgcatcgatgtaatgacttcaatgatcattgatgctcaccagggaaaactgaattcccgtgcttcggaagtaatggaatacatcgtacagttcgaggatgtatgcaaatacgccaaagctgttgatccggctgttcgcgaaatctaccgcaaacagttctaaaaatatcggccccttagctcaataggtagagctaatcactcataatggttaggttcccggttcaagtcacgggaggggccaccaaacaaggcaaggcacttagagaagcgggaggaacagaatctgattctgttggttgtaggtgcaaatcctacccttgccaccaaattagggtgcgtagcgcaatgccgttaaatggttcggaatatgcaacctttctcacggagaaggctctgttggtatccggtaataggttccccggaatgcggggtgaagtaaagaaactcccagcccactaattttaatgaggtttatatgaaatttcgtgaaactgtgaaataccataacgcggtcgaatatacacagatttttgttgatatgtctcccgcaaaattcaaagaacgttatggcatgacatttaatgaatggaaagatggattgcccgatggggactaccgaaaaaacttcaaattcaatgaatgttatgtggatgatgatccttacgatctggatatttttggtaaaacaacgcctctcattgagaattcgccagaacagctttacgaatcttgtattgactctgcatacgaaatttaaagagataacatgaaaaatttacaaaaactgtttgaaatgtctccggcaattagaaaaatcatcggagaaaatagcaatccaacgaatcgcaataaaaaattgatggaactttttgcaaaagagttcgatgattttgattctgaacttcataaagcgcttgaggcatattccaaacaagggttctttgcatcgccgcaagtaaatagcaagaaagagtatagcgaacgattctttgattgggagattgtcaatctcgttcgtagaacaaatatatctccgagcaatcaccaattgatttctcttgatacttcggtattctttatccagtatcttatcagtggtggtttcaaaaatcctgaaattccgtttacaaatgaagcggttagcagtgaatttgatgaatcatttgtatacatcaacacaaacaaataatcaaatggctatcttcggatagccttatttttggggtgtctatgcgctttttaaagtatgcaagttggatcgtactcgtccctcttgacattattactggagtattagcaattctgtttgccccgtttgttgtaccgttctacaacgagaaaacagggcatcttcctaaaggcttccggtggatggaaaccttcgataaccctattgatggtgatggtggacatatccgccgttgggcgtccatacgctatcatctgggggattttggggtgtacatgcaacgtgttggctggttgtggagaaacaaggcttataacttcgcatatcacgttttaggacgtgaagcgacaagcaaattcaactggaaaggcaacccaaaaacagaaggtgggccgaaccctgtaaatcatgggtatctgctcatgtggaacgaatcagcatggggtttgtacgtttacaaaccgtggctacggatccacaaagtgcaattctgtttgcgcgtttatgctggatggaaactgaaacaagaagttagcgacccagttaacctagatcgtgcaatgctggcgtttcatttcaacccgttcaggtattatgtaatcaagtaaaggtaatacaatgaaagcatttcaaattttagaaggtttgcatactggtacgatctatctggaagaaggtaacgacgttcggatcgtagtatcaaaaacattaactatggattctgtgatcggtaaagctcgcgttactccgtttgaaaagcgagagattgagatcgaatatcaaccaactgttaaggtggaaggtggacaacatttaaacgtaaacgtgttgcgccgtgaaactctcctggatgcggttgaacatcctgaaaaatacccacagttaacgatccgtgtgtctggttatgcagtgcgttttaactcgctgacccctgaacagcaacgcgacgttatcgcccgaacctttacagagagtctataatggcaattgatgatatcaagggttataaaccccatactgataaaaaagtagaaacggtaaaccgtatcaaagatgctgaaaatgcattaggtgcaatcctggaagatatcgaacagcgactatcaaattcagatattgattcactgatagaggaagaattagatgaggtgcttgaacgtatccatcaaattcaactagcgaaagaccgactgaaagaagcctctatgtgggcgtgtcgtgcggtgttccagcctgacgaaaaatattaaaaatcaagccgttgccgaaaggtagcggcttttttcgtttttggtgtaaaaagttgttgactcccttctcacattcccttatagttaatcccgtagacaagaaaacacttttatgaggatgacattatgaaacgctcttacaacatgaatgaactggttttcttcaaaactcgtcgtgaagcacgtgcttacgttctggcggctggtaaaaatacttctgctgttatcgatatgggtactgataaagctgttggtgctcgttgggccgctgttatcgttatcgctgctcctgttactccggttaaaactctggtacttggtgcgcgtcacactgaaactcttaacactgctgcaagcggtaggggccacgaagttaaagtgttcaagaagcgttcttatctttcatgtgtaaggggttaattatggcacgattcatatataaagtggaatacgaaaatactgagttatctgatacctttttgaagatgattcgtgatcacgggcaacgtctggaaagagtaacgattgatactgcgtttgattgtcctgttgggttggttctaacattatcttgcagcccagcaaaagaatcagcccgtgtcgaaatgttacataaactaaatgcattttatgaaggtggtagtgtatggcgagtattgtaaaatttttcaccgactcagtgaaagaaattaaaagcgctctggaacaatggaacactcgttgtgatgtatccattaaatcagagtacgaaacaacttatgatcgttatgatccggcccgtggtttgcacaataacccccatgaggtggaagtgtgaaatactacggattcaaaacgagtcattttggtaaagcgtatcgtacagaaaacatcgatcgcaaacgtccgtactatgattctttagtacgagcgggacgcaaacgcgctcgccaggaagggaagaaagaaggtgaagatcgtggataattggaaagcgtggatatcaattattgttggtgttatcatcggtcggggtttgtatgatttaatcttttcggcggaggttcattatggacattggttcgggtagccagtacccatcatgcgcattgagcaactttgctcctcatccattcacgtttgacggggtagaatgtgcatcaatggagggctttttgcaaagcctgaaatttagcaacccagatatgcaagcccatgtatgtactctggtaggcaaggccgcaaagttcaaaggcaaaaagaaaaaatggtggactaaccagaccttatactggaaaggtatccctattcatcgttcctctgaggcgtatcaaatcctgattgaaaacgcatataatgcgttattccttaatgaagggtttcgccgtgcgctggcagcaaccggaaaaagtaccttgacacattcaatgggaaagaataagatgaatgaaacggtgctcactgaacgtgagtttgtccgaaatttaacccgattgagagatctgttatgagtgaaaaagaaagagtagaatgcgtgttcctgttcaaaggcgcgattaatccattagcgttactgtatgcacaacatgcattacgttcaacgttgattcagagtgttatctataaagcaggtgtgtattatgttaccatcggcgcaaataacatggttgttattgaatcctatgttaaggaatgtgcatcaaacggcgttgtctttgataaagtcgattttgatgcaggggtagatgctgtttatatgtataagggttgatatgagttacgtagtttatttcgattgttcggatctcgatccgttcgtgcttcaacaggcaaagaaatatcatcaagatgtcgttggcattggtgtaacaaatgatgatatgttgtgcatcgaatttgaatattatcggacatttgagcgtgaacaattcctgggtgaattgaatgcattcaaaagtacccttttctttgatcgttatgaggttatatcttgaaacctgttattcttaccgatattgacgggatcgccgtaaaatggcagtcgggattgccgttctttttgtctaagcacaacatgcctactgatattgcattagaaatggttacagatgaaaaatttcgtgatatgaccgaaatcttcggatgtgatcagcagttggctaaaatccttatggaagaatacaataacagttctttcattcgttatctgaacgcgtatgatgatgcattgattgtgatcaaccgtctgaaaacgcaatatgatttcgttgccgttaccgctctgggaacaacaccaacagcaagccttaaccgaattgctaacctgaatactctttttccttctgcgtttaaagaggtgatggtcgtgggccacggtgaaacaaaaactcatcgttacctggaagcaaaagcaaagtatggtaatcgtctggtttgctttgtcgatgatctcgcgataaacttaaacgaatgtcataacgtcattagccagttgccgttattccatatgttacgtggtgaacgtgaagaaacaaatgcacctcatcagttagtaaaatcgtggtttgaaattgaagagaaattaaatgatcttgtcaatccttaatgaacttgcttccactctgaaaactaaagagaaagaagcaattttaaaacgtaatgcagataatgaattgttgaaagaagttttccgcattacgtatacaaaacagattatgttttatgtgcgccagttccctttagtagaagggaaaccaggtacaacaccgctttccgatgcaatcaaagcattactggaagatttagcaagccggaaatatacaggcaatgcagcgcgtgatcgtttactggatattgtatcatcagtgaacattaacgatcgtgaagtgctacgccgtatcattaaccgcgatctggaatgtggtgctggcacaaccttaccaaaccgggtatggaagaaactcattcctgaacagcctcaatgcctcgctacgccgtttagtgaaaaggctttacgtcgcatcattttccctgcttactcgcagcttaaagccgatggtgcgcgttgcatggctgatttgctggaagcattaaaccgtaaggtatcgagggcgggtaacgagtacgaagggttaactcagcttgatatcgatctgaaaaagattcgcgattatctgggatatgatgtagttctggatggagaattgatttatgttccttccggaaccgtaccaacattacctgaacctgaaacagacatgcctttttctttatctgctttcatggacgatgatgataacgacattgcgttatttgcggaagaagttcgcaaagtatcgaccccagaagaagaacaggccgaagcaaaacgcgaagaagggaacgggatcgtaaacaaatctctgaaagggacgatcaccgaagaagaacagcgaaacattgtttatgttgtttgggatattattccatatgaggtgtattacggcgaagctgaaagtgttcagacttatgatgagcggtttagcctgttgcgtgatatcctcctggatctttctctgccttctgttcgtttgattcagtctaagctggttaataacattgcagaagcgaagcaggactataacaattaccgcaatgacggtaaagaaggttctattctcaaaaacagaaacttcaaatggaaagattcgcgagtagccgatcaggttaagctgaaaaacaaaaccccgattgaactacggatcattgatatctacgcgcacactaaagaagaccataaggtcggcgggtttgtggtggaagatttatccggaatggctcgaacgaataccggatctgggttaactgataccgattatcgttacgatgatgatggtattacccgtgtatacattccattagatgaacgtggtgaactggatcgcgaatacatcatggcgcataaagatgaatacattggggccattgtagaaatggaagttgacggcctccagaagtcgaaaacgcgtaagaaaggggaaccggaatacagtttcttccttcctattatcaagaagataagacgcgataagaccgaaccagacgatattcatgttgtctttgcagatctattttaataaaaagcccttgactccggtcgggggctttgttatattgcatatcgaaacgtaaatcactgagagaatatattatgactagtagttatcagaaacacaaaacccttatggcaaacctgtccggtaaacatatcgacgaagtaaaatctctgctgacagtaaccgaaggttcccgcttcgaaaccaatcacattatcaaaccttctgtgaagaaagtactgaaagtgatttaccgacatccggtgtatcagtgcgttcatatcatgaacagcaacgcatttattttcgtatataacgaatccgatgataagtgtgttggtattttccgaaaacctaactttgaatgcatgagcgaagcggctgttgcaaccccgatcgttgaagaatatccggattatgttcaacgcaacatgcgttatgtgcaatcccgacttgattatgcatacgatttcaattctgacgcggtagaagcgctggcggatatcctttgcaaaaaccagaaagatcgtcaaatgacaaaatatctgactgatccaacaccgccaacaattcgaatttctgttgaagttccgtttgaaaatcatttcatggcagttgaagcgcttgctaaacttggtttagaagtgaaaacagaagccgtttaatagcactttttgttaaagaagcctcttgcaatgcagggggcttttttgtatattgcacacatcgaaacgaaacagacaaaaggaacatcccatgcaaatcactaaagaactcgaaggcaaagtaatcgttctggtaaataaagaccgtttggcacaactgggtaacggtggtgaaaaactgccagcggacgcactcgaaagcctttctaaaatgcgcgtgatgcgcgttactgacggttgggttacttgtctgcctctgaacgacgaagacaaagccgtatacgatgcacaagcggattcatgggatatcgaagtacctctggtaaacatcgaagttgaagagtgctacgaaatcgaaaaataatgcttgtgttctgggtaatgtaatggtacattacctacatcgaaacgaaaggagaaacatcatgaaagttatgcacactgcaaatcaacttcaaaacggcaactacgctatccacgatgctatcggtgcgctggttggggtttatcttcatggtatcaaactccttgaagtaagtgggaataccttttatggtgttgaaaacatcgaagcagcgatggaaattatcggtgacctgaaatgagtaagaaactcgaaatattcgaaactatcagcgaagacccgaatcttcgctggtgctgtgcgaaaactgggtttgatgctgcatggggtgatactccagaacaggcgcgtaaaaactgggaacaccaacaattgttttttgcctgtcgggttcctaccaattatgaggggagtcaattgttagcatgaaaaataaagaatatgacccaatagaagttaaagagcggttatcggtagcaagaagattccttgaatctatcgaccctgataaacttggaaaatgccctgatacgatttgccttaattgtgggcgttctgttcttgttggtaagtgttgcgataatccaaatatagttgtgatggaaaaggaacaagtatcccccgaaacatgggatcagatccaggaaatcattaaaaaccctccagcgccaactaagaaattacgtgaattgatgacaaggaaaatgaaatatgagcaaatttaaattgagtgcaaccgttcgccttattcgttggaatggtgaagagatccgttatgatgaccctgaattcgcccatgaaattctttcgcatcgtttgggattgaaaaacgcgtcattggttcaaactgttaaaacatcagcagagccggaaatttggcgttgtgttattctggatctcgataacaacattgattatgatgatcctaagaactatccgcttctggaagcacaagttgagaatgctccagaagacagacagtgttttttggttgagttgccacgcgaacattacgaaaacatcataaaggcccgtaaaaaggtcaataacaatgttttcgatctccacctcggattgtttgaggattaagtactgctagttgtgttcgtagtagcggcgctggtaggttcccccacctgtatacattcaagtgtttgcaggtggaaatcttttgatacgtctcgaacacattcaacgatcagatattttcctgcatactcttccccaaatacctcaatgattgcccctaccttaacatctaaacgaccctgctttatatcgaatcggatccggcgttcatagctggataacaattgcattttagacgcctggaaaggtttaccttctgaatctgggttctgaaagttggtatcatagattgcattacggtttgtgaagatccatgtattttctgtgtctgtatcagccagtatatcaccgtacatctttttatcagtcaatgacagactaaagaaactggcatctttaaacagcgttgtgttatccttatgggtaatatactgggcttctgtgaatatgacagtatcaccaacaaacacgttatcaacgttaaatttgtatgctgggatcggtgtctgggccagaatgtcagttgaacttttaaggaaaataccggaaccatcttcccacagataacagaagtcagaagaaactacactttgcccgttgtccctgatataatcaaatatatcctgatatgtgccatttagacatccaggagggatacgtatgttaccgccgtcaacttcgggggtaagtagtttcattttgctatacagtgccgtcatacactctgtaatcgtctgtacggcgttgttactaaatgaacgggcaaacttacgtctgaacgttttatgcagcggagagaggttcatacgcagcacagagcggtttttatcgtcggtatctacgttagagtaaagcaatccgtaataatgttgttcctgtgtaccgttatactggaaagatacctgtatgatcggctggataagttgctgatagattaactgtgcgtcgtatatctgcatcagcgtttccgatgagccgttaatcatcgtcttttcactaaacgagacaagagcgggtagcaattcagtatatgcgttatcaatgtatttttcgtatgatgtatataatttaatcgatgttattcgattgacgattttttcagccataaaaatccctcctaatatatcctatttactaaatagtaaataatgacccaggttcaatttgaggcaataatgaaaaataaaactcttgataaatttatgactacacggcttgaaatcaagaagactaacgttaaaaccgttcatcttccggatggaacagccattgagatccctaagatgtcgtatcgtcattttgtaaagattaagactctgaaagatgacccagttgcgatcatgcgattcatcattgatgacatcaaaccgcgtgaactaacagcagcggaaattgaatttgtgttgatccatatgtatgcacacaataacgctgattatgccaatacgcttaaagaaattgggctaaatcttgatgacctcaaaatctccgaaccttgctatgattttacgtttgacaatgtgcggttagtctttgacaaacccagcctgttaaatgctcaccttccgttcctcatcaaagaggcatatgttgacggtaagccagtagaattaactgaggataaacgagacgaattaattaattgcctgtaccgattcgaatatgatcaggtatcgcgtggtgtcctccaggaagtatacattattcatgaggggaaaaccatcaaagggcttaacatcattggtgaatgataatggctaactcttatttcaacgaagaacaaaagaaaaagtttctgaacagaaacagcaacaaacaaccagcggtcaccaaagtaacagcctcccttgatgctgaaagcgcccgtgacctaaaggaaatcaacgataacacccttgaaagtgcaatcaatactcttgatatcaaagaagggttgaaatcgttcgaagaaaaattccgtgacaaattcgcggggttcaaagaacaatacgaagaggataaaaaggaatcattagccgaacaactacctgatttcgtcggcccgatccgtcctatatccttaaccgatgataactcaaaaactgttgacaatacagtaaacgttaaccaaaatggtcagttcggtaaactggaagaaaacaccgaatctatttttcatgctattaacaaacttgttgatttatatgaaaatactgataagcataagccgcttcctgaaccagtggaagaacctgatccgtatgtagacactaagaaaaaacgcatcaatgatgatgatgacaaaagaagcaaaactctggatagtattgctaaaagtctggtttctattaaaggttttacatcgcagatccttagccgtttcattggttactctctggaagcaatggcaaagtttgctaaatggacgctccttattggttcgttaatctttacattcgatgtgttgcgcgtcacaatacgcaaatggttcgaagatatcctgaaagaaggggaatcctcaaaaaaactatttggtacatatctgggtaacgtaaaggctatcgtaacaaagatcgaagaaggtttgaacaacttcaatatgaacaacttaggcgaatcacttcgtgatttgttcgttgagcctatgaagttgttggggcaaactgtacaaacggcaatcactgagggtatcggtcgtcttattcaatcattgggtgaatcaactggcatagacagcattaccaatgccggacgcggaatgcagatcaccgctttacgtgataaacagaaatttggtcttgaattgactaaagaagatattcttatgatcaagaaacaggaactagaagaccaaaaagcggcattagaaaaagaagataaagctattgcagcacgtcatgcattaacaataactccttctcaaattcctaatggttctatctataaagttgctcctactgattatcaagaaagaaatcagaaaaccgtagatgctgataaagaacggcttgataatatgaagaaagcaacggaagaaatgcagaaacaatacgatttagctaaaagcagcgaagaggaagcacaaaaattagccgatgaggaaaacaaacgcaaccgcgcacgtatagaagaagcaaaaaggttagaacaagcgaggaaggaaggaaaacagccgccagaaggtgaagagaaaaaaggtgatgatctgttgggtaaagcaaccaactatgctaactctgaaaatctggatgcagccgatatcaaatacattaacgatgaactgttggatcagcttgaaaaacgtcgtaatgaaggtaatctggacgatgtacagaaggatagaatctctgaccttatcgagcaattgcaaaacaagattgcagcccgtacagaatccagcgccccgatcgacgcacagccaccgttagcagcaaataaaccggatgctgataaagcaagcaacattcaggttaacaacaaaactgttaacaacaacgtaactcattcagtacaacgcacagagcataaaccgctcgtagcgctggcataaggaacatataatgaagttttctattattgatgacagtataaacactctcaaaaatattaaaaatcgcggtatctcctctgggggtgccgcaatcacagaatcagtattaaagcaaactatcgttaccgccgaatttccggcccaacgtgcagcaggtatcgataacgcttataatgcttcgagtctgtataataacggccttctgttcactgcatatgattttaatggtgttggtagtaaagacaactatcgttcattacgtcaggcagcacagaacccaaaacaaatactatcatctgcgacgggtaatgttaagtacaaacaagtgttgaatagttctattggtactatggaacctgtttgccagatcctgctaccgcgaagcctgaacgataacgaagtaaacagccaccgctatcaagatgcaaacgatagtttcttaaccaaagggttgagccgtgttgtttcaaacatggtatggggcgctgtagaatccatttcaggcggtattatggcagaccgaagagaagcccttgatgttggtactaaagccgctttccagggttctgacaagcgaacaaagatgtattacaatacattcgtgatcgaaagccgtaatgatttgctggaactgattaaaatctactatctgtttactgttctgggatatggtacaacttctggcggtactgctaaagaggttgctgcattggttaaacagtattacggtgttctgggtgctaaaaccgcgaacgcaattagcccttccagtaacccagtaacagcgtcagattttgataatagtctgggtaatgacgtggttgatttcatttcaaacgtagaggttattaaatcgcctcctgtctggtttattcgtgatttccagtctggggattccttgcgtttacctcattcaacctttgggccagcaggtattaccagtgttcgctttggtcgttctattgataatattgtaaatacattaagagaatcaccaaataccccgatctcacttgaggtcgaaattcaatttatggaactgatcgatatgcgtcaggattctatttttgatacaaattactaaggagatatgatgttttacaacgtagatgaatttttatcaggtatggctaatcgcgattttcagcgtagcaacctgtttagcgttgtatttgcaaccagccctgcatcacgtatccttgacaacacgatcggtagtattcgagatactttgattgatggatctattagttctatcaacgcaaacaacccgaacgaattcattaatgctatcactggcggtgtgagtaaattgtttagttacaccgtcgataaggcgattatgtcgctgaacaaaacaggatttagcaaaatcatcggggcaattagcccccgtttgattacttccctgtttggtgatagcatgtatggacaactgctatctgaattccgtgatgaaatgatgtataatatgggtttaagcattatgggagttaacctccctggtaaatccattgggtacgaatacgtttataatggtggcgtacctcaaatcagattcactcgccctgagaatggggaattgtcattgacgttccgcaccgattcagaagcccgtaacctgaaaatctttaacgaatggatttccgctattcgcgatgatgtaacaggacaatacgccttcattgatgaagtgacaagtactattcaggttaacttacacgatcgtgatggttcaccgcatacaacatacgtatttcagaagtgcttgcccgtcaaaatcagtaacagtgaattgagctatgagaacaacaacgaaatctggacatttactgttgattttgcctataaaacatcatgggttgttgaggctgataaagaaggctgggaagggttcaaacaatccgtagaggaaggtttagccattgcagcacgtaccgcaattacaggacaataaaggggctacggccccttttgaggatcttatgtttgatattattcgagtaacattaccatcagggatcaaacgattccctatgtttacagttaaagaccagtttaaactaatgctgacccgtattgatatggaaggtcggccccttaaagagcaacaggaaatactggatgaagtgttggatctgctttaccctgggtattccaaaacagaacaggaatatattttcagccgggtgtattgtggttcgttcggtaaaaacgttatcaaggttgtgataggtggtaaaggtgggggccactccgaagccttcatggtgattaatgatattcaactggaaaacgaatacaagctgaatgatgaaatcacactagggtttaacttcccccatacacgcaatacaagcgaagagttgtttcttgaatgtatcagttatgtaatatacaacgaacagcgctatgaatggacatcactaaccgaagaaacgaaagagaatattcttgatatcgtcgaacttgatgatgtcgaaaaaatagttactatgctaacgaaatcggttgatgtgtctatgcgcggtaaatcatttagtggtatgttaaccctgttcaagatcctgtttagtcgtggggatctggatgaatttgtgaagaccaactatctgctaaataaaaacggcctgaacctggaacctatcatgaatagtagcccaatggaaaggcaaatttatactgcattgcttgcagaagacttgaaaaaacaaggtgctgttaaatgagaaagcatgaatataaacacgttgagaaatataatgttgattatcgtcctctgacacatacagagtttacccccaatgcagattttatcaaaggggatgtttacctgtatcaaagagaatatcttttcattctggcacttctggaaagtaaaaatatcgatacccgtcaactgttcatcaactgtgaagaatgtcaggaaagaatagaattccagcttaaacgcaatcaaatcatggttgaagatttcgacgataagctatacggcaatgacggaatcgcgctatctgttcaccctcgtaagactggtgatgaagagatccccgatcttatcgattacgtaatgatagacggcgaacagatcatgtggagtgattgtagcgacaaagataaagaaatggtgttggatgcaatcgactatgcaacctataaatcgatttctaccgccctggataagccagcagtggtcgcaaacattccggtaaggtgttcgtgtggacatagccatatcgtctctctgagaggcttacagcaatttttaaaggtggtctaaatgggtgtaaatctgaggttgctatatagcgatatagaacctaacatgcaacgagattggaataatgacgtagcggcttcaaaaggggccgcagcagtaagaaatagtttgattggtatcgtaaccacgatcaagggtacacgtccatttgatagtaactttggttgtgcaattagtgatatgctgtttgagaacatgaaccctctgacagcggaatcaattagaacttctatcgtatctgcgatccggacatatgagcctagagtatataatctttctgttgaagtcattccacagtatgatgataactcagtaacagtaactatctattacagcatcattgatgacccggatgacgtagagcaaatcaaactacagctttccgcatcataacaaaaagccccttcctttcggttggggctttctcttagaattcaatgaatcccattagtgtttgatatcgcaattcaaacggggagatataactttgcatctggttttgatcggatacgatgtaataatacacctcatcattatcatcgtatagtgcttctttgatgatgcaatatcgatcggtttccacgttcacataaagagtatccatgtactttgtaactttggaaccctgtgaactgatctcgtgaatagcgttatctatgaacagtgacaatgcttgcatgaagttatcaaactcaccatattcacagcccataatagaaattgcagtgtattggtgccagcctttgattgtgtctccacggcggatccatccaatttgtctacccccgatagatacacaccacactttaccaatagggctatagaaccgcaaaacttcttttaataacagggacatgaccccgcattttgtataaggattcattttaacctcatttcatatcaagtagccatgaagggctagtttcaagagaaatcgcagtatattcgtattttacagtataacctttgaaaccgaaaggaataattgcattttcattgagatattttactttatgctttgcttcttcttcattcagagcagcacagactgttgtttgttcaacgttaccagcaggagaagtaaatttttcaatgatgatatatacgcagttcatcctattgtcctctttccattttttcaagtttcatcgtatccacttgcagttgaagtttaagaatacaacctttcgatatgttatacaagtagtcactaacgatttttgactttacctgatcgtaatcagaagataacgtaatccaatcatacatcgtttggtatgatggaagatacgtacattgttcttcttttgataacgctttaaatgattggtaatcggttggaggttccgaagcaattgcggttgtggtcataagactaagtgcaagtagtagatatttcataatgtattcctcattgttttcgatagaaccaatatagcaaaaagccccgaccgaagtcaagggctttttcatcaatgcaagaaagatttcacgtactgttcgatcttttcacgacatgtatcaactgaggtgctttccgcaattacggcatgacataacgcctcgcctccgacccagaaactcatcatgtactgaatatcacgaccttccatttctttttgatgcgctttgattcgatcgaaagcgttttcgattgtttcagtagcagtaagcatttcggattccccgtcaacctccgccagttccccatcgatcatttcgctttcgacttcttcccagtatactatcgttatcatgcattaccccagtggttaaccgtcgtaatccccgccacaattcacattgccttcaatgaacagttcgcggttatcacgtaataaattatactttctttcgagttcaggcccgaacgcgtcggcgtcttcataccagctataattgtatcttccgcattcatcatcatattctggttcatcgccgcgttcattgaagtgaacaattttgatatcgtccatccccagttctttcaacttatcccagatatacgaaatctcaacgctatgggaaccgaacgcttccagtgagatcgtaccgttgctatcgacttgaggaataccccacttcgaacgagtatcatcggtgatcatatctattaatgactcaatattattctcaccgtagatatcagcaacttccttttctttaccagggcgaacaagtccgatcccgataataaagctactgcttgagctattgctcacaaacccagaacgaattttcatcgcatcaccatattaccaatcatgaatagagggattagcgcaaagacgataccccatagaatgaccttatcttcacgacggtcacacccatgatagataacacctccagcgaaaatcaatacaacaactgaaacgaacgcgaataaagaaatcatttgcgggtatccattctcatagaaacttctttcaggatcttattcagatcgtgaagcgcatcttttacgttaccttcgttataggtaagcatatcctggtacagccctttcaaacaacgattgataacatatgctttttcagaaggtaacattgttccagaacgattataatctctgaaaatgtccatcatcgtgccgttgttgccaggtaatgacgggttgaagttaaccataccagacatcaaactatcaacatacacaacggttgtgttatcagaacgatacgcgccaccaactttaaaccagttgctgaacacatacggagattcccgcacttcgctcaaatcggttccgatttcatcgatgtttacacgaatgttgttaaaatacaccgattcatcaatagaaccaggacgccatacgatagcaccgttgttatttttgaatccgactacatcaacctgccagccgttatctgttaaccggacatcatcaacgacgatgaaatcaggtagctgtgaatgaaagccgatgttttcaggacgggaattacgaaacccatcacgattggagaaataaaggatgtcaccttgattcagttcgcatatattcataagatttttaaagtccaattcaagtaattccacaagtcacctcaaagccccctttcgggggcgagatctcattagagtttaacttctttttcttccagaacgattgtgcaatcaaatttcacatctttccagaattccgctgcaacgatatctgttgcggtaacgcttacgctggtttcttcaaaatccagatccgcaaaccatgcgtgtccgacgacaataccgtacattacacgactcaggcgattattaagggcgcgaacctctttaatagtttcctttgtctgcttatcaagatactcgatcaggtcattcttgtcaagcgcttcgatctctttagatacagtatcataagcccacagaatgatcaggtcgccattgttgagtttcttcttaccttcggcgcgttttgcaacggtagcagcaacagccggaagtgatgaaacgcctttgattttcacgttcagttctttcgacatgtaaacatcagtcgattctgtgcgctcaaccttcggagaaaagccgtaatcacggatcccttgctcagacaaccattcaccagccgcctcaccaaagcgctgtttaagcccttctgcgttgcgtaaaccaatcgcgttatcacggaagaacttcattaccttctgacggcctttcaggatttccagacggacgttatcagcaacaaattccttaccagaaataccgcgagtcatcgaacggttaaccagaggcagagaggtaaagtcaaccagtacagacatacggtcttcaccaattttagccagcggtttgatagtcagaccagaagcacgtaagtttttcagagtcgggatatcggtttccagcggaagtaccttaacgttaacgataccatctttaacaatggtaaagttacgcacttgtttggtttctactttttccggcaatccaaactctttttgtttgctttccggaatggttacgtaaccttgtagatccgtattgatagaaatgttcggacgggaactgttacccaccaggtgtttcactgcaactttcgttgtggtttgggtaaattccggtttccatacttcatgcgctaccagttgcgccgccagtgctttacgttcttccggagtagaagcgtttgcaatctgttctgacagtttatccagtgtatcatcatctttctggacagtctgacggcctgtacgattgtacgcccagtgttcagaagacaggtcgatcacggtgtcggtttctgccagcagttcgagagcatcaaccagagtaaacgcattttcatcaggaaccatgttgtaatcaacaccatccatcagacgtttagccggatcaacaaccgcttcggagatcatatctttagcgttggaataatcctgtttggtaaagcagttatcgtatgctttaatcagacgcacatcacccagctttttcagaactttccatgccagatctggattcatggtatgaagcgcatgatacagaaccacatacagaacctgttcaccttctgctgttgccggatcgaagccgtcaacgtcattgatcgcgttttcacccagcgcccaaatgtttttgatatgttccggaaccagaacaacaccatttgcagcattcaggacatacacacggccttcatccaggtagatcgcatgggttgcatcgccaactttgacttcaacacgtgcggaggtttgcgcggtaatgatttcatcaaatgcaggtacatacgcatcaaacccttcaacgaatttgtgtaatgcgttggttgcttccgccattttttccagcagaggacggtttacataataaccatattccaggaaagcaatgttgttaaacgtcaacggcagagtagaacacgctttcaggatgtcatcagtacgccagcagttatcataaccatcagtcaggaagatcagactgttcagattgccattatccgcttgcagatcggtagcgacttcaaccgccagttgcagaggttcaacgaagccagtacatccggtcggacgcagataacgatcgatagcatcattgattttgctcaggtcggatacagagctaaccttttcgcccacgaatacagaaccgaactgaccacggctggagaaatacagaatagatacggtatcatcctgcttaaccagcgttgccaggttgtttttcaggtgctgacgaatgcgcgggagttcgttatacatcgatccggatacgtcacaaacaaaaacgtggttagtcggggttggtttggctacggcgtttttgaattcaatgttagtgatcataattttctcatttataggtaaattttattaaaatttcgtttacttttttgctaatagtatctaatgcatcatcgcatccaaacttactactcaacaatgaaacaaaatcatccatcgttgttgtttgagactcgccaacgtcaaaagacagagcgtaggcaacaggatttttaatccttacgatttgaatagtatactcattcagatcgaaccgttcaagatattttcgcaaagaaaataaatcaatcggtactggtagagtttgactaaacgttatttcttcccccagttgataggggggcatttttacacagatttcgtattccatcagtgatgactcttcatagtgtgttccagattacggaaaatttgcccgtgttcaagctgtgattggaattctccgcattcatcagagtaagtaaattcataaatgaatacaccgttctgattgccaaatttagcgttgtactcttcatacaaccacatcttgatcagagcgtctttctcttctgtttccagatcataccagtcacgcccatcataagcaagcgcaatttgaggattagaccgatatcgagtttcggcgctatcttcggtttcccattcataacgcttatcatcataatatgattcaaagccattccccatatgaccgcccaggtcgcggtgtacttgctgtacaacttcttccgctgtcgggcaagtcatccagctataaccacagttaggaacacaatcacccatcatttcgcggagattgttgatatcagtcggatccttcgggaaccggacgatgaaactacttgatgaactattgctcacaaaaccagatcggattttcattataatttctcccaacgttcagcatttttaaccttcatctttcacttccttcatgtttttcataacttcttcaaaagttacaggggtctcgttgtactgttgcgattcttcatcccatacatcacgatgcccgaatgttgaactttttgcaatgattttttcattttcccatacatcaatagtaacatgatcaccaagataagggaaattaggaactttgttcagcgcatcaacacagttttgcaatgattcagaaacatgaacaatttcagtgaattcataatcagcactataataagctacgtaaatcatcaccaccccctaacgatgctaatcaacagtaaccccaggatccagaacacagcaaccgcacaaatacgggccattactacatttccgcgactagtccactccgcactaaggaacaagagaacaaacgttaacgcgtataaaaccatttcaataacttcggtaatcatataaacctcacgaaaaagcccctttcggggcttgtttaattaatgcccgaacacaccacgaatagactctgcgaatgcatacagttcaggatttttagctttcactgtttcgatttgctccagaatgtaatctggtttatatttcgcaccgaaccagcagtaagagaaagagcgatcccacatgaacacgttatagtattcaccgttgcgaacttcaaccatcacataaccaggattagaacccagcgggtaatctttcagaagattgaatttcgcgccagcaccagtacatccgttaaacaggtcattaaaagtcatggtatgttccttttgtcagtttcgtttcaacaaggacactatactattcttctttagcctatgcaagatttaatttagcaaattcgccaaaatgttttatcgcttcctggtcgtatgcttttgcagcctctaattcatcactataagaaccgatatgcttaaccttaccatcaaccattatctgtgcaatgtaacgtattccggttggttgattgcgtacacatacacccttgaatatgctggttccttcctttcgccgtttcctgttctgagagttgcgggattggttcgcttcgcgcaagttatcaatcccgtcaccagcctcaacaccatttttgtgatcaatcacatcaggtagttttccggtcgcaacgtagtagatgattcgatggcgtagataccctttgcttttgaaataaacgcgggtatatcctcctttgatcttcgaaccaacttcctttccgatcaagtcggaacgtttatgcgatgttcgtataatctttcctgtgtggacatcaacagaaacagttttgaggaattcatcaattcctctctgttcttcttcaattgttcttaatccattatgtgacataacgccttcttaatttgttttgctatggcttcaatcactgggatggaaactgaattcccagcctgtttgtaagcctgtattttgctttcagggatgataaacgaatccggaaatccttgtaacctaaaacattctcgcgggcttaatcttctagggttcttaccttcctgcaataccagacattgaacaccgtcctttccatattgggctgttatcgtcccagtacacacagaatcaactgtaacggcctgatagccaaaccccttaccgtttgccttgtttcgttctttacgctctctaaagcccttccaggcacgatctgatatggtgtattgatcattatccggttcgagaatgtcaccgacccttgttggggtacgtggaggaacaggaaaactaaagaataccggatcgcgaaagcagacaataaacacacgctctcttcgttgaggcaatccaaagtcttttgtattcattacctgataatggatatcgtatccttcgtcctgtaacagcctgtagatggttttaaacgtgtttcccttgtcatgggttaatagctggggaacattctcaaagaacagcacagagggctttttagcccgtataatgcggagtatttcaaagatgatagtaccgcgaggatctaacattccctgttttaaccctgctttactgaacgcctgacaaggaaaccccgccaacaggatatcgtgatcaggtacgtcgttttcatcaatggcgaatatatcaccctgaatattttcatcaccccagttatcagcatatgtttgttgtgcatgtttatcgatttcagacgttaaaaggcattcgaccccgccgaatgccttatcgaaaccgagcctcacgccaccaacaccagcgcaaaggtcaattattttcatacgtcgaaatcaacctcatcgattttgtatgattcttcgccaatatcagcccatagctgaatattcacactttttgcatcacgataaagagattgaccacaaagcccacctgtataacaagtttctgtaatctcgttaacttccaggcggaggctattgcgcataattttaacaacagccttttccattgccgaatctagggttttagtatcacccaatactacatctttaacgttcaaaataacatcacccattatcgccactccgtttcaattccgtgtttgtatgcgtcaacgcccagaggggtgatcactaaacacatatcagtatttttcgttggtgaactaaacgccattgatgcgtaacctttttgaatcagggaatcacgccctgatttactgggaacatcgttgaaatctaaatccaacatttttgacgagtatccgtaaagtttacacagaacatcaatttcagcgccagataatttcggatatgtcatttatagtacctcacaacatgttcagaatacacacgttcaatgaaatcattccagaaatcgcgatcaacttctttcggataaccagatacagccgccagcttttcaacttcacacatcgttgattctagcgcctcttgtacggttgcgaaaggaacaccgccagctttaaccattttcaaaaatgcactatccggaagaggatatacaatatcaccttctttgaaaatctggatcaattgcataccaccgcgcaacgcatgagaaagagctttccagtcgatcccgttgttggcttctgcttgccgtgctcgttccccgtattcatcccagagtttatacacggattttttcatttccgctacggtgatcgtagactggaatttacgccccagaacttcataaaattcctgacaacccgatttcagtgttttgtctgtaacgaatcgacaaaactcgttcgtcgggaatcggttagaaatctcaccaactttgatgcgcttgccgtaattagattcatccacgttacccagcaatgatgtaccataccagtaatcgggaatcatttgtaacacatcaacaacttcacgcagtgccgccaggcgagaacctttaacgccatacttcgccgcttgcttacgaacataaccaaacaggccagttagttccgtagtgtagaagcgtgaacggttagcgcggagatattgccagatatcagagttagcgatcagtttgctatcatctgcatgaagcatatcaatcgccacggtgtcaccatcacatgcgaggctaataaacttttgcagactgtaaatctgacgatctacgtcattaacatcgttctttgagtttttatcaccagttgatgtatcgatagacttcttcgcagtacctaacaggatttcgcgaggatgagggagatagatccctttgtagtctttatcgcttgttggtgtttccagtccgtacaggtgagaaccgaatacggtttccataatcattttcatcagaattcaacctttaatgtttttgcgatcccgcgcaattcagcggtagtaatatccggaatgtttgttccgtagctattcccaaatacttttttaatcttatcacacaaatcgcggcgatacaccatttctttgtattcttcttcgctacgatacagttgataacccatccacccctcagcccatccggaattgcgcttgattttaatattagtacaacaatcagacccatcttccggtcggaaagatgcatacaggtactgacgcgcaactttttgtacgtaaagggttttggggttgcgattttgtcgctggtcactacggatcccagcatcatacaacgtatcaccaactttcacatcacttaaatcaatcatttacgtctccagcaattagttttttcacagtagtgaacgggaacagacacacccaacgtttctttactgcttctgttgtatgttatcacaacgaatcggttttcgccacccttaacacactccagatccaaaatctcgcgggttcccttcgtgttaatgtctgcaacataatattcttcgttgttgacaatcactatatccgacataatcaagcgaggtttcatgcagcgtacacctctgattcatcgatccattccagatcctgattgagtgattcaatcagctttttatcgcgtcgggaaatgacaacggtagaacctttgtcagctttcacgatgatgtcaccagaagaggtgatgtattcaaccacataatcacggcgagggcttccgagtctgtcaccaactttaacagcacgtctaaccgattcatgagatttttcggtgaacactaatccatcacctacatgggtaacaataccatcaacagcagaacgagaattaacataaattttgctaatctccgccatgaaaacactatctctcagatatcgagcagtcactttatctaaacactgagaagatactttatctccgccaggatatactgagataatcattacatgaccctgaacacgggcggttcctactttatgcagaatgtaaaccattgaaccatcagaatctttagatacaaggatcacgctgaaagattctttgtgttgcttctgagtttctccacaggtaaaactcacgtccagaaaatcaccaactttaacagcacggggttttgctacttgttcacgagcactaataacagggatcataatcatttcctcacagtttcaaattcttcatcagatttccaatatacgttaaaattacgacaatcgtgttcggatgtcaacgtatatttttcatttgttttctcatcggtgataaccatagtttcattatcgattgagttaacaccgtaaacgaaaacattctcaccgcgtttgtttaaaaacgcatcacccttttcaatcaactgccaacaggtaacaggcaaaccacccggactaaccgggcgggtaacaagacaatagggatgtttaatcatttaaattcttccattgcataggaagtaagatctttgaaataccttgcggtgttgccttctgggttgtttgtaatctccatcaggataacagcactatcaactcctgctttcttagccatgaatgaaagggcttcggtagcaataatcgttgctttcataacatcagctttagaaacgttgatcgtattcatttttcttccttttcattaatcacttggtatgtgtgtataatacaaaagccctcacgagaacgcaagggctttttattaaattccgtataaatctggattcataataaccgcacataaaagatcatctatatgtgcggtttcttgttctaaggtttgtttagatgaatgtgctttcaagcaaccccagtaaaggcgtttactatctggaaatgatcatcgaagaattccccttgtcgttgcacgacctcatgcataggtagccagaacgcgtctgctgcatcatcagcaccgcccatgatacgaggcaatgaaccatcgttattaggttcgagcttgatatactgtgctacagtcggttttgagaagtacaccgaacgtttcggatgatcgaacagcatcgaattacggatagaaccacgaataaccttttcaggtactttaattcgtacttcttccagcaattcacggatcgcgcaatcaaggaacgtttcattaccgtttttgtgtccacccggaagcgccaacgcatctttaccaggcgcaaacttacgacgaattactaacacgttgttattacatacgaccactgaatcagccgtgcaacagttcagagaatccggatacggatattttttgaacttgtcaatctctcgttgccagtgcgcatcttcatgggacaaacgctggaattcttttgtttgtgtccattcatcgataaaggaaaccgtagtgctaggcgcatattttaacaaatcttcgtcccagccttcatggtgttcccagataattttgcgtaaattggtcgaggatagatcctggtctccaaccttcacaggttcaaccggaatatgattccatccgaatgctttaagccagtaagaatctttgtctttttcgtacccaacgatcgcaattcgatcatttcgagtttcatcgattgccatacgaacacgggatttccatttttcctcgttatagaggtaatccggaatgtgagcgaatttgattctggctgcatcttcaacatcaagtttgcagatagaccagcgagtgatcattgcttgacgctgtttagcggtcaatgggtttaatgtgttcggatatgcataagcagaaccgatcagaatgtaaaccgtatcagcaacagcaagggcttcccttaccattttctcatgaccatagtgaaaaggttgaaaacgtccaattactacagctttatcatatttgtgtttcataacgtgctccacgtttaaaggttaatcataaaacagacgcaattattaaaacaccaaacaatccaccaatgaaaccaaagaatagtgaaatgagtattgtcaatacgatctgttttatgttcattatagtattctcgttttagatgtcaagcccccaaagagggggctttaaaacattatttacgagaatcgaaaatcactttacccgcataatccgaacccattacagtttgaggtacgccacctttatagcgggtagagtagttcatctgtacatccagttctttccagcggatcatttccggtgtaatggtgcgttgcagggcggcgttggcttctgcttctttcttcgctgcatacagacgggcatcagcatcacgttcgttagcgattgcagcgttttcacgcgcctggcgatcggcttccgcttgttttactgcttgtaatgaagtctgttctactttttgcagttcagctttagcagcgttaacctgttcttcgcggatcttcgtgttagttacctgttccatgataacttccggcagggtgatatcctgcaagaatacctgtttcacagtgtaaccgtaaggccgtgcataatcttctacttcctgctgaattgcggtttgcagttggttttggatcttcgcatcaaacaggtcttgcgcttttggtacggatttaccaaattcgcgaacagtggaaagcagtttttcagttacatacttatccagtgcctgatcctgattacccgcgttgatacggttgatcggtgctttgctaccgtcgaattgcagcattacggtcatatccacagtggatttaaatttatcctgggacggaacctgtaatttgtcgaacttcatcgcgatgtctttggtgctgaacgtatcaaacgttgccagcgggtttacaatgtggaaaccaggcagtacgggttttggtgatactttacccatgaaggtttcagttttaaccgtaccgtcttgcacaatggtatacatgttaggcactaaccacagtgctgcgactacgcccagagcgatcagagaggttttcttcgggttgttcacgatagtgtttaagttcatcataatttccataagttgttgttcaattcgatagttattctatcatcacatttcacgctgtcaaactatttttaagaaagttttgtcagcttgtagattgtttgatagcacaagcccttaatctcgtccaggatgttcttcaaagaactatctactgattcgtagatctcgtttgcttcgttggctattttacggagatacgccaccgtgtcaagcacattttcggtttttagcacaggtttgtatcttcccgtgattcctatgtggatttcggtgaatttatcaaccaaatcctgcatatcttcgtaaaaaccctcatatgctttatgttgtgagtatgaacctgttgcaaaatgtgcgctatgcatataggtaacggacataaggcacatgccaataaaggcatctatcttgcttgagttctcagattctgtaatttgtttaaatgattgcatgatgatccctttatgaacgatggatacttgcaaactcatacgcgaccctaatccctagctttgcgcattcggattcagatcggcattgtttttggcgccattttcgttccatgtagttgtagaatagttcgcttgtatttacgctgggagggatcgttgtgatgtatacttgaagggccgcattgatataatcgtcaaattctttctgaaccggacggtcggcggcgtgtgttgtgggtgtcatcatcaacaatccgaacagcacagccattgatatgcgtttaatgttcataacaattactcttttactcatagacccactataggtctactcctgtatatatttatagcaaaaacgaggccgaagcctcgttataatatttttgctgtaaagtcaatcaagtaatgtcataccaacacaaacttctttcgaaagcgcgtattttgttcacgttttctacgttttcatcccaaccgatcacaccagctttcatacgtttcagttcctgacgtaaacgggtacgtacttttgaatcaattttctttactgcaatagaaagcattgcgttcagatcgccatgagctttgttaccgtcgcgacacaaattattatcaaatcgaatgtatgcacatcctgatttgtgtttccagttggttgagtaccaacgtaacccatccggatcaataccatgttgagcataataacgagaatactcttttacttcttcgatcttttcgttagatgaacggtcacgaagaggattgtatttcttacggtaagtgcgactcataatgatctccttttgtttatgcttccactgtatcagggttgttctttagttgcaagtagtgttttcgacaaagtgaaacatatttgtcttctgccccgatctcaatctggtcgccattagcaacaaatttgccattcgcatcaatacgggcaacggtagttgctttctttccacaatgacaaacccctcgcaactccctgatctcatcagccagcgccagcaacatataagaaccttcgaacaagttcaactgaaaatcggttcttagtccataagtcattacgggtatatctaattcgtcaacaacccgacacagatccatgacatttttcctggaaaggaattgcgcttcatccacaaacacgcaagaaaccagtttctcgctatcactgtaaaaatgattgttgtgaacatcataatacaagtccatatcaggcgtgatcatggtgcatgttgcttccaacccaatacgcgaagagatactctgtttaccttctcgcgtatcaattgctggtttgtacatcaggatccgcataccgcgttcctggtagttgtatgcatcagtgagtaaacgagcactcttgccagcattcattgatgcataatgaaaatacagtttagccatttatcctctcaacaaaatctggggtattctggaattttccttccccttcatggtttttgcatgttttgtttgaacagtagatccaccaatcccactcatcataagggggtttggtaatgttcattacgcaaattaaagggaaatgacaatcccgacaacgaactttttctataatgtgtgcgttagccaattgaaaaccatcctttacccatgagtttttcattatgtcgcgcaagatactctttgatttctggcatccggatcgcagtgtcatactcttctttcgtcatggtatgatttgcgcaacccatacacccgcacacctgcgcgttgcaccaacggagtgttccatatgtcgcaatcaccttcattgctttagctttgattttgtcagtcatgattataaccactcatttcgttatcttgtgcttgatgtatatcaagataccacatattgattttacttttcagttcgtccatttccttactcagacaattgtcaacgatacatagaacattaacagtttctttacgctgcataatgttgatgttattcgctttcatcgcttgcgccaatgcattacaggttttaaccagtgcggcgcgttgtcctttgattacggcgatccgtttgttcgctttcttaatctcccgacctgctttgataggatccatcatgattaattcgccttacgaggatcgaaatgaacgacaatgatcgggtaatcaccagtcacctcattaataatgcgcttaatgagttcccagtcgcccccagcgaggccagcaccgattaaaggtgtgatgataggctttccagtcttaacggcgtcagcaagccctacagcctgtttaaaagcattgccgattgcgtcataatcgacacgcggcccaggtgtccagaaatcatattgagtatatgcattgaaaacaatgttgcctttttcgccaatgtaaacagaacaagttccgagcttatcacgggaaccttttaacgtgttggcatcaacttgaaatgcaccaggaatacgatcgcggatctcgcgagcaataccagcacccatattgcaataacagttgcatccgtggatcaaatggccttccccgttcagatacatgttgacagcattacctttcacttctttaatgatcatttttatttttccgatatagtagggccacaacaaggcccatcaaaatcacaaggatccacaatacagtgaattgaacccctacgctcattttctcgctttccgttcacggcggcgatcttcttgatgacacatatataaaacaccaccaaaaattataaaaccgataacaacgcctataaagtatccagcactaaacatagtcatcatccccgcaatagtaacaaggcccagtgctctcatgcttaccagcattgtacgccaagaacaccacaaccgccgccataataataaaaatccagatagccattagtaaagtcctatgccagcattgaattcgtcaaccaaataagtacggaacttttcgcaccgttccttatttggcgcttgtttgcatagattcatcattggttcagactgcaaaaactctttttgtttcagcaacttgccgcgtttatacaggtgagcattttcctctccccacatataagcaacatctaactgttctgcgatcacctgcttacatactgcgacatctttgatatcacgattgttgcataactcatccaggcgagcatcacccgcgtgagcaaatccagcaaccagagttaaaagcagtgctaactttttcatgatgattccttattcatcctcttcgataggagtataataatgcgcattacagatatacgcaagaacttttttcagagacatatccgagaatgtcggatcctggtttcgtctcatcccactaccagtttcaacagcccaacgtttgttagctggattgtatgtcagccagtaacaatcccattcagacagagtatgttcgaacagatcgaaacgcttacgcccatttgcttgcggcctgacaaaaggttcaaccatttctaaagcggttaaaactcgattaaggtttgaaccgtcttcatccatcgcgatccgcaaacagtattggttaatgtccggatccataccatcgatacccagaccgatagattcgaaaaattttgttgccgcgtgataagacacactggaagaacgatattccaacatcacggggatcttttccccgtccttgacgttgttaatgatatcctgatcgatgagttcaatcaggtctcttttctctttaatcaacgtggaaatttcttcttgcagtggggctatctgtgcatgaagttcttttatccgttgatcaattacggtcacttcgaacgctaagtttctcattgtacccattccccgtttttgtcaatgtacatgatccaatcagcaaccgcccaatgggaagtattgcctttcggagtcgctacgatgtaggaaccagctttaaacagtacgcgtttagtttcgttcaggatcaggtcgctcataatgtattcctcatttaaccaaagtgaatcgtgattcataagcatcgttcgggcgctcatacacagtatccgaacttgtaatgacagtgtacacggtttctttcacaagatccatgattttctgtgattctccccagacattgatactaaaataaatcccatttttaggaataggattgtattccatatcataatacatatccatgagttcacaaatgaacaggcggcgctgttcgttatcatatgtgaaataaatgttaaaacaatcgagagatttactcaaagtaatctctttgataacgatgttgtcttgtttgctaaaatgatcgcggattgcttgcacacaacgcaacaggttagggtaatcatatttttgtgaaacaatgacttgatgtgaaacgctcataatgtattcctctcaattagatgcactcataataaaaaagcccccgaccgaagtcaagggctttttgtcaaatgatttgtttttcttctaacagcttcgcggttgtattaaccatacgagcataatcacgggcttctttctttgtatacttgaaaccagcgttatagctcgcaagcgcctttttcaagtcgcctttgtggtaatcaagccagtactccagttcatagatcgcatacttcgatccaccttgaagagtttcgagctttttgattactacgcgtttaggatatgacttatccattcgtgcgctggcgctccttgcggtaacttgccagcatccataagcgtgatggccttttttacctttaccgacattctcacatgcgcgagactcgatccaggcaatagccgctaaatgatagcctaaacgtttagccttatctttttctacaggttttgcagtcttcaaatcatagttgtgtccaactcgataagcatactccaaaacctctttctgcttcggtgtaatgttatccaaatccttgatgtaggatggagaatttttgtttgccggaggcttcacagtagccttttgtaaaggcaattgatgagtaggcaaatccgcaatgaaatcccctagcggatccgtcgcagcgttgccagaaaaagagcacaagaaaatgctggcagcaataataattttcttcattttaatacctatgttgcaaaaagaggggcaataatacaccccactttatatttatgcaactattttagatagttttcgtgtcacgtagtttatcggcgataaactcagcaatgttataatttgaaatagcctcgttaggatcgtatagtgcaatgatttcatctaacgataccataacggcatgtttaaagtagacgctccagctagtagtaaggatctcacttttgtcaaatccacaatcagggctgaacaatgcgcggtatttgtacccactgtatttcgtcagacgatttgtgctgtgcgcatcactggtgatcagaaaagtcccctggtgagtttccacgacgaaaaagtatccgaggcgttctttgttgtccagcatcttttcaaacttgcgatcggtttcttcgcgaacaatacgagaagtcagcatttccaacactttatcgtattcgggccaatcattctcaatcacgatcgcatcaaatggtttcttaccattgatcccgcgcccgatttcgattttcgtgcaaatttcgttgaacgttttcaaatcttctggcgtcagttctttaagatcgctcaattttgctacataataacgtttttctagtttcatttatggaaacctcaattcaaaaataatttcacagagttaccacatttgggacatgtgataaattttttcacgacataatcagcagcagagaaaaatccattgtaaatcgattctctcttttgctgtatatcagatagttcatattctaacccacttttacagcaactgcaaacagtaatcagttttgggctatggataacagtaatcatatacacctcacaaaaagggggctttcgcccccatcattagaaattgtcttcgacaaacgccgcgagacgggaacgatacactgtatcaagaatgatatggcttgagtgttcgtattctttcagcttttcaacagcccatacaaacccgttgttaacggcagtgtttcgagggttgtcgatctgcttaatgttcccgcatagtatcagaagtgtgttctctccgcaacgagaaatgatagatttaatttcgtggttgctaaggttttgacattcatcaacaatcagcacagaacctttgcccggatccggatgtccgatactgcgaccacggaagtaatacaggctagggaattgcaccacccctttttcaatcaaaccttcaatgtatttttcagattccggattatccttaaacagaatgttcaggctagtaatacaaggttcgatagaaggccggagtttttcgcccaatgtaccaggaaggaagccgatttcacttgataacgggctatctgacttcacatacatcaagttagcgtaatgtccactattaaccaggtgcatagcaccggaaacagcaagcattgttttaccagaaccagcgccgcccataatggtagcaacatcgatttcattgctcataatggattcaacgaaagccgcttgcagagaatcacggggctggatagctttcatgagtttgcgtttcatagcctgttcgtgcttaacaggtaagacattcaagcaaatctcatcagcagtcaccacacgcccgactaactcaccatttgaggtaatgtactggttaggataaaaatcttcgtcaggaagcgaactgtaagtgatttgggctacattatctgtatatcccaacacttccacagtatcccagaaatcagggatctctacataaccggaatacaatacatcgctatcttttaacgtatcgtcgccagtatactgttctaccttacacccacgggacattgcgatcagcaacatcataatatcgcgagtaactaaggttgcatcctgttgcatacaagtttcaatgattcgttcgtcttgcttgtcaagagcaaacgttttgtttccgacataatcaaccactttaagggtgatagtgtcagacagtgctgggtttgtcaggtttaaaggaatacctgatttcgtaatcgcatcatatgactgaccgaaaataacttttgacagaagccggatcgccaatcgtgcttcgtgcgctgttcgttctttcgttttcaggtgatctaattcacccatagtagcagaggtaataatgatttctgtaccaggttgagtgaatgaatagattgaataggggttactaatcaaaacattggtgtctaatacgtattttgacatacattaaccttatgtggtttcgttaaaaaatgcaccgaaaacctcttttgctttccggttataaacggattttgcttcttctggagtgttatagtaccccaaaaattttctttttccatctatgtttatctgcgctttgtacttcccattggctttatgataagaaacacctttcaaccctgtactactgtttgagttacatttctttttcatcgcattttgctggttcgtcgctttctgtaaatttcttgctgtatctccattctcaacaccatatacatgatctacgataggaggaagataaccattctcaacgtaaaacactattcggtgtcgcaaatacatagaacctttaaaatgaatttgggaatactcgtttttgcttccggcttcacttccaggagacatagggccgcgctgaactttccaatacactttacctgtagatgtatcaacatctacaaaattcagaagagattcgatcccttgaatctcttcatgtatggttcttgatgaatagccatgacttttcattacatacccagcgaaattacgtgaatatatgctaatgggtgtctcttttgtacacaatgcatgattgtattatatacaatgtccatgcgttcattgtgtgtgagatcacactcatcaaaaataaggtttattgcctggtgctctattcgacgtccacggaaatgattaagaatcgcccctttactggtcaatacatcacatccggtagcaccgtgtagccgtttggcttcttgtgctgcatttaacgtatgcgctacgtaaatgttaagggaactatcggaacgtttcataaaatcaaacgcgcctttagtcttttgtgttcgtctacccagatccaacctggtttcaaataccataaaatcgttagggccgtaattatgcgttggttcttccaactctcgcataagatgcatcttacgacattcttcaattgtctttacataaaattcactattcatgttttacctttaaggggccaaagcccctttgttacgctaattccacatgcggggcatcaatgaattttgtttcgatcggaaggttcggatcatttttccagttgataccaaaacgcagtttaacacccagttcatcacctgcttgtttaacagcattcaggacaggcaaccacactttagggtttgtttgccaaccttgaggcaatacgctaggatacagatccacagcatcacccgtgatgtgttttgagttcattgtttgagatacacccttacggacgttctcgcgctgttgttcaacagtacgcagaccttcacgtacaccaaaatcaacaggagacagttgcagagcgcgttctacaactttcaccagttgaggtttaacacctttaaggttgttaaggcttttttgactgaatttaaacataaatcacctcttgtaaaaataccctgtttgggtacacagggtatttatggtttaagaggttcgataattaataatcgtaaagatcaccgaagcattcttcaaattcacgtttacgtttcatctgttcttcttttctctctttcatatcagaagggagacgatcttcattgacttcatcaatataagcctgtgcatcctcttttgttataaagaatgcatggaagttatatccgttgcgcccattcatactacggtcttcaagagagaactctgtgtggcagtcccagtcatcaaacagggtgatgcattttgcaaacagcccgataccgcgattcatataagggaaaccagtaacaataatcttgttacccatttccgccttttcgccattcacacaaaatacttcatacatgatcgcgcctggtttaacatctttcttaacagcacgtttttcaaaagcacttttcataatatattcctctcaattggtgtaactacagactactggtttattttctggatgtcaacaaggtttatcgttttttgacggaaaagttagagtgaacaaacgatcgtgaaggttgtctatccgttcacaagcctgtttcagtatggttttatcaccatcatttgttgtttcaatgcatccaagttcatcggcgtcaatgttcactacatcgctcatcaatgaagcaaacacgttagcatcaggatgtaacagttcttcgatttcggccttcatgccgtcgtgttcagaaaggatatcaataatatcgcgggttaaatctccctggtacgggaaccctgtttctaaatgattaatgatcctttgtgctttcgtaatcataattttacctacaaaaaagcccctttcggggctagttaattaaagttcacagcaacggcacacaccgtattttgtaaatggagcatcaccgctaacgtaggcccagaaatcacatgcttcttcggcagtatcgaagattgcagcatcatagaacccgtgggcttcgttaccgttctcatcgatgaaaaccggagtccagatattaggattgaagcaatcgtcaacaacaacccaaccttctttagctttcattgcttctttgttggcttcgatgtgagctaagatttcgttcatgatgtccattttacccaaccttctttagctttcattgcttctttgttggcttcgatgtgagctaagatttcgttcatgatgtccatttttctctcctaaagtgtgtttcgtttcgacagggctatagtctcataaccccgtatctacgtcaacacttatttgaagcgaattgtgctatttttgaaaaatagtccagagcacacagcaccttcaattttcacccctgtagggcttttagcaacgaaccctgttgcataggtgtctttctcatcacatgcaaaccaggcgtggcctgtgtacgtgatatcggtaaacccgttagcagtcagaatacgttcggcttctttctcatcagtgcatccagcttgtgctaaaacgacaatgacgactaaaaccaaagcaataatatatttcatgttaaactctttttaagttggttttactggcttcaatccagtacacgggatcagaatagttaccgcacatacccagtaacacagttgtacaccctaaatggtcggaaggtcgcaatccatcaggatgaaaaggcaattcgttaacaccaatactggtagcaaaaagagcacctccagtactgtaaaatgttttgatatgatcgtatgcatcatcaggccactgaaaacgataagttttattgtcaatggttactgtatacatatcatattccgtaaacaacggatcttttccttgtgttgccccatacagagcgccgcgccattcaaccagatttgcttcaatgtcgcttacacaaatttcgttacccatacgcaaatcatgaaggatcccttcaatggtacgaatagccccactaagttcattagttaacatagagtttcctttaaatcggtttaatggttttcaggtgtagtttagcataaaaagaaccaaatgagttaccattatgatcaaatttatagttttcactcttccagtatttccccgatttcatcaggggaacacgcttcttacctgctgttatcgtttcaaccattccggtatgagtaaatgtcatgatataccctcttctttcagcacttcccagatcagtttatcaaggtgcatcaggttccacataaccgaatcataagaacccagtgagcgggagtaaatcactccccatgaacgataacttttctggaatgcttctgcactatctacatcatacggcatatcatcaccggatgcaatcaaaagtttaaggatcatcagactgttcagaagttttgaactagcgtcttgtgcttgtacttttgcacaataattttcaataatcgcttttgcctttggttcggtgatgcgtccatttttgcatcgctctttgtacacatacataagttcatcgattatttcttgcatataacgcctcccgttctactgctgataacccgcgaatgtagttctgtgattctctatgcgcatctgctacagcgcgtcctgctcgttccgacgccagtatataagtaacaacttcattacgaatgtgccataggtaatccatcattacaagatcttcttctgtatgaaaacctttaatgtcacactcgcagcaaatagcgtctctttccgatagtgccagttgcgcggattgcgcgttgattggcatcatactgtacttgtcgatcaaactatccaacgttcgcggtttcacaataccaactgttacaggaacaggacgaagagtaggtttatccgaataaatcatagtattcctcttcatcaagtctagatgtcagtttagcgataaagtcgaaaatgtgttgtgaaccatcttcaacataatgacggtatgcaagcaaagttgatacgtgacacatatcgaccgattcaactttgatgcttgatgcgatcattgtatcatcatttccatatccgtcaatatcacggagtaccatttcttcagtcgggaaacgctgaaggagtgacgcttcccgatccgataccagagcaactaagcgattatgtcgcgtgttgtacgataatattttcatttcaattccaccgcgtaaacatcaggttcaggggctttgtgtacgcgcatatctttaccgcataccgcataagccggacagttacgacaaccgttatgatccttattaccgatcagttcattacggaactgtttggttttcggatgttcccagatatccttaatgaaatcgttcgcttccaggacattcaaaccttcttcccaaccaccttcaacccagcgttcggtaaacgaacaagggaagaactcgcctttctcgttaatgtacgagctaaacatagttgcttcgcaatcttcggcatattgcttgtactgttcgaagtttgggtgtccttccatcgcttcaacaaaagcaggggctgaacagctatcgaaaccaaatcctacaccagaatcgaggcaatattcaacaagttttttatattgttcgcgggtaactgtgtcccagttcttcccacggcctttttgtttcagacccaggaatacgatcgcgttaacttgcttcaagcgcggatcattctttacagcatcaaccacgttaaacgcgtcatcataggttttagagctaaccatgaaatgaaggttgatttgctgttgtccggcttctgcaagattagccactgaattaaacgctacatcgaatccagcatgtttgtatactgataccgcaacagccccagcaacagccgctaaacgcgctgcaacgtcttttgatacatcagcaatggtaaggtttggtacaatgcctttagaacgcgcataggccatcatatcaaacatatcagggtttgtttgtccctgtgcatcagcaccgagggcgcattgtgttaaccagggcattttatcaatgatagatttgaatgtatcaagatccatattgaagccgttagggttattagacttgtagcagaaaccgcaaagtttaccagcagggccattgcatttagttgtgatctcgatatcgagaatttcggggaatggggcataggtaggatcagtttcgaacgatgttccccagcgagcaaactcaccagttttaacgttgaaattgtagttataccacttagagcgagcgtaacggatatcaccatcttgatagatgaacagggtaggagctttcagaacagtttgtgcgttattcataatataattctcaaaatctaacatgggattggaagacagcgcgagcgagactttcattatcaaacggtattgattggtgttgccctttgctatcaatgttaacgcgccaaaattcactagaacaattttcagtggagtagttcaacagcgttaccgttttattcttttccaaaaatacgcgtttgtcaatctctgttttgattacgtgttccatcattttacccaccgttgtttgcgttcgtcagccagttcttttttgtacaccttgatgtattcgccgttcaaggcacggagatttgaaaatacacgattgaaaagatttttcttttctttgtatgccggagacatacggatcgattcaatagtcatacccatttcatttttaggatacgctcttaactctgcgccgatctcatcgatccatttttggtacagatcacgcttttctttgtactgttcaaaagtcaacatgtccattttttatccccgtttcgtttcggtatgggtgtaagataacatcatcctacacccagcgcaagagttatttgtattccatgaagaattttattgcttcttctggcgtcataccgtcagagaaaaatccaaagaaagtacagtgatggtcgttgtatgaaatattcaaaggagatagtaaacttcgaacatgttcagcccacaaacgatattttttgctgaatggttgatctctcattcttcgtccccttgtgcgtagtattcacacactgcatcttctggggtgcagccgtccgagtaaagagcatacatcagatcttcgtcataatcagaagaacccagcatatgttgaacagagcgtttccatttgttgtaatctttttcgccctgggtttcgctgttttctgatttaagcatttcgtacatgttcatagaaatctcccgtagtcggttgcagcatcttccggatccgcatcaagttcgtacagttcgcgagctaatgcgctgggtttaatatcgcgccctaagtgggcgctaacattacgtagccatttcatatagggttcgaatttgttcattttatacgtaccgcgttaaaagcctggttccggagatcatacgctttttcaagctgttcagtagtgaacagaggactatcagtgttagtggtgaaactgcaaatggttttgttgtcggcgttgacttcttcgacaacgatttcataaccccagatcccgctatactcacatttcacgttccggtacttgatgtaaaccgcagcaacatcttcttttttgtagttccggcttttgtagatgatttccatgatttcctccttcgtttcgatgtgtgtacaataacagatcagggttatcgagttttagcaatttgtgctaattatgccattttcttagcgattttccaggaggctttgaacgccggaacgtcttcaatatcaatccagaaaccagatccgaaaccatcactatagcaagggcaaccgtcgcagtagttttcccaggtcatcacttcaccaccaacagaagcaccagtttccatagcacgtaatgcatcttcaactttttccagtttttcggcgttgtcgtcgtaaatgacaaagtaccatttaccattgtattcgttacccagtttgattgattcgcgaacaagtttcatgatgatttcctttttgtctgtttcgtttctatgtgtgtaatataccacaaccagaatttaatgcaacatttattttgcttcgagttcaatatttttccatgttttcatcggaacccctatcgcatcccaaaacttaacatcttccgctgcaatcagagtaaagaagatcccagttttccagtatttcccgtttctgatttcgtttgcgatctcattcaactggtcgcaaaaatgttcagtccaactaacatcaccatcccaacgagttttcccgttgtacagagagaatatgaaactatcaatataagaagattttccggtagagatacccatcaaaacagccaggattgtgcgaactgcatataaattctgaacctcaacacttctcgttttaatagtcatttcatgattcctctgttttgtttcgatgaatgcaatataacaaaacccctcaccataggcaaggggtttttgcaaaaatcatcgtttgattggggtattatctataaccctttgaatttccgaacgcatcgtagaatactgacacaattcggtaagcgcccgatccaggtgcatcatagcataagaaaactcttttccgcatttgtcacatcgagcgtataaatgtaaatggatgcgcccgatcccatctacctgactatatttctggaatatgtaaggatctgcacctcgatagccagttgcttgatgcttacactctcgtttgaaccatgacattaataatatccttgtatgttgaagcgatcacataacaattttcttgtttggttagtatcgctttggatagaatgcaacatagcgctgatcatgtttaggttattttgcatcatttccgcgctcatgagaacttccatacgcgcacgtaagcgtttattttcttcttccaactcaaccatacggtcatatgctttgatgcgctctaagggcatatcagggcgctctttgagtacgcgagcacgttcaacctcacaagcatgatttgctttccagtggttcgattccgcttcaaatttattgaggcggcggatctcttcaaccagctttttgatcatgtgtggatccatcatgtcgatgaatttcatcaagcaattggattttgtttggttgtcagcaacagaccaagacgaattatacgtaaccgtaaacgtgcggcccatttcatcaacaaccccgatcttgttatcatcggtgattgcagccgcccatttctcccgcatggctgtacaggttccgctggctacactatgcaacttgtttaatgttgcgtcatcaaacacaatttcatcactcatatatgcctcacatagatttcaaaatacgcagaagtgcgttagtaaagatatcaggaacgcaaccaccaaacaacttatgattcatcagcgccaatttcatgctgtgattttcagtatatcgcccgttatggatcccccaggcaacgacattaccaggttcatgaataactaaattggtgagagtaacggtcatgcgctctttatcattgatagagaatgaatagcggtagccggatccgatgtcgccgtaaaggttaaggtctttcaatttcccttgctcatgcaagcgtttcatatgaactgcacatgcatggttaatagtcatttcgtcatccctagcccagtcatcaataccagaggtataacgaatattgaaatagttagtcagttcatttgatacgctcattagaaacctcacttttataaaattctttaccagtcccattacagctactgcatttgggggaacggttgttatcataccgccccgaaccgttacatgcaacacatttccttaatttccagccatacacgaacctcatgtaataatcggttcgtgcggccttgcgttcatggaaattcatgctttgtaaacctgaaccaaccacatttcgatgttaggcgcgtaagtaacgtttaccttatgcatagtgcggtatttgtaagcggctttgtacgcatcgagttcagtcggaacacagaaagaaaaaccgttatcatagcgttctgcgttagaaacttcacaaccaactacagcggcaatgtttttattcatgttcatgatgttttcctttctctgtttcgtttcgatgtgtgtaatataacaaagcccctgcacgaatgcaagggctttttgattattttggtaatttttcgatggttgcttttaactcattgattttattaaagagttcatcgctatatttcatcaactcactacggcgtttttcggcccacttgatcaggaattcatgagaatctacaccatacgtgtaaccttctgcactcagttgaatacgagcacgggaaccataatcaacagaactttgttcaatgagaaacttaaccgcatcaagcagggctaaatcttcatgacttaccatgattccttctgcctttggaagatccacaacttcatcctgaatgagttcacgacgggttgtttcttccagtgtttcatgattctggatcatcgtttcgaccggatcctttgccacggctggtttgttttcacctacttcttccaaaaacatcaacatccatccaggaattttagtccggaaagaactttgtacttcactggtgcatgaatttcccagaatgtggatcgcgttgccatgcatatcaactttattgatatagataacgttctgctgttcctgtcggttgctaccataagaaaggaagcggcgtaacgatgtgttatgaccatacttccctaaatcgatttcagccaggcaatcaatgatcccacggttagaaaccttgtaacgcttaccctgtttgaaaaataacgattcttccaggtgagtagtggtaaactcttcataaagaacatagaattctttaggaattttgcgctgaaccaggctcagtttacaattattagaaggaacaataacagcgtgaatgtttccttctgcgtcacacatagcttgcattacttgcggatagtaaagatggtctttcttgcaagtatagctatggatacgactctgccgttttttgaagtaccatttaccagtttcaaaaggcgctgttgtaaaattcattttgcattctcatacatagttaaaattgcttgcatatgttccggtgattgtggaacccctgcaaagttcactttcaaaaagaaattcaaccgatcttttatgttgcactcatcgagtccaagcgctggtaatgaaatgttttcaaaagcacgttgttcatgtctttccatttcaccccaaaacaaacgggaaccgttaggcatcggtattccaatttcattgttccagaatttcatgatagttgtcaagcgttgttttccgtcgatgacttctacccatcgagattcgttgaattcactatcaaccgcgatcgcgatgataccgcaaggaaacccagtaatcaaagtcttcatgaaagcatcttgctctttctgcttccacacgtagggccgctgataggacggattcagatccagatcgttgttcttgaaccagtgaatgtaactaccaaccatgatcgcatgatcgcgactttggaaagtttttaactcacgaatacggtttcttacaatttcgtctgtcattataaaatcaccatccagtatataatcgtaatcataaccgctacagtgaaacacattgcagcgtacacccgcgcattatgaacctgtgttttcaattctgcgatctcttgatccttttcgctttcaaactcttcgcgagtaccataatacccaggatcgttagcagttgccaatctaaccgcatctttttcaaccagcgttgcataaccgctttttatttgtgtcgccccgtaccatccaccccgatcgttgttaatgatcagatgatcgcctttttcgttatgctttgattcaccaacgacaataacccgcttaccattcataatatgatcctcaaaggggccgaagcccctattttgcgttcttctgtagataatctaacagatttccgctttgatgtaaatccaaaactttagaaaacttctctgcgtttctttcgtttgtgagttcgtcgaaatgccatacaccatcatcagctattaacgcgccaggtgatgaacctgtttctacatcacgggaaagcgcaagccccagagggtgtaagatttcgcggttaatgcgccaaacaaggcccatttcagatagagtattaaaatcgacgtatttcatattatgcctttggtttcacaccgtaggccaacataccaaaacgatgatcattatctgcatctttaaacagaacttcgttaccatcaatgcagatgacctttgcttccggatcgatgtatggaagcaaccacaaagggatcaggcgtaggccgctatgttcatcccagcgactgaaattgagttcttccagttcatcaagggaaagatcattaggatcgatataacggaaccatttggtatttttgaggcggtcggggaagtttacgatttcttcatagccgaattcagaactccatgaagagtaaacagtgacttcggatgctttggttaaaacagcatcacgaattgatttgcagatatcgattaaagtcagttgattttccatgatatatttctcatcttgctaaaattttaggcagtagttgccccatcgttttacgtgcatgtgacggaatctgtgagatcgggacatatttaaaatcatccatttcacgtatagtccgtccgttcttaacgaaagttgatgcacaatagcattcttccgctactggataatcttgccctacatagaggaataaagcaaggttttttgttttcgtgtaatcgagaacacccaggctaaccaattcctccgcgaacacttcaaatcctgtttcttcgaagcattcgcggatcgccgcgtcaatatgagtttcgcccttttcaacatgccccttcggaatatcccaatggggcgtttcagtggcatggcccatcaacacggcaccatctttaacaaagataatacccgctgatagttccatttattcacctgcaaaagcgttatcaaatgcttcaagtgcgttgttagcgcgagcactggcttttgtcacaccagcctggagattttcaaagaaggtatgtttccacacttcgcggcgactggattcatgttccagactgtttttgtgatcgccgcgaatctgttcttccatgtcataacggtacagatcgagttctgcgtttaatttctgttctaatgcctgtgcaaatacatgttcaatattcattttgtatagcctatttcagatttaaggttttcgagggtggagtgataaacaacattcccttcgtgtcgagtataccatacttttccgttctggttacactcattcattacattttcatctaaaccagggatcggcttcatgctgggagaaaacgcgatagacatcatttgttccgcactatcagcaaacccacaagggaaaacagatccagttggtttatcaagatacatcaactctactttagccatagatttcttcgaaatcctcacaatcaggcaaatacgtttcacagaaggtgcaaagcgtaaagaatgcaggttgacgaataccaggattatccggtagatacatccagaaggtgttagcaaacacgatgaatgttttcaggttttcggtggtgatttcgctaacaccatcatacccggattgattgatcgcgcgttgcagtggcacctcatactgttcgcaatagtcggcataatgatcgcttgttacaaggccattagccattttaatcaaatcgacgattttcatgattttacatattccactttaacaggttttgcaacaaatttatctttggtgcgcccatgaccattacacaggtcacattctttgttgaaatctttcatatcttcgacccatccagaatctggcaacccagacggatatgcgttataacgaatggtttcataaccttttccgttgcatttcgggcaaacatgaggacgttcttttttagcagactctgccagttcgcgaagggtggtagaactaccataagcccgacacatgttttcaaagtcttttaaagtcattctataaacatcaatgacgttatattttttgccggatggtttagccataatatatttctcacttaaagaattttttgatgaaagagatagcaaggccgataccaaagaaaattaagtaaccttttccgtcaccgtgcgccaaaacatagagtgagctgccgtatgcgatgagttctgcgatgttcattaagtttctcatgatatcctcctttttctatattaagtatcttaccataatataaaccaaagtcaacaacaaagttttatcaacccacttatcaccagtcattagtaatcccctacaggttgagacgccgcaacactcaggatcttgaaagtgcaattgttccactcacaatacgtttttgcacagtgaacagttcctttcataacaaacccgtttgagaaaattaaccagtaaagtttcatgatagcctcctttgtttcgacaaggccaatataacaaagcccctgcacgaatgcaagggcttttttcagtttttcaacatccaaagttgcggaggacaatctttagaagcgattagacgatccaggcgggacataacccgacgataaccgtcgtattcaaaattaatttttggtggaacgtagtttacctggattgtttttctgttagctaaagaaacatactcagggatcactgttcgcaaccgtatagcgatgactggcttctcttcgccttcgttaaagaatatttgaacagtgataggacaggcaaaaattttaccatttacccgacgataaacaataacttcctgtgtcccttctgttttggccttcacagcgtaggttagaacataacacgaataatgatttgctagactcatcatgatatcgcgataagtttcaatatcttttttaatcgatactgaacggtctttaaagcgatctgcaatgtggtcagcagtagccgctaccttgattgtataccagtcacctaacgcgctagtaaacgcctcgctaacttcttttcgtacactgttaacaagatacattaaacgtgttctgttcatataatcctcactgatttttgaagtattcgatctgacgcaaacgcttttcagcggcggctttcgaatcgtattcaccaagttcttttgtgcgatcgtgattcaaaacaacccacttatcgccacgctgttcaatgtgttctgtaatatcttttaacgacttatccagatccagtgattcagcctcttcacagataatagtcaaatccacgggcagtgtcaacaaccttttcactccgctgatatcatcaagcatcgaatcgtatgcaagggttacgtgcggcttgtaatccggataatcgtatgttgcgccagcatcaatagaatctttgaaacggctatgcaggtattcagattccaggatccctacaatagtgctaccgtattttgtgtcccacttttcaacatcaaccagtttagcaggttctgtgatgtcctgttgcgggaacaaatcaaccgttttccggctgtatacgatcgttgtatgcatcttttcggctgaaacagcattctttgtgatacctaatgtcttttgaacatttttcaaagcctcacatgaagcctgatcgaatttagcacacatgtagataccaggatctacaacaggttttgtgatttcaagaaatgatttcataaaacaccccaataaaaaaggggccgaagcccctttgtaataaatttgtttttacgcttcttcgccaaaggcggcttcatcttccgcgcctttttcgacttcaacggaagggatcagagcggataccgcgccaatcactgcttctggggttactggctggcttgcgtcaatacccagtaccgaacacaggtcggacagaagttgacgatgaacagagagttcactttctttttgcgcgattacttcgttcagatcgaatgcgcggcctttcagtaccagtacttcattttgcagtttttgaatatcagacattttattacccattgttaaaatttaaaagtatcgagcactttgctctttagttgtttcaaagtaccttcgttagtgatgatactatctcccggttgaggtgtcaaacctttttccgtggaatgttcatcaacaattccggtatcctttacaataaacacaaacttagcacccaagcgtttcaggtatttatattcgtgttcttgacgacagtcagtgaccagaagatggttgtattcgtcaccagtatatttattgacgaatctttccaacgtgtaacgaacccaaaccgtgttatcatacttgcatacgatatcagttccaaacacttgcatcaagcgtctgatactccagggagtatcgttactcataatcaggttatcaatatcatcaggactataaacaatattgtatccacgttctttgaggatttcaagcccgattttgaaaatatttagaacatcttcattagacatcacaagaggtttctctcgatcgcctttgtaaaaaatagcatccggatcagaatattgtccttcaatcatattgcgaatgtatggtttatcgtaaccatatcgctgcattgctattcttagcgttcttttgataccaaatgccagtgcttcacactgaacatcattgtacgcctcttgaataaatttagcaaccgtatctttaccagttcgcttttttccactaatcacataaatcattagctcattctcttttgagaagtgactacttttccgtcaatttcaacttccatatgaaggaagccaaaagttgccatacacgtaaccgcttcatcactatcgttagtataacccaattcaacctcacccaagtttgttgggaaggcaccataaaatctaaatgtggcgatcgttttcatctgggagttatccaggatatgcacagcgaatgattgcttaggatcatcccacgcaacagagttaaactcattgtaatcgtttgtgctcaacatccatatgtaaatcccaagatacgatctcatttcctcatcgactacaaagcggatcatcaaaggatcaaactcaaaagccgaaccaggtactttacctcgaaccatcatatttgcaggaatatcaactgctgggaggttcattgatggtagtgtaaccccttgaacttgtaaagtcaaacctttcatgtaactgttatcaggaatatcaacccgaaagtttgtaggtgagatttggtttaaaatcatttctgtagacataggatctcctttcctctatttagcggggaacgggatcaaagcggcctgacggggtaatataaaaaattgaagaaaatgcttgaccttttaaaatctttgatctataataattattaattaaaattttatcaaaaagatctaacaagatcaagtaaaatttaataaataatttatcaaaaatttttagatctgatcttgaattcataaattttgtgatctataatatattatatattttattttatcataaatttttatgaagatcaatacctagatctaataaattttatgctttttctgaaaacttttcctttaccccgtcactaaatactggtactatgttcccatattggaaatcaggaaaaacaaaatgactcatttgaaaaaattcaaagaatttctgaccgaaggtaaaaccctcgctcgtaccgtagcacgtggtcaacgcgctaaaacttccgataaacattcaatcggttttcttcacttcaaacatggttctgacttcgaagttttagcaccggattctcacgatctggcatacttcggtaaaaacattgtacgtttgaaaggtatgactactggtaaagttcaagcggcttatgtcgattgggctaaaggtactgtttctttctacagtggcaatccggatgatgatctggatttcgacaaaccagaaaaattcaaagctgctactctgtatgaagaggcggaagaaaatctggatctgtataaccagttagcagaagatttcgaaatcgagatccctatggatgaagctctggtgaaaggtaaagtttacaaactcccaagcaacgatatgcgtcttctgtacactgggcgttctaaaactaaagcaagcggtgaatatgcagtgtttaccgtagtcgatgcttccggaaaacctcgcctggtatctggtaaaaaattcacccaggaatataaaggcgatatggtttctaaactagttctggttgaatccgaagatctgaatgaagcggctaaaggcattcgcgaaaaagttattgctgtgatggtgaaacgcgggtttaacgaaaaagatgcagaaaagatggttgacaaaaacctgaaagatgctatgaaagttagacctggtgcgacccctggcaaacttgcagaaatagttagcatcctgtaaaaataaagccccttcctttcggttggggctttttgattagtatttgctccagacttttttcgcgccgtaaggtttccctttggacataaattgctgagtcggtagccaaacagctttcgcccaatctttaggggcaatctctgctaatggtgatttgaggtgtgatggtagatatgctttgatcatttctgttgcgcctcgcatacctttcacgttaccccagttaattttaagcacggtcttgttagagaggcgtttagtggatccgtacccacgcttcaataactcttctaaaaactcctgtcgtgctctgggtggcgcatagtgcaagttcaaaccatagaacactaagttacccgctttcgatcttccggatcctaagaaaatgatcagtggaaatctatcccaatacggcagggtgtctttatattttgcatcatatgcaaacgtgtacaggcgacccgttgctggttttgccacacggtgtgttttgatactggttttgatgaaattaccaaaccattctgttgaatctttctgtcgctttgctgctgatacaccaacagtgatctttttcagactattacggaaatcgttgatgatctcgatcccgtgttttttacggtagtcattacgttttttacgggcttctgtctctgcggaacgtcgttcaatctcatcatcgatctgttttttgtaacgatgcattgactttgtgaacgttgcgtagtttaatccctcagaatcggcaaaacgtttagcagaaacacctttcgtttttgccttgcggaatttgatccccagttcaacccaatcactcaatttgcgtttgggtggtgctttgggtttatcctcttccgcgatgatctcaaactcaaaaataaaactcatgtttccctccagggattactgacctcgccacccaaaaacttttttgagtgattcttctgttacgattttgaactgccagcctttttgacggcatagctcatttgcggctttccacttatcaatattaactgtataggtgtaaagagcatcaataaatttctttttattgtgtacgttgttgtttactggcttcggtggaggcatggtttctttaaggggcttaacctcccaaagatatgtagtaccattttccatttccacatagaaatccatgtaatagcgtcttctcttaccgtctgcattgcagaaatacgggatcactatacattcagaattccaacgttttacgtgtgggtttttatccagccacttcataacgtagcgctcccacgatgacctatacgtaatctttcgcggatcgcctttatacttctgtatgttttcgggtacaaacgaccctttatacgtctgtcttccagccattgcgtaaatcctaaatagaataatataacgtttagataggggaacttatcgtgctattttcatacttcccgcctgttgattacaaaggcacccagacaactgatattttccgagactatcgattttattttaatcgtgtgattggaaaatataaaacccgtagttaccagataacaggcacactacgacctgaacaacttgcagaatcattatatggaaaccagcaatactactggatcctgttgatgcttaactctgtttatgaccctttctatggttggatctccgatcaggaagccgcgtatcagtgcgctatacagcgttattctgaggttggcggtgaacaggttctgtatcatgtagatgaaaacaacaacaagtattataaccttgtcgaagaccccaataaccctggtcattggtatgacaaaggtgacaaaccaatgctgtatttacagtatcaaggtgtattagctcctgtagatatttatgaagatgcagtgttgcaaaatgaagcaaaacgaacaataaaaatcattagtccgtctgacatccaggcgtttctgaatgattttattaaagaaatggaaaaggctaactcatgaaattaggcggaaatttacactcacctttctttgatggggtggttgaaaacgttgatgatccgcgcgggttgggccgtgttcaagtccgtgtatttggacaacacccagcccaaaaacaaaaatccgatgcaatcggtgttcctgttgaagatttaccctggatgatgcctattcaggatattagaagcgctgcgatctctggtgtgggcttctctccaactggtatcactcgcggatcctttgttgttggttattggcgtgacaaatggcaccaagatggtatgataatcggtactgtcgctggtgaatatgtcgaacaaccagacacacagaaaggtttttgcgatcctatgggtgaataccctcgctatgttggtaacgatgttaactcccttgcattaggtggtttgaaaggcaaaggatcatcaagtgtcatcattcgtgattcaaacacaagcatagcagtaaacccagacgatcgcccactggatgagataccagaagataaccgccctgatacgggtggatttacgatcgaaaagatgctcaagcaggatgaggggatccgcacacgatggtatacagacagtgaaggatatccgacaatcgggatcgggcatttgcttatccgcgaaaagactcgcgacactgcaaaaattaacgctgcgatcagtaaagcggtaggtcgagaagtaacaaacgggacaatcacggcagaagaggtatcaaccttatttgctcaagatttagccaaagtaagatctgatattcagagaatcgctaacgtccgtgaagtgtatgtgaacttaaaccgtcctcgtcaaatggcgatcgaaaacatgtcgtttcaaatgggcgtcggtggtgttgctaaattcaccaataccctaaaagcgatgaaaaatgaagattggcaagcggcttataatggtcttcgaaattcactgtgggctagtcaaactccaggccgttcttctcgcgtgtctaaaatcgtcctcacgggcaaccttgaatcatatggggtgcaagtaccagatccggaagggcgctctctgagtgctgcttacgctgcgtataacggtgctacattgtcggctactagtccggaagatccgtttactcctggtgatacccgtgtgatgtttgaagaaccagcatcatcttataatgcggaatatccgtataacatggtgtttgaatcgagatccggacacattcaggaattcgatgataccccaggatacgaacgatataaccgtgttcacccagcagggagttacgaagaaattcgcccggatggaacccgcgttgttaaaatcgtaggggatgattatcagatcgtgatgcagggccggaaactcaacgttaaaggcaacttacaggtagttattgaaggcgatgcgttcatttacaacatgggtaacgttcaacaaacggttgatggtaacgtaactgaatttgttcgtggaaacgttcaacaaacggttgaaggtgagtacgttggcctgattaaaggcaatgctgaactaactgtaaacaaagatgcaacagttaacgttgatcagaatcttaccgcaaatgtgaaacagaatgcaaccgttgctgtaacagaagacgcaacggtcactgcaaaaaatgcgaaaattgagattgaagaaacgatggatatcggtgctaaagatatcaatatcaaagcaacgaataacacgtttattgattctggcgcattaacaaaaatcactggcggcacagtacaggtaggctaacatgattatggattatgaatcaataattgatggaattatgcaaaattatcagcatccttgtgatgctgagatccccgctggctattatcggcgggttatctggcaagggcatacagaaaattatccggctgttggggttgagtgggataccgagataatcaaaatcggtactcatctttatactcaagaaccattcggacatagaagcacggatctacctgttgtcaattcaccaggaacagatccaaataccggacaatcaacagggatccttgttccgaagattggctattatttcaacactcaagcagaaattgatgcttacattacatctattggtgcaactaaaatcaatggtggtaatgattggtatggcgcggatctgtcaaaatcaaacctatacaaaaaccctggcgaactggctatgtataaggtcgaaaacagtggtgggtatctttccggaacaaaccctgtatgtgatgctcgcatacgtcagacgtataatcaggacactggcgcattcaccaatattgattattattggaatggtaatcgtatagcctatatgaagcatgatgaaacaggggcgcaccaatgcaaatatacgggtatgcaggttaacaccaacgcagatacaagcattcctcctgttcctcctgcaatgccttccacttatggggcattaccgagtgaattaagccgtgctgatatttcgtgcattccggcaactgttggtttcgcatatacaaatatcagtgatgctatgttacaggcatggaacgaaacccgtaatacgttcaagctacagtttaacatgttaacgggtgctgtacagaatggattcgggatcgcgacgatgtttgatggtttatccgtatcgatggaagaagtaatggcgggggcgctcgcattgtcacagcaagcatggcaaactgctatgaaagttttcagacaagtgattagcgctgcatttaacattatcggtggtgcatggggattgattaatcagttcttgcctcaagtaaccatcttaggtgttgcgatcaacatttacgatctggtgtttggtgataattctgttcagactttgaaagatgcgtttaatgcaatcatcaaatccggacaacaaacatatgaaaccgtcataaacgcaatatacggggccataggaagcgcatacaattactctgtggaatatgtcaaagctggcgctcgcgaccttgtggatgcgtgtagcgcgttatttgattggtgtttaacgatgttccaaaacggttgcgttgcattaatcgacttatacggtcggatcatgcaaacatgggctatccctccggaagtcccaaacccgttatggtctgcggtgctggctatccgtaacatcatgatgcaaatcaaaccacttgatataattctgggcggtaacttccctggattcactgcaatggatttgtatcaacaagcacaggaaaaagtcaaggcttttgttgatgagtcatacgaacagatccgagggctttatgaacaggggcaggaactttacaaaacgttaaaaaatcaaattttcgaacgtgatgcaattcagagaaaattcaaccagtacttaaactggatgtggggcgctgtaacagacgaagcaacagcggcttatcaatctgcattggatgctgcaaacgctgctgtagccgcaacacaggccgcgtatgacgctatacaggaacagattggatctctacaagatgcaatgaaagatacatacagcatggcgatggaagaattaaagaaattgcctttgatgagtacaataaacgagtttttaggcttctgtggtgtcgcatttgacgatcttctcaagtcatatgaaaatgcgattactggtgctcagtctctgtacaaaaatttcattgatagttcgcgatcgtttaaagatcactgcaaagtaatctataaccaaatttgtacgttggcgttgagtaaagtcacacaatatgtgaataaattgctgtctctcataggattagcaatcaactttggttcgattagtgtatgtgttccagtactgaaatactaaatagtcgaatgatcaagaggaatttataataatggctactgctaagactaagactgtcaaaaaacagattaaccaaatccccgatatctttatcgggggtactttcgaagaaattaaaacagatctgattgattggctgggtggacaagaagagtttaaggattacgatttttccggctcgcgaatgaacgtactgatcgaccttctgtcgtatgctactctttatattcagcagatgggtaacacagctctatttgaatcgtttattcgcacggctgcattgcgtagttctgttgtacagtctgctcaagaactgggatatatgccagattcgcgcacggctgcaagtacagcagttatgattacggctgctaacccactgaccccaacatcgatccgtatcccgcgcggtacaaaattcatcggtactgtaaagaatacagacagttattcttttgttgtatcagatgacgttgttatcgttcgtgatagtaataacaactatacatcaatgctgaacctggtgcaaggccgtttagttcgtactgaactaatttatgacggttcgagtatcctgatccgagatccaaacattgaccgtagtcaggtacgtttaactgtaaacggcgcacaatgggacgactggacaaacgaaagcattgtaaacgcaacaggcgcaagcacgatttactacatgcgtgaaactgttgatggacataccgaagtttatttcggtgaaggtgaagcaagtcaacaagtggcgggtggcgcactaaccgccgaatatatcgggggcttgaaacctgctaatggttcgactatcgttattgaatatctgtcaaccgatggggaagcggctaacggtgcaaaagattttatctatgtcgatacattaaccaatattagcatcacggcgattaaagagaacccaaccaacacccctgattatgtcggtgctgatggtggtggtgacccggaagatattgagcgtattcgagaactggcccctgttatgcgtgaaacacaacgccgttgtgtaactgcatcggattatgaatccttcctgtctcacaggtttggatctatcatccaggcggtacagtgctttactgataacgaaaaacctggttatgctttcatttctgttaaaccaaagtcaggtttacgcctaacatcggtacagaaagaagatatgcaaacgtatctttcgaaatataacctcgcgacgatcaccccgtcgattatggatcctaactatctgtatattgtgcaatctgtaaaagtaacgtatgatatcagtaagttgacggaatcagaggaatggttacgcggtcaggttatttcgtcgatcgactcttactatactgacaacgttgaaattttcaacaaatcgttcagtgtatctaagatgttgacttatgtcgatcagtctgatacttctattatcggttcggaagcagatattaaattgctccgtgaaattgacaactattacagtgctcctatgtctgggatccatttcttgaaccaggtggaatcgaaatcaatcatttccagtacgttcaagttcaccaacgaagaagacgaaagttatgttgttcgttatgcttctacggaaatggatcaggatggtaacgcaaaaattgtaataggcccgttcaaggatggggatatttcgatcgctgcttatacaggtgatgactttgaaaaattaacagatgcaggaacccgtaataaatattacgaagtaggatcggtgtctcattataccgatttcattagctttgacctgggcgttctgaacgtatccgccgatagtttcagtgctgcttatatcgagctaaccgcaaagcctctcgaagaaaccatttttactcgcgatggatcgttgatcgtgtttgaaaatgacctacgtcctcaatacaccacattgactatgaatcctatcagtcaataatcgttaacccctgtcttcggataggggtttttctttttataaatacgtgatatacataaccgcaaatttggagaaatataatgattaaagcgccttcgattacgagtttgcgcgttgataagctggctgctaacttcgtttaccttaaatgggatgatgttggcatggatttctattatgtggttgaattggcccgtagccgtgatatggacggaactattattccagacgaagagttaatctggagtcagttgggctatagctacgaaaacgaatggtttagcgatcaggttgccccaaatacacgttataaattccgtattcaaacaactcatgaagggtttgaaccttctgattgggtgatcagcgatgaattatggacgtttgatgagaacgcctacgcatatacaaccatgcgtgaattcacccctgctgattcgtttatcaatgaaaaattcgccaaaaacaatcgtgattacgtcgattttaacgatgatgttattatggcttctctgatggttgaggattttgtatactctcccctgtattctgatgtaagccagatcagcgataagatcctgaaacaagaaagctaccatgaaattcaagatcacatcgaacacgtttgtaatgatatagatcgcacgttcctggtatactcaaacggattgctttacctgtttgaacgttttcagaatatggctaaagtgtcaaatgacaaaggccaaacgtggtattactacaaagcattaaacgatcgtgtaggcaatccggtttcccgtaccgttgcttatcagagcgctaacactacgtatgtgttaggatacgatcgcatattttacgggcgcacgtcaacagatattcgttggtcttctgatgaagttcgtttttcttctgatgatgtaacgtttgcgaagctggggaaccagtcagggttagattttgatgttgattcatacaacacatatgcgcgtctaccgggaggagtgtcgaagtatgccgaagctatagcttgttctaatgaatggctctacgtggctgctaagaacgttatgcgccgtattgcgttacgtaacacaccaattgatactgatcctggttcgccgacctttggtgaacgtatttttgatgaagtttcatataccatcgtaccaggaaatgataaaattgttgttaaaaaaatggacgtgctgaatgaccgtctatacgttctggtaactggtgaagttaaaacggcgatgatggatccgactgtcaaggctaacgtgatcccatcaaacgatgctggcgtttatctgtgggatgagaatgcaaagacgtttacccgtgtttatggtaaaaccgaagatgaacgtttttatatcactcatgaatataccaatatgtcaaccaatggcgatgaagtttacatttctgttggtaactacaaatatccaggcactttgccagatctggatctggttgaaaagtatccggaagatgtgcattcagcggtgaaatacgatcttgttcctggttatactgcgagcatttcgattaactttgctacagttcgtgcaaatcagaacgatcctacagtatggaactttgggccgcaagagtactacaatgaagcaaactttagctggcatttccgcgataaggttagcacatggatcaccaatgataaccgtcctctggtggtttatccggaaaccctgtatactctggttactgatagcgcgtctcctgcgtcaacgattcgtgtaaaccatgaagtttgggacaaaggaacagttactatctacttgaataatatcaagtttactggttttacgaagtacacaaacggtgttctgttgtatcgctcaggtggtaggataattggattctatgaactgtcataccgcgcaagggatgaactcactattttctggaaacccgataacactttaatggtggcaagtctggttaatcaggaacgtgaaaacccatatacgccggatattgaacctggattaatcgaccctgatctgagtcacatgatcactcgttttgctccgcaaagctatctggacaaccaacagttcgagaaatttggtgaatactatctgcaatacatttcgttgggaagcaacagttactataacaaattgctgaacctcatccggaacaagtatccgagagagaaaaacaacgtcgaatatttgtggtctgaaattaaccgccgtaacatttacctggataaaaccaaacgtgaggcagtggttagatttttcgaatcacgtgcaagcgatttctattcaacaaaagggatcgaagcaagttatacgttcctgtttaaattgctgtataacgaagatgtttccgttgagatcgaaagctccaacagtctcgaatatgatattttggttagttcaacaaatatcagtcaggatatcgtaggccggacgatctatacaccaactggacgcgctaacgttacatacatcgaacgtgactatgaaaatggtcaattgcgttggtcaatgactctgcataatgctcaaggtaactttatcgaagggcaggttgtcaagtcagaaaaaaccaatttcaccggaatggtaattcgtggtgttcgcggtaaacaaatggctaacaactcgatcgactatatcaaccgtggacgatcttactatgtgatgaaaattcgttcaaatctaccgacttcccgttataaggatgacgtattgaggtttgttcatccggtaggattcggctttatgggtatcacgatgttaacagtattcatcaactctggtttgtcaatgactcataacgagacaatcattgatattctgagaaactaccgtttcgatagtggttatcctaagttctggcctgatcgcattgcgagtatggacggtaacggaaaccaacaattcgacctggttactggtgaacctctgtacaccgcacacccgcgagcgggggaaccttttgatgtacctccggaatatgacattgaagaaaaacctcttaacggtgttcttccttctgcgcgacggttcgatcaaagtccgttgttcgattgctcaggcgttaaatattcacagttccgtaatttggtggataaacgactgaaagatgatgcaggaaacccacgtgatccaaatcctccatcacagattaaggtaggaaattaaatggcacaacaaaacttgtatcggtcggtaattactgcaaaattccgaaccgaaaacttgatgaacttcaaagatatgatcggcgatgccgccgatctaaacacgatttacatgtctattggacgaactgaatcgtggtcggataacgaatccgaccctaacttcgcccctccatatccaaatgatagcaccgatggtgttagtgatatgtggacgcatatgatcggggctactaaagttcctggtgatatgatagatgcaattttaccacgtaaagactggggtgatactcgttatccaaacccgaaaatcttttactttaacgatattgtcgttgtaaacaccgcgccttataaccgtaccgatccgggtaaaggttggatggtttatcgtgtggttgatgttcctgatatcggttcttgctccatttcgagcattaccggaaaacttgaatgtatcaggatcggcggtatctggagtccatctcatgaatctagtgaacctccacgcggagaagctaacgggatcgacatgggcgacggttataaatgggaatacctctacacaatcccgccagatgtcgtgatcaaccgctgtacaaacgaacatatcgtagttcctttccctggcgaactggaagaggatccggtacgttggggttatgataacgtgattcaatggtatccaggacaatacgatctagtgtatcggttgaaagtgaattcaatgcgttttcgtgcatacatggattctcttttcttcccgcaatctacgcttcctggtaacaaagggttccgtcagataagtattattgtaaacccgttgattaaaaaggcaagcccgaccgaacctgaaaagaaagcaactggtgattactataatgctaacgcgcttgaacctgattccggacgtatgatttacatggaaaacagacaacctattattcgctcccttgatcagactgaggaagtgagtattgtattcgaattctaaggaaaaacaatggcttaccaaacagcaaaaaaactaattgatgtcggtgaaatcggcaacccatcaacaggcgacccgctttatgatggtggtgttaaactgaacgaaatgatcaccaacgtttataatgcgtttggtgatgtgcgtatgctgtctgcaaacgaaggtgtcggtaacatggtgatccatgctaccggatactatcagaaactaccacgcacttactattcaagcacaccgatcgaactgggttccctgcatgacatagatacttcaacaggttcgattaccgttgttcttccttctggtaaggttggcgaaggttgctacttcataaatagtacgggtagtgtctctgttgatcgtcctatcgcgtttcgtcctcaagttggggatactatcgcgggggttgcagaccagttgtatatcacgtcaccttacacctttgtaaaaatctggtgtaccaaaaaagaaggtgcggtaacaaaatgggattattctgtagaatctatgttcggttctaaaacgatgcctgttgacactacggcgcttgtactgaaagcaaacccgactgctattcctatgttcggatatagcgaatttagcggggctaaggtgcttgtatacgcagaaaacttagctggtacagttaccaaaatggcagaagttttaatgaccgtggatcgtgtacacaaaacgatttattcaacggaatacgctattttgaaaaacagtgaagatgaaatgtttacattaaactttactgtcggtgctggtgatgtcgtatacgctaacgtgcaagcgatcaaagaagatcgaattaaattcacgattaaagcaatagatacgattaaatcagggatcgcgtcatgaaacaagaaattttaataggtcagattgtagacgatggtacaggcgattacctgcgtcgaggtggtcaaaagactaacaacaactttacagaattgtataacatgctgggggatggtgagatcccccatccagcaggtgcctggaaaacttttgcgggtacgacgctatcaccaaaatttggtgaatcatgggcgttgaataccagtgcaaacaaaatcaccgtaaacctcccgaaaggcggcgtaggcgattataacaaggttattcgtctgcgtgatgtgtggtcgcgttgggctaccaacaacgttagactgatccccgcaactggtgatactatcaaaggttccccaactcctaaagatctgtttaaagattttatggatgtggaattggtgtattgttctccgggccgttgggaatacgttgaaaacaaacagattgacaaaatcacaacttcggatctggcaacagtagcaaaagaaacgtatattgctactcagggacaaactgacttccctaacgtattcggtgttggtaatgaatacaacctgcaatcgttcgaagtttactatcgcggtaacttgctgttcatcgatgagaaagacggattcaatgctgataactcagactatggatcgattggttctgctcctggtgaactggttgcacttgatggtaattcagtacgtcttaaaaacccgtgtaacgctggtgacacgcttcaatttgttacctatctagatgggttagcaacatggcgatctagctatgaagcgtatgtgatgcgcatgtatcagactggcgatacttctctggaaaccgttcctggtgaacagtgggtaggtgatctgacaaccaaaaaagagtttacacctgctgaatttggtgtaaaccctcgcgtgttgattaaccctaactcgtttgaactgcttctcaacggtaaacaactggttaaaggcggtgacgctgactatccggcgttttcctgtgaaggtgcggaaggtgttgatgaaagtacgtgtgttggtaactctggtgtatgggttccgtcaggacaggattatagtttagtattcactgattctgtagtgacttcaatcaagtttgctcaggaactggaatccggcgacgttgtaacgatccgttggtttaacaatgatattggtactctgatggattgggaaggaactggcggtattaaagaaaaatctgataaggtttatctcaataacgaagaagaagttatattgacgaaccgtatcgaatataccgattataataacccttctcagaaaacaatgcgtaatacaggggaaacctatcaggggcgtattctggatattcaggctatgtttgatattatccacccgatcggaaccatctatgaaaacgcacataacccagcaaaccctgctgattatatgggatttggtggttggaaacgttacgcagaaggttatttcttggctggctggacatcaaatgtaacggatcctgatttcgcattaaacaataatgatttagatagtggtggtcaaccgagtcatacggcaggtggtactggtggcgatcgtggtacagaaatcaaaatcatcaacgttcctgaacttgtatcaaaagataaagttcttattgctgatgaaaatggtgctgtgatcattggtggttgtcagttagatcctgatgcttctggccctggatacactaaataccgtgaggatacattgaaagtgaatcatggtaacacattacctgataaaatcaaaactattccaccgtatatgactgcacatcgctggataagggttgcataatggcttacaaaaatatttcaaaaacaagggagggcgctcgcgtcctctctaaagaagcagattacttacagtatgatacttatggtaagttgcctctgatcggcggtaaacgttcgatcggcgaaccaaacattgaccaaacaaaacgcggtgttctgtatggaaacgtacaatccgcaattgatgacctgtatacgcttatcgagcaaatcccgattaacggcgttgttaccatgactgaggatgcccctccaatcgctgtacagcaggttgagagcgtttcttttgatggtattgtacagaacatcgattcagaccaagaacaggctgtagttcacgtgtacggctttcctttcatctttgataatgggactaacgccgcaactgtttgtgaaacggcatacaacaaatttactgaattcgttgcagcggaaaaatatttcgcagaagttaaccgcaaaggtgttgatggtacgatccttgaatgtcgatttattgatagtgttccgcacccggcaacaaatatctcagaaaacggtattcgtcaaatcggaactatcgacgtagccgcaaaaagtggctatggttcatgggttaagttgggttctggtttcttacctgatgttactccgcaagtaaccgtgtattacttcaaacgaattgcataaggataacacatgagtaacaatacaatcaaccacgtaagtgataaatccatttacgtgacatttgacccaacaggtactgattggcctgataccataaccaacgtacaagatgcgttggaaaaaataggtagttgggcgcgtactgatactgggcttcctatcgcaacaacttctgttcgtggtattgctcagatcgcaaccgaagctgatattgacgctggcacggataacactaagattgttactccgaaactgttagcatatcgtatgcagaaccctaaagcatcacaaaccgtatggggttatacgaagtattcgactgatgcggaatccacaaccgtaactaacgatgcatcgtctattactccgcgatctctgaactatgtgttcaataaccgcaaaggtacagaatcggtttggggttcttctaaaattgctaccactgcacaggcggttgctggtacagataacactgtaactatgactccgcttaaagtcaagcaagcaatcgcgtctctggttcctgttcagtcaagtgcgaccgaaagctcgcaaggtttggtacaactggcaacagttgcacaggttcaggctggtacgatccgtgaagggtatgcaatttcaccttatacgtttattcgtttaactgcaaatgaaagcaacctgggtgttattcgtattgcaacacaagcagaagcaaacgcgggtactgatgacaccaaagcgattactgcgaaaaaattaatcaatacccgtgcaactggatctcagttcggtgttgtcaaattagcaacaactgttggttatgtggcaaacactgcactttcttcaaacgctgcggtattacctagtgatcgaaatgcggtaattaacggttctctttatgagaatagcgcaatatataacaacaaatatcagacgtggacagatcttgattggcatttcccagtaggtgctattgtcatgactggttttcagactgaccacggtagtttgtatatttgtgatggtcgctcactgaataaaaataactatccgttactttttgagcgtataggttatacatttggtggtggcggtgattggtttaaccttccagattgtcgaggcgttgcagtacgtggtcatgaccgtgggcgtggactaaaccctaatcgtgggtatggtacatatgaaggcgatatgttgggctggcatgaacacccattacagcttatctaccagaacggcggtaatattcctaaatggcaagcagtttacgaactgaaaagcgccgaaaagaatgaccaaagcgctcgcgtatttgatgcttctataactaaagccactggtgtgggtggggaagaaacccgcatgaaaaacatcgcattaaactacgtaattcgtactcaatagaggttattaaatgatcatcgacaaattaaacccgttgccgaagatcccgtttgttgatggcgtcccagatgacgccacgactcaaacgaagattatttggatcaaaaacggtgaaactctggacggttcgccagataaagtgtcaaacactggtagtcttaaccgaactggtgtaaacatccagcagaacgcggttcagttagaacaaaataccatcacccataatgataaaatcaacgaagtaatcgatcaggttaacttgattactgaaaacattgatgctattggtgatgagagcgtaatcaaaaaagttaaccagttggatcaggatgttcgggcattaactttatctaacacccaaacacagaacaaggtagcacagttaaccctttctgtaaatgctcaaaacgatgaaattggtgaatacgatccagaaaaagatcctaaacaccgcacaattcgtaatgatatcatttacattaagaaagaagttggttcatatcctggatttaacgttgatggtgatgttgacccctcttctactggtactggccttaaataccgcgtactgagtaaccaacgtgctatttctatgcaggaaactcgcataaccaaactggaagatgattgggcgctttccgaagtaggacaactgacagaagaggtaaaagaacttcgtgctgaaatgggtgattctggtcttgccacaacccgatcaatctatgcgcgaatcaagatccttgaggatggttctattgtaatgcaaaatgaacttgatgcgattaatagttatatcggtcgcacgtcaggttcaaccagttccattaacgatcgtgtgaacagtctggaaaactccgttagttctctggctacacaaatcaatgatccggtaactggtatcactgcacaaattgcaaccattaacggtcaaatcggtacggcttctgctcagggtagtatccgttatgatattgcggaaactaaacgcagattgatggatatggaaatgattctgggtgaatccggcgatgatggattgcagggacaagttgcgatcttaactggtgacgttggtgaagattcagatcctaccagtatcaaaggccgtttgagtgttgttgagggtgaattacgcaccaacactagcgcactctgggaactgcaaggcgttgtaggtaactcttctagtggcctcgttgcaactagccagcagattaacaaagaaatctatggtgatggtgttagttccgatcctgttactcgcgctggtttgaaaacgacaacccgcaacctgttcactcaggtaggcgataacgcagaaggtaacgaaacgggcatttatgcactgattgccgaccttaataaacgtgttgaggatttagaagcgttgaacattgcacaggcacttgcagatcgcgtaactatcgaagatctgaatgctaaactggctctgtacatcaaagaagctgacgctgatctccgttatgagagcaaaaacccgcctctgtcattcggtactaacctaactggtgatactgaatatactactggcgacccattgtctctaagcgtaactatgactggtggcgtttctccgctgtcttatcagtggacgaagaacggcgtaaatgttggtactaatgctaacacatttaccattgattcgctacagccttctgattccggaacctacaaagtaacggtaactgatgcaagccataaagtcatcgtttctgatgaactggcgatcactgtcgcttaacgattaacaaggggcttcggccccttttgaggatctttatgattacgaacaacccagcacaattaaaagatgaaattctgcgccgcttaggtgctccgatcgtcaaaatcgaagtgacaacagatcaggtttatgactgcattcaacgagcattagacctatatgcagaatatcattacaatggatctaacaaagggtatatcattcttaccctggggccggataacccgaaaaatattttcgatctgagtaaagaacacattttcgcaattactaaagtgttgcgtactaacatgggttcccttgtatcgatggatggtactgcggtttatccgtggtttactgatttcctgatgggccttactggtggttctctgggcggtggtggttgtgcatcacgtacctacggaatgaacgcatatggcgcggatatgggctattttacccagatgatgagctatcagcggtcaatgcaagatctcctgtctccgcttccggattactggtataacgacgacacaggacagtttgcagtatacggaaccgttaaagatggtgatattgttgttatcgaagcaatgatcagatcctttgttgatgtacccagtatggtcggtaacgtctctggatacgctacagcgggttctgatggcgaagataagccaactatagcagatatatacaataacccctacaaagctgtctcaggcggtgtgaaggctggtcaaggtacaagcgttcagggttcatcctctgcgtataacaaccgttgggtgaaagattacgcaactgctcttgttaaagaggtaaacggtcaggtgctggctaagtttcagggtatgcaattgcctggtggtgttgctccggatggaacccgactgatacaggaagctatgcaagaaaaagaaaacctccgtcaagaacttctgttactgtctgatgcacttccagtgttgatgatgtaaggaggaaaaatgcactatagattgtatcttgttgtttttgaaacttctactggattaaaaatttatggggggaagcgtcattccccttatgacaatccacataatgacccatatacaggatcagggacatatataaaaagagctattaaaaagtatagccattcttgtattaaatgcattcgatggtctaaagaatttcccaacagagaattactagcagaagcagaagaattattagttgatgagataatggattattattccagttgtgttaatctagtacggggaggaaaaggcggagtttctttttatgatccatcaaaaaacccaaatataggttcaaaacgaagtaaagaatctagagataaaatgtctatgattgccaaaaatagaaaatatagcgaaattggccttaaaaatagacaagaagccacccgtataatgacaagaaatagaaaacaccatgatgtttctggtgataaaaatcccgctgcaagaaaagttatcgttgatggcgttgaatacccaacattgaaagaatgcggagaccactacggcataacaaaaaattctgtatttcacagaataaactctaagaaatgggagggatggaactatgcgtgattgggatgaaaacttatttgcacaactggaatctggggaaggtgtagacaataacctaaaaacagaagttactaataagtatgttaactggtacaagtataaccctactcaacagttacatgattcactaacagccgaagcaattcaaatgaaatctccggatatgtattacgtccgtcgagaatttgttaatattgataaaattttgggtgaagaccgtgaatcgaagtttacaaaatcgtggaaaattgcagcatacatcgattcgtatgcaaactacgaaggacagagagacttttacagcaaattcggtatgatgtcaaacgatgaaatgacacttgtgatcaatcctcgtttatttgcacatcaaactgatggcgggatccctgttctgggagatttgatttatttccctatggataacagtctgtttgaaattacatggattgagtttgacccgttcttccagttcggcgatcgtcctcaacgtaaaatcaacctcgttaaatttatctatactggtgaagaattggatcctaaactgcaacgaaatgaagggattaacctttctcccgatgccgatctggatctcgaacctattcgaaatcttgatgggttggcggataccaatattgaacaatacgaagaagatcaagcctttgaagatgaaggtgatgaattcattgaatcgtttgatgttgttaacgggcgcggatcaccgttcgcacagttcccataaatataaccaggggaaaccctatacatgtaagggtataggagaaatcttatacccgctttaacccatacaggaaaaagaaaatgtttggctactggtataatagttcgctgcgaaattatattgtcttgatgggttgtcttttcaatcacgtgcaagttaaacgcgttcgcggcgaacaagaaaaatttatcaaggttccgattacctacgcatcaaaagaaaaattcctggcatccatgaacaagctgaactatgcatacagtcaggaaaatgttgctaaaacggaaacaattttaccacgtatgaatctatccctcgttgatttgcagtataacgcaattcgtaaaacggggatcgcggtaaaccaaaaaatgacgcagttacgcgcacctggaaaaacagtaacgcagtttaaccctgctccgtatcgtctcatgttcgaactgggagtgtatacccgttacgaagatgatgtgtttcagattatcgaacaaatactgccatacttccagccgcatttcaactgtcgtattacagaattacataaaaacgacattaaaatagaccgagatattaaaatatctctgcaatctgtttcccctgatacatcgtttgaaggcgatgcaacgacacggcgacacattgaatggtctttaatgtttgaattacagggctacctgtatccgcctgttaacgagattaaaggcgagatcagaacagtatacacggatttcttttccaatatgaacccgttggacaaagacaattttgaatccgttgatgctcaggtggatccggttgatatgcctatacaggattacacgggagaagaatacattaaaacgtatgctaatgatatcccaattcctagcggcgatcaacctcctaaaccgaggggccaataatggaagaatttagcgtaaaacaactacttgatcttgaaaatctccccggtgctgaaactggggaagaaatggttgtatatgaaaaactcgaactcgttgatgtcgagtcacacccagcagatcgaaaaccggatttagaggaagactatgcacttgcgcgtaaaaccgcgcattacatgaatcagatgatcatggatatggcacaaattgccttgcataacgctaaaaactctgaatctcctagacacgttgaagtttttacaaccctgatgaatcagttaaacaattctaaccagggattgatgaaaattcataaagaaatgcgagaaattaccgaagaaacaacaaaaccaggatctgaaaaaggtaatggcggcggtaatgaaatgaacatagagaatgcaactgtatttgttggttcccctacggaattaatgcagaaatatggtagtgcatacgaaccaaaagaaggcttcattaatggtgaagcggtagaggtaaaccctgatggaaatggaaccgacgatcgatccgagtaaggaatcagatcacccaatcggattaatgcatcccgattatctgaaaaagaaaattgatgaatttgggatggagtggacgcaaagcgaacatgataaaaaatggtatccgacaaagtttagcgattacctaaaaattaacggtatccagaaagttgatattcaagcaaaagacagttcaaactttgcgacgtataaaaacaaaggaaacaagaaaactcgatataacggaaacccaaacctgaaacgcgcgtacatccaaacgaaatggacgcaacagatgttgatggagtgggttaagtgtcgtgacgatatcgtttattttgctgaaacatattgcgcgatcacccacattgactatggtacaattaaggttcagttgcgtgactatcagcgcgaaatgctgatcgaaatgcataaaaaccgtatggttgcctgtaacctgtctcgccagttgggtaaaacaaccgttgttgctatcttccttgcacactttgtgtgtttcaacgaggataaatatgttggcgttttggctcataaagcctctatgtctgcggaagttctggatcgtacaaaacaggcgattgaacttctccccgatttcttgcaacctggtatcgttgaatggaacaaaggttctattgaacttgataacaaatgtaaaattggtgcgtttgcatcttctcccgatgcggtgcgtggtaactccttcgcaatgatctacattgacgaatgcgcgtttattccaaactttattgatgcgtggttagcgattcagccagtaatttcttctggtcgtaaatcgaaaatccttatcacaacgacacctaacgggcttaaccacttctatgatatctggaacgctgctatagaagggaaatccggcttcgtaccatacacggcgatctggacatcggttaaagagcgtttgtatacagacggtgatgatggcgtatttgatgacggctattcatggtcttcgaagatgatcgccagttcaagtaaagaagcatttttacaggaacattgtgctgaattcatgggaaccaacggaaccctgatcgctggctggaaattgtcaaaactctcatgggttgatactgatgaaacggaaactaatttttatcagtataaagctcctgtagagggacataaatatattgcggtactcgacccagccgaagggcgcggtcaggactatcacgcgatgcatattatagatattacatctatgccgtttgaacaggttgctgtatatcattcaaacaaaacatcgcaccttattttgcctgatgtcctgttacgttatcttatgatgtacaacgaagcatgggtttatatcgagctaaatagcacaggccactcagtggctaaatctttgttttctgagttggattacgataacgttatttgtgatagctataatgatttggggatgaaacaaagtaaacgatcgaaagcgattggatgctcaaccctaaaagacttgatagagaaagataaactcatcataaataacaaaaagacaatacttgaatttcgtactttctcagaaaaaggtgtttcgtgggctgcggaagaaggtttccatgacgatctcgttatggcgctggtttgctttgcatggctaacaacacaaatgaaattcgcagaattttgcgagaaagacgatttgcggttggcaaatgaggtattcgcacgtgagcgcgaactgctttatgaagatatgttatgtcctgttatcgtaacgagtggcgacgaaacaatatctgtcggccaacacggtatttcgtttatataaatttagaggaaacttaataatggctttaatctctccaggcattgaaactaaagaaacatcggtacaatctaccgttgttcgaaattcaactggtcgtgctgctattgttggtaaattttcatgggggccagcttaccagatccgtcagatttctaacgaagtcgaactggtaaactattttggctccccagacaatgacaccgctgattatttcatgaacgctgtaaactttttacagttcggtcaggatctgcgtgttgttcgtgtcgtcgataaagaagccgcaaaaaacgcaaccgcgatctataatcagatcaaaaccacgatcaccgctgctggttctaactatgcagtagacgatcagatcaaagttaaacacaataacgttgttattgaagaagatggtgttgttaccagcgttgatgatcagggtaaagtcctgtctgtgttcattccgagcactaagatcatcgcacacgctaaacaggttggtgtatatccggatctgtctagtggctggactacagaaatcgtttccagttcttctggtgtttctgctacgattacaatcgacggcgtagaagttgatccgggtattactctgctcaaccttgacaccgcaaaagaaactattcaggcaactgctttccaggaactttgcaccaaatacaagctaccgtctgttattgcaatttatcctggcgaaatgggtagcaccgtaacggttgaaattctgtctaaagctgcatacgattcttcggctgtcattaagtcttatccttctggtaagtctggtaaaaacagcggtcgcagttcgatgaactttggccctcagaatgataaccaatacgcgtttatcgttcgccgtggtggtattatccaagaaacgtttatcgtgtcaaccgctaaaggtgataaagatatctacggttcaacgatctacatggatgatttctttgcaaacggtggttcgcagtatctgtatggtacgtccctaaactggcctgtcggattctccggcgttctggaactgggaggcggtacttctgcaaactccactgtaggcgctgatgaactcatggctggttgggatatgttcgcagatcgtgaatctctgcatgttcctctgctgattgctggtgcttgtgctggcgaaactgccgaaatttcgtctactgtacagaaacacgctgtgtctatcggtgaaacccgttcagattgcgttgtattcgtttctccgccgcgttctgctctggttaatatcccactggctcaggccgttgataacctcgtagaatggcgcacaggctacaaaatcggtaatactaccccagttgataacaacatgaacgtaagttcaagttatgcgttcatcgacggtaactataagttccagtatgataaatacaacgatgttaaccgttggatcccgctcgcgggtgatatggctggcctctgtgtttataccgatcaggtatcgcaaccgtggatgtctccggctggctacaaccgtggtcaactgcgtaactgcatcaaactggctatcgaaccgactaacgcgcatcgcgattctatgtaccaggtacagattaacgcggttactggtttctctggtggtgccggatacattctgtacggtgataaaaccgcaacgactgttccaagcccgtttgaccgtatcaacgttcgtcgcttgttcaacatgatcaagaaagacattggcgataacgcaaaatataaactgtttgagaataacgatgatttcactcgttcttccttccgtatggatgcaggacagtatatgtctaacgttcgcgctctgggcggtgtatacgattaccgtgtggtttgtgacactacgaacaacacgccggatgttattgatcgcaatgagtttattgcatcaatctacgtcaaaccagcacgttctatcaactacatcacactgaacttcgtagcaacctcaactggtgcggatttcgatgagttgattggatcaacgtcagtataacatgtaaggggctgaaaagcccctataaatacacatagaggttagaaaatgcttactgatattgtacgcgcctttgaatccggtgatttcgcacgtccgaacctgttcgaagtagagatcccgtacctgggcaaaaactttaaattaaaatgtaaagccgctactatgccagcgtctaccgttgaaaaagttccggtaggttacatgaaccgcaaaattaacgttgctggtgaccgtacctatgatgactggacaatcacggtatataacgacgatgcacacacaacccgtgatgcaatcgtagcatggtcaaacatgctgcatggtatgggtgaagacattacaggggatatccctgcaaactacaaaaaaaccgctacggttaaacagaaaaaccgtaacgacgaagtaaccgccgaacataccatttatggcctgttcccgaccaacgtgggagaggttactttagactgggatagcaacaacgaagtgagcacttttgagtgtactttcgcgctagactggtgggtttaaacgctataaatacaggggtagcaataccccttatcattatttttcggagttgtaaatgaacttttttggattagacaatgtgttagggtttttcaaaaatttcgccaaacaggatgaaatggaatttgaagcccaattaaaagatgatacaggttcgattgcgcctccgaaaaataacgatggggcgcacgaaatcgaaacggacttatcaaaccagcgttattcttctgtgttccaacagttctattccggacaggatccgcgaattcagaacaaaacacagctaataaatacataccgtggtatcatgacatatccggaagtggaaaacgctgtttctgaaatcattaacgaagcgattgttaatgaacaaggaaaagatattgttacgatggatcttactaaaacgaattttagtaaaaatatccaagataagatcatggaagaactcgataccgtaatgaatattcacgatttcgataaccgaggatctcgtttattccgtgattggtatgttgattcgcgtatctatttccataaaatcatgcacaaaaatgaagctgacggcatcaaagaattgcgccagttagatccccgttgcatggaactgatccgagaatcggttacagaaaccctacccggtggggttaaaattttccgtggctatcgtgaatacttcgtatacaccgcaccgaaaaacggttatagctacaacggacagatttatagtcacaatgacaaggtaaaaattcctcgctctgcgattgtttacgctcatagcggccttgaagattgcgacaacaacattataggctacctgcaccgcgctgtcaagccagctaaccagttgcgtttgctggaagatgctatggtgatttaccgcattacccgtgcgcctgaacgtcgtgtgttctatatcgacgtaggtcagatgggtggccctaaagctacacagtacgtaaataacattgcacagggcttaaaaaaccgtgttgtatatgacgcgagcactggtaaagttaagaatcagcaaaataacctgtcaatgacagaggactattggctgatgcgtcgtgatggtaaagcagttaccgaagtttcaacgcttcccggtggcactgccttctctgatatcgacgatgttaaatggtttaaccgtaagctgtatgaagcgttacgtattccgttaagccgtatgcctcgcgatgatggcggtatccagttgggtaacgatggcggtattacccgcgacgaattgaactttagcaaatttattcgcgaattgcaaattcaattcaaccctgttcttgcggatccgttaaaaactaacttgatcgcgaagaaaatcattacagaagatgaatgggatgaaaacgtaagtaagattgcttttgtatatcagcaagattcttactattccgaaatcaaagatattgagattttggaacgccgtttaaacctgatgggccaacttgaaggggtggtcggcaaatatatctcccataaatacgtaatgaaagaagttctccggatgtctgatgaggaaattcaaagcgaagccaaacagatagaagaagaatcaaaagaagaacgttttaaaaatccagaagcggaagaggaaaacttttgatgaaagaatttatcgaagcaatcaaaagcggtaatctggtggaagctaaaaaaactttttactccatcatggaagaccgcacagaagcgcttcgtcacgaattacgcgttgaacttgccgaagctgtacgcatcgaaggcgaagaagacaaagaaaaagacgacgaaggcgctgataaagatgacgagaagggcgataaaaagccagccgaggatgataaatccgataaagatgatgagtgaggtgtgtaaatgcaacttgacatcgaaatcaccgccgaagatctccaggaacatttagacgaagcgaaagcccgtgtagatattctgggtatcgatgaaggcacggttaaaatcatcgaaaatttggcggtcaccgaaccaaatttagcccttgctatgatggcggttgttgaaggtttaacacttgatgaggtaattgtcaagcatgttgattcccgtggcaacgtagaacgcctcaaagacaggaaaacccgtgagcgtaatgcgtatcagactaccggattaactaaatcccaacgtcgccagatcgcgcgtcgtgctctcaaaacaaaacgtgctaacccgtcaattgctactcgcgcacaacgtaagcgcaagaaagcattgcgtaaacgtgctgcactggggctataaatatgaatgaatcccaaatcaacgaaaacggcgatatgcttttaatcgaagaatggggtttaccttgcggtgacgtttcagaatctattttagaatctgttggggaatcaaaagacggtaaattgcggatcgaaggtattttccttcaagccgaaaaggttaaccgtaaccgtcgtttgtatcctaaaaacgtacttgaagaagcagttaacgattatattagaactcaagttaacacccgtcaagcattaggtgaaatgaatcaccctccgcgcccgaatgtggatccgcgaaatgcttgcatcctgattgaaaaattgtggtggaagggtaacgatgtttggggccgcgctgttgttgttgaaggcgacggtggtgatggtgacaaactggcggcgttgattcgtgctggttgggttcctggtgtttcttcccgtggattaggtaagctctccgattccggcaaaggctacggcgttgtacaaaagggctttaaattagctgtaggcgttgatgtcgtctgggggccaagcgcacctgatgcatacgttaagcctatagtggaaaatcagcaaagcaaaccgcttgttgagaataatagtgctgatgacgcttttctggcattgtccgagcgtttgaaaggtctataaatacattaaacaaaacaacaggaaaatcaaaaatgcttaaagaacaactgctggcggaagcccagaacctggatactccggtcgagttagacagcattttcgaatcagttgaactttctgatgacgtgaaagcgacattcaccactgtattcgaacaagctgtaaaagctggcgctgcaaaactcgctgaatcccacattacccagatcgcggaacgttccgacgaactggtcgaagctcaggtaactgaacgtgccgctgaaatcgaaactaagctgtacgaagatgctgataaatattttgcgcacatttccgaagaatggctgaaagaaaacaaagaagccgtttcccgtgacatcaaagccgacctgtttgaatccctgatcatgggcctcaaagaagttctggttgaacataacgttgtcattccggaagaacaggttgatgtagtcgccgaactggaagacgaactgactgagaatcagcaggaagttaaaaccctgtttgaagcgaatcaggaactgaccaaagaaatttcagaaatgaaacgcaatgcagtagtttcagagaaaactaaaggtttgaccgaatctcaggtcgaaaaagtagaatctctgattgaagggctggaatattccgcaaccttcgaaaataaactcagcgcaattgttgaaatggtagcaaccaaagctgaaaaacccgttgacgagtctgtaaatactccgcaaacgaaagatgactttgttccggtagttgaaagtgttccggcagagaaatccaagatcaataaatatgtacaagcggcaaaagccctttcttaatttcaaaaggtaagaaacaatgtctaagaaaaacgaattgatggaaaaatggaacgatcttctggagtctcaggaaggcttaccggatatcgctaccaaatccaaaaaacaactgattgctgccattatggaagcacaggaaaaagacgcagaagttgatccggtttaccgcgacgagaaaatcgttgaatccttcggtggtttcctggcggaagctgaaattgctggtgaccacggttacgacgcaaccaaaatcgcttctggtaactcaagcggtgctatcaccaacatcggccctgctgtaatcggtatggttcgccgtgcgattcctaacctgatcgcgttcgatatctgcggtgttcagcctatgactggccctactggtcaggtgttcgctctccgcgcagtgtacggcaaagatccgctggcttccggtgctaaagaagcattccatccgatgttctccccggatagcatgtactccggtcagggcgcggctccgagcaacggctttaccgaactggcttccggtactgctatcgctgacggcgctatcgtgttccacgatttctctgaaactggtcgtgtgttcctccagaacgtttctggctctccggttactgtaactggttctaccgccgatgctctggatgctgctgttatcgccgaacaggaaaaaggtactctggctgaaatttcttacggtatggctaccagtgtagcagaactgcaagaacagttcaacggttctactggcaacccgtggaacgaaatgggcttccgtatcgataagcaggttatcgaagcacgtagccgccaactgaaagcacagtactctgtagaactggctcaggatctccgcgctgttcacggtatggacgctgacgccgaactgtctgctattctggcaaccgaaatcatgctggaaatcaaccgcgaaatcgttgacatgatcaactataccgcacaggttggtaaaactggtttcactcagaccgttggctctaaagctggtgcgtttgacttccaggatccgattgatgttcgtggcgctcgttgggctggtgaaagctacaaagctctgctgattcagatcgacaaagaagcaaacgaaatcgcacgtcaaactggtcgtggtgctggtaacttcatcatcgcttcccgtaacgtggtttccgctctggctcgtatcgatagcggtatcactccggcaggtcaaggtctccagaagactctgaacgttgacaccactaaagcagtattcgctggtgttctgggtggcgtgtataaagtatacatcgaccagtatgcacgtggtgattacttcaccgtgggttacaaaggcgataacgaaatggatgctggtatctactacgctccgtatgttgcgctcaccccgctgcgtggttctgatccgaagaacttccagccagtaatgggcttcaaaactcgttacggtgtaggtatcaacccgtttgcgaactctcgctctcaggctccgtccgaccgtatcacttctggtatgattaccaaagaaatgttcggtaaaaacgcatacttccgcaaggtttatgtgaaaggactttgatcctaagttattgaaaaataacgatattaaagggaaccttcgggttccctttttcatttctataaatagtgaaaacaattgaggctatattatgaaacatattatctacaaaataacaaatttggttaataataaaatttacgttggtgctcattcaacagaagacatcaatgattcatacatgggttcagggatcgcggttaaaaaagcacaaaagaaatatgggatgaataactttgtaaaagaaatattacatgttttcgatacccgtgaagaaatgtatgaaaaagaaagagagatcgtcaatctcgaattcataaatcgtccagatacgtataatgctggtataggtggtaaaggtgctcctatgtcattgattggttggtctgacgaacaaaggaaaaagatttctgaaaatactgcaaaggctatgcgaacaccagaactaagggaaaagatgagacaatcccgtttaggtaaaccacagtccgaagaatccaacaggaagcgctcagagacgttaaaagctaaatacgtgaacggacgtatagacagagagtataaacctctcacagaagcgcacaaggcgaaattaggccgttctgtatcgatagatggagttgtatactcatccgggtcggaggcggcaaaatcccttagtatgtcccactctggtttaaaatatcggattaatagcgacaaataccctacctggaaatttgttgcataaataccattatacactttacgcaggaacataaaatgagtgaaaaattttacacaattaacaagctggtgcgtcagtcacagctaccgcctggcctgtctaaaaaggttcttgatgaggcaaccggaacagaaacaattaacgtagctaatacccgtccggatctggtatctcttacccgtgcggtaaacaacctgatctacggtgaacttgtagcgattcaggaaactaatttacctaccgcaactctgttcggtgtgcgttatcgtaaccctaaaggcgatatgacgttttccagcgctgctacctattccggtaagtatgcaagccgtgataacattccagttggtgcggttggtactgcctacaccaaaggccaagttttcaaacacccgacaagtgatgttgtatacgaagtaactgatagcgtaactctcgcaggtgctgatattaatgaagcgattatggtcgcattattcagcaataaattacgcctggcaagcgaagccgcgccaacaagtcagtatgaaaccagcgaagatattagtacaacttctttcgaaatggatcgttggaatatcaacgttcgttcccgtaaattcaaaactgaaatgaccgtggaacttatgcaggatctggaagcaaaccaattcaacgcagaaaatgtgattgaagatgttttgggtactgttgccagtgaagaagtaaacaaagatatcattcagactctgatcaacgtatcaaatcgttacaacgttgatggtgtggtcacaaacggcatttttgatgctacaaccgcatacactgcaaaggatgctccggctttaggtcgtttcctgtatcaattagtgtgtgaaatggggcaggaaatgaatagaacgacttcatttgaagctacctatgtcctggcctcttctcgcgttgtaggcgttctggctgcgtctggttggatgcatgaaaccgatgaaacccacccgttagcgacagggcgacttaaaaacggttattatgtctatactgacaccaatacaccgtttgattacctgctgactggttgcaagtacgatctgggtgaaatggatcatgttggctctctgttctatacgccatacacagaagctgatcaggcaggttcgatcaagatttctgttgatcctcaatccttacagcctaaagttgctattctgatgcgctacggtttatcggttaacccgtataccactgctgctaatgaaagacttgtgaaaggtgatgactgggtaaacctctcaggtaaatctaagatgagtcagattgtgggtatcaaacttcctaaactgggttgatagtataacccaacggggataatattcaataggtggagtagggaaacttactccatcttttaataattataattaatattaaattagatcttgaaattataaatgatttatgataaaatttattaattataattattatagatcaaataatttttgaaatcaagtaaaaataaatttgattttataaattagatcatgtataattattcttttaataatatattagatcaatttaaatttgactacaaattaatatagtatattatagatcaactgggtaaattggtgagtatgttatgagtttgaaattagaagatctgcaaaatgaacttgaaaaggatatgctgatagatcccctcaagttgcaatcagaatcagcggatatccctaagatttgggctaaatggcttcgttaccattcaaacgcgaagaaaaaactgatccaacttcatgctaaaaaagaagctgatgtgaaggatcgtatgttgtactacaccggaagacatgacaaagaaatgtgcgaagtggtgtatactgggactactgaaatcaaaatcgcgatcgctggggatccgaagattgtagaaaccaacaaactgatccagtattatgacatggtggtagatttcaccagtaaagcactggatatcgtcaaaaacaaaggatactctatcaaaaacatgttggagatccgtaaattagaaagtggtgcataatgtctactgaaaatgaaaaatgtgtagtgtgcaagtgtccggttccttctactggttatgtgactgaatccgggcgcgtgtgtagcactatctgtgctgactacatcgcagaaaaaacaaaaagcggcgagatcaacgaatccgatgatctgaatgaagttcaaatgttgctgtaggagaatcttatgattggatacggtgaaggaattacagatcgtgatgaacgtccggatctgttagaatctgacgaacaccctgatttttagggtataaatactagcgtacccgaaaggggcttgataaaagaatgctggatgataggcgtactcttttgcgccgtccgatggagtttaccttcggcggggtgattgataacataccttcgatcaagggcatgagtaaaaaaagccagaatagtacctcactggctataatcaaatgtacgtgttgggctgattgcgtcccaaaattaaaaagccccttcctttcggttggggcttttttttagaacttttcttcttctccgctttcgagttcggcctttaattcttcggctcgacctttcagcgcatcgcgcatagaaatatcgtctgacggcgcaacatcaacttcttttacacgatttttgtaatatttttcaagctctttaaggccgtccatagtacggcaagaggcgaccttgctcatgaaatcatcaatagccgcctcataaagtcgaaaatcgttgaaactcttcattttgacctctaaatttcgatttgtttgatcacgtagtcaaacttttcttcattgtaaatgcgtactcgttcgattgcgtgtttcataccatagtttttgtatgaatatttatttttagcatttttggactttgccagcgttgctaagttatcaaccaaatcccaaacagtagcaagagatttagaatcatgtttacgcagtacgcgcccaattgactgtttgactataacagcagatttgcaaggatgtccgaagatgatgtgatgcaggttcttgacagaaatacctgtactcagtacaccaatagaaccgattacgatcagccccttcgttgattccgcgatccgtttcatttcgtttcgctcatcaatccccgtttccccagaaatgtatacaacgttgtcatatacctttttgagttgctcatacagccatttaccatgtttgatctgattgaacatcacaaacacgttttcatctttttcccttgccagtttcaacgccagcttacagatccatgcgttacgcctggtatgcgatgttatatacttgatttcgctttggtaatctgcccccttcattttcttaatctcatcctctttatatctcatgaagatggtattaattcgaaggttggtaacttgaccttcctgcatcaaccgatttgtatcaactggcttgaagatttgaccaaaagcgccaatgtattgcatcatgtttgctttgccttctttcagagaaccagaaaggccaaacttgaaaatacactgatccattgtgttgatgatcttctgtatgctttgtccggttgatttgtggcattcatccaccatcaaacacatgaactgctgaaaccactcaggaggcattttaacagccgattgccacgtagacacgtagatcaatgcattactgtttttagcagttcctgaccgtattccaagcattgcctcgcgaggtaaaaggcgatagttgacgatatcaccgatcatctgatcaacaagggcagttgttgggacaatgattagtactttgcctgtgtaattttccagacaccaacgagatatcaatccctgaataagagatttacccgctgacgttgggaggttaagcacagcacggcggtttttaatcgcatgaaacaccgattgtttttgataccaatacggatcaatttgcttgtttccgtcgtatactgggtgttcttctaaccacttgtcaaaatctggctgggtaatttcttctgtttcgtggatcttaggatccatccagatagaatacccgcgagactccgcgaattttgttacaagataggctaaaccgtagggcagtttcccgttatagtccatcaagtatatgtagccgttccatccaccatatttgtattttgcctggtactgataacctggcggctggaagctgaaatagtcgcgcaattcatagactatgttagcctctgcctgaatctgcacatgactagtgttaaggaatttgacttcgatatccactatgtgtatcctatatacggtttatatgaatatttataggctaaataatgataaacattggagaactacaatgagtattgattacgaaaaggttgaaggtttcaaagccttagaacaaaaagaagccaaattacagcttgctacctacgcgcaagaaacgtttgatgtcaaactgaaccgtcagaagtcattcgaaaatatgcttgctgatctggaagctgccgtaccggaagaaaaaccggaactgttgatcgactcccctgatccggaaattgttacatacgaaggtgaaccatctgttcctgatgttgctccggaaattgccgaccagattgaaattgttccagacgctctacaagctcctacaagcgattctgagacggtttctgatgaactggcatggatggaagggtttaccccgtctatcatcatgatgggccgctctgtttcgaatgctggcttttatacgtgtccgtattggatctatgattggatgaaacaaaatccggattggtataagcaccctgatggttgtcctcattattcagcgcgtcaaaccctcaagtcactggcatggtacatgcaccgtgatgggatggttactgtacgcgaaaccagaaatagccagttcgacacgttcaaaaaataattttaaaaagtagttgaccttaccctgctgttcgagtatatttgtattcgaaggcgggggaatggctctcgcagtgaagaaggaaatacaaaatgaacatgatgaaaaatgcttactacccagttctgtttgtttgggctaatggtgaagttaagaaaatcgtcaattctaaagctccttattacactgtaggtgaagcacttcgccacgctgcggaagcaaattatcctgttcatgccgaacctggttatgctcgttggaacggttctaaatgggttgctgatacctgggacaactacgaagaagaaagaatggagtgtgatcctgattacgtatctcgtcaaatggaagctcatatgattgcagatcgtagactggataatgaagctcgcggattctattgattaacaaggggctacggccccttttcttttaggtgaaatatgaacttaaatcacgaatgtttaaaagatttgagcgatggtaacgagattggtaacgttatttttcttgatatcgatggcgttctaaataatatgcggtgcatgaaatttggtgaacatatggacatcgaatgcgcacgacacttacgccggatagtgaatcacgctaattgtgatatcgtcatttcctctacgtggagaatcggcaacagtacccataatctacgtgaaatattttatccgtggggattgtatcggatcattggtaaaacttgcactaacttccctcatagtactggaatgcgtggtgatgaaatcaaggcatggatcgatactttcggatgtaaaaactatctcattcttgatgatgataccgatatgctttcttcacaaaaagaacattttattaaaactgatgggtttgttgggttgaccgaagaacaatccacttatgcgatccgtaacattttcggggttactactccgttttgtcctgaatgcaatgggtatggacgtgttaacggctacgacaaatgcggaacgtgtaacggtaaaatactccggctataaataccaataaacataagaggctaaatttatggcaattccttctgtaacaattagcgccaacaaaaacgaacttttgattggcgaaactttgaccttagaggttgaaactactgaactagatccgggtgatgtgtttctggcctatcgttggcaaaaagacggtgtagatattccaggcgcaaccgccgatacttacacaactacggttgacggtacaactgctggtgattataccctgatcttaaaacacggtgctgatgaagaatcagcaacagaaaccacgtctgatacaatcaccgtgaccacttattctgatgatcttgtttctaaatggacggttcacccgattccgtggcgtgataccagctttaccccgatcggttattgggtacttgatgaaattctgtatcaaaaagcacagggtaaagattggaaaactgattatgctgattacaagtatagtgaggaagtacaaacgatcctgaaagcgttcatggaaaacggtgaatgtgagatccaggattcacgaaacggctatattcataaaatgagtgaaatctaagaggctttaaatggcaactgaaaaatggactacggttcatcctattccgtggagaaataccagttttacatatcttccatactggctatacgatattatcgttgatgcttttgagaaaggcgacgactggcgcgattatgcggaagaaaaatataaattagagtttgatactctgaaagaggcgtttgaagattatggtgatattcatgtaatcgaatctcgtaatggtaaactggttagtctgttgtcattgactcctgctcctgaaccagatcctgaccaataaaataaggcaaacaatgaatacacttctttttgatttcgacgacactttagcagaattttctcaggctttttatgataagttcggtgtacgtccggaaggaacgccaaaggaacgatatgatgaaatggcggcttctttggtgcgtactgatttttataaaaaccttccccgtattcaggctgggattgacctccttcaatggagtttccaacgccgaatcggtgatcctgctactttgctgcttcgcgcggaagcggtcagccctctttgggttatgaaagaaaaactgaactatacagataagatttgcgctgaactgggaatccctcgtctcgattttagtcgcattgactatccggaacagttcgcagaacatgcctatcgtggtgttctgatttcccgcaaccagaaacatcttgaaatctggaacaattctcatctagctaataaagttcctggtattttccttgcggaaaccctggaagaaaatattcagctagtcacggaagcgcttgcaaaggctaatcaataacaaaaaagggaaccgcaatggttccctttcttttacaatctttttaattcatcaagcgctgttttcttatcaccaacaaagaggattgctttacctcctgcttttctgaaaggcaacaccgcttttgcccgatcgtcaaacagaattcctttaccagcgaatgctgctttttcatggctacttttaacgtagtggaattctggaacgtaacccaatactttttgtaatgctttacgtttttgttcggcaacaccgtcagaattgaatttaccgacactggttagtattgctacatcaccaagtgttcttaaatgatggaataattcaaatccttctttgattggttccagattttcgtagaaatcagttttggcaatttttgctttgcactttttcaactcatcttctgtcatcatagagggttcgccatacattggcacaaatgaaccttcccagtcgaacaatacaccatccatatcaaagaaaaacttattcatatcaattcctcagtttgtgtatgcatactataatgtttaatcattaatgtcaaccccaagtgtcagttttcggtgcgtatgctgcaactttagccacaatttccttatccagttcagctacagatttctgaggcttaccacgggctttaactttgatgtagtttgacttaacaacaaacatccctttgttacttgatttcttgatctcgctatcaacaccaactttgttaaagctgatccaaatgtcgccgtccatatactgtttaagagaatcacccatgttcaggatcttcgccatagtaagggccgcgccttcgtgggtatccatgagaatttctttaggaactacacgatcgcgtttctggttctgctgcatagcaatatgcacatcgttcataacccatacgatatgtacgttttcttttttgtatcccagcgtttcgacatcacgtgcgatgcttgccagcttgctcatgccttttaacgttacgtcaaagatgaggttaggtttacgatcttctggtgctgccataataccggaataaacacggttttggtttttgttggaaatgttgaaaacgtcggcgatcacatgatggagggtagatacgttttctgggtttttgaggttcattgttttgacatcatgacccgtttgtttcttgatctctgctgcgagtttatcgctacccattacaagttttttcagggcgtcaacgtccagggtaataccttcgatgcctagcagtttttccagtgtgaatcctttaccggaaccagcaccgccagcaagaataacaacctgaccgaacttaggataagcacggcctccgaaggtgatcagcgcttcggttaaggtgctttctgtgaattgtttaaatgacttcatgtaaaattctccagtttattttctattatttattgacatgctttctgacagtggtgtatggttagggtgttcgacggataggccggaagaactttaaaccataaggtatatgatatgaaaatcaatttacatcgcttcattgtagaattttcccgcaaccgtgacatggactcttacaactattactcccgtgagattgaagatcgttttgcggctcatgttggattccgtcgccaccatacccctaaaatgcgtcctgaccacgatccgaagtatagccctattacatggcaagcccctatcgatggttatgttgaagggatccggatcatgacgtttaacgcgatgtatggaaacgcgttgatccatatcgcacgtgagaaaagggccgaattccctaacggatggcgtattgatgaagtgattaaaaaccttatgcagttacgacgtgaatacaaagcgggtatgtgtctgcgtaatgaacagtatcagatgtataaaacgtatgcatatatctctaagcacctaattaattccatgttttacatcgttggtaatcatggttccgctatagatatcggttcttatgaaatcgtggcttatgctcgcgaacaaggaaaggccgctgcactgaaaatcattgaatctggtgctatcattcttaaccatcgcattgatactattgcttactatggtgatcaggttgaggttgaaggcgtacaccatgaacgattcaacaaagccgtatttactaaaaatggttatgcgtatggtaatgacattataacttctgcggttcctttcgttcgtctaactgttgaaggatttggagaaaggttgtcttatagactgtcagaagctcaaatgtgcgcggctgctgaaagaatagccagaaagcggaaaatgtataccgatgaatacctggcgtatgtcaacaaaacaaaagaagatgtagaccgagaaatttcttgcatggatttatccatttgatataatgtaagcatctttttaagggaggatacatgaaaacgatacattgcagaaatgaaaacgttgtttattatcacggttcgtgtactgctgctggtattgaaagcatgttattgcctccctgtgattctgatactctgtctgaaaagggcagaaagaaaaatttagaccgtgttttctttaccgctgatatcgggttagctcgtatatatgctggaagggccgcacgttctataggtggggatcctgttctgtacagggttgtgtgtccggttgatgttgtatgcatgaacgaagacaaaggcgcgagcgtttaccatgcagcatgggcgttttgtgaggaattatgaatgataaagtgttggcgtatctcgttttcttgttgggatatcgcttagaagtgatgggcgcgtattcatcaatgtatggtgatttaacggctatctggatggtcgggttaggggttgcttttacattcctttcctttgcaattgttaatgaatcggaaaaggatattgtatgaaactatatcatgtgatctactctggtgttttaggcattgacaaacaaatgttagttgatgtaatgtgtaaaaaactcgatgaacgaattggaactcgatacaaaaatcatgtatcggaaagtattttcatcaacgttgaccatccaaatgacatggaagaaatggttaatactcttgatgatcagcagatcccgtttgttgacaatttcaacatgagcgctggagtgtatacggtagtaacttttgttctaaaaaatgttgacatccgaaacgatagcgtgttgaatgtagttgcaaaaatcgattctaccaaaggaaaataatatgaaaattgtacaccgtagcatttccgaactgtctcaagccgaaaaagtgcaaattcatttcaaattcaatgatttgcgtaaaggttatgccgaaattgcccgtgaacatgggttagataacggcgatatttaccaggtagtacaggaaattgaacgtatccgcgcgttccgttctgcaaatctccctgttaaaaatgcaatgcgccgcgaagcgatcgaaatccatcgtaagcgtgtgtacaatttagaacgtgctaaacgtccgatgaagaaagaaaagaaacctcgcccgtttaaacgcgaacatcttaacacctctatggcgctggcgtttcaagatgcggggattatctgatgcgtaaatctgcgatggatcgttgggctagtattgctacttcaaacgtaaaaccaaatcaagccgctcctgatgtagaagcggttcgtaaagcaaaagaacctgagattgtggcccttagccccgaactcattgagcatcgccgccgtgcgtctgctattgaactggatctgcgtattgcgcgttcatacaatctcaagcatgaacacgccgcaaagaacaaccattcttttgaccttactctggaagattggaaagtattgatgacaactgaacgttgtcagtattcaggcaagatgtttagcaataaacccggtagcccgtatgcccgtacaatggaacgtattaatccacgtctgggatatacacaagaaaatacaatagcggttatcaatgctgctaatgctgaaaaatcaaatctagatgcattcgttaagggtgatgtcattctggatgaagtaaaagtgaagttgctgcgtaaagcactttatcaagtcgaaaaacgtgtgaaaatgaaaggttaaattatgtttaagaaatattcttctcttactaaccattatgaaggtaagttcatcaatggtgtaattatgaacgggcttactggcggtgtgtgggttgcgcgtgaaaagatccacggtgctaactttagttttatcaccgatgacggaattaccgttacccccgcaaagcgtactgatgttgtgaagccagccgaagatttttatggctgttcagcagtagttgcaaagtattcaccagggatccgtaagatgtgggaaaccctcaaaaagaccggaacgtatgatgatttggttattcaagtctacggtgaatttgcggggcgcggtgtacagaaagatgttgattacggcgaaaaagatttctacgtattcgatatccgtgtaaatggtgaattccttccggataacctgtgctcgctgatctctcgatctcatggcctgaaaatggccccgctgttgggatacggtacttttgaagagatcaaagaactgccgatcacgtttgaatctgttgtgaataaagcaaatagcggcattggtagcgataatacagtatatggtgaattcgtatatcctatcatggacgttgaagagggcaacattgcagaaggttttgtaatgaaacctgtttcacctgcttttatgccaaacggtgaacgcgttgcaatcaaatgcaaaacaaccaaattcactgagaagaaagcgaagaaagcaacccgctttaatgctccggtttcactgtcagaaaaagacaaaaaccaactcgatgagtttgtttgttaccttacagagaaccgtgtgaaaaacgttctttcgaaactggatctggcttcgatcactgagaaagattttggtcgcattatgggcttaactgttcaggatgctatcgaagaaatcagccgtaatcacgggcctttcctcgaacagttcgaagacccagcaatggctaagaagctgtttgtaaccgaagcccaaaacatgattcgccctgtatggggcaaaatcctgaaccatgaattttaatcagattctggttgatgcaaaagcggctaccctgatcggtagccgtaaacctcctgaacgtatcgcaaacattgctgttaaaatcggacgtgctttgaacgaacgcgggatcagggcttattctggcggcgctcctggtatggatagtcattttctgtttgactataatccggataacagatgtataatccttcctgagaacggttttaacggccttttcgcaaacggaaaggatatcatcgactttcaagatttaaacacacagaaagccgctgacgaagccagaaaggtagcaggtaacttcgatacacagaatgaatacgttcaaagaaggtatgcgcgaaacacgattcaagttcttcgtgaaaatcttgacaatccaactgattttgttttattttgggcggaagaacgtgaaggatgtgttaaaggtggaaccgcgatcgctgtaagattggctaggttgtacagggttccatgtttcaatctcttcaaagaaagtgtattgaacgatgtgtgtgatacgttagggatcaatatcaaacccccaacgttggattttttatggtaattgaacatgcacccttacttcgtgaaacatacgaaagatgggctgttaataacgcaataggtgaaaatatgattcatgtacgtagtatcggtgctgacggcgaaactccagtagaaggccgatcccccactctcgcagaacgagcaagagaaattatcaacgatcagaatgctaagatgatcgaacatgcgcgggatacaatcacaaaaggtgttctgaaacacgcgacacaacaaaaccttatctatgatatgaagcacgatatcggctcttgtctgggtattgaatgtactcgctatgcattccaacgagtttctgaatggttggaagaagaagggctaaaattcgatacagaagaaaaacgcaacgccgctaagatcacaaattctctggctagtaattacaatcaaacgtatcgaaaccatgaagaacgtgaagtgttcggtttcaacattcctgaaaggaaaacagatcgccgtgtaagtgaattcactttttacattagttggtaaaaaggtgttgacgggggttggttatagtagtattctaactcccgtagacaagacactaactcagaaggataaacatcatggaaatcgtaatgaaagcaacttatgctggatactgcctggaagcaaaaggtgttgctaacaatggtaaaggcttacgggccaatgttgaagcaatgctggatgaattacatgcaatgtacgaatacgacaacgtagcgggtagcgttcttatccaggcgttggaagttgatggtgttgattgtgctggttggtgggatgcttacattgactacaacgataaccgggtttacctgttgagcaacaaagattatttctaaggaaccactatgagcgatgaagctgaggctttagaagattgggctgattttgatgacgaagaagacggtgaatatttctgcgttaatcgtggtgcttataaagaccgtttagaactccgtaaacttttatcgggttcctctcaaatatcaggatccaaacgaaaaagtagtaaacaaaaagttcagtatagtgatggttctgtacgtgatgaaactgttgttgctgaattccgtggtcgggttatcacaaaagaaagacaaattgatgtaaagaacttgtatgaagtggctaaggctgctaaaataggttctgtgattgtttgccctgtgtgcaaagaaaaacacacaaagacaacgtatcacaaagttttctgttcgaatggcagaaaaaccagtaaggattgtaagtctaaatatcacaatacaatccatcccgaacgactggatcgggtattttaaaataaacctaaaacgtggagtacgtttatgaacaacaaaactttcgaagaactgaacagcatcatcacttccgtagattcctataaggtttctcactggtcgcaatatccaactggctccgaagaggcgctgttttatattgaatctcgtggtggtaaatttgatcaagtagttacggctggctgtaaccgccttgcgcaaatcctatcacgtccggtgactatggaaaacgtagattttgctaatcggttgtacaaaatgcactttgggcgcgaaatcttcaactacaaaggttggaaagaaattgcagaactgggttacatccctcttgaattcagagcgattccggaaggaaccccagtagcggttaaaaatccggttgcaactttccacgctgggaaaaatgcgctgtggttagcaggacacgtagaaaccctggcgatcaggggagtatggttcccttcaaccgtagcaactctatcccgcgaatgtaaaaaagtgttgaagaaatatctcaagaaaacctccgatctcgaaggtgaagcatttgatatggtattacgtacccgtttgcatgacttcggcgcacgtggaacttcttctgctgaatccgctggtattggtggcctcgcgcacctgtataacttcctcggtactgataccgtagaagcgctgattatggctatctctctgtttgaagattgtcagaaagcgtttgatgatggtgaaatggcggctggtatttcaattcctgctcgagaacattccactaccgtttcttacggcaaagaaaacgaagaccttgcgtacaaaaacagtattgagatcttcggcgaagggatgtatgcatgtgtgtatgattcctgggattttaaagcggcggttcgccgtatcgcagaatataaagattcgattctttctaagggcggtactctggtagttcgtccggattctggtgatatggtagacaatatcatgtacgctcttgaagaactgggccgtatctttggctatacagtgaactcaaaagggtataaagtactacacccagcagtaaggatcattcaaggcgatgaaattcatggccctgaaacaatcaatcgggtgttgaactggatggagtctaaccgttgggcgtctgaaaacatcgcgtttggtatgggcggcggattgcttcaagaagttacccgcgacactcaaaaatatgcgatgaaaatgtgcgcaatcaaaattaacggtgtgtggactggtgtgtataaatgtccaaaaggcgctgaatggaaaaagagtaaaaaagggttgttgatgactatcactgatggtgttaactttaaaaccattgatactctggaacagaaagtgccggaaggctggaaagatgctatgatcacatactatgtcaacggaaagattactgcccgtgacactttagaggaaattaggaaccgtgccgggatttagtatccgcaaaaacgacaaaggaaccgtgattttctatgacaacattccccttgtagctcgcaaggggctttttgctaaaatcgctgggtattcctttaaactggaagaagtcaacgacgaaacactaaaagagatcgtaagaattgccttacaattaagaggtaagaaagacgaacagaaagctattgacatgatcaataaattgggtgaaactcaatgctttatagtgaatcgtggttacaagtacgataccattgcaaaatttgaaaaagggctttgtgaattatgagttattatggtgtgatcccatacacaggaaacaagcaatcgctattacctgaactattcaagctgttccccgaaagaagttcatacatgcgtttcattgattgtttttgcggtggccttagtgtgtcgctaaacgtccctaaacccgttctaagcaacgattatgataagacgctgattgatatgtatgagcgtcttaaaacgcttcctgacctgtctccggtgcgagaattgattgcatcgaaggggctggggaaagacaagaaagaagagtatctgaaattccgtgatgaatacaaccagaacaaagatcctttatggctctatgtcctgatcctgcattcattcagcaacgttaaccggacaaacgacaaaggcgattttaacgctgctgtaggaaaacgaaccctcaactttatgacagaaaaacgtttcgaacatttcaaaaagaatgtgacaggaattgaatttcgttctggttcatactctgatattgaaatcaacgataacgattttgtttattgcgatcctccgtatctgatcactgatgcggtgtataacaaattctggaacgcagatcacgaacgcgagttatatgctttccttgactccctgcatgagcggggtatcaagtttggtttatcaaacgtgacacatcatgcaggaaagcaaaatgatatcctgatcgagtggatgcaaaaatataatgtgcataacctcgataaaaagtatctgttaggccagcatactgattcttacgaacaaaataaaacgcaagaagtctacgtgtgtaactaccagaaacgcgacgtaaatacataccctgaaacactggatgacttaatgtaaggtaacatatgtttaagatttttggttatatcccttctgtttataattgcgctccatgcctgaattctaaacgtctcctggacgcaaaacgaaaagaatatgagtttgtttctgtagccgatgaaaaagacgcagacggcaaaccgatcctgaatgaaacggtcatttctgaactcgaaagcctgttaggtactcgtagactgaccatgccccaaattttccacgatggtaagcacatcggcggctttgaccaactgcgtgagtacgttcgcacgttgggataaatattaacacctttatttgattggtgttattatgctcactaaacgtattactaagaaagattatccatccattaaacaagctctttttgaacagcaaaacggcttgtgcgcgttatgtggtcgccctttagagggtgaccttgaaaaacatcaccttgaccatgatcatgctctatctggctctaatgccggacgtgtgcgcggcctcctatgtaacctatgcaacggtacagaaggtattgtaaagcacaaatttaatcgttctggtctggtttcccgtgatgttgattacatcgaatggctagaaagcctgcttgcatatctgaaacaagattattccgaaaaccgtattcatgacaaattcataccagataaggtaaaatggttttcaagacttaccaaacctgatatgattgccgaaatggtttctatgggcttcgagtacgccgacaaagacgaacgcaaagccttaaccgcaaaatatagaaagcaattaatgaaggcaacgaaatgaaatatctaaacgctcgattatcaacgcaacagaagaaaaagctgatgatgttgatatcctccactgacaaaaagatcatatctctacatgattggatgcttggaaggggtgactctgatttgtgttatgtcaaaccgaaagaccgaacgatgtttgatgatcgcggtcgcacattgactaatttttctcctatcaccgttattgatatgtgggaactccttgagattgtaggacgggatatacctgttgacggggttgaactgatcaaatatcttaacgagattggacacaatttagatattatccataaggcaacgaaatgaaagtagaaaaacgcgacggcaaaaccgtcgatttcgatcaagaaaaaattcgcaatgctgtgtataaagctggcggtacgatgacggatgctgactccgcgatcatgcttgtgttgcgtagtcagatccgcaacggtaaagcaatgaagatttcacaaattcaagaacttgttgaagaatctttaatgaagacaaatccgactgttgcccgtgcatatatcgaatatcgtcatgatcgtgatatcgcccgtgaacaaaacggaaaattattccgtgatatcaagggtttgatgactcttagtaacaaagaattaaccaacgaaaacgcaaacaaagattctcgcgtattcccgactaaacgcgatcttctggctggtatcgtttctaaacatatggcgcgtaaccatattctaccgaaacatattgttgcggcgcatgattccggtgatattcattatcacgatctggattacagcccgttcacgccatacacaaactgctgtctggtggatttgaaaggtatgctggctaatggcttcaagatgggtaacgcagacatcgaacccccgaaatcaatcggtgttgcgacggctctcatggcacagatcaccgcacagattgcttctcaccagtacggcggaactacctttgctaacgtcgatttagtattggctccttatgtggagaagacattcgctaaacatgtacgtgatgctcgcaaatatcaagtagcattagtaaaagattatgctatttcaaaaacagaaaaagacgtatttgatgctttccaatcgtatgaatacgaagttaacacgctgcatactgccaacggacaaacacctttcgttactattactttcggtactggtacgggaatgtttgaacgcatgatccagaaagcgattctgaaaaaccgtattcgtggactgggtaaaaagggcattacccctgtattcccgaaactggttatgtttatggaaaaaggaattaaccttgatccagaggatcaaaactatgacatcaaacaacttgccctggaatgttcttcaaagcgtatgtatccggatattattagcgcggctaataaccgtcgtattactggctctagcattcctgtatctcctatgggttgtcgtagtttccttagcgtgtggaatgatgagcacggtaatgaaattcttgatggacgtaataacctgggcgttgtgacaatcaaccttcctcgtattgcgattgaagccgaagcacaggaagatgaagacgcgcatgatgcattttggcgtatccttgatgaacgtctggaactgtgctttgaagccctgatgactcgtatcgatagcctacgcggtgttaaagccagtgtagccccgatcctttatacagaaggtgcgtttggtgtaaggttgaaacccgatgatgaaattctggaactgttcaaaaatggacgcagttctatcagtctgggatacatcggattgcatgaaactctgatgcttttcggatctggacaacacccattcgaccggatcggttctcagaacatgggtagactgattctggaatatctacgcgctgcgaccgaagcatggaaaaagaaaaccggatttgggtttagtctgtactcaacccctgctgaatctctatgtcatcgtttctgcaaactggactatgagaaattcggaagtatcaaagggatcacagataaaggctggtacactaacagttttcatctggacgttgaccgcaaggtaacaccgttcgagaaaatcgactatgaagccgattatcattacattgcaactgctggacatatcagctatgtagaattccctgatatgaaaaacaacctggaagcccttgaaaaagtctgggattatgcaatggataaactggactacttcggaactaaccttccggtcgataaatgctttgaatgtggctctgatgatgaatttaagccaacagaagacgggtttcattgtacccattgtgggaaccatgatccggaaaaaatgagcgtcacgcgccgtacatgcggctatttgggtgctcccgctgtccgtgggttcaacgaaggtaagaacaaagaaatgatgcatcgcactaagcatcaaaattaatcaaaaagcccttgacttcggttgagggcttttgttatattgggcctatcgaaaaggagacatactatgaaactgactaagaaaatgaccgatgtagtggcatgtgcgtttgcattaggctacaaagttgaaaatcacccaactcgcgttgaagtcatcaaccctatcaagggccgtcctggtttggttctgtgtgaagacggtacagcatatcgtaatgatgtctctttagaactggcaactactatccgcaccgcaaaacaaatgaaagatgttctcattagcggcgcaaaattgagggctttatgatgtattggacaaaagataaatttgtttttcgtgatgatacgtgctttgggactgcataccgaaacttggctattcgtggcggttcgttttcggctaatgatttgtctaaggtagtatttcctattaaagttactgagtatgacgtattcggtgttaaaggatttactgattactttggtacaaagtttgaatcagaatcttacatttttactaatagcgatcgtgaattattcaaaaaacacgttgttgttaaagagaaaccgttattaccaaaagaggacgaagcaaaggaaatctatgatctcctgaacatgcttgacaatctcggtacttgtcatctgttcggtaaacgcgcccgtaaagcgaaagatgttctcaacttgttgcgctctcgccggaattatctgatccgggaagctgaacgcaatctgaaaaattcagaaaaacaggctgaaatccataaatcaacccttgctaaattaaaggctttgtgatgtttcctttatacgctaaagtgcgtcgaaatgtcgggaattcatatcaggaatggagtgaatggctacgtgaaacaaagtcattctacatttcaaaagcaactgatatgaaaggccgtaacattcgctatcgtaaacccagtggtaaacgagtgaatgggatagattacattgttcttgattcgattcgggatgatatacgataatttaactttgaggcaatattatgattttcaacaaaacaaattcacgtaatttgaactatctacgctgtgaactggaagctaacgaaattgaactgtttttctgtggggctacagatccggaacacaaattgcattgggtatcaggtgagattgtaagcctaaccgaccagattgttgaagaggctacccgccgcgatgcaatcgttaaaattggtgctgttgatgtgaactacgaaggacatccttcatttttcattcaatattatccataaaagtattgacctgtatatatgaatgtagtaacatccttcttgtcaactaaggaggatgttatgaaaatcaaaaacactgctactgaaactctttgcaacgaaattgcagaaatgtactggagtaaaggtcacttagaggctatgaaagagtttcaaaagtggtgtgatacccaaaagttagctaaatgggaatacatcgttattgttgaacggatcaaagaactgatcctcgtgaagaaaggtaataaataaccatgtaaatcaacatggaacccaatatgaattatcaaaaaatatacgattctctcatatcgaaatataggggagaatctccaatatcttacagacacaagaaatcaggttacgagattcatcacatatacccaaaatcaatgggtggatctgatgaaccagataacttagtatatcttacaccaaaacagcattatactgcacatcatcttctgtctaaaatatatggcggtagtatgcataacgcattttggattatgtcattttctcgtgggtttcctatcacagcaaggcagtataaaactgcaaaagagaataaaattctcaatcaaactggaagaaagcattctcctgaaactatagaaaaaatgataaaatccagacaaggaagaacatattctattgaatctcgtagaaaaatgagtgaatcccataaaggatattctcatagtgaagaaacaaaagagaaaacacgaaaaagctgtttagtttctaaagctagatttgtgaaagttgctatcggaacgaatatcaaagatccgtcaattgttatccggctgtgcggcaaaactgatatacgcaatcatggattcagtcaaggcaaggttcattcttgctgtcgtggtgaaataaaaagttataaaggctatacatggagatttgaatgaattatattagaatttataacatggatgtggtcaacggaaaagggatccgcgttgttttgtttgtggccgggtgcaatcataagtgtgatgggtgctataatcgcagttcatggaatccttgcaacggaacaccgtacacggaagagacagaaaatcatctgatttctctgttgagtaatccgcatgttgatggacttacattaactggcggcgatccgctttaccgtgacaactatcctactatcctaaaacttcttgagcgcgtttctaaggaacttccaaagaaaaacgtatggttatggacaggatataccctggaggctttacaggccgacccagaacgttctaagctacttccttacattgatgttctgattgatggtaagtatgaaaaagatttaccaactaaaaagccttttcgcggctcagataatcaacgtatgatcgaattcgctaaaaattcgatagaaattaaaaatattgcttgacctaatgtgtaactatggtaatcttaccacatcgtaaatgacgattaactttaattgagagataatatcatgatcctgaatttcaaaacccgtaaagaagcgcgtagctactgctggaagtggaacattcccctgaaaaccatccgtaatacagggcgcggttcttgcccgtggacagttcaagcaaacgaactgaaaacgttcgtggttggtaaaacttacaaactggttgaccgtgaagggtttactaccaattcacacggcggatctaacaccgcaaacactatccaggcgatgcagatcgaaaaattcctgaataacgaggtaaaaattatctcgaaaatcaattcagatactttcaaaattgagcatactccggaaatgacttttagctctctgcgttcgtgggaagctcgttattttgtcgaagttggcgctgctccggttaagaaaacgaaagccaacccgaaaaaagccaacgttacggctccggttgcgcctgtttcaccagcaaccgcagatcttgatcaaatgcttgatggtggttcggcaatgtcggttgaactggattctactaaatttgttgaaggccgttcgtatgttctggttaaaccgcagcaatttaaaaatcgttgtggcgctaaccacgggatcaaatcatataccgatgaatacagtaatggtgtatacaccgtttaccatacgacttcgctcggtcatcatcaattgagcaaaacggtagaaaccattgattcccagaccggaaaagttggttactatctgcttgattctgaacgttcgttcttccgtgaactggcgacaggaattgttgatgaacctgttagcgtttccggtaatagcgctatcgctatcaatgtagacgaagcggctaagaaagaagaaatcgcaaaagcaatgacacagcttgaagaagcggttaaggcccatgatgacgcgcttcaaaatctgcgtactgcttccgacctggttcgcaaagctgctcgaaaagtagcagaagtaagcaagtaaattaaactgggtgctccggcacccttttttatgaggtgacacatggaattattagaaggtaaatcttataccctgaacatcgacgctaaagaatttgcagaaaaaacctggcgaaatgctttagctgaattgatcaaaaacaacggctatatcacaatcgatcgtattgcgattggggatactgaggacattgcttatgttctgcaagatgatttcgaatacgagatccctagccatatctggaaatacttcaaaccatatgatttgccggaagaagaaccgaagattgctactaaagaagaaatcgccgcgcctgttttaaattttgtatcttctgatcctaaactgtggatgactgtaaaacctgttcaacaagatatcaatgatctgcgatttgattatccttttgtcaagcggatcacttcgatttctgtactaccagcgccgactgattcacaggcacttgaatttgcattacagcatgttttcggtgataataagctgtacgcgattaacaaggaagctgctattgatgaacagaaaaaggaaatcatcaaccttctttctctgcatcaacaacttgaagcggtggaattgattgagcgtatgctttctgatacaaagaaagatatcattagcaaaatcactccggcacgaaggaaagcaattgatgaaaatcgagatttacggtattcccgaatcgcttcataaatgttacggctgtattgaagctcggaaattacttgatgagcatggattagaatacgaattttattctgttctaaagccagcaaataacagtgtggggtttgattacgatcgaccccgcattgaagagttagcgaaacgtgttcgtagtcgaagcatggcatttacttaccctcggatctttgtagatggtaattttattggcggttatatgcaattgaaagagtatttgggtgaagcatgaataaagaatacattcgcaaagtagcaaacgctattcacgcaacaacgattgattttctggaagggtttgatcatattatccaccctgaaacgctggatagttgggaagccaaactgtttaaaagtatcaatgaacagtttccggaaaaggttaagcgctggtttatcagacaggaaatcgtagcaacgatccttaatgaacgtggtgttgaggcgttcggtgtaacccctctatataaacgaaaccagattacagacgaaacaatcaagaaatataaaaagatggttcggaagtaataaataatcagttaaatggccttcgggccattttttgtatataaatattggtattgaatacaatataggaaaaaagataatggtagctaaatcattccgcgcacgaagtggccttgatgctgctggtgaaaaagttatcaacgttgggaaggctgatcgtaatacgctgagtgacggcgttaacgttgactttttcaatgaatttaacggaatccagcagtatgacccgactcgtggttattctcaagacatggcgatcatttatgcgcgtcgtatctggtacgcaaaacagaatattgcttcccctgctggggctttcgacgaatccaaatggatcgcaactcgtaatgacccgaaatgggtttatagtaacgtaaccactccagacggtagcattattgaatctggtagttacattatggctgatggacgctttactgaacttctgtacctgctgccggacaacccgacagagggcgacgtaatcacgtttaaagattgtggtggtttagtaggtgtgaacagtatccttgttaagtctaacacccgtcagatccgtttacgtactgtacaatcggcacagtatcgactgacccacccgtacatgatcgcaacgtttatctataacggtaacgtatggcgtgttgctgaaactctggataaccgcgattctgagatcgtgaacgcaaccggaacaggttcattccagttacaatctggcatgacagttttccgtaacagtgctacaggtaaaatcactctccagttgccgaaatatgcaaatgatggtgatgtgatcacaacctatgacgctgataaaatgaactctatcaacgtagccgttttgcagatttatccaggtagtggacacactatttctgacggtgcaattactggtgttacttcggtaactagccagaaatctggctttggtatgttcatctttgatgcacagaatagccaatggaaagtatatgatgctgataatcgtgttcgtctgcgtcgtatctatagtgatttaaacacagttcctaacgattacgtttttgttactgcaaacccttctgggactataccaaacgttacagttacccttccaactgatgttgctgatggtgatcgcgtttacgtatccctttatatgatgggtaaaaaccagaactgtacaatcaaagttaaagatggtacaacggacaagatccgcaccaacaaaaatatgatgcagttcccgcagcgcaaagactatccgcctgatgattggtttagtgtaacttcattagcatttaatgctgctagtgattacctcccgtatatcgagttttcttacatgaaagctacgaaagaatgggttgttgctaattatcgtccgatcgttgaacgtgttgacgcaactaacagatcgcgtactggtgttattgctctggctgcacaggcagaagtaaacaaaaacttggaagacaacccgaacgacgaaactgctattactccgatgacgttagcaaataaaactgctacagaaacccgtcgtggtattgcacggttagcaacaactgctgaggttaacaaactttcaaccgatacctatctggatgatgtgattgttacccctaagaagctgaacgaaagaacagcaactgaaacccgtcgtggactggcagaaatcgcaactcaggcagaaaccaacggaagcaccgatgatattactattgtaaccccgaaaaagttgcataaccgtattgcatcgccgaccttgactggtatccttgcccttgttgctactggtggtgctcctaacaccaacacggatcgttctcaggctggtactggggtttatgaccattcagattatcagaaagcggtaacgcctaaaactcttcgtgagtataaagcgactcagttacaatctggtgttgtatggctggcttctgaaaccgaagttattaacggtactgttgcaagttcaaacgttccgaccgttgttactccggaaatgctgcacaagaaaacctctactgatggtcgtattggtttgatcgagattgctacccagacagaaaccaacgcagggactgattacacgcgagcggtaacgcctaaaacgcttaatgatcgtgctgcaacggaaacgctgacaggtatcattgcaattgcaaccactgccgaagtatcagcaggtactgtaacgaataaagcgatcgtaccgtctaaactgaaaggttatctggacgatacaagccatattactgttgctactgctgatgggttaactcaatctggtactatttggactacggttaacatcggtattcaatcagcaactgaaactcaacgtggtactttacgcgttgctacgcagtctgagacgaacgcagggacattagatacagtatttgtcacccctaagaagttacacgctaagaaagcgactgagagcgcagaaggtatcattcaggtggctacggctgctgaaactaccgctggcaccgttgcaaacaaggctgtttctcctaagaacttgaaaaatacaattcaggttgatacttcatggcaagctaccgatctggtacgtggtactgtgaagctgtctaaggggcttggtacttggtctggtaatgatgtggctggttctactcttccggatgatggttatgccgctgtaggtgttgctgtttctccgtatgaactgaacttaacactgaaacactatctaccgatcggtgctaaagcggttgatgctgataagctggataatctggattcttcccagttcattcgtcgtgatattgatcagacggttaacggggcattgactctaacgaaagaaaccactgtacaggctaacattaactcaaccgccgacgcgagtttccgggtaatgaatgttagtggagatctgaacgttggtgatggctcatcgatgggtaaacttcgtttgaatggcggttcatctaacgactggtcaattcaagcaagttcatcctctgggcgtattgcaatgatctcaacgggtaacactggcacagttcatctttctgtgtataatgatactcgcggcgttgtagctaacgttaaattccaggctcctgaaattcaggcgattggcaaagtgactctgggtaatgatacagtgatcacggctgctggttctgttctctctatgggtacgaacaacaagacaactaagatcctaacttcggacgctggtaacattttggcagaagaatcagggaactcttataaagtctttactgagaagaacgcgcaaaccttgctgaatcctacgtatgtacgtaaagcaggtgatacgatgtctgggcgcttgacggtaagcaacagttcaattatcattgcaggtcaagcggcttggtcaacgctggatgcagtaacagaagcatccaggggcaactggacggctgagatcacagcatcggcacaatacaacttgcttcctggttatgcggttccggttcttgaaccagatccgattaatccagaaatcatgattgtgacccgttatacctatgttaaagcaccgggtactttaacgcagtttggtaacggaactgcattcacttatcagatttgggcacctcgtccgacctctggtactggtgttaatgcgctggcgcaatccttctggatccgtcaaatgaacccaattacgggtaaatttgatggttggggccgcatgtatactagcaacaacccgcctactgctggtgagattggtgcaacgtctgctgttggtactacggttaaaaacatgactgttaccgattggatcaaagttggtaacgttaagatttacccagatccagttactcagacagttaaatttgagtgggtggcataatgtcaaacttaatggcggggttcggccccgattttgtagaaacgcaaattctatcggaaacaaacagcgtaacttacagaataaccgcaaaggcaacacatcccaatgcggttcctaatcagtatgagtttacactaaatcaaaaggcggtagggacaccgcctagtgttgggatcaacgtatggagaattaacaatgctgtagttgatccaattaaaaccttcacattatcgaatgataattcagcaactgcaaataaagcgtttgttgaatatatggatgctcaaccttctgggctgtatttgataatgactaacggtgaatacaaaacaagccaaatcgttgatgattggtttgctaaaaacagatccgttatgtggcaaggcgctgatttcgctcagagattcccaaattctgcatatgttgcattgtatggggcatcaaaatctcgtatactgattgaatcgttttacgctaacgatggaattttaaaagaagattcacgcgcatcaatcgatcttgtctatgataacgttggtgatgttgggcgaactggtgtacccttccgatctgttgaagatacggaagaatacaattcaaccaatggatctgaatataaagtatatcctgttgcaaacccagtgatctctaaactagctgattacggtatggctcctggattggctatgatgattactggtgatttttacgcaagtaaagcattattggatgctggatcaacaacaagggttactgttcgatggtttacgggtactgctcaaacttcatcatcggtgattgaagttcctgcaaataaacctgatgagtggttacgatttgaacagttctatacgatccctagtggttgtgatggatttaacgttgctgtatctcgttatcctaaacccgctacggatagtttatctgcgatccgtaacttcgtgatggttcaggtatctgctgccgaagccgatcaaaactttgctgcacagtttggggttaacggtatcagaatgaacaacatgatcgatggtggaacaccgtatatatttgaattgccgaatactaaggtttatcctggtggcgattatactgcttccgaattccgtgaagttgatgcataaacaaaggcccggatcatcgggccttataaatatgtaaaaaggggttattatggcagatttaaaagctggttctacagtcgggggtttacctatttggcactccggcacatttccgctggttccggttggtaatactctaacctatcgcggatataaggtttatactgaaaacgataaaccgcaagcatcaaataacgacttcgtttctaaagcaagcggtggtcaatatttgggtgtagttgcctttaaacaggggctacaaattaacgctactttcacaggcggaagtgaccagaacggtttatattctggtgatggtgatggcgcgacattatcaaaagccaacattgatcttgtatcatggtatggtattggtattcgttcatcttttggtactaatggtcgcgtattagtcatcaacgctcgaaatggtgatttaaacactcagggtaatattacggttgaaaaacaaatcagtattacaaccgctaaccctactgacgcaagtcatgcaacacgaaaaagttatgttgatggacagataaataatgtcacaacaaatgctaatagcagggtattacgcgctggcgatacaatgacagggctgttaactgccccgcaattcgcgagcacaggcgcggcttcccgtcccgaacacgtaccacggctcgaccaggtaattactaaagggactatcatagattttggatcttattaaggtgaaacatggctgatttagaaaaaattcaattcctacgtagcacagttgcggggaaaacacctactacaagtcagcttgcagatggtgaactggcgatcaacatggctgattatgccatttacacgaaaaatggttcttcgatcgttcagttagcgggtaaaggtatcccagaaacaaataccaaaaaattaacagttgatgggcctagtgctcttaatgataccgttaccgtagcggaaggtaaaactattactttcaccaacgagaatttaagtggtgaaataactcgtcatatcgtcggtaaatgtgccagcaatgatggatggtacatcggttccggtggtacaagcaataacggcattcttgaaatcggtactattgacgatggtactgaaacaatccagtttgtacaacgcggtgctggtaacgttgaagcccgaaaattggtcttgcttgacggctcgggtaatactactcttcctggtgagttaagattaactactaataagactgttaaaattaacaatggaagcacacttgtccttgaaatgggcgtaggctctaacgatgcctatattaaaaaccaaagaggcgtaggtgttcttcaattaactaatgatagtaacctgacgttcagaaattcccaggtttattatgctatgagtggaagaggccctggtaaagatggtactcttctgactaatgtagaaaacgcgcgtcagcttgagcaagataatttccctgtaactacaggcaacgaaactcgttggattaaagttgctctgttaaaagatcccggctcaggtacgagtcgcttgcaactgatggtgactaacggtggtaactatggcaatacgcacagttctattgactttatcgattgtagcgctagaagcattcccgcaacattaacaagcgcaaacattagttcttatctgcaaattcgtcgaatcggcgatcctggaattgataacactaaccaaatgcgttatagtctggttcgtacctccgaaggtttagaactgtggtttgctcaacgcgcattcattggtggtgttaaagttgctctgctgtctatcgctggcggtactgttactgaatattatctgcctactggttacacaatctctgcaactgctccggaaggtttagttgagagtgtggctattcgtatctatgacgaaatgaataaacctaaccttgacaatggtactgatggtattctgtctattgctaaaggtggtacaggcgcaagtacagcggatgctgctcgtacaaacttagggttgggtactgctgcaacccgtgatgttggtacaggttccggacaagtaatgctcgttggtgcttacggtttaggcggtaagggtacatcatacaccgttgctaactctcgcgattacctgaaacaactgcgtgctgatggttctcagttcatgcgaaatacgcttggtactgaaattaactatggtatgggtgcaagtttttatagctctgtatcagatgttcatgcggtgatctcggttgactgggctactggtcgcgttaaagttggtgcaactaatgatgctaacttaaactcagataccggaaaaatcagctctcaggaactgtacggtactgcatttaaaccaactccggatgacgtaggggctgttgctcgtgctggcgacaccatgaccggtaacttgactattaaagctaacttaaaggtcgaaaatcctaatggaacgatggttgatttaggttcagagaactcagacaagtacagcagattaacccttgcacgtaaagttggtagcggtgctaccgtagcaatgcttaaagttactcctgaaggacacgtgcaatttggttatcaagatgcagttgctactccagctcctagtaaatatattctagttaaatccagcggtcttgaggtagaaggggatttagtttttaatcagacctatcgcggcaccgaagaggcagttgatattactgataagactgttgaccttaatggtcttgtcattaaaggaaccgacccaggtactcgtcagatgtataaatgcttctcatatggtggtggttctaatatatcgaacaaacctacctctgacggcaactttgttcttgaagttctatctttgcgtaaaatttctgatactgattggacttgtaagcagacctttactacaaaaggtaatgttgaaggtacatatgttcgatactgccaaaacggcacatggtctgcatggaaagaggttgttgcaggggttcagccaattaatttaggtggtactggtgcaacttctgtagatgctgctcgtaataactttactatcggcaaaacccaatctgttgaatttggttctttaattttaaacggcgtcggcgataacgatgctactttagattttaaaggcggtgctagaatacgtggtggacagcgcaccggtgagggcgctatgatcctttcagccgcagcaggcgcggttggaaaatatatcgcttttcgacccttcggtgattcgtctgttactgagattagagtaaaagccaatgagtcaagtgagccattacttgagtggtcttatggcccaggtattcgttcaaattcatctggcgcttttgttatctacgcaaaaacaggtcaggcactccatttaagaccaaacggtgataattctaaccaagccacagttattgaccaaaacggtaaaatgacagtcggtggtgaatttgaggcccagaactcaaaaatcactggtaatttgaatgtatctgaagataacagaatgattgttcttggcagaaataccgatattggtttagtcaagaaaagtaatatgccaggaaaaatggctatcagtaaatctaactcgtttactgttatggtgtcaaccaataccaacaatcagattaatcctgctgatacgtttaatgatatattcaaagtagatgctgatggaaaccagactgtttacggaaatgcccaagtcaacagacagttaactgtttctagttcagctactgttgcaggtgttattaatgctaacggcggtattattgttcctactaccaagtatgtgcaaattgccgatgctcctacgcagaataaccaagccaccaacaagaaatatgttgatgataaggttgcttctgctattagtaacgctggtgatacttatcttccgttaactggtggtactgtaactggtagattaataattacaggtgatcagttaaaaactacatcgctttgggctactggagacgctgctgttaatggtgctttaactgttgacggtaatgttgttagtaattacggtattggtagctttgttggtgctgtagatgttaaggctcctgctgcggataatggtacaacacacctttggttccgacattctaacggtggtgagcgtggtgtgatttatatgccgcgtgacaataataccatgatgggtttaagagccggtggaagtgaatggcaattacatggctctgcaggccaaatggtagggccaggcgcacgctggagaattcatcctgatggcaacatacagggtgatgtttatggtggttatatcactaactatatcaacgataggtttaaccaatgtgctcaatgggttcgtactggtgctcaacaagactttggcccaattggtcgaccggcacctggtaaaactgttcctgctggttgggtacttgttggtcttaacggtaacagcaacgaagctaaccagaacatgcaacttatcggcggacggttacaagtatggaaaccgggcgttcaatgggttgattctgctacttgataataaggggcttcggcccctttaaacttaaaggtaaaataatgattgttaaacaaatgaaaggtattaaatggcatcacaattttgaaggtggtgcttactatcgagattgtaatgataagtgttggtattcttttagaaactctcttgataaaaattcccatattattatcgttgatgctaaaacaaataagataattaattactacaacggtgaagatcctactatgataggtttgtttgctgataaagaaatgattttagatgtatatcagctcgacgattttcctgttgattcgtgggatgaattctcaaaaaggaagttcgaatttatcgatggcaagaccataatgactaaagatgttgaagttgaaaaagaaagaaccaaagaagacatactggcggatctaatcaagctacaaaaagaattagaatctatgtaattttaaaggctaccatacaggtagccttttgttgtatcctaaatatacgtatagtaacctaagaagagtcttataaaaatggctgagagaaatcccgtggataaactagccttatttgatcgggtaatctcgtttgtgatgggtgtgaaaacatggaaacaattgctgataaaaataattctaataatggttatgtttcttatggtagtaacttggtacaaatggactgatatattcccgatgataaaaggtgcccttgtagtcgatacaagggctatcgaaatggaaagaactgaaaagtttaatcaatccgcgttggaacagttgagcatagttcatcttacttccaacgcggatttttcagcggtattggcattcagaccaaagaatataaactattttgttgacattgtagaatatcagggaaaattaccatcccagatcgatcctaaaaacctcggcggttatccgatcgataaaacatccgaagagtacacgaatcatataaatggcttgtattattcatccactaaagcaagttcctacctaccgacgcgtgattttgtgccagtagcttatacttttagttgcccttattttaatcttgataactactattctggatcggttttgatggaatggtacgcaaagcggcctaatataccagatatgaagctaaacatcatatgtggacaggccgcgcgtattttaggtcgagtgaggtgattaacgtaatgctggtgttaaattgtgtgttcttccaatagcccgtttgattgctttaaagaagttcatcaccgggctatttttctcgtaaatatcccaaactttcaatttgtcccacggatccggaacataatcttcattccttgccgaaacccccaacgtaaccctcctgtatccagcgctgtcgtgataatacacgaagaatggcctacctattggcgcaactttacaacctctcttagcggctctcatagcctcatcgaacgtcattgatacctccaaaaatttctatgcatgtttggtcgaattccgatagtttcactcaaaatgaatatcggatgatctagctcatcgtggttttcttcgtcaatgacgatatcccaatcagtagccttttgttcttctaccgtggcaatgaatacctggtttacttcacacttgcggtgtgtacgtctgatgattgtatccccttcacgaaacacaatcatatcagggttggtagtgcggtacgcggttttacccgcgcacacttcattaagcatatcttcgtatgtcattataaaacctttacacgttgaacgatggtttgtttaacgtctttgtattctccgtgctctttaacggttgctttgaaagtgatttcatcaccttcgtttgcaatgttattaccgaagtaaacaacaacattaccatcaacattaattttggtcatgaatctttctacagaagtgtagtaagaaacttgagtatatcccagtgaaatcactttctcaacggttccggtcatttccagacgctgtttgatttcaccgatgtggttagctttagaaatgcgttcctggcgctcttgttcccactgttcgcggatttcttcgcgtttggcgatataatccttctccagtgcaacacccatgcagtaagcacacacggcgtcaaatacagggctgtttttgttgtcttctttagactggtcagcccaccaaagaacagtaaacattggcatttctgcaattacttcgcctttacgcttgccaatcggcatgatccctttttccagcagttccagtttttcagtatcgaacactgacagtttaccgcgacgttcgaacagatcgaaatctgcaaagccctggaataccattttgaaagtatcagtttcagttaaacgggctgaaacacggtcgaaatactcacgcgctttcgcttccgctttctccggatcggtagataagttgcagatatagttatcagaagtataaccgccacctctacgctcaacacgcaaggtgtacattgcatttttacgaccagaagaaatgaagtaagtggtagtaactacggttgcgttagtcatggtatttctccttaaagggtatctcgtttcgatatggctaatatagcaaaagcccctgaccgaagtcaagggctttttaatcattcattcgaatctttcattgttttatgaagatgaatatcaaaaattttccagtacgcctttccgcgaggataaatttttgctttgtcaatatcgttgttgcttccccatgtgttgtttgggccacgacatcgattttttatataatctgtatgccagaataagcgctgaaccgatgattccgtacctaatggatcttctttactgaacagaatttgtatactcataagaagaaccctgttctaactactaaatcgatctgtttttccggtatcagtggcgcatctgcatcaacgttgcactgataatacatcccgacatactcatgaggaatgttggattcactcgcccatgccaggttgtcgtctgtacgcggccctaacatgaggttaacgatatcgacagcgcgatcctgttctggggtgttgttgcatccgttcacataatgcccgtgagcggttttgaggatttcaatgatatcttcgtcggcttcaacgagatacagccccgtgttttctgggatttcctcaagaataatcaaagcggttttcatcacacttacctttatgtttctgtttacgttttgcttctttaagtgctcgcttgcgatcgcggtgagtagaagcgcggttaatccatgcatgtttcgctaccagattgttcatcgaggatataatggcacatgatgttgaatactgacttcaccatacatttttacgatagttaagctatcagatcctttaacaattctgtatttttctggaacaacgcggtcgatttcttttttgacgaagttaagcaatccgaagtcatctatatcttttggtgctttggaaatagaagacagcgatactcgttgacgcgaatcatagtacgaagaaattacaaacatatattattttccttattggggcttttcagccccattttagagaattaatccagcagtttgcggatcttgtctgcgatacgtccggcgcgggttgcacttgcagtatgatcgctttcttttgaagccagttccgccagcttacgctgatgttcttcttctgctgcttggcgatctgctgcaacctgtgcaacctgctcattatcgtgagcaatacgcgcttccagttcagacagggttttgtcgaaagttgctacgatttcatctacagaacgaattttattaaacagtttcataatttatctcaattggttagttttaatcagtatacatcaatacggctggaattcaaaatcataaatgtcattcagtgcgcggttccactcggtgtagttttcaccagcaccataacgcatttgaatagcactttcgaacgttgatccgttgaggttcgggaaaccgaacaggtttttgattttgtcatgtgctacatagtacagagaagcactttccagcatcgcaaccatcgcagacggttcgtgttcgcggcgcttgatacgtaacagagtacgactagcaccagttttacg

SEQ ID NO: 13 - DNA, 3834 bp, unidentified
  source 1..3834: mol_type = unassigned DNA
atggctgatttagaaaaaattcaattcctacgtagcacagttgcggggaaaacacctactacaagtcagcttgcagatggtgaactggcgatcaacatggctgattatgccatttacacgaaaaatggttcttcgatcgttcagttagcgggtaaaggtatcccagaaacaaataccaaaaaattaacagttgatgggcctagtgctcttaatgataccgttaccgtagcggaaggtaaaactattactttcaccaacgagaatttaagtggtgaaataactcgtcatatcgtcggtaaatgtgccagcaatgatggatggtacatcggttccggtggtacaagcaataacggcattcttgaaatcggtactattgacgatggtactgaaacaatccagtttgtacaacgcggtgctggtaacgtagaagccagaaaattagtcttacttgatagctctggtaatactactcttcctggggatttaagattatccactaataaaaccgttaaaattaacaacggaagctctcttgtccttgaaatgggtgtaggtgctaatgacgcttacattaaaaacttgagaggctctggcgttcttcaattaactaatgacggcaatctgacattcagaaattcccaggtttattatgccacggatggaagaggccctggtaaagatggtactcttctgactaatgtagaaaacgcgcgtcagcttgagcaagataatttccctgtaactacaggcaacgaatctcgttggattaaagttgctctgttaaaagatcccggctcaggtcagagtcgcttgcaactgatggtgactaacggcggtaactatggttctacgtgtagttctatcgactttatcgattgtagtgctcgaagcattccatcgacattaacaagcagtaacatacgttcttatctgcaaattcgtcgaatcggcgatcctggaattgataacactaaccaaatgcgttatagtctggttcgtacctctgagggtttagaactgtggtttactcaacgcgcgtttattggtggtgttaaagttgctctgctgtctatcgctggcggtgctgttactgaatattatctgcctactggttacacaacttctgcaactgctccggaaggtttagttgagagtgtggctattcgtatctatgacgaaattaataaacctaaccttgacaatggtactgatggtattctgtctattgctaaaggtggtacaggcgcaagtacagcctctgctgctcgcacaaacttaggtttgggtacggctgcaacccgcgatgtcggcgaaggtgctggtaatgttttagaaaatggcgcttatggcttaggcggtaatggtggtaaatccatcaacgacattatctctaatgcggatatgttgacccgcttaaaatcatacggcggtactttctggcgtggtgttactaaatctggtgttagcgttcaaaatggtctttatagtcatggctctggtatttttatgaatgctggtgataccatgtcagccattaatatcgactatgctagtgctaaagttcgtgtatacgcggctaacaacgcggctcttgccgcaggagatgtcaaatacaacgaactttacggtacagcaaataaaccgtctaaggccgacgtagggcttggtaatctgacaaacgacactcaggttaaaaaagctggcgacaccatgactggtgatttaactgttcctaatttacatgcttccggtacggggactgcatcggtatatgttaatgccggaaccggaaatgctcatgtatggtttagaacagacagtaatgaacgtggtgtaatttgggcaactccaaatacagcggacttaggacaaattaatattcgcgcaagaaccactggaggcacttctgctggtgattttagcttccgttctgatggccgccttgatgttcctgtagcagttaaaattggtggagcagcaatgctaaccaaagacgggaatattacctctggttcgatgtttggtggtaaccttaacaactatttgacttctattaaaaacgatatcgttgctggtgataataagcaagtaagcaagactggtgataccatgaccggtaacttgactattaacgctaacttaaaagtcgaaaaccctaatggaacgatggttgatttaggttcagagaactctgataagtatagcagattaacccttgctcgtaaagttggtagcggtgctaccgtagcaatgcttaaagttactcctgaaggacacgtgcaatttggctatcaagatgcagttgctactccagctcctagtaaatatattctagttaaatctagcggccttgaggtagaaggggacttggtttttaaccagacatatagtggtgctgaagacgcagttgatattactgataagactgttgaccttaacagtttggttattaaaaaatccggtttaggcacccgtcagctgtataaatgcatgtcatctggtggcggaaataacatatctaataaacctacatatgacggcaactttgttcttgaagttctgtctttgcgtaaggtttctgaaactgactggacatgtaagcagacctttactacaaagaacggtgatgttgaaggcacatatgttcgatactgccaaaacggtacatggtctgcatggaaagaggttgttgctggtgttcaaccaattaatttaggtggtactggagcaacttctgtagctgctgctcgtaataacctcggtgttggtgaaggacagagcgttaagttcggcggattagttgttgatggaaacatcaacgttgcttctggtaattttgttattgcaggccaagctcctactgataactcgcatctgaccaacaaaaaatacgttgatgatcgggttgcttctgccattagtaatgcgggtgatacttatcttccattagcaggtggtactgtaactgggcggttaacaattacaggcgatcagttaaaaactacatcactttgggttacgggagacgctgctgttaatggtgttttaactgttgatggaagggctaggtttaatcaagagttcagtgtatcaacctcagttaacgttcagaacaatggcaacagtcatgtgttcttccgtaaagcggatggtacagaaaaaggacttctttgggttgatgaccctggtaacgttagtataagagcaggtggtggttctgggccagtatggaatttctggaacagtggttcttgccaattcccaggtgctattagtaactttaatggtgttaatagtactactaattaccctggcggcggtattggcgcatatttaaatacagcgggcctaacaagtagatttagtaatggtgcttatgtttccttatacttccaagaatatgtaggaaattatcaccaggctattcttaatgttaacggctatgggcaagataacagcttttatttccgggctggtggtgatttcatatgtacccgtaatggttcattcgataacgtcgagattcgttctgaccgtagagccaaatcggatatcaaagttattgaaaatgctttggaaaaagtagaaaaactaaccggtaatacttatgagcttcacaacacatccggtggtactactcgttctgctgggttgattgctcaggaagttcaagaaatcttaccggaagcagttactcaagataatgaagaagatggcggtatgcttcgtctgaattataactcagtaattgcacttctcgttgaatctgttaaagaactttctgccgaagttaaaaatcttaaagcagaaattgaagaacttaaatctaaataa

SEQ ID NO: 14 - DNA, 3804 bp, unidentified
  source 1..3804: mol_type = unassigned DNA
atggctgatttagaaaaaattcaattcctacgtagcacagttgcggggaaaacacctactacaagtcagcttgcagatggtgaactggcgatcaacatggctgattatgccatttacacgaaaaatggttcttcgatcgttcagttagcgggtaaaggtatcccagaaacaaataccaaaaaattaacagttgatgggcctagtgctcttaatgataccgttaccgtagcggaaggtaaaactattactttcaccaacgagaatttaagtggtgaaataactcgtcatatcgtcggtaaatgtgccagcaatgatggatggtacatcggttccggtggtacaagcaataacggcattcttgaaatcggtactattgacgatggtactgaaacaatccagtttgtacaacgcggtgctggtaacgttgaagcccgaaaattggtcttgcttgacggctcgggtaatactactcttcctggtgagttaagattaactactaataagactgttaaaattaacaatggaagcacacttgtccttgaaatgggcgtaggctctaacgatgcctatattaaaaaccaaagaggcgtaggtgttcttcaattaactaatgatagtaacctgacgttcagaaattcccaggtttattatgctatgagtggaagaggccctggtaaagatggtactcttctgactaatgtagaaaacgcgcgtcagcttgagcaagataatttccctgtaactacaggcaacgaaactcgttggattaaagttgctctgttaaaagatcccggctcaggtacgagtcgcttgcaactgatggtgactaacggtggtaactatggcaatacgcacagttctattgactttatcgattgtagcgctagaagcattcccgcaacattaacaagcgcaaacattagttcttatctgcaaattcgtcgaatcggcgatcctggaattgataacactaaccaaatgcgttatagtctggttcgtacctccgaaggtttagaactgtggtttgctcaacgcgcattcattggtggtgttaaagttgctctgctgtctatcgctggcggtactgttactgaatattatctgcctactggttacacaatctctgcaactgctccggaaggtttagttgagagtgtggctattcgtatctatgacgaaatgaataaacctaaccttgacaatggtactgatggtattctgtctattgctaaaggtggtacaggcgcaagtacagcggatgctgctcgtacaaacttagggttgggtactgctgcaacccgtgatgttggtacaggttccggacaagtaatgctcgttggtgcttacggtttaggcggtaagggtacatcatacaccgttgctaactctcgcgattacctgaaacaactgcgtgctgatggttctcagttcatgcgaaatacgcttggtactgaaattaactatggtatgggtgcaagtttttatagctctgtatcagatgttcatgcggtgatctcggttgactgggctactggtcgcgttaaagttggtgcaactaatgatgctaacttaaactcagataccggaaaaatcagctctcaggaactgtacggtactgcatttaaaccaactccggatgacgtaggggctgttgctcgtgctggcgacaccatgaccggtaacttgactattaaagctaacttaaaggtcgaaaatcctaatggaacgatggttgatttaggttcagagaactcagacaagtacagcagattaacccttgcacgtaaagttggtagcggtgctaccgtagcaatgcttaaagttactcctgaaggacacgtgcaatttggttatcaagatgcagttgctactccagctcctagtaaatatattctagttaaatccagcggtcttgaggtagaaggggatttagtttttaatcagacctatcgcggcaccgaagaggcagttgatattactgataagactgttgaccttaatggtcttgtcattaaaggaaccgacccaggtactcgtcagatgtataaatgcttctcatatggtggtggttctaatatatcgaacaaacctacctctgacggcaactttgttcttgaagttctatctttgcgtaaaatttctgatactgattggacttgtaagcagacctttactacaaaaggtaatgttgaaggtacatatgttcgatactgccaaaacggcacatggtctgcatggaaagaggttgttgcaggggttcagccaattaatttaggtggtactggtgcaacttctgtagatgctgctcgtaataactttactatcggcaaaacccaatctgttgaatttggttctttaattttaaacggcgtcggcgataacgatgctactttagattttaaaggcggtgctagaatacgtggtggacagcgcaccggtgagggcgctatgatcctttcagccgcagcaggcgcggttggaaaatatatcgcttttcgacccttcggtgattcgtctgttactgagattagagtaaaagccaatgagtcaagtgagccattacttgagtggtcttatggcccaggtattcgttcaaattcatctggcgcttttgttatctacgcaaaaacaggtcaggcactccatttaagaccaaacggtgataattctaaccaagccacagttattgaccaaaacggtaaaatgacagtcggtggtgaatttgaggcccagaactcaaaaatcactggtaatttgaatgtatctgaagataacagaatgattgttcttggcagaaataccgatattggtttagtcaagaaaagtaatatgccaggaaaaatggctatcagtaaatctaactcgtttactgttatggtgtcaaccaataccaacaatcagattaatcctgctgatacgtttaatgatatattcaaagtagatgctgatggaaaccagactgtttacggaaatgcccaagtcaacagacagttaactgtttctagttcagctactgttgcaggtgttattaatgctaacggcggtattattgttcctactaccaagtatgtgcaaattgccgatgctcctacgcagaataaccaagccaccaacaagaaatatgttgatgataaggttgcttctgctattagtaacgctggtgatacttatcttccgttaactggtggtactgtaactggtagattaataattacaggtgatcagttaaaaactacatcgctttgggctactggagacgctgctgttaatggtgctttaactgttgacggtaatgttgttagtaattacggtattggtagctttgttggtgctgtagatgttaaggctcctgctgcggataatggtacaacacacctttggttccgacattctaacggtggtgagcgtggtgtgatttatatgccgcgtgacaataataccatgatgggtttaagagccggtggaagtgaatggcaattacatggctctgcaggccaaatggtagggccaggcgcacgctggagaattcatcctgatggcaacatacagggtgatgtttatggtggttatatcactaactatatcaacgataggtttaaccaatgtgctcaatgggttcgtactggtgctcaacaagactttggcccaattggtcgaccggcacctggtaaaactgttcctgctggttgggtacttgttggtcttaacggtaacagcaacgaagctaaccagaacatgcaacttatcggcggacggttacaagtatggaaaccgggcgttcaatgggttgattctgctacttga